European Patent Application EP 4 477 069 A1, published December 18, 2024. Title: UNREDUCED CLONAL GAMETE FORMATION AND POLYPLOID GENOME DESIGN IN THE SOLANACEAE. Applicant: Max-Planck-Gesellschaft zur Förderung der Wissenschaften e. V. Application EP. The sequence listing filed with the application follows.

SEQUENCE LISTING (160 sequences)

SEQ ID NO: 1 - DNA, 6992 bp, Solanum lycopersicum
  source 1..6992: mol_type = genomic DNA
ttcctgcataatttcgttacttgctataaaaagttcttgaaaaaaacatattgaaatgtgtgaggatacttgatctgctctttttcttatttagtaacaaaaagaaggtggagcttaattatcttacctttttcatagtcaaactgtatttagatcaataatttttttggccaatctgacgttgaagtgatcaaaatattgattttgtcttgtatttgagtttcattctacattattcaaagtgaaagtctccaacaaatgttgttctagaatattcaatctcgagccgaaacctaggtcaagcagtggtttgagactcaatctcaatcatgatttcaaatcgagatcggaaatccaacctcgagccgagattattggaccttaatctcaagtcaaggtcgagtaccaaatcgaggtcaagtcaagtcttgaattgaaattggggttgagtctcgaattcaagactaattcaaaaattaaaacagagggggcatcatgacttaaaaagaaataaaaaacctatgcaatataacgccataaatttaatcaatgcatccagtaagttatgattaatacaccctcaagcaactaggtaggtccgcgctacgtctcgaatcaaagtcagtgttggaaatcatgaagttagatcccaactcaaggttggaaatagggcttgaggttgaggtcaagctaaagatcaagatcaagagttaggtattgagtgagggttgagatcaaaagttggttccttgaatggatagggttggtggtgaggttcgaattttttttcttaattttaagtggaatagttattatatctcatattgaaaaaatatttttcaaaatattttaagttaataaaatataaaaatttctaaaatatttttttttctaaaatattaaccttcatgcccaacacgccgagctaacttgcgcgcgcagctataaagctcggctttaccaatttacaaacaacgtgaacctgcagagcgaagaggaaatggagggaaagcgttcaaacacgcggccactaacactcttaaggaaaatcaaaggtagctagcgcttccattgaacttaaattttttctgagaaatgcattacgattctcgcgttcaatacattgattctcaacaaatcttcttcgcgtttaagccacatatactttggttttgttttgcaggatttactcgttccattgttgaggatctcgctcgaggtaggccgccgctgatctacatcgaacggttcagaaattactgtactgacacttctggaaattggtaagacgcagtgtatgtatgagtatatgaaatgatcagtcaagttatgcgtagtgaagtgcttttttgttatctgttccttcttattcgaagatctggttgaaaacaataaatgtatgttgcagttgaaaatttcattgcaaatagtgttttagaaaactcaaaaactaacactgaatttagctgtcgatttcctatgaattaataaaaaaactacctccattggttcagaaatttatctactgatacttctgaaaatcggcaagacgcatatgtgtgtgagaatgttatttggttgcttgagtatatgaaattatcaataaagttaaacttagcgaagtttttttcttctttccttctttttcaaagatctagttgaaaaaaatgaatgtgttctgcggtctgaaatttcattgcaattaatgttttagaattctaacacaaaattttactgaattattgttgatttcctatctattgatagaaatacaggaatgtatgattcctttctgtattacaaggcctccaaacagattctccttgacgtaattgaactgaaaattgcaactgatgaagatccacataggtgtaaaacgcccccagcacccccaaaacaaacccttacaaaaaataaaatgtagagatatcattattctaaatgtcttgctcagaagaagaacgagcacagtctatactgagaagtttgtttgtagaagccatatcctaatcctattctaagacactaataagtacaattagtaatagttacgttgaacagagttctaaaaacaatgaaatttattgaagttggtgtttgaatggctaattaataccatccaaattttctgatagtattaatggtttttgttttatttatgtagctcttgcagctccggtttatcgactggcaaggaagctatttccttgaagagggaatgccatgcacgtaggcttggtgagtctagggagagtaaacaatacttgtatatttcatctatagtcctcattacatagttgacaagaaatgaaatgatcaagaatggggtaggaatgattattaaaagttgctatcctcactgaaaatgacaaaatttccaggagaactatatttccccgtttagttgattttctatacttttgttgtcctatatgagcctccctttcattgatgttacacaggatgcaccatgtagggtgggggacggggattgggatggggtagtacaaggtttctccctcagttatcttttctgtttggtcgaatcaacttgaaggcactttttgctctccaatctccttaacatcttagaaccttgcatggttacttcctctttatgtttttgtttcagatgttatgttgagagttctactgatagttcaacaacttctgcaagaaaacaggcatggatcaaaaagagacatatattacatgcatcctactgtttttaaaggtaaatctgaatcggcctctggtgttacaaagttgttactcccctgttaatttcgtaggacatggttggactttatgtactccagaatcagttttgaaatattcttgtgattgcttatgaagtttttattcggtggaaaattcgtatgtgctgttgtattgttcagcgttctcagttggtagaaatctgccatgatttagatctctaatgcaaaatttatgtattcaaagatctcgtcttccttatatgctcatcattttcttttgcactccataatgcagaacaatctgttgttgatcgggcaattaatgacatatgcatcctcttgcaatgcagtcggcataaccttaatgtggtatgtcaatctactttcctctccatatcaaaatacactcattttagatgtatatccacatgtcctcactattagcagagcccgttgaaattctcttctatttttatttagcaagatgttcattttcacagtggaggattcaattagggttcagaatattgatattagaagtggtcattctgctacttatacatgcttttgacacacgaaacggtagatcacaagtatctaactctgccttctctagtgtagttgattagaaggatgtgaatactgttctcatatagaacttgaatatcaatttcagagaatgaaaatgatattgctagactagggtaaacccatcattcaaatgattagtttgttcttcttttattgctagtcttgtaggaaacttgacattttatatacttttgatgcttgccttctgcaggtgtctgttgggaatgggtgcgtacctctacacagttaatatttccttgcaggagtgtgattctagacacatacagtttgagttcattatatgcaatgttctttctcatacttgacatttataattccccatcttttcttcttgaaaattcaaatgtttcttcttcagttgattatgtttatacctcttgcattgtctgaatgttgctacattatgtatctaaatttctttttggggagcaaagttacttcatgattgagagtgttgacatagtctatcatgttacaataagcttttgcacttttagcaaggtaaaatttaatgataacccggagaaagcatgtcaactctcaaggagtactattgcatcatcatttttggcctacttttaaagatattggtggtaggtgtagatcaagtttaaacactcaccagtgaaattcacaataaatctactgttgttgcattttgctcatgacaatttttgttccccaagacggatatatagttggttttcttctttgtgtatattgtaatagttcctttagttctcggtcataaaattcttcttccaactatttttggtctagattggtgatgggctggctgcggtatgtggaatctgggaggaaaattgactgcattagcaatcctaacaccgtaagaatgataagtagaagctaagatgggtttctgtagttgtgtaacaatctaattatgatggttcctgcaggcataccccattccagtccttgttgaagaagttgatggtatccttatgagtataagtattcgaattatgaacacaacgtggttatatttgagcatgagtttgtggacttcatacatgtgcatgtccagttattgctaaacataaatggatgctttgttattgaatatatcatgttatttgactttatggattgctttgtcaggctatggctgtaactgttactcccttaatgcttgaacaagatattattagcgttgctcaatacgttatagttgtggagaaggaatcaggtaaaactatttataagcagttcaaggctataacagagtcatgaaaggtattcctagttcttaagtgaggccattatttgttgtccatcatgcagtattccagcgactagcaaatgatcagttttgcaagaggaaccgttgcattgtgataacagtacgcatcttttgttttctgagaatttccacacatacttgactccataatttctttttgaacagggaaggggttatcctgatgttcccacaaggaggttagacccatgttgctcaccttgtcagacttgttgcagatgaatcctacatcaattaatcatatttctgtcttttcatgttgcttgcctgtggtaggtttctgcgtctcctcattgacaagctgcatttgcctgtgtacggcctggtagattgtgatccatatggctttgacatcttaactacatacaaattcggttctttggtaaggattactcaatttggtgttattatgatatgaacaagttgctaacacacctccttttcacttatgttcacatttctagaagaaaagtcatacattcatcaccgttttcctatcacgagctatcaagcattcattcttatatcttgatagtaactacgcgagacacttaagttgaagtgtatgaagtaccggagtagttagatttaatggattaatagaaggatgtgttcttcggtaacacatatctgtaacttttttgaagcaaatggcttatgacgcaacatttctacgagtctctgagatacaatggcttggagtatttgtccaggattgtgacaattatagcattccacagcaatgtctcctgcctttaactgctgaaggtaacattcacacaatcatcatctcgtttcattatagctttttgtcaaagcaactcctcacaaatgagtggctgtgtaatcttgtcagataagaggaaaatcgaagcaatgttacctagatgttatttgcaaagagaagtaccacaatggaggtagaatttcatactactaagtaatgttaatgccaagacttcgggttctgaaaatattcatatcactgttcttcatgtcctaaggtttgaactggagctgctgttgcacaaaggagttaagtttgagattgaagcattgtctgtgcattcactcactttcttgtcccatgagtatctaccatcaaagatccacaatggagggtatatctaaatcttttctatctcggtatttttgatgtgctcgcggaaatattatttgaaagaacaaccgattagtcacttatgtcaaattcatcctgttccgccgttttggctattaagtttttcacgaccagttgttgtggatatcgagatactaatgtgcattaacattaagcagattgaaaattttgtcgctgaatcaaatgatactacatcagaatagattgaagaccccaattagccttaattcttaaatttattagtgatgtaagttaaatttccgtgtttaacttgttatgacactatattggttgttgtttttcccaggaaaatagaatcatgataatgtagacaataagaaatacaaacttttaaaaaggattcaagttatatatactgacgtacggatatcatgtttgtaaatactttattagtcatttgattgtgtgtaatttttttacacgaagagattatgaacgtagtaattggctaagatgcaagaagaacccagtagtttgatattgaacaatgattatatgtcttcgtcatgcaaaaagaaaaccaacacatgctcaaactcatttatggattctgataacagactcaatttgtcttatgcaaagtcacattttacctatacatttgaattgctaaagtaatttatttttattacaaaccaaaattagataacactttgaaaaatattttgtttgttttgatctagttttataaaacttcctcaacctaggttgattcatctttaggaatgaattaatttggttgcaatcatcatattccttaaataatgacgtcattcactaatgaatatttgggcaattaatgtgcaaattattgatcaagtttgacaccaatacaacatgtgataaaggattaattaaaaattaaaagaaaataaagaccaagcagaatagattcagagtattctactgaaaatctcaaaagtaacaataaaaatatagaataacattaataataataaatatttccgtgacataaataataagaagaaaatcttggtaaagatttgatttataaattacttaaacatgacaaaaataaaaccaaatgcagagaatttagtacttggtttgttatatgaaaatggtaataaaatctttggtataattatccaattttctttctccttttaatcacgagggaatatcttcataaacaaacaataattctacctatacttacattgcactcgttaatttgtcctccatttttttt

SEQ ID NO: 2 - DNA, 1435 bp, Solanum lycopersicum
  source 1..1435: mol_type = other DNA
tttctaaaatattaaccttcatgcccaacacgccgagctaacttgcgcgcgcagctataaagctcggctttaccaatttacaaacaacgtgaacctgcagagcgaagaggaaatggagggaaagcgttcaaacacgcggccactaacactcttaaggaaaatcaaaggatttactcgttccattgttgaggatctcgctcgaggtaggccgccgctgatctacatcgaacggttcagaaattactgtactgacacttctggaaattgctcttgcagctccggtttatcgactggcaaggaagctatttccttgaagagggaatgccatgcacgtaggcttgatgttatgttgagagttctactgatagttcaacaacttctgcaagaaaacaggcatggatcaaaaagagacatatattacatgcatcctactgtttttaaagaacaatctgttgttgatcgggcaattaatgacatatgcatcctcttgcaatgcagtcggcataaccttaatgtggtgtctgttgggaatggattggtgatgggctggctgcggtatgtggaatctgggaggaaaattgactgcattagcaatcctaacaccgcataccccattccagtccttgttgaagaagttgatgatattattagcgttgctcaatacgttatagttgtggagaaggaatcagtattccagcgactagcaaatgatcagttttgcaagaggaaccgttgcattgtgataacaggaaggggttatcctgatgttcccacaaggaggtttctgcgtctcctcattgacaagctgcatttgcctgtgtacggcctggtagattgtgatccatatggctttgacatcttaactacatacaaattcggttctttgcaaatggcttatgacgcaacatttctacgagtctctgagatacaatggcttggagtatttgtccaggattgtgacaattatagcattccacagcaatgtctcctgcctttaactgctgaagataagaggaaaatcgaagcaatgttacctagatgttatttgcaaagagaagtaccacaatggaggtttgaactggagctgctgttgcacaaaggagttaagtttgagattgaagcattgtctgtgcattcactcactttcttgtcccatgagtatctaccatcaaagatccacaatggaggattgaaaattttgtcgctgaatcaaatgatactacatcagaatagattgaagaccccaattagccttaattcttaaatttattagtgatgtaagttaaatttccgtgtttaacttgttatgacactatattggttgttgtttttcccaggaaaatagaatcatgataatgtagacaataagaaatacaaacttttaaaaaggattcaagttatatatactgacgtacggatatcatgtttgtaaata

SEQ ID NO: 3 - protein, 383 aa, Solanum lycopersicum
MEGKRSNTRPLTLLRKIKGFTRSIVEDLARGRPPLIYIERFRNYCTDTSGNCSCSSGLSTGKEAISLKRECHARRLDVMLRVLLIVQQLLQENRHGSKRDIYYMHPTVFKEQSVVDRAINDICILLQCSRHNLNVVSVGNGLVMGWLRYVESGRKIDCISNPNTAYPIPVLVEEVDDIISVAQYVIVVEKESVFQRLANDQFCKRNRCIVITGRGYPDVPTRRFLRLLIDKLHLPVYGLVDCDPYGFDILTTYKFGSLQMAYDATFLRVSEIQWLGVFVQDCDNYSIPQQCLLPLTAEDKRKIEAMLPRCYLQREVPQWRFELELLLHKGVKFEIEALSVHSLTFLSHEYLPSKIHNGGLKILSLNQMILHQNRLKTPISLNS

SEQ ID NO: 4 - DNA, 7259 bp, Solanum lycopersicum
  source 1..7259: mol_type = genomic DNA
taatttgaagaaaaatgaagattgttcaaaatcggtgaaagcatcaacccaccattttaaaaacttcaaatttctctgtcttttgttatgattcatttttttttttcattttatgtaaataaagtacctgttgaattttcaagaagaagaaaaaatggaccatttgagaaatagcatataacgaagaaaatgaaagaggacaacatttggtggatgaattcggaatgagatggggttaggcatttttttttgttatgaaaagaaatggtgattgtggaacaacagagaagaagaagagaagaagatgaagaaaaaagggtagtaagttagatggggtgggggttagggtggggagaaagatttttttttttatcaatttaattttttatatattattaaaggaaggaaaatattctttatcttttaaaattaaaattatgggcccatatgccacgtgtcgtagttctattcgtaatttttgtcaaaataaggagtgtgcattacacgcacaatatttgtaaagataattattattttatgtttgataggtaaatatttattaatattaaaatgtctaattgataagagtctcagttgaggtgtctaaatgaattatgcggacaactttaagggctatcgatgattgggccattaaattaagcctcttgaacaagaatagtaggggacacgtggaagccattcaggaacgatagcacaaaaattccattcacttgagctgtgacttgagttcatcaaacattcattctgcaatagggtgcggtccccacaatatactctgcaaaatgcaatcgcaatcgcttctgttatggcgggtatactctacagtatatacagacgcacaggcacaaaacacacacactttcacctttctcactttgcatatgatctccctctctctctccaactatatatacaaaaccttctagcttcaagtactctgcaaaatcagtgctgaaatttccttcttcacgacggcaatatgttctactctcatcagcttcttgctcgcaaagctccgctcggccaaatatggtgaaaattgtcgattactacttgtcatttcaattttttcctttcgaaattcgttatgttcatatgcatacgctacatttttggagtttctgattttttacttgcatatgttgtatatcctgagctagattgtcgttcttctttggtcgctggttaatgatattcagtagcttcttcaacctatttctcgtaatctgaagttatgagttatatgttaagttgtcactgttaaaattggatctgtttctgttcagaaaatgcttgaattcaaaattgttttatgaaggtattgatccagtttactacggcttttgttttgattttctattctaaatttgtttaatacatatagataagttgcatgttttgtgtttctgcgttttttaactttcatatatcgcaatccctgtagtggatcctcttttcgtcatttgctttctgtgtctaatgttctgtattcgttgaagttacttcataggattttgtgtatatgttaagttctcatatttcaatttggctacgaagaatgcttaaattgaaattgtttatgatctttctctttgctgtgaaggatggcggccactctgcactcaaaactcaataggaaaaagcttagtaaactcaatattattaacatctggtgaggcgttttcttctactactacgttgaaatgccttaattccttgttgattttgagtattcgtcttctgcaatttcttttgtcaagtgaacaaatcttaaatccatcagtcccgatggctctgaggctttctggaattctcatgggtatgcttcgaaaaccactgactgtccgcaattgctgcttttgatttagatatctaatcgacagttctgtttcaggtggagtagtcattgtttacgaacacaaagtgaaactcctatacggtatgaattgccatgatgacttcatcatttcaatttgaatttcacgttaattctttgaattctactcctactttacccttccttatttcttcatttttttttctttatgttttctttaatgcagaggatgtgactcgtctcatggtagtaacatttgtcttcgatcctaatcaaattaatctctttctttgctctgttttcattaaattccgcatttatgattgggtactttcaggtgcaaatcaatgaagcttggaaagtcaaagcagctaccgatcctacgttacttcccaagggtaaatcgcaagccaagtgagtaactcatctccaattcgacgtcacagtattttgccgagaagcagagattgtaaggccgacttttaacaacttctaatactttcagttacctcaatagtgcttcagtaaattaacaactaaagtatgactgccaccaattagttgaaatgattaactcaatttattatgatttctttcactcaatgtttgggtcagtttcatcaatgagttatttaaggcctgcttatgctgtgagtcctttatacctaaggtctttgtacttaaaaatacctagtttagcgatgaattggttgtaaacattaaattctgattcctgtgattgtttttcctaatgttgatgaattttcattcctcatttcaattcctgtaggtatgcagctattactctgccagagaatcgggaggaagaactcccagagattgaacagacattacggaatccagacacagtcacaatgatggatttcgaacaaacctcctatttcacgatggtacattatggaaagctctgtcacctcctcaatccacgaaataacttcaaaagcagaaacaaaaattgttaggaaaattaggaatttgttcgaactgatctaattaaaactattgagcttgctttagattgttaaataagtcatatttcattattcagcaagtctgcaagctcaacaatagaaagttaacaatgataaagttgtttgatttcccttcgccttttggttactctatatgttttgtagcttgttctatgttatttccactcttgggttttctcagtgttcatgaccttgttgagtaggcaatcttatctgataccacttggataagagcaggaaatcttagtgaaaatcagatcactacatgagagtgcagctaaacttgcggatgttcaatgtgcagagactagataatgctgatctctatgataaacccaatgcacaggaggaacctgctaaggacttgcatcaaggtacacctagatcccacaatcagcatagattatgctactttcaccatcacaatagaatatataactatatcctagtcaatgctactttgttttccagttttgtcttgttgtgcccatctctaaaacaatcctgaaacccttgttgcagttgatccagataatatcaccctcgctgaacgctttgaatcccatcatacagatatgttcaatcattttgagaggtatcacgatgaacagtttgtaggctctgtatttctaagtttgtacgatcagttcgcataaaaacttcacgtgaaccaaactatccaccattaaatcacaggaggctaattagccccatttttaattaactgcaaagctttccttctattatccccctattaatttttaagcatgaattgttctgcaggtttgatattgaaggggatgaagaaacacaaatgaattatacccagccagaggatgctcaaatcccaagtactcctgtgcaatctccacctcgagaacaagcccatcaacgtaagaacgtgttactatcttctactttagataaatgaagttttttgagatgtaaatagtagatggagttacgatatttcattatttcacttggttttctgatagagacataatggcaataaacccttcctctcaaataggaacatgaatgcaagtcgtacttacctactatgagatcagttaaaatactttgtagctacctggctgcttaccattaaacttccggtttacatatgaagttccttcaagcacagaactcttttggattgagttgagcttgtaaaagtctttagatttccttaggtaattaattatttctgaaaattggttgaatggagcgaaacattattgcagctgatgagatccctgacagacatccagaggaccaagtgaagcaacaatctgatgaagttaaagaagcttttgaggtagaaactccacaagcaaccaagctagaaaataatgtaaagaaaaactgtcagcactaatgttacgtcttgacatgatattgtagcagcggcaggatcaacaaaggccaaagccagctcgacgaagaacaagaaaggccacaagtcttgcaattgatcatgagcaaactattatttctggtgacatatatcaatcctggcttcagagttcttcagatattgcatcaagaaaaaggaaaaagagaaaggtacttccatacctcccaatctagatcttccccatttcaatttttccattgtgtgcaccgtataacctttgatatcaatggctagtctttgtgtatcccaagaatagcatgtgcatctctctctggaaggtaaccttaactaaactaacatgcagcatcatttattagtaaccttaagtttctattctgtgcagactttgagtgtcttaccttctatgaagatagccagaatgatggaaatgcctcctattgcactactagaaggattgttcacaaatggaaataaggaagttcactatccagcaccactcctaaaattatggatgaggaatacccaacctccgcatgattcaccttccggtctggtttttcatccatgatattagactcttagttgccaaaactataaacaggtggtaattacatttgacttgcaggaaaaacctctccaccctttcctcctgaaccatcctatacatctccaggtgaaaggatgggtaatttggaaccgcctttcgaatatttccaaggcggtgtaggctccccagcagtaggaatctctatagaaaaacaaagggcaaatctcaacaataacaagattccacctgaaattctcatggaggacctcagaaccaatcttacaaatatgggactgcatccaacagagactaatggagtgaaagagactgatcacatggccacacctggctctggtatatcgatttttttatgaatttcccaatctccatgatttgttcggcaatctgatatggtggtataactaacatttttgtgaatctataggtgatgagcctagatccattccaagctcaggatctggtcatggtttactatcacagaattctgtaaccgattcaagtcggttagtactactagtagatatatgttgagggatttgtctaaagatgaaccacttgaatcatacagacaatgacagaaggaaataatgaatatcatggatttcagcaccatagggaactttaaaactttgcttctttttaaaattatgaaggtctcaccatatagcagcatctggttacattgatcaaaattgttaactcttcaggtccaacaagaaaagaccccattcttcattgaagcacagtggcaatggtcttcaaccagtagcagaagagaacccatggcacgaccccactctaaatttcaagttgactagattatctgaactatctgaaaatggttttacacaagacaacggttcgtgaatagtcagtaaccttcccattttagttctggtcattttctttaatgtggtttagtttgttatgaacctcccttcactattttggcagagatattgatggaaaccggaccaacacaaacccaacatccattcattactcaacctcttgacatgatgactgactctatcaggatgtaaatccttttccatttgttcctaaaacttctccagcttcactgtatatcatctgattaattgatttttcacctgataaactgatgtctacagacagctaaagagtcattttgacactcccggatcggcagaagcagaatgtttgaatgaactaactcttggaatgacaaagaaacaagcagcatgtcttttttatcagacttgtggtatgcaaacttctttcatatcttttcctcttgcattgcagctcagagaaacttcatagtttccagcttctcattagagagaattaatgtttgctccattctacgtgcagttctggccactcgagactttgttaaagtcgaacaggagcttccatatggaaacatcctcatttccagaggtgcaaagatgtaacaacggataaatctagtagatgctaaatcctcacaagtcttatagattcatctattgttatagctgatacaaatttatttttcggttaaggtattggagaattgaggcacagatttatagctcaaattttcaggagaaagtatttttattgttaacctatctagtgtataatcgtagaagcatagttatctccaagagaatatagatagaagtatatgattggtcattctgaaactagctaattgtactagcatttggtgacagctaaaaactatgggcttcctttgtttgatctttataaaaacgggtcaggtaacttaaagtttctgtacgaattgacctatttcttattgatctctattttgtgaaataaatttaacttctatttcttgcctggaatcaattttataataattaaattttcttacatcaatcacatagtatataattcattcaatacaagttctaaaaaaaattggacaagttaggtcttttgtgtaatattagaatacaaaattctgtcttgctatttccatttttcttttttaatattaaggatatttttcttaccaaaaattaaaaaaccacccaaaaataggcattcgtgccaatgacccacgccacttccgcccggtccaaaatcaaatgccctacattatcttatctttgaatatctagagtctagtctccttctcgcattcgcaagaaaattactgccgtagaagttaaaggctctcattgtttccgacggcgacatggcaatgacgatgaccactgcaatggcatcgccgtcgcggcggctgcttatcaactctcgacatagcaccatctgcactatccccaagaatgtggcaatttacccagcagcagcagttacaaatcaggggttattgaagcactgtatatcctcgcaaagatgcctaagatctctggtaaaaccagtatcggctgctagttcaggttttgaggcagatttgggtgacgatgaatctctgatacg

SEQ ID NO: 5 - DNA, 3225 bp, Solanum lycopersicum
  source 1..3225: mol_type = other DNA
ttttatcaatttaattttttatatattattaaaggaaggaaaatattctttatcttttaaaattaaaattatgggcccatatgccacgtgtcgtagttctattcgtaatttttgtcaaaataaggagtgtgcattacacgcacaatatttgtaaagataattattattttatgtttgataggtaaatatttattaatattaaaatgtctaattgataagagtctcagttgaggtgtctaaatgaattatgcggacaactttaagggctatcgatgattgggccattaaattaagcctcttgaacaagaatagtaggggacacgtggaagccattcaggaacgatagcacaaaaattccattcacttgagctgtgacttgagttcatcaaacattcattctgcaatagggtgcggtccccacaatatactctgcaaaatgcaatcgcaatcgcttctgttatggcgggtatactctacagtatatacagacgcacaggcacaaaacacacacactttcacctttctcactttgcatatgatctccctctctctctccaactatatatacaaaaccttctagcttcaagtactctgcaaaatcagtgctgaaatttccttcttcacgacggcaatatgttctactctcatcagcttcttgctcgcaaagctccgctcggccaaatatggatggcggccactctgcactcaaaactcaataggaaaaagcttagtaaactcaatattattaacatctgtgaacaaatcttaaatccatcagtcccgatggctctgaggctttctggaattctcatgggtggagtagtcattgtttacgaacacaaagtgaaactcctatacgaggatgtgactcgtctcatggtgcaaatcaatgaagcttggaaagtcaaagcagctaccgatcctacgttacttcccaagggtaaatcgcaagccaagtatgcagctattactctgccagagaatcgggaggaagaactcccagagattgaacagacattacggaatccagacacagtcacaatgatggatttcgaacaaacctcctatttcacgatgagactagataatgctgatctctatgataaacccaatgcacaggaggaacctgctaaggacttgcatcaagttgatccagataatatcaccctcgctgaacgctttgaatcccatcatacagatatgttcaatcattttgagaggtttgatattgaaggggatgaagaaacacaaatgaattatacccagccagaggatgctcaaatcccaagtactcctgtgcaatctccacctcgagaacaagcccatcaacctgatgagatccctgacagacatccagaggaccaagtgaagcaacaatctgatgaagttaaagaagcttttgagcagcggcaggatcaacaaaggccaaagccagctcgacgaagaacaagaaaggccacaagtcttgcaattgatcatgagcaaactattatttctggtgacatatatcaatcctggcttcagagttcttcagatattgcatcaagaaaaaggaaaaagagaaagactttgagtgtcttaccttctatgaagatagccagaatgatggaaatgcctcctattgcactactagaaggattgttcacaaatggaaataaggaagttcactatccagcaccactcctaaaattatggatgaggaatacccaacctccgcatgattcaccttccggaaaaacctctccaccctttcctcctgaaccatcctatacatctccaggtgaaaggatgggtaatttggaaccgcctttcgaatatttccaaggcggtgtaggctccccagcagtaggaatctctatagaaaaacaaagggcaaatctcaacaataacaagattccacctgaaattctcatggaggacctcagaaccaatcttacaaatatgggactgcatccaacagagactaatggagtgaaagagactgatcacatggccacacctggctctggtgatgagcctagatccattccaagctcaggatctggtcatggtttactatcacagaattctgtaaccgattcaagtcggtccaacaagaaaagaccccattcttcattgaagcacagtggcaatggtcttcaaccagtagcagaagagaacccatggcacgaccccactctaaatttcaagttgactagattatctgaactatctgaaaatggttttacacaagacaacgagatattgatggaaaccggaccaacacaaacccaacatccattcattactcaacctcttgacatgatgactgactctatcaggatacagctaaagagtcattttgacactcccggatcggcagaagcagaatgtttgaatgaactaactcttggaatgacaaagaaacaagcagcatgtcttttttatcagacttgtgttctggccactcgagactttgttaaagtcgaacaggagcttccatatggaaacatcctcatttccagaggtgcaaagatgtaacaacggataaatctagtagatgctaaatcctcacaagtcttatagattcatctattgttatagctgatacaaatttatttttcggttaaggtattggagaattgaggcacagatttatagctcaaattttcaggagaaagtatttttattgttaacctatctagtgtataatcgtagaagcatagttatctccaagagaatatagatagaagtatatgattggtcattctgaaactagctaattgtactagcatttggtgacagctaaaaactatgggcttcctttgtttgatctttataaaaacgggtcaggtaacttaaagtttctgtacgaattgacctatttcttattgatctctattttgtgaaataaatttaacttctatttcttgcctggaatcaattttataataattaaattttcttacatcaatcacatagtatataattcattcaatacaagttctaaaaaaaattggacaagttaggtcttttgtgtaatattagaatacaaaattctgtcttgctatttccatttttcttttttaatattaaggatatttttcttaccaaaaattaaaaaaccacccaaaaataggcattcgtgccaatgacccacgccacttccgcccggtccaaaatcaaatgccctacattatcttatctttgaatatctagagtctagtctccttctcgcattcgcaa

SEQ ID NO: 6 - protein, 628 aa, Solanum lycopersicum
MFYSHQLLARKAPLGQIWMAATLHSKLNRKKLSKLNIINICEQILNPSVPMALRLSGILMGGVVIVYEHKVKLLYEDVTRLMVQINEAWKVKAATDPTLLPKGKSQAKYAAITLPENREEELPEIEQTLRNPDTVTMMDFEQTSYFTMRLDNADLYDKPNAQEEPAKDLHQVDPDNITLAERFESHHTDMFNHFERFDIEGDEETQMNYTQPEDAQIPSTPVQSPPREQAHQPDEIPDRHPEDQVKQQSDEVKEAFEQRQDQQRPKPARRRTRKATSLAIDHEQTIISGDIYQSWLQSSSDIASRKRKKRKTLSVLPSMKIARMMEMPPIALLEGLFTNGNKEVHYPAPLLKLWMRNTQPPHDSPSGKTSPPFPPEPSYTSPGERMGNLEPPFEYFQGGVGSPAVGISIEKQRANLNNNKIPPEILMEDLRTNLTNMGLHPTETNGVKETDHMATPGSGDEPRSIPSSGSGHGLLSQNSVTDSSRSNKKRPHSSLKHSGNGLQPVAEENPWHDPTLNFKLTRLSELSENGFTQDNEILMETGPTQTQHPFITQPLDMMTDSIRIQLKSHFDTPGSAEAECLNELTLGMTKKQAACLFYQTCVLATRDFVKVEQELPYGNILISRGAKM

SEQ ID NO: 7 - DNA, 5596 bp, Solanum lycopersicum
  source 1..5596: mol_type = genomic DNA
aagaaaacatagtaacaaccctatttttactaacaatatcaatataattgccaataatagattgttatttatggataagaaatatttataaaataatattatcttttaaatataatagaatataaaataattctttttgagatatatataataatatttttccaacataaattataaagatgcaataataatgacatatgcaatcgaattttagacatacatcaattagatctacaacacaacaccaacaagagcaatccacaccgagaacaagatacaacttcatgaggggttcaagagcgcacaagtaacggaagtccgaccctgggatcacctaagaagaagagaaaaggtaccttacatagaaaatcatgtatttttctaaatttaaattcaaatattactttcaaatttaactcaatcttatgtagtataagctcacatatatcattccttattaccaaaattcatttcttttttatataataaataatctgtcaattactatataatttgaatttattttttccaaaaaaaaaagaaaaaactgtttttttctttttgcatttggctttattacagtgaataaaaaaacaaagaggaagcttgagctttttttctgggtgcactaaagtcaagaacgaatcccttcaaatttgaattcaaaaaattacacactaaactcacagaaccttcatcacccacagtacaaatgttttcatctgattggtcggtcacttttctattctcaactccaattaaacaaatgatttttagtgggcccaactttgtccgctcctaacgaatacctaaatcaaatggacggttcagattaaatcaaaattcaaatgtatttatttatttatatattaataacttcacatattgagagtaacacacagcgttcttcttcttcgtttatcttgaagaagaggattgatgaaaatttgttgagaaattgttaaattttttttgatcatttttcgatttgaaggaggaaatgatgacaacccagaataggcggtcgtctgcggtggcgaagagacaagcaatggcagcgaattcatcggggttagagcataatcagaccggaaaattgaatgccaagaaacgaccggctttgtctaatatctcgaataatacaactgtctctgctcggaactcggtttctcattcctccaaactcgtgagtatttatctgtttttgtataaatggctttattactctaggaaggtgattagagtactgggtctttctctttctttgcgttttttttgttactgttcgatgattttactgggtttgtctctttttggtggtggttatggtttttttctgattgctggttcagaggaggaaaatgtaggttggttttgtgattttttttttttggggggggggggttctttcttggagtttcataaacattacaactttctcaaaatgatcgaagatactgtgtaaaaatcagtttgagaaaatcaagtgaagtgatttttgatatgaggagatttgtgggttttatttttttttggtcaagattttgtaaattggaagttaatttctttgttaattgacttccattttttaaacaagttcactgttttgtgcaggaaatgcattagttatcgagggatttgttttttctttttttaaagtttgagttgaagtattcttttaatgataagaaagtgttatgaatggaaaatttgaaacaatcttcccccagttcctgctttttgtttatcttccactttgctttttgaatatttgaagaaagttctaatgtttatgttattaagttgaacaaaagttcttgctttctttcaaatggacatagtataattggacaattatgaagtggaccagtggcattctagattattattttcagtgttaacatgaattgtttagcatgtcattactgtgaactagtggaccaattcctgctttttgtctccttagatgattttattactgttcttaattttattacacaaatgagcagagaagttgagcaacttttgctaatttttagttttcacagttgggttaaaccttttctttagtaagctgttttgcaatgtgtgtaaattgaaaaaagactgtttcttgtatctgaagttgtgactaacttgaggtcatttttggctttggaaggcaccatgtacatccaagattgtaaacattaagaagaacacttctgcttgcaacagtaatgcagtttcctcagggactgctgttctgccagcatcctcctctgtgagaccaagcagcaaacctgtttctattcaaagaagtgatgcagttgtgcctaagatcactgtcattcctgttcctgccacttgcagcatggacatttctccatctcattcagatggatcattagtctccatggatgaatctatgtcaaattccgacacagtgagaagtccggaggtcgaatacatagatgaccatgaattagctgcagttgattccatcgagaagaaagcgtgtagcaccctctacatctcagaacatgtcaaagccgcaggttttgatcttttcagcagagaatagtccttgttctggcatttcatttttttaactataacatctatttaatacaatttatctatttttgattccagcagctgatatatgcaagagagatgtacttgtggacttggaatcaggggacaaaattatgaacattgataacaatcttgttgacccacagttatgtgctacaatggcctgtgacatatacaaacacttgagagcctctgaggtataaaaatgtttaccctcttatcttttttaagctcgttgaattggatgctgctgctaactttaaactgaattgctgttttactaacatttatcattaaacatgttttaatgtcatctttgatcactgtactaggcaaagaaaaggccttccacagatttcatggcgaaagtacagaaagacatcaatcctagcatgcgcgctatcttaatcgactggcttgttgaggtaaacttctaatatcttttttctctaaagctatgtccctgatgaaatgtcaacctgcccaacttatgacttaattaatgtggatgagctcagaaattcgtcaatttgatagggaacttgtttgatggtataggttgccgaggagtacaggcttgtcccagacacgctgcatttgacaattaactacattgatcgatatctttcgggcaacctgatggacagacaacgactacagttgcttggagtagcttgcatgatgatcgcatcgtaagaaactaccttctgacctctactgcatatgttttctccatgatctttacaaatttttccttgagtgtttttcatattcttgtgtcctcaattatttcaagcatatctgtaagaaaatgctctaagacattaatatgggaaatgctttattgcagaaaatatgaggagatctgtgcacctcaagttgaagagttctgctacataacagacaacacttacttcaaggaggaggtatatgatcttgattcacagaacctgcagtggtcgaactttgtagtggcactaagacttaacatattatgcaggtgttgcaaatggagtctgctgttttaaattacttgaagtttgaaatgacagctccaacagccaaatgttttctgaggttactattcttatcaagatctagttcttttgagtatgatgatttaggaacttattgttgagatatactgcaggaggtttgttcgagctgctcaaggacttaatgaggtaacctcttcacttaaagttgataattctccaattctataggaaacaagagttgattaaaactttaagatcttcaggttctgtcactgcagttggaacacttggctagctacattgcagaactctctcttttagaatacaacatgctttgttatgctccatcactcattgctgcttctgcaatttttttggccaaatatattcttcttccttcagtgaaaccttgggtatgtacgaattagcattgtgacaatcctataagctgttataatgcattttcgcttcttattctcctttcgacaaatatattcttataaaatttgacttttggaaactcctaatacagaattctaccttgaggcattatactttgtatcaaccctctgatttacgagactgtgtcttggcactacacagcctttgctgcaacaacaacaattctagcttaccagcagtccgggaaaaatacagccaacacaaggtttgcataattctcttttcagttcattccaagcaagtatactggggtctggactgcacttgaacattcatattggaaaattagtgtctgctgaatcttattggataagctatcaacaacctatctgagggataaaagatcaaccttctctcaacactagtcaaatgacgataactgaaaattgacttgatagacatgtattttcatgtacatacagagtcatgtaggcatctgcataaatttcctatcgagtttattctaatgtttggttttcttaaacagtacaaatttgttgcaaagaagtattgccctccaactgtacctgtagaattcttccagaacataagcagctaagccagggagataatgtgagaagaggcatctacttcagtagttccaattgtctgttggattaactcatggcattcggtcttatatagcctttaacttgcaatgtccatggaagagagcttcattcttggtttttctctccttgaggggccttagcagagcatctttgtttgtagtcattaacattgacattgcaggattagtctcttgtactctactgtttttctctggcttagtttgtctagtcaatttgtgtatagaagaagcgccactggctgtttcattagctcagaaactattcagtaatgattcctttatggaactattggcagtttgtgccaattagtattgagaagaacatcccaactgatcaaagccttgacttctagtcctgtcaactggtgcaactcaatatcgagttgtacagaagttgggtgaagaaaaaagacacattgttattgcatctattaattcgctcataatttatattgatcaaggattcaaccgtatacattggcaaaaatattttacagagtcacaatagacaacagatacataattattctataatttacatatagcacagacactctagccctataagagaagttcattgagcacactgaatcttggcagaatctaagccgaaggatgcattagtcctaacattcagccagtgacaatcttcaaaagaacagggctgaccaccgttaggccattctacatccataggttctatgaaagtagggccccaagcgggcgtaccatcctcgtatgaattgtgtgttaatcttcgtatgtctgagccgtctgatttgatcacatatatatcaccatatggctgataatgatgaggattcgagatgggctcagctgatacggcggcgtaatctgaagtgaacactatatacttgccatccgggctgaaataaggatggttagtcctcccacctataccactctggatcaccttcttgagtcctgttccattagggtgaatcat

SEQ ID NO: 8 - DNA, 2036 bp, Solanum lycopersicum
  source 1..2036: mol_type = other DNA
cgtttatcttgaagaagaggattgatgaaaatttgttgagaaattgttaaattttttttgatcatttttcgatttgaaggaggaaatgatgacaacccagaataggcggtcgtctgcggtggcgaagagacaagcaatggcagcgaattcatcggggttagagcataatcagaccggaaaattgaatgccaagaaacgaccggctttgtctaatatctcgaataatacaactgtctctgctcggaactcggtttctcattcctccaaactcgcaccatgtacatccaagattgtaaacattaagaagaacacttctgcttgcaacagtaatgcagtttcctcagggactgctgttctgccagcatcctcctctgtgagaccaagcagcaaacctgtttctattcaaagaagtgatgcagttgtgcctaagatcactgtcattcctgttcctgccacttgcagcatggacatttctccatctcattcagatggatcattagtctccatggatgaatctatgtcaaattccgacacagtgagaagtccggaggtcgaatacatagatgaccatgaattagctgcagttgattccatcgagaagaaagcgtgtagcaccctctacatctcagaacatgtcaaagccgcagcagctgatatatgcaagagagatgtacttgtggacttggaatcaggggacaaaattatgaacattgataacaatcttgttgacccacagttatgtgctacaatggcctgtgacatatacaaacacttgagagcctctgaggcaaagaaaaggccttccacagatttcatggcgaaagtacagaaagacatcaatcctagcatgcgcgctatcttaatcgactggcttgttgaggttgccgaggagtacaggcttgtcccagacacgctgcatttgacaattaactacattgatcgatatctttcgggcaacctgatggacagacaacgactacagttgcttggagtagcttgcatgatgatcgcatcaaaatatgaggagatctgtgcacctcaagttgaagagttctgctacataacagacaacacttacttcaaggaggaggtgttgcaaatggagtctgctgttttaaattacttgaagtttgaaatgacagctccaacagccaaatgttttctgaggaggtttgttcgagctgctcaaggacttaatgaggttctgtcactgcagttggaacacttggctagctacattgcagaactctctcttttagaatacaacatgctttgttatgctccatcactcattgctgcttctgcaatttttttggccaaatatattcttcttccttcagtgaaaccttggaattctaccttgaggcattatactttgtatcaaccctctgatttacgagactgtgtcttggcactacacagcctttgctgcaacaacaacaattctagcttaccagcagtccgggaaaaatacagccaacacaagtacaaatttgttgcaaagaagtattgccctccaactgtacctgtagaattcttccagaacataagcagctaagccagggagataatgtgagaagaggcatctacttcagtagttccaattgtctgttggattaactcatggcattcggtcttatatagcctttaacttgcaatgtccatggaagagagcttcattcttggtttttctctccttgaggggccttagcagagcatctttgtttgtagtcattaacattgacattgcaggattagtctcttgtactctactgtttttctctggcttagtttgtctagtcaatttgtgtatagaagaagcgccactggctgtttcattagctcagaaactattcagtaatgattcctttatggaactattggcagtttgtgccaattagtattgagaagaacatcccaactgatcaaagccttgacttctagtcctgtcaactggtgcaactcaatatcgagttgtacagaagttgggtgaagaaaaaagacacattgttattgcatctattaattcgctcata

SEQ ID NO: 9 - protein, 490 aa, Solanum lycopersicum
MMTTQNRRSSAVAKRQAMAANSSGLEHNQTGKLNAKKRPALSNISNNTTVSARNSVSHSSKLAPCTSKIVNIKKNTSACNSNAVSSGTAVLPASSSVRPSSKPVSIQRSDAVVPKITVIPVPATCSMDISPSHSDGSLVSMDESMSNSDTVRSPEVEYIDDHELAAVDSIEKKACSTLYISEHVKAAAADICKRDVLVDLESGDKIMNIDNNLVDPQLCATMACDIYKHLRASEAKKRPSTDFMAKVQKDINPSMRAILIDWLVEVAEEYRLVPDTLHLTINYIDRYLSGNLMDRQRLQLLGVACMMIASKYEEICAPQVEEFCYITDNTYFKEEVLQMESAVLNYLKFEMTAPTAKCFLRRFVRAAQGLNEVLSLQLEHLASYIAELSLLEYNMLCYAPSLIAASAIFLAKYILLPSVKPWNSTLRHYTLYQPSDLRDCVLALHSLCCNNNNSSLPAVREKYSQHKYKFVAKKYCPPTVPVEFFQNISS

SEQ ID NO: 10 - DNA, 4826 bp, Solanum lycopersicum
  source 1..4826: mol_type = genomic DNA
gctcgatgattagtcgcccatggataaggcgccggaatcgtttcgcttttcaatgtgcgctttcgtttacgtggacggcgagatggtggtggcggtggcggtggtggaggtggcggtgctacgacgggagacggagaaaaagacagagacagtgtaagtaagctatggtcgatttcattgctgtttgtcgccattgttttgttgtttgtctacagagaaatggttttatatataaggaagagaaaaatggaaatgggaagaagtttgttatgaatagtactgtaaagtgtacgagaagataaagacgaaacagaaacagagcaggtagtaattccatttggtttagacttctttttttttttgaatttcgaaaaaaagttggccttttcaaattctgttttagagggaatgaatttgttatgtgtttttatgtacaattatttttaataataattaaaaaaaaagttcacagattattttttgtttaagttaattcttctagattttttaaatttattcgattgaagctaataaattatttcctattttgtggtggtctttaatttctaggcttcaaggtgaaaaaattaaaaattaactcatttaaacgataaattatacaattaaatgattgaaatttgtccaattaaatcgttgaggtgtttcacgctttttaaaaaaagaaaattacaacataaattagacataattttctatttttattgttattgtattgttaaatatatgattaaaataactaaacattaattaataattaatttcaatactaataataaaattgaaagaacattttaaaaatagtcttgaaaattaaacaattaagttcatttgacaaaaataaaaatattttaaaaattcaattaatataaaatgaaggagaataaattcacccggatatgcaaaagtgggccaaatcaaacactatataaatgcttagcctctgaattcaaaattgcagatttaccgccattttgaagctatgggagaattctgcagatcaaccattttcttctccgatcaacacctctgctatgccgatatccttccttcttcacaggtaactctccgtcaccaaaacattcgcagatttctagcagtgttgaatgtataaattgcttcatttggaagttcaattaaattaaatcggatcgatatattttagtccatgggaaaagatgaactggtagattcaaagttctaaccatgtcgcgattgcagcatgtatttgttttctgatataatcgaatttctgtgttcaggtccgagctcgaatcgaagttgcggtcctgaattttcttaaagctctaagttcaaactctccgtcaatttctgatctatcactggtttgaaattttacatcttcatcttttcgaaacgaaatctctctataatttgcacttttagcttacttcatatgcctgctgtaagcatcatcaagttataaacaaatccaaaaaaaagttgataaatccattggattgatgcttcgttaattgttcagaatgcttattgttcttaattaagcaactttgggagatttatatgtgaacctctctgtcacctcaaagaacaaatgacttaccagttttgggatgaattaggcctgaacataaatggatatagatgattcatatagtggacgtcaaaaagaggcatagttgatgatttatatatggcatatgtgatgcagatcagtaggaactccagcaatagcagagtgagccgtgggttacttaccggtgattcatggatcttcctgtcccattctttttgcacgcgttctttgacgagagagaatagtgctaagtcattcataagaggtaaaaggctacaagtttcttaccatcaaattacttattagacaaatcaatgacgctggcaatgtttttgtgatcaagtttggaaggttatggagatgtgctaccaaattctggttcaggaaaagagggtgacacagagagagctatactacaagctgctctgtgattcaccagattacttcacttctcaattgcaggttaataggaccatccaaggtcattgttctttcttctttcttcatcatatctgaatatgatctgtgtgttcggttgattttgttaacacgaggtccttcatttactatctatgaggaacagacttggtggctttgcttcgatgcagccgttacagccttggaataatggcatcaagcagaggggcaatagcaggccgtttattgttacaggtactattatcaaccctttggttgtaatttcaaatgtttatattttaatttaatcaaacgcgtagcagtattagtattttgacttggccagtaacatgatctgtcatattggaatgaaataggccatgtacaacaaatggatatagagaattcatatagcccatctcaactagtttatgattgaggcacaaccgattgtttgatttcaacatgagccaacctagtcaaaactttcaatgtttccaaatttctatagttgataagagctagctgctggtagccgtctatgatcaactattttgctttgtatcttgaatttgtgccaaaactcaatgaacctattacttaaatgatgtacaagtctctaagttcctatataaagcttgttcaagaatttgaaataggtagtttatccaacagttagaacttggtatttctttcttcaaagatggacatatgacttaagtttgtttctttacaccactgagataggagccagacaaggaagttattgactgctctgcttgtggatcttcgggttatgctatatcaggagacctggaattgctggaaaaattaaccatggaaacagatgctcgatacatcatcatggtggaaaaggtattttatcacttgttgggaactctagtcaatcatttttgcaagaaactaaaactagttccactttttagcatgctatattccagcgactagcagaggatcgtgtattcaatcacatcccatgcattctgattactgccaaaggatttcctgatattgcaactaggtgacgtgaagatttataaacatcttcaaatagaactttattctgatgttctagcttacagaatagctgctaggagattgtccattcaagtattaattcataacatattctaatctgtaacaacttattcaggtttctgcttcatcgaatatgtcggatgttccctaatttgccagtcttggggctggttgactggtataactgacttgactagtattgccatcacatagttacagagcaaaactcttacaaatcaaattgtgatttttaaggaacccggctggattagcaatcctttgcaccttcaagtttggaagcatagggatgggacttgaagcatacagatatggtgctcttttctcttaaaagttatgttgaatcatgtatccttgttgtcttcttaacttcacttataggagtctgtttctctgcatgtttttttaagcttgtaatgtcaagtggttaggactgcggaaggatgatattaatcaacttatacctgaagaatgtttggtccctttgaaacctcgagatctccagattgccaagagcttaatgtcatcagagattctgcaggtataattccagttacaacagaaacgcaatctttctccattatttggttcggaaaattgttacataccggttttttccaggatagctacaaagaagaggtggctgctatgattcagagtggtagaagggcagagattgaagctctctattgtcatggatatgattacttggtgaagttccttgcgacaaaaatagtacaagccaattacctctaataatttgcctactcatcgaaaacaagtactgagaaactattggatttccagaattgaatgcttaactgaacggtgtaggaagttcagcacttaaaaatcaattcgtattaggaattgataccattacggctttcttgtgcattgatgcggtctatttagctagcgcctcatttcggagtgtcactgctatcaagacttattatgtttaccaaaacaacaggatctcttacattgaaagatctaagattacggcattcaactgaagttcgactcgatgaccatcagagcagatatgcaatcttcaacttaacaaaggaaacaaattcccaaaataaactgaacacaccagactagtgttatgaatgtgcggaaattcagagctcacagggtccgttatgagcaggggagcctgcaaagtattcgcacaattaaaccatatagagacataccgaactgaccactccataataaaagaaaaaaaaaatggccggccattcatcagggaaaaggggggtgaaacctcccatctcatttgtgcaataacaaattataaatgtgtaacaatcaaataattatgcatctgttaataatacaacttatactcacctctattcttggccaaaaaaacacaaattatcacccaaaaaaaaagatcaaaacaaaacagtgaggagggtggtagaagagaaggagaagaaaaagaagaagggcagatcactgggtgaagaaatgactgcctaaatgctgtactcccctaaacgcaatgttgtgctccttgctatatctctcagcaaaacaaaataaacttgatttactgtgaacctagtctcggtggccatctacattacgttacagctaaactcagctacggcaaaattctttcagttctctttacgaaagagacaccctctttccctccactgagaacttgtcactgccttcaagctgcatacaaggagacaagtcaatcagtatgctaaacgaacaacccaaaaacagg

SEQ ID NO: 11 - DNA, 1853 bp, Solanum lycopersicum
  source 1..1853: mol_type = other DNA
tctgaattcaaaattgcagatttaccgccattttgaagctatgggagaattctgcagatcaaccattttcttctccgatcaacacctctgctatgccgatatccttccttcttcacaggtccgagctcgaatcgaagttgcggtcctgaattttcttaaagctctaagttcaaactctccgtcaatttctgatctatcactgatcagtaggaactccagcaatagcagagtgagccgtgggttacttaccggtgattcatggatcttcctgtcccattctttttgcacgcgttctttgacgagagagaatagtgctaagtcattcataagagtttggaaggttatggagatgtgctaccaaattctggttcaggaaaagagggtgacacagagagagctatactacaagctgctctgtgattcaccagattacttcacttctcaattgcaggttaataggaccatccaagacttggtggctttgcttcgatgcagccgttacagccttggaataatggcatcaagcagaggggcaatagcaggccgtttattgttacaggagccagacaaggaagttattgactgctctgcttgtggatcttcgggttatgctatatcaggagacctggaattgctggaaaaattaaccatggaaacagatgctcgatacatcatcatggtggaaaagcatgctatattccagcgactagcagaggatcgtgtattcaatcacatcccatgcattctgattactgccaaaggatttcctgatattgcaactaggtttctgcttcatcgaatatgtcggatgttccctaatttgccagtcttggggctggttgactggaacccggctggattagcaatcctttgcaccttcaagtttggaagcatagggatgggacttgaagcatacagatatgcttgtaatgtcaagtggttaggactgcggaaggatgatattaatcaacttatacctgaagaatgtttggtccctttgaaacctcgagatctccagattgccaagagcttaatgtcatcagagattctgcaggatagctacaaagaagaggtggctgctatgattcagagtggtagaagggcagagattgaagctctctattgtcatggatatgattacttggtgaagttccttgcgacaaaaatagtacaagccaattacctctaataatttgcctactcatcgaaaacaagtactgagaaactattggatttccagaattgaatgcttaactgaacggtgtaggaagttcagcacttaaaaatcaattcgtattaggaattgataccattacggctttcttgtgcattgatgcggtctatttagctagcgcctcatttcggagtgtcactgctatcaagacttattatgtttaccaaaacaacaggatctcttacattgaaagatctaagattacggcattcaactgaagttcgactcgatgaccatcagagcagatatgcaatcttcaacttaacaaaggaaacaaattcccaaaataaactgaacacaccagactagtgttatgaatgtgcggaaattcagagctcacagggtccgttatgagcaggggagcctgcaaagtattcgcacaattaaaccatatagagacataccgaactgaccactccataataaaagaaaaaaaaaatggccggccattcatcagggaaaaggggggtgaaacctcccatctcatttgtgcaataacaaattataaatgtgtaacaatcaaataattatgcatctgttaataatacaacttatactcacctctattcttggccaaaaaaacacaaattatcacccaaaaaaaaagatcaaaacaaaa

SEQ ID NO: 12 - protein, 382 aa, Solanum lycopersicum
MGEFCRSTIFFSDQHLCYADILPSSQVRARIEVAVLNFLKALSSNSPSISDLSLISRNSSNSRVSRGLLTGDSWIFLSHSFCTRSLTRENSAKSFIRVWKVMEMCYQILVQEKRVTQRELYYKLLCDSPDYFTSQLQVNRTIQDLVALLRCSRYSLGIMASSRGAIAGRLLLQEPDKEVIDCSACGSSGYAISGDLELLEKLTMETDARYIIMVEKHAIFQRLAEDRVFNHIPCILITAKGFPDIATRFLLHRICRMFPNLPVLGLVDWNPAGLAILCTFKFGSIGMGLEAYRYACNVKWLGLRKDDINQLIPEECLVPLKPRDLQIAKSLMSSEILQDSYKEEVAAMIQSGRRAEIEALYCHGYDYLVKFLATKIVQANYL

SEQ ID NO: 13 - DNA, 10939 bp, Solanum lycopersicum
  source 1..10939: mol_type = genomic DNA
ttaagaacattaatcattaaatcagagagacttttattttgcagcacattgcataatcctaccgtttcgccagtcttctgcagatgcatgtaacctcacatgttctggttgagagaaagaggcttgagattagccattaggtgaagtgccaagtgatattggcccgttcagtcgagaaaaatagacttgagattagctataggtgaagtgccaaggggaggatcgacttgagctatggactgattgacatagtttaggaggctaaactaagtctattaaagagagaaatttcaagaaataagtatggcttcggttttattactttgatcaggtgtagctaggctgaagtcgattagtccgagtattaagtgacacttgaattatgtcttcctttgccaatataagataggtccatgaacgggagcgacgtaagcatattagtggtttgtacaagttaaaatcaaatgtcaatataagataggttgttgtctgggttccatataagaatgtgaaatataggtacaactcaagtgtattagttgtatgtccaagtcaaaatcaaatggagtaaatttaaattctactccaaaaatgacaagtttcttttaataattctttcattttatatgaaaactttaatatagtattccatattattatagaaaaataaattataatctatggttgcttaagaaatgaagttctcaaatttagagacgtatgatggatatttttttctttgactacgaaagacacgatatacatgtgaaaatataaacagcaacgaaaatgaaatttataataatgttaggttcgattcgttgttacaaaagaattatggatatgaaagtattggttattcattaatttaaattataattctaaatttgttcgaggctttaagcggcaatataaacacacccgaagcacccaaagttccagatgattgcaattggcgggtatacagtgcgtgcttcttcctctgcatactgcaacttcaatggagatcgaaatctcttctgtgaaaatgctctataaacatgtgattttttttcctcccaaacatagccaccatgcatttctaatccaatttcaacttggcattacttacaatttattcactttactttcactcttcttctacttttgcagctcattttctgcgccgttcaacgatgccgcatgtccgatgaactttgtagattatccgtgaaattgacctcgttttctcgatttgcactcccgctcgttcgaatatcaggcaatatctctctctataagagtgtgtgtttcgtatctgttgtctcaacgtaatgccgtacttctatatatttatgtctatgatggtataagaagatgtgtcatgcgagagtgattcagtttggaaggcgcatggactagttttttctggatttatgaaaatcacaattgcgagtaatttttccttctttctgatccgaaacttttttgtgcttgtaatgggaaaatgaaattgctgtttacataacaatatgcagagttgtaatttgaaattcgagctgcagttcgatttattgtgttaatacagttagcagaatgaatctatgataatgaatcattaaatttttctcaccaacagtttctgatactggtgttgggagcaaaccggaggattaccaatatctgaaatacggagacgatcctactctggctaatcaatggggtaagaaattggcgattacatgcttattaagttttgactctatttttcccaacttatatttctcagagagttatacctgatacacacatagctttggtttaaggttcagtagacacagagctctcatctaaacatatatgtgtctcgtacatatgaaggaaacaagacctcacactaaaagaacttcgaccaacattttaagatatattttttcaccacattgatatgtgaagaattgcaacttataataattttcgtattgtttttgggatatttaaattttaattctaaagtattggtttaatctaatccaatattgttttgaagtttgaagattagtcaaattgactatcaaaaagtgaaaagtgacacatattgggacaagaggagtaacgatctattttcgtgtttaggcacaacaccgagacaattgctcatgtggttccagatggtgcatgtcccttaatccatgactaaaatttattctgaccaactaaaatgctgattaaagtactagaaaacatcactgtctactccatcccttggagtagaagcataatttgatgcacaacttgagatacttggaagttggaacattgttcttcagatttgagctaacagattagggagctgagaaagaggagtatattgtggggtgagatgaaagagaaagaaatatgatgattctaggggaaaaagtaagagaatattcatcaagtgtactggttgcataaatgcctttgttttactcccatggccgccaaacaagaaaaatggaaaacaacataaagagaggaaaaataaataactaacataaaaattcaatttataattttctcaccgcatttcacaggtattgcaactcaagattatgtgtttcggcctttaatgtcgtcctgcctggaagatactattgaaaagccttccatgagtttttttataccacctgttaggagcgctgataatatagtatatttacattgcagatgggatgatttctcttgcaactacaagtaagtcttacccttctaggtgaataattcttttgcctagtcagatttgtcgttaggataaaaattgagaaattttgaaaatagtagtaatatttttgtgatgtatgattgaagttgtatcaataaagtactgtaactacttcaactgtagaggatgaacttcttgcttgccttctgctcctctgaactttgcttcattagttttctaaaactcttgtgagctgagatttgattggtttttccattagtctatggtttggtggcagtttatgcatgacagctagctagtcctgttctttcctttgtactttgagggatttgataatgacctgaagattagaggcagctttctaaagtgcagatacttagaggttgaataacgccacaacattttggttttgctattcgaacagtctcagaaccttgaaacgctaaaatagaaaagaggcattaccaataaagcaactatacattttcttatggtaaattacaacaactacttctcatatgtggagtctagggagggtacaatgtaattccacaagtaaggtctggggagtatagagtgtacacaattcttattcctacctcgtggaggtagagaggctgtttctatgagaccctctgctcaaatacaacaaatcaaaataattatgtaaaaggcagtgtagaaaacaggtcaattaataagcgaagtagtacatactgtccaaagaaagaacagttccaataacgaaataatgcggtaatcgaattacaaaaaagatatatgataacaactatcaaaagcaagaaaaaaaacatgtataagactaatactacaacatacgcgatacttccagactcctgacaagcctaatctcgctgaaaagtgagatagaactcaactacctactaactttctaccctaatccacgatctccatatcctcgtgtcctcggtaagttgaagctgcaccatgtcctatctaatcacctctacagctctacccaatacttcttcggtcaacctctacctttcctcttacccactatatccagcctctcacgcctccttgcatctgtacctctcctcttctatgcccaaaccatctcaggcgttcgcttccctcagcttgtccaccacggaggccactgccactttgtcctggatatcttcaattataatcttatctctcctagaatgcccacacatccatctgaacatcctcatttttctaacttgtatcttgtgaacaatgtaaattgggatcaactgtttactcagaacgtctcatcgctaactcttctctgaatcctggctaatcacgtcttgaatgatacagttccttaaccagtaaattttaatgacagaatacatgatcatctgtgtcaacttcacaaaggttgtatacactaaaaagcggaattgatgcagtttgacagttcatcgaactttatgttggtatccaacttaacaaaaaccaatcaagctcacacaacttgtcttttagcttagggtgatcattatctcctagtaataaactgttggaattgctttggaagaatggcttctggatataattatctttcataatgacaggtttataactttatataagttttacatatataacatatttcttacctttgacaattagacaacgttggaagtactcctatatctcataggattgagaacatttggttgtctaaactgagggatgaaagttgcaggcacatctgatagtgagatacacaatttaaacgtaaatctaaaagattctaattctgctggaagactgacaaagctaccctcaactgcaaagaatggtgccaaattcaggtatgccattttcaggggctccatccatgtgatgctactcttaaattagttttctcttgaccatacccatctagtcttttccttcctttctatgcttctgtctttccgcacatggttaattacttataccttgcagtgggactgaagtatcaatatcaatatccaagagccttgatgacttgttggcagagattacttgctttcttcaaaaggttcattttcatgtctatcagctgattctagctatgatttcctaaattgtatgaaaaattctctaactacagtttttcattgctatctacgcagatgatccttctgaagattccggttagttcattacttttcttgaaatgctttatattcaaatcaaatgcaactatcttctctatagacccctcttataaatcatagctactaactgctcagacagctcaaggcgttcagtgtgaacctactaaatgcaagtgtatatattttggatgagttcaccatgtcaaaaatatttcttttgttaccagattcgcattaaaattcgaaagttttaagcttttatatgtcattttaacctacttctttggccttgttatattttgaaaagcttacctttttccctatcctgtttcctaggagttacctaggagcctaggaccactacctctctgtggctgatggcttgtttctcttcttacagaaagttgtaatggaactcttagtatgtggtgatgatcctttgagttcacagattgaaagtcgtattctggcaattgagggcagctctgcatattctcctattgaaagcatagaaagcttgaaagtgggactcaaggattatattcgcaagcaccaaacttgcttctcaattgggtaagtactagaaaggtgctaggttttggttaatgaatgatgatgcattccaacctctagtttttgttgaaggttggatataatgtattagtaggtctaacttccacatgttgaaatcataattcttaggtgctaatataaaaagataacaaagagtacactttgacatagttaccctgaactttgtcatttccttgttttacatgaactatttcatctactaactttaagctagcctttcattctacaattttcccattaaaaagtgtgacatttgcagttcttctctctttcttatgtggttttgtctgtatgcctgaccgttcattaagctacttcagtgtgatataaagtagtgcattattgttctgaaatatacaatttgtagattttaccttcttgaaatactggttacaaatagttagattgagtgaagatgggaaaaagaagcttgggatacactggaccaggtgagagaaaatcaggatcaaacataaaaggaaatgctagaactccaaccatagaagcagactgaaggaggagtagaggcaagacaattgatcacatgtagcatgcaggaagtagtacttaagttatttaaaatctggttgacagctcaattgactccttcaatttgatgtaggaggatttaagtttgataatgtaatttagttaagatctatttgtggtgctaaacggctcatatggtatatgtaaaattgcagcatctcatataagatctttggagatgtaactgttgtgcagagccaaaaacaaaacgaaaatatcaatgtgcattgcattaaacacggctgtacataaagtcgttgtttcttatttcagggaaaacctgaaggttggaactggggttgctaattcttcagatagttctcagggaaatagccaggtggtggaagctgttgtgattatcaatgagatgtcagaactagttcattcttccagcatcagtgaacaagacatgaaaacagaggtttgctttggattaattgaagaagactcttaaaagcataaaatatgtttgcattccaatatctgctttattaattatgttgtgatcaaatgttagataatagttcactgtaaagatgccatgttgcatattctttcccaacatcttttaacttgtgttttgagttcatttgttgtcctagaatgtgtggattgtgaaaactaatgataatatcacagatatgcattctttgggatttcaactttccgggatcttttatcactatgaatgtcttgttttcatataagcatggtgcacaaggtgaagaaccttgtgcactttatggtgtgtggaggctaagatttatgcaatttcccctacatcatggagtagatagctatttatgtgagtaataactgaaaaatatttttgaacttctgagggccaagaagtggacctttttctttatggccatcttgatgacattggattggatatgttacattacacatacaacaactatgtctcaatcccaagcaagttggggttggcaatataatcctcacggaccatgtggctccatttatgttcataaatagatttacatatcaggaaacaaaattctatgtggaaagtgtgattttcatattgtaatataaaataaactatttcctaaaatctagagtatacccagtgtataccaaacaggatacattaataatccgatcttattatactgtggacaaatatagtctctggtattgagtctaattaaatattgcttattaaacttcgaggatatcaaaagtttttgctaagtgaactatacaagttataggttggctgtcccagccatttctagtccttacagttgtttccaaaagtatacgatggagggggacttaatatctaatctccaaagtaaacgaaatacaagtgaggacacaaaggaaggttttggagaaatcctatttatcagttaagctcacaaaacaggtgcgatgaacatatgaagattccaatatgaatcctcacttactcactaaccttgaccaattccttttttctgtgtcttgattctaaagttagcaaagccaactttatccatgatataaactcctctcactgcttgagggagctcattagcagatatagaaattctgtaagattgtttgatagcttcaaacttagctagcccatcttccatggcattgagttccccttccgtttgtgcttgtcaagatattctggattctggatatcaagtagctttgatggttcactgatgccattgatcatatccactactattttaaagtccatttcgagtagcacattgtaattccattatctggaaacccctgcaagccagcgctagctgcaacacccagcatttctagaacttaaaggaagaagccctaagaaggccatgacaatttttccctgatgacctcttagaacccccccttctccagctagttcccttctaacattgaactgccatcagtgttgagtttgacataattttgagtaggcttgttccactttttttttccgatcaaagggttactatattataatatttaaagattgacagtagtaacaggttcttcgcccgttgccaaggacagatcgttgttaatagtttgggtcatattccgaccctgaataatacaaattgagggcttgttccagttgacagtaatacaagtgagctttggcttaagttatacactaatcacaaacctccctcctgttggagtttaagttaatcaaccccaagatctttgaaatggcaatattcagattaacaaaatatttaagcaatttttttaaaaattaagttccatatatctgttgatgagctgctgttgaagtttttaaaaatttatcactaagcattacttgctcgtcttctttcagttaagccagcatcttgcacgccttcacattttcttttcagtattgtagtttgtttgtgtttctttaatttgtattaatgatcttctatgcctgatttcagatcttatatttcaaagactttgtaccttgttctattgctccgtcatccctcgatgcattcacaagcatcaactggaaaagctatgggttggctctgcggagtgttgcagatcatgatgatagtgtaatgctggaatgggagaacctggcaccagatttacaaattcatattgccatccattgttaccatagaaaatatccatcataatataatacatatccatgagaattgacatggtcatacactcttagcattaacttcaaacaatgagtattgtcttttgcttaacttgctgacaaggtgaaacagtgggttgcagaaagcagttcacctgatcgaaatctagctagaaaagctatcaagtgtgctttggatgacttgaaagaaaataatcaaggggttctcctaagtacacgtgcacttaaggtaatgttttcactcttctttgcattctttatggtcattggattttctagttcctggtattggcttggctatgaacaaaatacctcccgttgttcgatctattctgcattcttatacgtccatacccaattgtgaagcagaaaaagtagttttttcttcttcttcttcttcttcttcttttgatacggatttttaaagagtgctaagcagacagcattcagtaattccagttggctaggtaattcacatacagaaactaggcatgctgtggaattaacattctttagaccatatgactagtgctgattgaatctgaataagggatgacaattattcaaacataaataagagcatcgattggcaagaaatctattctcattgcctcattggggatgaaagcttcctagaaaaaattctcctttttactgggaatggcttttacagcatcatctatttagcaccgttgttccaggttgtcagatatatagcatttttattagctggaagtgcatatgctttcatatgtttctgcagaatccttttaaattcagtacccatatccatggtcaggggcgtacgtagtttgacagtagctaatgtatccgcaacctctatatcccagacatttgctatatatttgaatagttttgtatataacttagcaataggtgcaataggatttccacatgaaccaatttaaaatctcgatacaccttctacctgattatgatcttgtttgagcttgaaatggccaaaatttcagttttccttcgcgtacatagctaaggttctaaatttgtttctcccacagacctgtgattatgcacctgaccttgcaaaaacgcttgctcacctgatcttttcctccaatgacttgaacttccaagaagaatgttgttctcttctcggggtacagtctcaagaggttaacattaataatattggaaattgcatcagggagaagattatttcagtcatcggattaaatgatcgtaactcccataagcataaagaagccccaaccttcctatttgacgatgattgtttccagaaagaggatttcatggacgaggaatatcaagaaggtttagaatcttacaactctttggatctatagaaggttaggagcattattagatgtccaattattaatctcttctctaatatgtttatagtttacctcacaatcaaattattctagttacttctgcttggctttattattgctatggaaaagggtaagttgaattttttggtccaaagtagataaactgatactcaattatttctacaacgttgtggtgaaaaagagaatatatatattcaaaatttcattctctcagttttttccatgttagtgaaatatctaaggattcattttgtcacagattttggaagtatcttgtagaattattatctttagtcagaaatcatctagtttttgggagatcagttttcaaatctcaaaagctacttcaaacttgtttttgccccaaaatcttacattttataaaagtgccccatcgattacttcagatttattttgcttgatttgtatactaatattttcttaagaattgtaaacccttgtcaacatatatgtgatttttcatctcctaccttgaatactacttgcttataatgaagtcattaaaaatattctgtataatttggaaataatatgtttcatttctgtctttcgactaatatctcattactaactcagccttgctgctttgaaaattttctcgtataataattaatatcagcctaagataaattcttttccttgaggcttgaagcacttgagatctttggcttcttccattcatttttttggacctcgcatgttcttaagatataattactagtgttagtattttatcacaaatactcatataaattggtgtatagttttttgtcttaagaaatgatttggaaataaataattgtattatatatttttaaaatattagacaagtaaaaatgaatggagaaagtattttttcgcttaaaaattagtgaaagaatacatttaaaaatttggtaaagttcttcgttgatataaatttccaaaagtgaaaagcacacaaatcgcaatgaaacagtcaaagtcg

SEQ ID NO: 14 - DNA, 2499 bp, Solanum lycopersicum
  source 1..2499: mol_type = other DNA
gaagtgccaagtgatattggcccgttcagtcgagaaaaatagacttgagattagctataggtgaagtgccaaggggaggatcgacttgagctatggactgattgacatagtttaggaggctaaactaagtctattaaagagagaaatttcaagaaataagtatggcttcggttttattactttgatcaggtgtagctaggctgaagtcgattagtccgagtattaagtgacacttgaattatgtcttcctttgccaatataagataggtccatgaacgggagcgacgtaagcatattagtggtttgtacaagttaaaatcaaatgtcaatataagataggttgttgtctgggttccatataagaatgtgaaatataggtacaactcaagtgtattagttgtatgtccaagtcaaaatcaaatggagtaaatttaaattctactccaaaaatgacaagtttcttttaataattctttcattttatatgaaaactttaatatagtattccatattattatagaaaaataaattataatctatggttgcttaagaaatgaagttctcaaatttagagacgtatgatggatatttttttctttgactacgaaagacacgatatacatgtgaaaatataaacagcaacgaaaatgaaatttataataatgttaggttcgattcgttgttacaaaagaattatggatatgaaagtattggttattcattaatttaaattataattctaaatttgttcgaggctttaagcggcaatataaacacacccgaagcacccaaagttccagatgattgcaattggcgggtatacagtgcgtgcttcttcctctgcatactgcaacttcaatggagatcgaaatctcttctgtgaaaatgctctataaacatctcattttctgcgccgttcaacgatgccgcatgtccgatgaactttgtagattatccgtgaaattgacctcgttttctcgatttgcactcccgctcgttcgaatatcagtttctgatactggtgttgggagcaaaccggaggattaccaatatctgaaatacggagacgatcctactctggctaatcaatgggatgggatgatttctcttgcaactacaagcacatctgatagtgagatacacaatttaaacgtaaatctaaaagattctaattctgctggaagactgacaaagctaccctcaactgcaaagaatggtgccaaattcagtgggactgaagtatcaatatcaatatccaagagccttgatgacttgttggcagagattacttgctttcttcaaaagatgatccttctgaagattccgaaagttgtaatggaactcttagtatgtggtgatgatcctttgagttcacagattgaaagtcgtattctggcaattgagggcagctctgcatattctcctattgaaagcatagaaagcttgaaagtgggactcaaggattatattcgcaagcaccaaacttgcttctcaattggggaaaacctgaaggttggaactggggttgctaattcttcagatagttctcagggaaatagccaggtggtggaagctgttgtgattatcaatgagatgtcagaactagttcattcttccagcatcagtgaacaagacatgaaaacagagatcttatatttcaaagactttgtaccttgttctattgctccgtcatccctcgatgcattcacaagcatcaactggaaaagctatgggttggctctgcggagtgttgcagatcatgatgatagtgtaatgctggaatgggagaacctggcaccagatttacaaattcatattgccatccattgttaccatagaaaggtgaaacagtgggttgcagaaagcagttcacctgatcgaaatctagctagaaaagctatcaagtgtgctttggatgacttgaaagaaaataatcaaggggttctcctaagtacacgtgcacttaagacctgtgattatgcacctgaccttgcaaaaacgcttgctcacctgatcttttcctccaatgacttgaacttccaagaagaatgttgttctcttctcggggtacagtctcaagaggttaacattaataatattggaaattgcatcagggagaagattatttcagtcatcggattaaatgatcgtaactcccataagcataaagaagccccaaccttcctatttgacgatgattgtttccagaaagaggatttcatggacgaggaatatcaagaaggtttagaatcttacaactctttggatctatagaaggttaggagcattattagatgtccaattattaatctcttctctaatatgtttatagtttacctcacaatcaaattattctagttacttctgcttggctttattattgctatggaaaagggtaagttgaattttttggtccaaagtagataaactgatactcaattatttctacaacgttgtggtgaaaaagagaatatatatattcaaaatttcattctctca

SEQ ID NO: 15 - protein, 471 aa, Solanum lycopersicum
MEIEISSVKMLYKHLIFCAVQRCRMSDELCRLSVKLTSFSRFALPLVRISVSDTGVGSKPEDYQYLKYGDDPTLANQWDGMISLATTSTSDSEIHNLNVNLKDSNSAGRLTKLPSTAKNGAKFSGTEVSISISKSLDDLLAEITCFLQKMILLKIPKVVMELLVCGDDPLSSQIESRILAIEGSSAYSPIESIESLKVGLKDYIRKHQTCFSIGENLKVGTGVANSSDSSQGNSQVVEAVVIINEMSELVHSSSISEQDMKTEILYFKDFVPCSIAPSSLDAFTSINWKSYGLALRSVADHDDSVMLEWENLAPDLQIHIAIHCYHRKVKQWVAESSSPDRNLARKAIKCALDDLKENNQGVLLSTRALKTCDYAPDLAKTLAHLIFSSNDLNFQEECCSLLGVQSQEVNINNIGNCIREKIISVIGLNDRNSHKHKEAPTFLFDDDCFQKEDFMDEEYQEGLESYNSLDL

SEQ ID NO: 16 - DNA, 8325 bp, Solanum lycopersicum
  source 1..8325: mol_type = genomic DNA
gcaaactcggtgacgtcggaaagatgattaaattatttttaatttgatatatcatgggtcacctaattcatttggtgctaaaatatttgagcgtctgaagttgacccaatatccatttttctctaatataaatgttgaccctcacctatggccaaacctacagtccataggtccaaccatggattgtactagttgaccgtgggtgggatcagagaccatcaaactctggactccaacgacgaaaccaatctatggttcatgggtccatcaacggaccgtggaccatggttgtatgtgttatctttacatcctaattttttcgtaagtctgaaactgaaccacgagatcccacctacgatctgggatctgacacacggttcgtcgatgactttcgttgattcaaacatcagatattaaagagctgtaatttttcatcttctcaaattaacagtgttacaaataaaatttaggcggagtgtatctattctcaaaaagttcaacaaccatgtgtacaattagtgaatgaattcatgtttcttgtgtttatcctttttcttcttttctctatttaaaaaagatcgattttgtttttcttttaatttgtttataaaaaatatctttttcttcttttctctatttaaaaaagattgatttgtttttcttttaatttgtttaaaaagaataatttttttctgtaatattttaattttaattttttatttgacaagtttaagagtacaatagggcaatccactatcatatcaaaattataattttctgtagagaagtccagatttttccaatgtaacttgctaaaagagaaattttataagttcaacataactttattattattattattttttttatacatatttggaatttgaaagcagaaggcgtcaaagattttttctcccgctttgctatccatcccacaccttctccatcgcactagccagtctcttcactcacgcacacagtagtactacagcaacaaaatatgtatttcgccacttctcaactcccccactcaccaccgtcgccatcgctggaaccaccgttaacatgcgcacaaggccatagctcgactttgattatcccaactgatgaaggaggatcaatttgtctgctctgcttgtctaatctcatttccaatccgagatcgccgaccgttcacgtgtcctatgctctctctcagttatctatcgcgcttttccaaccgagtttccgccaaaccttcttcacattccactctcatttcctaatctcgcctctcgtcggtgttctatcttccttctatgatgaacccatagccaagcaaactatggatttgattatgcagttgtgtgaagctccagactgcgatgtgcatgcagagtttgtggctcggctagcagatcgcctttccagcggctctttagcttggagtcagagacagctccactcggtaacttttccctctgtactaactcttaaatttccaatttatggaggtgtaatttagaagggagctgtagaaggtatagttacatagatatagccttacatgatacaacatatactcctacaatcaagtgatttattaatttgcatagaagtgtgtcactctaaaatggactaataaggaaataaaagtggaactgagttaagtatctgatttttctaatttcctcagtgtccttcagcattgtgcaactttgttctgtggcatacagccgactgtgatcagtaaagctttcagcactgaaaatgatcttgaagatcctattaaaatttatactaagaacaggtttagcattatagctatattgctcactcttcaatcctataatcaaatatagcttttatagtagcttttccacagttatttggcactgctttcagtttcagtgagtcaatgacattgactaacagcttaagtttagtcaccgacactgttgcagatttgattggaaaatcacagtcagaatgattcctgagaaaatattagttttatccagagcagtgagtaaagcttaaacctgcttaggtagttatttcaagtttcaatgccagtgttcaagtccataagaagacttgtggaggaaaacacttatacgatgttacaaaataagcaaataaaagatgggaggaactgtaaatgattttgaatttgggaaaaatttgagttgcattgtaatgacaccaattatatgtttcctcatgatgattcacaacctttttagagtagcttcacattctattcggttcatgtttgctgctgacgtctatgaacaaattgctcattttggagatggtacactgtatgtaattgattttctcattgagaagctataatgaacaagaaataggaagaagttatacttagtggttctgtcttggtatcattggcctgatatctgtcaaatacacattggattttaatgagataactcagccttcaatttgcacagagaatttgtagtttctatatttatttctgtatttgcagtgacatatgttttcctctaatacatgtaatctgacccttttttttaaaaaaaaaagcttcactgcttaggtcttctcttggattaccaaaaaaaccattcctattgtctcgaagaaacggatgccctcattttcaatctcgtcagtggccttcaattgtccaggtgactcttgaaactgagacagtggctatctcattttgccttaaacaaagccctgaaggtcaattccttcttgagtacagtgaagatattcagggggaaatcctgtttgttctatacaaattattcctactcaatgggtctcaagatggtgaagatcctcctagtttatttggtcatttctcgaagctcctacacttagcactggcagttctgatgaaagctcaaagtgatgatgttcgcttaaactgtataggtaagcttctttcacattaccggtttctgcttcttgagcatttgcatctctgaatttgattttccagcgaatatcttgacagttaaccattttatacttggattattgcaaaataagaggagtatatggtgataattgactaatttatgatatatttgacaagtataccagggaagtatggttgctaaaaagcgagaatgcattataggaatagccatatatctccttgagaaatcatttgaatgtagagattttgtggctcttgagcctaatgttgtggtaaacaggctccataaatctgttcacacctcggatatactctgactgataaaaagttttgcgtgtatatttgctgctgacttgactagcaaagttctatgcactcttcaccagagctctgattatctctctcttctcccctcccttcccccaccattcccataaggaaaaggagataagatgctgctgatgttggagtttctgcaagataatctcatctctcgcatttgtcaaatcagtgatactctttgtttatgcagcattcttaacagtaatgatgcaaagaggattctttcaaactacttctataattggcacaaggagcaggagttgttatgatgttgaccacttgatggaaacaaatgagcagatatcagatgggcctctagctatcttgtttgcagaggcagtcaaaggccccctgctttcttctgataatcaagttcaaatagcagcgctagatttactttatctttatctgtcgaggaaagatgtcttagaaaatgaaatccaagtatttgttgaagagaacattgcagactatgcgtttgaagtgctgaggttgtcaggtaagaatatcagctatacacagtgtctgagcagttagatttatacgtattagttttggttgaagaaatgaaagatgaaagagggcgtttcagtcgcactctattctatttgtttttccgtttacaattaaactatcttgaaacgaccacttctctggcgattacagtttctacaataaacaaattaccatgggtacaatgtttgttgtccatatggttcgacaagatctaagttctctaacgacaatcagctagagaacattctaattatattaggtcagattatgcaattaatgttgtctataatgactaatgaagtaactcattagtttgcaggatgcaaagacccaacaattaaatcttgtattcagcttcttgatattttagcaactgctgagcaagcatttaggcagagacttgcaattgggttcatggccctgattccagttctgcatcatgttgctgaaattcccttccaccctgtacagactaagacactcaggcttatttggaactctgtggagaactgcccaggggtggtatccaagtctcaggtagaagaaataagcctttcattgacaggaatgctcaagaaaaatcttgacggagaaataggcatgcttccagaaacattagctctggtctgttcaatatttgttgcacttatgaaatgttcatctacctgtgggatttcaagtttctcactatcaattcaggatgcatcaagaaattgcatcttaacttgtttaattaattatggcaaatacccgggtcaacttttgaactctctttacctactgaaagaggcatattcatatagtgttgggatgaattcctcaagctcaatgaacacagatcttagaagaagcattatagatgtatgcaaaacacatatattaccgtggtttatgaaatcccttcatgagatggaagatgaggatattccagctgcaatacttgaaaatttctattccatattgctacaagattcagacaccgaaaccaaaatatttgcaaatgttctgctcacatcttcctggttcagttttgcatatggatgtttaggccttttcccttctgaaaagatgaaaaggaatgtttatcttatctttagtgtgatgacagatatcattcttggggttgattctgcgcgatgcattagcgatgctgctccacatcttccatctgatcctatagatttgcttttccttttgggccataaaagctcccaaaatgttgaattgtcttctcggcaactggcagttctgttgttactgtacatcagctcactgtatgacgatcggtaaatagtttctgggatcttaatcttactctttctgcattttccctgcttatgttatcagtcctcagttgatcatctcaccccttttccagaattgcagatgataagcttgtgttagcttcattggagcaatatattctactaaacagcagcgaaaacatgcatggagcttctgttttgggaatatttataaatctttatgcactatacagaggtttagccaaggtgagctaccaaatcccctacagcccagaggctgaaaggattgtgttccacctacttgcggaaaagggctgggatttgctatctacgagaatccacgtaacatctttgaaatggttgttccaacaagagaaaatctgcaacgtgctgtctgcccagattttgaaattttgcagatgccattgctccaacataaaccagataaatatccatggtgaagccaatcagaagatagatgtgtatgttatgacagaacttgtagctttgggggataactttgtaggtacgctcatggtgtttctattgggagaggctggagaacaatattccgagtatgacgttgtttcactggtgaataccataaaacgtataatagaaatctcaccaagtacttcagatcaattctgcttgcacgggatagctactgcaattaagaacctttactataagtttggtcattctttatccccagatactttcatgtcaatctccgaactagtatcctacattcttcaagcagtacactctgaatccctctctgatgatgaatcctgggttgcaattgtggtgaaagtatagtactgactcttctaaatactgtttgctcacagttcctctgtagtaaatagacttttccttgattgcagattatcgactacctgatcccctcagtagctgcagatggatggacaccgggaactcttatatcaattggcattctttctatggttttgcatcactcagtgaatcaagtgatggttgaagcttcgaaaaccataatccttagtactcatatgctatcattggttaataccactatcgccaatgcctgttccaaaggaccttcacttcttgaacaaaacgaaggagcaagatctgtagaagctcttgtttttgtgctttcacttcttttcttctctttgagaaggtatcagttcctttaacataggttctatgctttcttttattttgttttttattttgaatctaatagcttattttgctagtgcgcatgccattttaccggggattatggacttccaatatctgctggatcctaccaacataccgcaaccctggtcttatattagtatacagtgccacgatttgtgcaagttattgcattttggatctattcctattaagttacttagctcgcaataccttctggagttattcagtggaatagaagacgagaaaagtagaaaatcagacacattagaattcagaactaattatttgacgtctataatggctgttttagaaggccaactattttcaagtgacatgtctgtagcaatgaactgttccctctgtttgtctatgctcattgggtggcaagatgtggaaacagaagtatcagctatacaaaggaacaactggtgtcggtttatagtagaagaattagtgatatccttggcagctccatctttggcttcaaaatctttcatgatccatcacaagcctgcaattcatattgcagttgaactgctgagaagaaagaaagttctccaatggatgacttcaatcttcgatgaatcttgcatatttgccattactagaaacattacaaattctaatttgagcgctgaattggtgttcctcttaaggaagttacttaattatggttttctgaatgatgaacaaattgctgctctaaatcaagtattccaggtaatagatactttatctttgaaagatcattggttcctattgtgatctggtgtcatgaagcttgcttttagaaaaaaagaagaagagaacactgccaaaatgaaataatggaattccgttattattgtgtttgcctgcaggaatgcagaaaatgtatctacacagacaaacttcaacatgctggggcagaggagaagacatggaacgtagcagctgcttcagattatgtaggtaaagtttgtcagtttctcattagcctcgtaacgactcagccatctagtggtatggagtcttcaagatttcaaagtgagaaaagggaattgctggaagaaatagacttattttcaaaatgtttaatgagggaagattgagcatgcaccactaaagttaggttttgcagagtatcatatacgttcttttcgaagaacaattcagatattttcctgttttgtcactcataaactaaaaagagcagtggcatctgctagtataatcctatatctgtcaccaaaataaaattaaaaaagtcttccgtttcattggccacatacaaagcactgccttagtaattctactttttgtgcatcaccaagttctacatattttctttactctttgttttgttattccaaaagagggacaaagaaaatgggaaaaaagcagttgagctccccaaattgattggtagaagaggtcctttcttccttgagaaacatttgggctggactgggcaggcccatcgttgtggcaaagcaagcctgagatcctaggggctaggccctagcattaagcaaacaaaataattccttgatacatgttgttggtttttcttgaagtgtacataggaatcgctaaataattgatgggacatattactttctagtttctcccacagacgtaatagttcctcccatctcagcattataaaactcccttgcatgaaaaagatagcccaccatccaataatttaatacaccttttactatatatacttgttgtcctaacttgtacatttacgaaggctaaagaaaatgatcaaagagatatgggatggaggacccccactcactcgacctcaaacttggggacccttccagtacttattgtataacgaatttatcagggtgccgtagaagtggatggacattgtcttctacttagaattatttgttatatacaaatgaacaattatgagtacaatgacaatctacattcataaaacaaaaaagaacacaacaaatgaagtttcctccttcataaatcatgcatgagatgagaaacatgataaaaaggcagaggatttgcaagagggatgtggtccctgtgagagggaggttatcttgttaaatcatgaaaagcaacacccacgtc

SEQ ID NO: 17 - DNA, 5352 bp, Solanum lycopersicum
  source 1..5352: mol_type = other DNA
tttttctgtaatattttaattttaattttttatttgacaagtttaagagtacaatagggcaatccactatcatatcaaaattataattttctgtagagaagtccagatttttccaatgtaacttgctaaaagagaaattttataagttcaacataactttattattattattattttttttatacatatttggaatttgaaagcagaaggcgtcaaagattttttctcccgctttgctatccatcccacaccttctccatcgcactagccagtctcttcactcacgcacacagtagtactacagcaacaaaatatgtatttcgccacttctcaactcccccactcaccaccgtcgccatcgctggaaccaccgttaacatgcgcacaaggccatagctcgactttgattatcccaactgatgaaggaggatcaatttgtctgctctgcttgtctaatctcatttccaatccgagatcgccgaccgttcacgtgtcctatgctctctctcagttatctatcgcgcttttccaaccgagtttccgccaaaccttcttcacattccactctcatttcctaatctcgcctctcgtcggtgttctatcttccttctatgatgaacccatagccaagcaaactatggatttgattatgcagttgtgtgaagctccagactgcgatgtgcatgcagagtttgtggctcggctagcagatcgcctttccagcggctctttagcttggagtcagagacagctccactcgcttcactgcttaggtcttctcttggattaccaaaaaaaccattcctattgtctcgaagaaacggatgccctcattttcaatctcgtcagtggccttcaattgtccagtgaagatattcagggggaaatcctgtttgttctatacaaattattcctactcaatgggtctcaagatggtgaagatcctcctagtttatttggtcatttctcgaagctcctacacttagcactggcagttctgatgaaagctcaaagtgatgatgttcgcttaaactgtatagcattcttaacagtaatgatgcaaagaggattctttcaaactacttctataattggcacaaggagcaggagttgttatgatgttgaccacttgatggaaacaaatgagcagatatcagatgggcctctagctatcttgtttgcagaggcagtcaaaggccccctgctttcttctgataatcaagttcaaatagcagcgctagatttactttatctttatctgtcgaggaaagatgtcttagaaaatgaaatccaagtatttgttgaagagaacattgcagactatgcgtttgaagtgctgaggttgtcaggatgcaaagacccaacaattaaatcttgtattcagcttcttgatattttagcaactgctgagcaagcatttaggcagagacttgcaattgggttcatggccctgattccagttctgcatcatgttgctgaaattcccttccaccctgtacagactaagacactcaggcttatttggaactctgtggagaactgcccaggggtggtatccaagtctcaggtagaagaaataagcctttcattgacaggaatgctcaagaaaaatcttgacggagaaataggcatgcttccagaaacattagctctggtctgttcaatatttgttgcacttatgaaatgttcatctacctgtgggatttcaagtttctcactatcaattcaggatgcatcaagaaattgcatcttaacttgtttaattaattatggcaaatacccgggtcaacttttgaactctctttacctactgaaagaggcatattcatatagtgttgggatgaattcctcaagctcaatgaacacagatcttagaagaagcattatagatgtatgcaaaacacatatattaccgtggtttatgaaatcccttcatgagatggaagatgaggatattccagctgcaatacttgaaaatttctattccatattgctacaagattcagacaccgaaaccaaaatatttgcaaatgttctgctcacatcttcctggttcagttttgcatatggatgtttaggccttttcccttctgaaaagatgaaaaggaatgtttatcttatctttagtgtgatgacagatatcattcttggggttgattctgcgcgatgcattagcgatgctgctccacatcttccatctgatcctatagatttgcttttccttttgggccataaaagctcccaaaatgttgaattgtcttctcggcaactggcagttctgttgttactgtacatcagctcactgtatgacgatcgaattgcagatgataagcttgtgttagcttcattggagcaatatattctactaaacagcagcgaaaacatgcatggagcttctgttttgggaatatttataaatctttatgcactatacagaggtttagccaaggtgagctaccaaatcccctacagcccagaggctgaaaggattgtgttccacctacttgcggaaaagggctgggatttgctatctacgagaatccacgtaacatctttgaaatggttgttccaacaagagaaaatctgcaacgtgctgtctgcccagattttgaaattttgcagatgccattgctccaacataaaccagataaatatccatggtgaagccaatcagaagatagatgtgtatgttatgacagaacttgtagctttgggggataactttgtaggtacgctcatggtgtttctattgggagaggctggagaacaatattccgagtatgacgttgtttcactggtgaataccataaaacgtataatagaaatctcaccaagtacttcagatcaattctgcttgcacgggatagctactgcaattaagaacctttactataagtttggtcattctttatccccagatactttcatgtcaatctccgaactagtatcctacattcttcaagcagtacactctgaatccctctctgatgatgaatcctgggttgcaattgtggtgaaaattatcgactacctgatcccctcagtagctgcagatggatggacaccgggaactcttatatcaattggcattctttctatggttttgcatcactcagtgaatcaagtgatggttgaagcttcgaaaaccataatccttagtactcatatgctatcattggttaataccactatcgccaatgcctgttccaaaggaccttcacttcttgaacaaaacgaaggagcaagatctgtagaagctcttgtttttgtgctttcacttcttttcttctctttgagaagtgcgcatgccattttaccggggattatggacttccaatatctgctggatcctaccaacataccgcaaccctggtcttatattagtatacagtgccacgatttgtgcaagttattgcattttggatctattcctattaagttacttagctcgcaataccttctggagttattcagtggaatagaagacgagaaaagtagaaaatcagacacattagaattcagaactaattatttgacgtctataatggctgttttagaaggccaactattttcaagtgacatgtctgtagcaatgaactgttccctctgtttgtctatgctcattgggtggcaagatgtggaaacagaagtatcagctatacaaaggaacaactggtgtcggtttatagtagaagaattagtgatatccttggcagctccatctttggcttcaaaatctttcatgatccatcacaagcctgcaattcatattgcagttgaactgctgagaagaaagaaagttctccaatggatgacttcaatcttcgatgaatcttgcatatttgccattactagaaacattacaaattctaatttgagcgctgaattggtgttcctcttaaggaagttacttaattatggttttctgaatgatgaacaaattgctgctctaaatcaagtattccaggaatgcagaaaatgtatctacacagacaaacttcaacatgctggggcagaggagaagacatggaacgtagcagctgcttcagattatgtaggtaaagtttgtcagtttctcattagcctcgtaacgactcagccatctagtggtatggagtcttcaagatttcaaagtgagaaaagggaattgctggaagaaatagacttattttcaaaatgtttaatgagggaagattgagcatgcaccactaaagttaggttttgcagagtatcatatacgttcttttcgaagaacaattcagatattttcctgttttgtcactcataaactaaaaagagcagtggcatctgctagtataatcctatatctgtcaccaaaataaaattaaaaaagtcttccgtttcattggccacatacaaagcactgccttagtaattctactttttgtgcatcaccaagttctacatattttctttactctttgttttgttattccaaaagagggacaaagaaaatgggaaaaaagcagttgagctccccaaattgattggtagaagaggtcctttcttccttgagaaacatttgggctggactgggcaggcccatcgttgtggcaaagcaagcctgagatcctaggggctaggccctagcattaagcaaacaaaataattccttgatacatgttgttggtttttcttgaagtgtacataggaatcgctaaataattgatgggacatattactttctagtttctcccacagacgtaatagttcctcccatctcagcattataaaactcccttgcatgaaaaagatagcccaccatccaataatttaatacaccttttactatatatacttgttgtcctaacttgtacatttacgaaggctaaagaaaatgatcaaagagatatgggatggaggacccccactcactcgacctcaaacttggggacccttccagtacttattgtataacgaatttatcagggtgccgtagaagtggatggacattgtcttctacttagaattatttgttatatacaaatgaacaattatgagtacaatgacaatctacattcataaaacaaaaaagaacacaacaaatgaagtttcctccttcataaatcatgcatgagatgagaaacatgataaaaaggcagaggatttgcaagagggatgtggtccctgtgagagggaggttatcttgttaaatcatgaaaagcaacacccacgtccctgtgtcccctttagtccttttattctcatcctgccccttactgaacaaatagatttagcttatctatacagcagtcagaactactgataaatcattaccttatatatgtattaattaataagctcatgatttcagggtctttttgggatgaa

SEQ ID NO: 18 - protein, 1294 aa, Solanum lycopersicum
MYFATSQLPHSPPSPSLEPPLTCAQGHSSTLIIPTDEGGSICLLCLSNLISNPRSPTVHVSYALSQLSIALFQPSFRQTFFTFHSHFLISPLVGVLSSFYDEPIAKQTMDLIMQLCEAPDCDVHAEFVARLADRLSSGSLAWSQRQLHSLHCLGLLLDYQKNHSYCLEETDALIFNLVSGLQLSSEDIQGEILFVLYKLFLLNGSQDGEDPPSLFGHFSKLLHLALAVLMKAQSDDVRLNCIAFLTVMMQRGFFQTTSIIGTRSRSCYDVDHLMETNEQISDGPLAILFAEAVKGPLLSSDNQVQIAALDLLYLYLSRKDVLENEIQVFVEENIADYAFEVLRLSGCKDPTIKSCIQLLDILATAEQAFRQRLAIGFMALIPVLHHVAEIPFHPVQTKTLRLIWNSVENCPGVVSKSQVEEISLSLTGMLKKNLDGEIGMLPETLALVCSIFVALMKCSSTCGISSFSLSIQDASRNCILTCLINYGKYPGQLLNSLYLLKEAYSYSVGMNSSSSMNTDLRRSIIDVCKTHILPWFMKSLHEMEDEDIPAAILENFYSILLQDSDTETKIFANVLLTSSWFSFAYGCLGLFPSEKMKRNVYLIFSVMTDIILGVDSARCISDAAPHLPSDPIDLLFLLGHKSSQNVELSSRQLAVLLLLYISSLYDDRIADDKLVLASLEQYILLNSSENMHGASVLGIFINLYALYRGLAKVSYQIPYSPEAERIVFHLLAEKGWDLLSTRIHVTSLKWLFQQEKICNVLSAQILKFCRCHCSNINQINIHGEANQKIDVYVMTELVALGDNFVGTLMVFLLGEAGEQYSEYDVVSLVNTIKRIIEISPSTSDQFCLHGIATAIKNLYYKFGHSLSPDTFMSISELVSYILQAVHSESLSDDESWVAIVVKIIDYLIPSVAADGWTPGTLISIGILSMVLHHSVNQVMVEASKTIILSTHMLSLVNTTIANACSKGPSLLEQNEGARSVEALVFVLSLLFFSLRSAHAILPGIMDFQYLLDPTNIPQPWSYISIQCHDLCKLLHFGSIPIKLLSSQYLLELFSGIEDEKSRKSDTLEFRTNYLTSIMAVLEGQLFSSDMSVAMNCSLCLSMLIGWQDVETEVSAIQRNNWCRFIVEELVISLAAPSLASKSFMIHHKPAIHIAVELLRRKKVLQWMTSIFDESCIFAITRNITNSNLSAELVFLLRKLLNYGFLNDEQIAALNQVFQECRKCIYTDKLQHAGAEEKTWNVAAASDYVGKVCQFLISLVTTQPSSGMESSRFQSEKRELLEEIDLFSKCLMRED

SEQ ID NO: 19 - DNA, 6492 bp, Solanum lycopersicum
  source 1..6492: mol_type = genomic DNA
gtttgttttttccatcgtagctagccaaactctctatcttgcggtacaccactctcttcctacctcactgaggtttttaggtgtgtaagctcgcactcaaaagtcttttggagctattacttgactgattccgctttatttgatataacgtaattttattccatcgtagttagccatgctctatttgatatatcgtttgtttattccatcgtagttagccaaactctctatctcgcggtacaccaccctcttcctacctcgtaggatttcactgagtttttaggtgtgtaagctcacactcaaaagtcctttggggctattacttgactgatttcgctctatttgatatatcgtaattttattccatcgtagttagccaaaggagattcataagtaggatcaagttgtccttgttgtgctcctttaatatgagtacaatttaatgtcgataaccaaataatgcattggttatgcagtatcattttctcctatatgattcaccaacacctatattaatatataatattataattttcaactcgttcaactaaatacttgtattatttttgtatgttaaaatttatgctggaattattttctcaaatagagccaccatatttaacgatcgaagtgcataaataaatactccaattattgtactatgaatattcgttttactcaagacacaagtgcttcagttacttttacttgtactttagagaaatatgatcaatttgactattttgtgcgtgaataacgtccgtatgtacttaaaatttagtcatttataaattattacatttttttcaaaatgaattaaacgttcaaatcacatgtgaagttactctaaaatgaattagaatttaaatttcgtttaaatatgatctatgaaaacattgaactattatgtaactaagcaaacgtattatactaaaaagactttttagtacaaaacccaaaaactcacgcgagtcccgccattaaccacagtgtgagagaaatggagattttgagagagcaaccgaagagccactccgatgaatcgttcaaactcgccatcgcaatggcactcgtccgatcaaagcttcttcacaaaccgccggcagcaacaccggttccgccttcttcctgcccgcctctttctcattccgatgatgctgttaaatggaaacaaaaagttcgatcaatttcctttaattccttcgttttcctatttctattatcagttaattaactttcattttcaggcaaaagagcgtaaacgagaaattctcaggctcaaggaggatctcaaagtagccgaaggttagtatttaaaattttcgttatagtttaagctagattttttaagtttattgctattttaaaggcttaaattgaaatttttgatgatcaccgcaatttcgttaggatctgttattatgtgatccaattcgattggaaaataacaatgtgtagttatgaccatctaggttttacatttttgatcatcttgctatgtatattaatcaaaattgaatgataagaaggataaactgaggattttttgttgtgtgtttgattttgatttactaatgtgttgtttgtataggtagattcacattgatcggctattttgttttgattatttttactttttttccccctggagtaagatggttcacagtgtgatatatttccaaaaaatgcatcatgcaagtgttatttctttgataagttgggattattgagtcctaagaaaattggagctggttctgaccaacggttcagtgatgtgttgcggagaagatttcttagacaaggtttggcatttttttgaatgctgttgtatttattggtctaaagttgtcaattcggccttcatatacattagctgtattcatttacttgtatatttttccagtgaggattaaggagagaaagaggagaaggccagatgattctttgcttcaccgaatttcaggtgaaagttcagttagagatcttcttatggatctaattttgtctttacttttggtggttaacttgcaaagtctcatgatttttaaaagttacattgagttgagatcttatcatacctcagccatgctctcatttactacgtgtgctgtactttgatctctggaaaaaactaggtcctatttgcatttgtctgaacatgaattttcagctatagatgagaagtatgaagattatgtctttttcttaaatggcagattgtgacaatgataataatattgagcaactgagcgcttcagttgattttcttttggaactttgtgacactatttctcttcacagcgtatgttgtttctattaacccaagctagtgatgctttgtcttatgttatgaatatgatttccatgtatcttttcacttgctattgttctaaatctgtaacagttggaggagggtaattttaagaactggtgccaccaagctgtggactttattattggtaatgacacaatattttcatttcctttgccttcctgtgtacagttttttcataagcaacatctgaaaattttaaacttgaattcctgatatgcttttttatttgtaatatgccaacgattaatcatatcacagatgaactgttattttctaatctctagtgtcgaggattgtgatacaagctgtattcaaggggttagtaagtgcatgtattatctgttctgaaacttaaatgaaaaaaggattgtctactgaagcttcattctggatttgggtgttcatggaaagattgctccaaaggacttcactttgagaaccatcttcatggttcgtactgctattttgaatgaagctttctaatttttacttgaaaatgcaaaaggttcaccatttagccttctttgtcaacaccttgttatgcaagtactgaaccatttcactgcatagaatgccttaatttttgagatttcagttgtatattaaggtagcaagcaccagatgggttcatcgattactatctagtcttttttccctaatgacttccaaagtcagcagcattcttatttttccacttctaaggtacactggctacaatgtcaccaaccgaaaggaatagagaacccgtggaaggcattatcaacagtttaatcatgcgtttattgagaagaatgtgcagtgccttgcaaggagatggtaactatgtgctcttgttgttattcatactaggttttctaagactattttcaactggcagattacggaagtatatattacatacctttagtaatggtagtataagcatgttaatcagttacactgcttaatgttgtatgcggagaacttgtcaatccttgcgtgcatgtaggctgtagaagtagatgtagtgtttagattgaggaagagaatagcttcttgatgtaatgtggaccagtcaggtcttcatttctatggacttccatgacggttatgagtcagagaaatcagacttgaaatgtaaacattctcagcagaacggaatgttcttaattgagctccgagattctggcagcaggcactaaaaatattttggtagacatgtaccaatatatgcatgtacagaacgaagaaatagttgcagcatgatactgacaaaagtctttggtttgatacgtatttaatggaaacaaattaatttcatataataagtggatgtttggtttattatactccggtcttcccatttatggatcattattggataggatctaagttaaacatgttaattcgacttgcaagttataagtagtaccaataaaatagtaaagtagtgctcaaaccgttaaacaaatctgaattgttaaatttatggaagttgtataaaagatattattggtagaacggtgttgaaagtttttggatatgtcaaaaataaatatagtatcataaatttggatggaggcaagcaatatttgtgatgaaactatccgcttactgtagaaagacaccttgataattttccagcagaaaaaaaaagagattgtttttcacacaactattaaattcctcaatgtaacttacttaaatttccttctacatagcttcttaactcttgattccttaatgatatgtttcagaatctcatcactttgacaatgctgttcagttctatattcaacatttgatgcgtaaggtcggaaatgaggcttttgtcggccaacgtataatatttgcagtttcacaaagaatttctgcaatggcagaaagtttgctattcatggatccatttgatgatgcctttccaagtatgcataactctatgtacatgatgtaagtccgaccagcttgtatatagtttcttatctttatctaaattaattattcttttatgcttcttttagtattttttttaactttcttatcacataatagatggccacagaaggggaagggaagggagacgggggcaatgggagtcaaacccatacatgttgtatacttatttattctttctagtattctcaagtcgagtgattgctactgtattgtgtgatcatcttgactatcttatttattgtaaatggttgtttaagctgcaggattacttggtattgccccccttttttgtgtatactattcattgtttagaacactggaattattaagtgatcagaggtgccctggctatgcagcttgtcagtctctcctaattgtagaggctgtgcctgcttcagatccaaaatatgttccgttttttacattaacgaagtactgtattctgcctgaattgctagattagttagttaaattggggatgtccattcacctcaaaatttatcataacaattatgtttaaacttgacatttggaaccatagcttaagcttgcgagattttctgtttgtaaggggctgttggaataatttggcatacagtttactgccttgtatttgctcttttctgcacccatacttcactttatatttccatgattttcttgaaactgtaacagcaaatgagattaaaattatactttcttaattgcaggattcagctttttgaatttctggtttcagattatttgttaatctggtcaaacacaggggattttgacttgagtgagcttcttttgatcacttgatctttataatctgtttccactcctcccctggggtccaagttagttctgcctctggcagagtaaaattcaaatctctaggctataggccctaaacatactgcatgtaagatatgcctacaaggataattagcaggctcccacaattaacctatctggtgaaggttatatttaatactgttaatgatggaaatgaatctgacatatatatccatatgtttgtatttactctgtagggctttttgaggaatgggttgtatcaatcctccacggaagaaaagcgttggaactactagaaaacaggaattctctttatgtactgtacatagatcgcgtaatcggagttgtggccaagcaagtgagacagttgtcatttctgcaaaagcttagcccacagattcttgagaacttgtttagctaagcactggcatgcagctttttccttgtgaactgtaagtaacttgctttcaacccaaatcttcttttcttgtgcatagaaaattcaggtgtgtcgtagaaaatgctttgttattaaaagtcaagagttcttaattaattaattaattcccagagcatcaaagatcaaagttcttttaaagtgaaagatgctcttcaaatgtgaaaagatgaaacatgtaaatggtgaaatccacctattgaacaaaatctacatgacattagcacagcatcatgtgtcgaaagttggaaaaatatcccacatctctttttgttgaaccagattcctggttgaaatttgttccaccaaattgtcggcttaaataaatctttgacttcccgtggcatcactatttttcatattccttatcgtcgtagttaagatcttgcataaatgaggttgttggacggcttgacttctagctcttcgtagttaattccagacatgttcttttctcatcttcttcacttttctttgtgatattgagtgtggtgggaatctgaatcagattagtttacttataaacaaagaattcctattctagtactacccattgtcttttccatctttagagttgttccttgtccccaccatgttcatctttcaaactacatttgaagggtgattactcagcccttgaaacttttttttttcccctttaggatggattactaataccaaaaagttcgttttatatttgaaagatgcaaaaaaggtgtattgtattggacacacttctgctttttgctagatatatagtttccttcccgacttccatctaaccaaacttgctcctagctactacattgtatatcatctctctatctaattcttgcttactagacatgattcaagccaaaaccatactggttctctcattattagcaactcttttatcatcccaatactgcaaaacctcagcttctactgatattccgccatccactttcaggcctccaagcca

SEQ ID NO: 20 - DNA, 1146 bp, Solanum lycopersicum
  source 1..1146: mol_type = other DNA
atggagattttgagagagcaaccgaagagccactccgatgaatcgttcaaactcgccatcgcaatggcactcgtccgatcaaagcttcttcacaaaccgccggcagcaacaccggttccgccttcttcctgcccgcctctttctcattccgatgatgctgttaaatggaaacaaaaagcaaaagagcgtaaacgagaaattctcaggctcaaggaggatctcaaagtagccgaagatggttcacagtgtgatatatttccaaaaaatgcatcatgcaagtgttatttctttgataagttgggattattgagtcctaagaaaattggagctggttctgaccaacggttcagtgatgtgttgcggagaagatttcttagacaagtgaggattaaggagagaaagaggagaaggccagatgattctttgcttcaccgaatttcagattgtgacaatgataataatattgagcaactgagcgcttcagttgattttcttttggaactttgtgacactatttctcttcacagcttggaggagggtaattttaagaactggtgccaccaagctgtggactttattattggtacactggctacaatgtcaccaaccgaaaggaatagagaacccgtggaaggcattatcaacagtttaatcatgcgtttattgagaagaatgtgcagtgccttgcaaggagatgaatctcatcactttgacaatgctgttcagttctatattcaacatttgatgcgtaaggtcggaaatgaggcttttgtcggccaacgtataatatttgcagtttcacaaagaatttctgcaatggcagaaagtttgctattcatggatccatttgatgatgcctttccaagtatgcataactctatgtacatgatgattcagctttttgaatttctggtttcagattatttgttaatctggtcaaacacaggggattttgacttgaggctttttgaggaatgggttgtatcaatcctccacggaagaaaagcgttggaactactagaaaacaggaattctctttatgtactgtacatagatcgcgtaatcggagttgtggccaagcaagtgagacagttgtcatttctgcaaaagcttagcccacagattcttgagaacttgtttagctaa

SEQ ID NO: 21 - protein, 381 aa, Solanum lycopersicum
MEILREQPKSHSDESFKLAIAMALVRSKLLHKPPAATPVPPSSCPPLSHSDDAVKWKQKAKERKREILRLKEDLKVAEDGSQCDIFPKNASCKCYFFDKLGLLSPKKIGAGSDQRFSDVLRRRFLRQVRIKERKRRRPDDSLLHRISDCDNDNNIEQLSASVDFLLELCDTISLHSLEEGNFKNWCHQAVDFIIGTLATMSPTERNREPVEGIINSLIMRLLRRMCSALQGDESHHFDNAVQFYIQHLMRKVGNEAFVGQRIIFAVSQRISAMAESLLFMDPFDDAFPSMHNSMYMMIQLFEFLVSDYLLIWSNTGDFDLRLFEEWVVSILHGRKALELLENRNSLYVLYIDRVIGVVAKQVRQLSFLQKLSPQILENLFS

SEQ ID NO: 22 - DNA, 7238 bp, Solanum lycopersicum
  source 1..7238: mol_type = genomic DNA
taaaataattttacatgatatctcgaaataattattcttattccgctaattaagcgagccataaggggtgtgtaagtaaggatgtatttgctcaaacatcacatcatttctatttgtttttcgacaaaaagtcaaagctgattaatatccagccccattgatactgtctaaatttatgtgacattttttgttcttttagaatcaaataattaaatttaatcgaaaatttgcatataaattttttatttttaaaaaataatatatatatatatatatatatatgtatgtatatatatatatgtatgtatgtatcaaaactacgtaaaatagtactataaatcgacaattcaaaaaataaacataaaagatataccataaaaatagagttatttgaatctcaaaatttaaaaactatcatataaattgagacagaaaaagtattcagtttatatatgatagtgtatatgttattttgagtttatatattgttactccacttttttgaaaccaataaagttctaagaaaaatctaaacatatcagataaaagggacttaaacatagattttaattactgaagattaaataaatcataaattgcaaggatggaaatcaaaattttatcaaaataatgagtacgaatatccctatttaaattgtctgaactaaacgggcctagtgtcagataaaatgactgggccataattattgggcccaaattaatgagtagaggtccatcaaagcccaaaattcacataagaggcccatatgtaccattttccccaaaatatttgaaatttccgtgtatataaacccacactctcccgctggataatcaacgcaaatcatacttccaagttccaactgttcgacggagcaaaatcgcagaggaattcaaatgtatttacaaatttgattatatcttcgtctgttagggttctgtaattgttcaaattgaagttttaatctctggaagatttcaatttttatagtatctgcaaatgaagttgaagatgaacaaagcatcggatctcagctctatatccgttcttcctcctcatgcaaggtaaaattctatctcagtttcacgatttcatctctttgcattgtttagcatgaaattgcgtagctctctgtgtttctgccttttgttcgcatgcatttccaatttgaatgttttgtgtgcgacgcacatagcgtgttggagtgagatagagagaattttactgtaaatttgagcttcttcgggaaaatttaaggaggaactaagcgcacatctctctgtttgcttttcttcgaatgtatattttgaagattttgatgttctatccacacatatgcatatgtatacatgttatttgttacatgtatgtttatatggatgagagaggtagaatttttctataatattgagctttatttttgtgtgatgatgatatgagaagaacgccaagtgcggaaccgctctgtgttttggcctacttctccgtgtttgtgcgatttttctcatacattacaggtatttttaaatgttttcgtgtccaatatacacaaactgtatatatacataaatctgtctatgaatgcatgaagagagatagagagattttataataatattgatcctatcttgatgatatgcgaaggaggccaagtgtggtaccaagcgcagcagagtcttccgtttttgggaaaagccaaccctcacaggttcggtcacagcagcaatcacaacaatccttctcacagggattttcatctcagcaagcagtctactctcagttatcacagagctctctggatgattttgtccctaatgagcaagtaattcctccatctcgctcctatctcttagttattcgaagagaagttgttgacgaaatgtcatttggtatactatacgaaggaactagttcatttggtgtggaattgataatgatagacctaaaatcatttttgttagcaacttctgaagaatgctttagattgtctaaaatgtattttgatgcttagcaatacttgaatatattatattgttgataattgttgcctaggttacttttcagtgtatttttgcattagtatgctttattatgcttgaaatagatgtatttagcttctgactatgatttactttgttaactgttgcgtcaacacaacactcactttatatgacgtgtttgatttaagtgttatattagtgaggcttgaaaaaatattaaatttaagtatatttgaacagctttgaaagttatggaagttgcataaaagatgaatgatgccaatattttgcaaggtccttatatggaaagtaagtcaaacaaattgggatggagggtgaagtaaatattatttaccatcttcaccgtactggacagtgaatcataaattctgttgccgcatctgtcagaatgtttcttatcggtatatgaaaaaacaggagattgtcacagtgcactttgaagtggttgtcggcagtaggtcgtagatcttcttggtgttcatatacaattagttaactaatggactttttacttttaaattaatcatatgtcttcatgttttcaactctgtcctgtgccagggcacatagttccatagaacttcccactttatacattggaactttttctcatctcataggaaacaatatgcttttatggcaattttacatcttaaagcaaacaaatgttgtaactgttaataattttaatgcagagattgggttctcaagaaagagaaaattcagcaaaaaggatgagctgtttgcctcatatcaactatacacgagaagagactcaaatgcagttatcaaaaccttcgactaattatttgcgcaaatggtcagttcctgaaagcaaatgtaagcaccaagccacaatccaccaccataaactacatgctctcaacttctgtttaaaagttaaggaaaatgtactcccgttcagtgctaatttgcagctggaatcatcggactaaacatgtttatgaattctaatttttctgggcagaccagattgaagaacttgaacacaaaattggaatggtagagactttattaagcaggcaaggaatgatcttagattctattcagagtgatattatgcaagttaaccggggaacaaaagagatgttgatggagagtgagtattctctgcccttctaatttacgtgatgtggcaaataattaggaactcaaagagcccatatcattagtctacgagtgtggagttttgtcttgagaagcctgctggttcgattaaaacttttacttgcaaatattctggtggatgtaaaaataatggcaaacctaagacatttgtttttcttctgaattttctttcagtggaaagcttacgaccaaagttagtttctcatgatgaactgttgcaattgatggtaactatgcttagcttctctgcctacatccagaaattaagtgcctgtttgatttatcacatttcctaatccacgtggcatacaatatctagaacaaggacagggaagatctgaaagctagccttgaggggaccttcaaatctatgtttgaagagcttagggagaacaaatatcaagagaacatcagagatctttcatcactgcttagagctatgcccaacaaacttgagatgtgcattttgcaacttcaaactgatttgagcaagaccttagctaaagagattcaggcatgttgcatattgaaactgacttttttaattcatatttaggctaccctctgtggttggattaatactgtttcatctatattcttattgcttgcagataattgccccccgcccagattttcatggacaaaaacatgaaaccgctccagtcgatcctccaaaagtatgtttttgagtactctttcttcaaattccatatgatttatatgagtatttagtctattgaagaacacaatcagaagttataatgcatttgaacatttgtagggcatcaatgattgtatccctccccgtgaagtgaagttgctaaagaagtaagttctcaaacttccttctcatcgccatcactgcagccttagttttgaaatctttaagtagcaattagtaatcggtagctctccagtatgaaaagttcataatcacttggtggatctcttattatttgcatcatttgtgtgcaataggcataagaggtagtcatttcacaatgcctctgaaatgtgtgcattgacatttgagaacacttgaggatgggatacactctctgtcatcaggaactacttaggtgacaaatagatgtgaagattcacggcatagtgtcttttgatccatatcataaccagaaagtgagtatccccatttctcacattagctatatgaaggaagaaagggaaaacaaaggaaagcgctacccttattcgtcgaaagctagccttcatgataaaccaaatgaaattagaaaaatttaagaactttgctatagcttcaaagaaatcttttagattcttgtttacaaagttttgctgatctttcttacattgagcgacttaattcttcattgctgtgcattgcaaatcaccaaacatttcttttcaattctggttcaactacgaatctcagagatcagaaaacaactactccgccgaagatagaaatgggaagctggactacagttaaaattaatcaaacttgtatgaagcagaaaattcccatcagaagtcacacacagaatgaagcatttcaacaggtaactctctcattgtccttaagcaaacaattgtttgttgtgttatgagcaacagttgcttcctttgtatgaaatgggaagctggactacagtaaaaaataaccaaacttgtataaagcagaaaattcccatcagaagtcacacacagaatgaagcatttcaacaggtaactttctcattgtccttgtgcaaagaaatgtttgttgagttatgagattcagttgcttcatttgtttgaaatgggaagcctggactacctgaaaaaaatgaccaaacttgtatgatgcagacaattcccatcagaagtcacacacagaatggagcatttcaacaagtaactccctcattgtccttatgcaaagaaatctttgttgagttatgagaaacagttgcttcctttgtttgaaatgggaagcctggactacagtaaaaaaataaccaaacttgtatgatgcagaaaattcccatcagaagtcacacagagaatggagcatttcaacaggtaactccctcattgtccttaattgttgagttatgagcaacagttgcttcctttgtggcatgaaacatccaaaaaagaaaaaattgtcttttagatgttgtatttgttatatgtcatagtccaccatgtcttaggccttcaagttgaagtaacaaaacgtctttgttcagcacaccacattttttgataacttgaaactgtgtcatccttattctcagagctgacatctggctatccatttcaggaaaggggatgtagaattaccattgaatctgatgaggatattgacgcgggattttcctgcttgcttgaagaaaatggaacaggtaatttgcacttcttgcctgcatcattcatttttgaggatttcacaataagcaaagttattctacatcctgtaattgatcaatgtgcttattgacccatgcttgttgaacttatctaatgaatccaagatctatttagatgtatatcaaattatatcttatatctcaagactgactactgacaagaatgactttccatacttctagtcaagcagaacacctaagatttatactatgaaatcaaatacattaggtaacaagtcagaacatgtctgaaatcctgaagcatctggtacactccatactattatgttttttctcaaaccaaagagaaactgatagctctctcttccctttgtctgttggggtacagtagggaatttgaacctgttctcaggttcagtgtcccgagggatcttgtttatttttctctggaatagtcacatttcgagtctgtctaaaataagaaattttgagcatcataactgcagcagcagtgttcttctacacacactgaaacaatcaatcatatacagtattttttttgtcatttgctaagatttgagtgcttaaactgtcttcccttaaaacacccaggaatttatccactagatgatgcaaaggaagagagtgcacgcatattaaggaaagcaaggaggcgaaagagaaagcattttaacactatcattatagattgaaggtacacagtgaatttataatctgctgaatcaaggtcctgtgatttgataagcagtaaaaaatgtattattgattcttccgtctttctttagccaatataggacatgtttgctatttgacttttcattattattaggaagtccacgactgaccgttacatagcaagcaaaatctttgttgctgctgcaatactaagtcttaggtgattgtataacgagatgtcaacagactcagttccataagaatatgtaatgcactaggtttatgtaagcaaatgattacgatgttttaaattttgaattgcataaagttgcctgattagatcattgcatcttctgtatacaatgttttattagctaatgagagtaaattttcagcgtgtgatattataccattatagaagtatataatatggaaatgagaatccttttcaactatggaagagaacttcgaaacacctagtagagaatgaaagcatatctaccaagggaagaaaggaaggtacttattcctggacttggatggtccgtattttttatttggttacattctgtactactcttttgtcaagatcctgcagcctaaataagagaatcactctctcctcgtaactcttttcacgtaattttccttagagcataaatatcgtgtggaatttattcttgtttgctcataagaatctatagatcatctatcatgttccttgcctgttgcttttggtgtatgttgggttccttattgacttagtccaagtctaagtagcataggcattaccagccacatcgaattgcactcgtggtgtatttttaataatgtaattaagaagcatgctcaatataaattctctacaagagtcatgcgtgggttgcttctccttttttaataccatccaaaagtccaaacaaactttcgttggctgtataaggaagtttcccttcctgcactacctactatgcctccatacatgactgtaaaactccttaagttcaaaacagtccc

SEQ ID NO: 23 - DNA, 1763 bp, Solanum lycopersicum
  source 1..1763: mol_type = other DNA
cacactctcccgctggataatcaacgcaaatcatacttccaagttccaactgttcgacggagcaaaatcgcagaggaattcaaattatctgcaaatgaagttgaagatgaacaaagcatcggatctcagctctatatccgttcttcctcctcatgcaaggaggccaagtgtggtaccaagcgcagcagagtcttccgtttttgggaaaagccaaccctcacaggttcggtcacagcagcaatcacaacaatccttctcacagggattttcatctcagcaagcagtctactctcagttatcacagagctctctggatgattttgtccctaatgagcaaagattgggttctcaagaaagagaaaattcagcaaaaaggatgagctgtttgcctcatatcaactatacacgagaagagactcaaatgcagttatcaaaaccttcgactaattatttgcgcaaatggtcagttcctgaaagcaaataccagattgaagaacttgaacacaaaattggaatggtagagactttattaagcaggcaaggaatgatcttagattctattcagagtgatattatgcaagttaaccggggaacaaaagagatgttgatggagatggaaagcttacgaccaaagttagtttctcatgatgaactgttgcaattgatgaacaaggacagggaagatctgaaagctagccttgaggggaccttcaaatctatgtttgaagagcttagggagaacaaatatcaagagaacatcagagatctttcatcactgcttagagctatgcccaacaaacttgagatgtgcattttgcaacttcaaactgatttgagcaagaccttagctaaagagattcagataattgccccccgcccagattttcatggacaaaaacatgaaaccgctccagtcgatcctccaaaaggcatcaatgattgtatccctccccgtgaagtgaagttgctaaagaaagatcagaaaacaactactccgccgaagatagaaatgggaagctggactacagttaaaattaatcaaacttgtatgaagcagaaaattcccatcagaagtcacacacagaatgaagcatttcaacagaaaattcccatcagaagtcacacacagaatgaagcatttcaacagacaattcccatcagaagtcacacacagaatggagcatttcaacaaaaaattcccatcagaagtcacacagagaatggagcatttcaacaggaaaggggatgtagaattaccattgaatctgatgaggatattgacgcgggattttcctgcttgcttgaagaaaatggaacaggaatttatccactagatgatgcaaaggaagagagtgcacgcatattaaggaaagcaaggaggcgaaagagaaagcattttaacactatcattatagattgaaggtacacagtgaatttataatctgctgaatcaaggtcctgtgatttgataagcagtaaaaaatgtattattgattcttccgtctttctttagccaatataggacatgtttgctatttgacttttcattattattaggaagtccacgactgaccgttacatagcaagcaaaatctttgttgctgctgcaatactaagtcttaggtgattgtataacgagatgtcaacagactcagttccataagaatatgtaatgcactaggtttatgtaagcaaatgattacgatgttttaaattttgaattgcataaagttgcctgattagatcattgcatcttctgtata

SEQ ID NO: 24 - protein, 441 aa, Solanum lycopersicum
MKLKMNKASDLSSISVLPPHARRPSVVPSAAESSVFGKSQPSQVRSQQQSQQSFSQGFSSQQAVYSQLSQSSLDDFVPNEQRLGSQERENSAKRMSCLPHINYTREETQMQLSKPSTNYLRKWSVPESKYQIEELEHKIGMVETLLSRQGMILDSIQSDIMQVNRGTKEMLMEMESLRPKLVSHDELLQLMNKDREDLKASLEGTFKSMFEELRENKYQENIRDLSSLLRAMPNKLEMCILQLQTDLSKTLAKEIQIIAPRPDFHGQKHETAPVDPPKGINDCIPPREVKLLKKDQKTTTPPKIEMGSWTTVKINQTCMKQKIPIRSHTQNEAFQQKIPIRSHTQNEAFQQTIPIRSHTQNGAFQQKIPIRSHTENGAFQQERGCRITIESDEDIDAGFSCLLEENGTGIYPLDDAKEESARILRKARRRKRKHFNTIIID

SEQ ID NO: 25 - DNA, 4656 bp, Solanum lycopersicum
  source 1..4656: mol_type = genomic DNA
tttgcaattgtctttcatacgtgtatctcacgtggattctaggagatctattaatatgataccttcagttttggttatttcttgtagattgatacgtgattggtaataatgggacgggtctttcggaaattatttttctgtttcacaatatataaataaggtttaataacattttttacaattttatgacgtatttgatacatgctaacaccagcattatatcatatgtttaatgatcacgtttactttaccactctcatcccatttatctcctcctttacttattagattgccttattctttttaaattttcatttattagaactccttttaggccttattgtttattttgttttgtttttccctagttgacacattatattctaaaggaagacctagtcttttgctttgctaagatcacatcaaattattcacttccaccgaagtatgaatagaagctttttgccatcgaccactacttccttctcttgaactattcttttttttattaccgcaaaatcacacaaagaaaggtaaacataccaaggcaagtcacctgtgacgagctctaccaacctaagatctctattgggaaaattcctttgacttgacaactttgtgggtcataactattctgtaggaattgttttatttaaagtaagaaatcaacatttattacatgtttaaattatttttatcatttcaatttcattgtaatttacattatttttaatggctcgtaatttcaacgcaaagttaaaaaagaatattaatattaatttactttgttagaccaatactttataatcataacgttactgatgatgttgaagtcatcaacatcgcagggaggaaagtgtagtttttatgtaacaagaaggagctctttgaaattaacccaaaataaaattaaaaagggaacgcggaaaatacaaaattcgaacagactataaattagggcagtttgaaacctgcagctcctcatttccttctcgtgaagatgtcaactgcagtttcgcaccaaatctcccttttcagattccaagtcgagagccgtaggtttgttttcgataatcaaaacttcaattctgattcaataaaatgcacttgtgagcatgatttttgtgcagactggatgaaggagctcttcgaattctcgagtccgttttagcttgggacgattacaaatctctggacggagtggtatgtattttgaaacagttcatgagacacgaatctctccgcattattgaggaaatcgctggaaaagctgcagagcataagcttctgatcgtagattttctagttcgcgtttttgctctcatcggagatactgaggtatacagctttgactctatcgatttcaaattggtacatttgactttgatttgattatttggaaacacatagttactagaagacagagataatcggaaagaacagtagttttcagtaggatgatgttgaagacactgatgaattaaaccatgtatttttgtggaatttgtgataagttgaagagctgcttgaaattttgtagcctgttgtgttcggtatttgttttatcttcgaaagataatctcatgctaatattgttttgctaaggaagttatatccgtagttttaaacttttagtgttcgaatgcacttcaaataagtattagtagtagacacagataacttatattcctgtacaagtggctgtgattttgatggtggaggcaggtggtaatgtgagtagtacaagatgtaaacaatgactgctgtatgcagagaaaattgtatctgtaaaggaaatatatccttccttatgtatatacaaaaactcttttcggttagagtttgtgaaaatgaagtaatcagtagaagtgacattaaggaacacgagacctgtctatccaataagtgtaatgattggatagctttcatggtatattaaaaacaatttgacagagcatgaggttaagagttagctgtagtcttcaacagaacgttgatgtagttgacgagaattcatctgattttaaacatcacatcatgctttaaattgtccttttgaaatttgtgaaagctgcatacaaaatttatcagagttagtgtgtcgaacattttgggacatccaaagtgtagacatatcctatgttgtgaaagctttaagaaaccacaactattgatgattttattcttctattatagaaattctggttttgcctttttattttcggttccaaacacgtgacttttaaccattgggtatacacagagttgcttggcgttgagatatgaagcattgcttatgagagagcagaaagcaatctgtgatcagaggcttcttgtttcatatagtgagtggctcacttttgctgagcattcacttgaaagtggcttttgttccatcgcaaagaaggtaaatttctgtcaaaattttgggcacttgtaagtattttacacgtgcaaatgatcaaggaacaaaactagtatatgctgtccattgaaaatttatgctcaggtcagagttaatgctaaatgctacttcttgtactgttatgtttctatacttctgtgatcatagcttgaagggtcttatcatgtcatattgttttccattttggatgtgtttgtaggttctatctctgttaatttacctgaataatttgatctgtcattcagatgctattgtggaaatcactaaactttgttatctttatgcctcttgttggaaatttgttagatgcaaattaagtacggttcttttgcattctgaattaggaattagactcactgctgaaaacatcttgttctaattagcctcctccacctcagcaattagtcctcctttgtctacttcagaaatacaatatggacagtttgtcatggccttatgtgtagtgaaagttatgataggaattagatcaatctagctgtgcaactattgcatgtttaacatcttgccgacactaagagcatatgtttttgacttgatgctatctattttgtacgtttattttgagcctggtaccttatggcttcataaatattgtgaagttacaacatcctactgcttatagtaagtgtattccaatatctacctctgacctttacttttcaggcatgtgaaaaggcgctcttatgttttgacgtgaacatcgtagatgatcctgaaaactatttcgtaattgaaaaaattaagaatcttaaagatgttgctgtgatctcagcgtcttcaaaatctggtatgttcaaatatttcattagatccctcctttgtttcatagttaatgctttgccgttatatgttcctaacatgaaagtgaaatgaatttggtggaatgacatcaaagtcttccattagatcatatgtaactggaagggtggtgaagggaaagctaattattaactattcattactgctaaagctttcttgtggcacattagttcaggctcaggcagcaacgtacttcaagaacaagaatattcagcagaactcacaaggatcctacgttcctgtggaagctaaaagttcaggaagcactctgtttagagatggaatcaaaagaaggcacagacgccaattggatgaataccgacatctgaaactgagtggaataactgatggaaacatgcaaaatattttggtaggtcaatatgctaagtaaaaaagatcttatttaatttcgtcaattgattacaattgatagtgcaggaatgatttttctctgaagtaatactattacggagtcaccaatatgatcaaagattaacttctcttcttattggttagtatcttggaaggtaattactctgataaatataccacaacaccattgctatgatatgtttaatacttattaaaaatatggtcttataacaaaaatattgtgctgtggtaagaacctctagtttcatctattgacttttttgtttcttgtctaactgaaagagaatttgtttcatcaattgaaaactcttcaaaatttatttttgtaccataataagcaattttttgcatttttaaattactgataatgagacaaggtcagactgcttgccttgtctcttctcgaccttggtcctgcaataggaacctagcatgctggtgataagccttcaataaaatatatttcttagggaatctgtaattaagtctaagcaacaaacaaagagtacatttgcagcaagatattagcttcagcccctctccatgcaatcacgtgcctatgcagttgattgttttgtcaatttttagaccttcgccaaattggataggtgtaacttactagtcaaaatcagagagttggattagtaagaaattttgactctaacaattaggaatttgtatacctttttagaaatccaaatcttctttctttatataattgtatcacttaaagaatcaaatatcatgcaccgttttgaacaggaagaattaggtgcggatatacgatacagggtaatacatagataacaggttgatcgaatacagttgcttagcataaatcttgtatgcgttaaaactctcactaaattgctacttccttcgtcctgatttgtgtattttctatattcaataacaaatttaattttaaaatgcttaatttatttttaatgatatgatttacaatcgcataaatatttataattatatttttttacttt

SEQ ID NO: 26 - DNA, 2888 bp, Solanum lycopersicum
  source 1..2888: mol_type = other DNA
tcgaacagactataaattagggcagtttgaaacctgcagctcctcatttccttctcgtgaagatgtcaactgcagtttcgcaccaaatctcccttttcagattccaagtcgagagccgtagactggatgaaggagctcttcgaattctcgagtccgttttagcttgggacgattacaaatctctggacggagtggtatgtattttgaaacagttcatgagacacgaatctctccgcattattgaggaaatcgctggaaaagctgcagagcataagcttctgatcgtagattttctagttcgcgtttttgctctcatcggagatactgagagttgcttggcgttgagatatgaagcattgcttatgagagagcagaaagcaatctgtgatcagaggcttcttgtttcatatagtgagtggctcacttttgctgagcattcacttgaaagtggcttttgttccatcgcaaagaaggcatgtgaaaaggcgctcttatgttttgacgtgaacatcgtagatgatcctgaaaactatttcgtaattgaaaaaattaagaatcttaaagatgttgctgtgatctcagcgtcttcaaaatctgttcaggctcaggcagcaacgtacttcaagaacaagaatattcagcagaactcacaaggatcctacgttcctgtggaagctaaaagttcaggaagcactctgtttagagatggaatcaaaagaaggcacagacgccaattggatgaataccgacatctgaaactgagtggaataactgatggaaacatgcaaaatattttggtaggtcaatatgctaagtaaaaaagatcttatttaatttcgtcaattgattacaattgatagtgcaggaatgatttttctctgaagtaatactattacggagtcaccaatatgatcaaagattaacttctcttcttattggttagtatcttggaaggtaattactctgataaatataccacaacaccattgctatgatatgtttaatacttattaaaaatatggtcttataacaaaaatattgtgctgtggtaagaacctctagtttcatctattgacttttttgtttcttgtctaactgaaagagaatttgtttcatcaattgaaaactcttcaaaatttatttttgtaccataataagcaattttttgcatttttaaattactgataatgagacaaggtcagactgcttgccttgtctcttctcgaccttggtcctgcaataggaacctagcatgctggtgataagccttcaataaaatatatttcttagggaatctgtaattaagtctaagcaacaaacaaagagtacatttgcagcaagatattagcttcagcccctctccatgcaatcacgtgcctatgcagttgattgttttgtcaatttttagaccttcgccaaattggataggtgtaacttactagtcaaaatcagagagttggattagtaagaaattttgactctaacaattaggaatttgtatacctttttagaaatccaaatcttctttctttatataattgtatcacttaaagaatcaaatatcatgcaccgttttgaacaggaagaattaggtgcggatatacgatacagggtaatacatagataacaggttgatcgaatacagttgcttagcataaatcttgtatgcgttaaaactctcactaaattgctacttccttcgtcctgatttgtgtattttctatattcaataacaaatttaattttaaaatgcttaatttatttttaatgatatgatttacaatcgcataaatatttataattatatttttttacttttttaattaaatattatcatataaattgatacaaagtcaatacaaataatagattcaaaataataaattattgactataataaaatatagagtttgaatagatgaagttcaaatctaaattcgcactcgggagagaatgatgtgatgaaccctccatcgactgtgactgatttcaggctctgacgtactctctttcgataaacctcattgaaaattttaggatttcagggaattgattttcacaaaaatatttgccacccttttttttctcttcaatattttattgttcaacaaaacccgaagccttgaatttccaccactttagagacggaacaaaagaaaagaaaaagataatttttaaatttaaataaataagaaaacatccattttcccaataatcgaatcttccatatcaccaagtgcaattaatggatgcattgaagctcgcatgttttttattttctctaagacggtactgaagatgtctgtttttcactcttattttattcatcaccttatagaattaattattccatcaaatcaataaacaatatttacaaggttctcatcctgtcgaccacggctcttcttcttagctataagaagttactgggtttgaaaaattctaaattggaaactgaaacagaagataatctttttttttgtattttatgaggttaggtgggggacccataactttttatttttgtcttagaaggaaaagtgatttggtcatttagactagttgaacatagaaaattggatatgatgaattatataattcaatagagtttttagtagctgggaaagagagctgttttcctcggaatagaagataaaaagtttggaatcatgtggaaagcattaaatgctaaagagtgggaatcgaagcttggggttcttcaactcttattgtttatggtgtatcatttcagaaacctcgtgatacatttgctctaataagctcatgaatatttttttaattatatgtctagcttagccatactgctcaagaatcttttcattttcattccaaattaattaatggtcaatcagatgtggaagctgtta

SEQ ID NO: 27 - protein, 251 aa, Solanum lycopersicum
MSTAVSHQISLFRFQVESRRLDEGALRILESVLAWDDYKSLDGVVCILKQFMRHESLRIIEEIAGKAAEHKLLIVDFLVRVFALIGDTESCLALRYEALLMREQKAICDQRLLVSYSEWLTFAEHSLESGFCSIAKKACEKALLCFDVNIVDDPENYFVIEKIKNLKDVAVISASSKSVQAQAATYFKNKNIQQNSQGSYVPVEAKSSGSTLFRDGIKRRHRRQLDEYRHLKLSGITDGNMQNILVGQYAK

SEQ ID NO: 28 - DNA, 8582 bp, Solanum tuberosum
  source 1..8582: mol_type = genomic DNA
tttttttttattcggtgaggagaaaattaaagttttaccgaaatttttatgggccaaatactatttttaaataaagtgatagtatttcgaaaaaataataaatactccataagtattatttactttcctgaaataatatttatagacaaacaaaatatattttctgaaaaatatttgattttcttatttaatttttagtgtttgattagtaataagaaaatattgtctccataagtattattatatataatctattcaaatactataacaccacccttgaatccccaacctttaaaatgaaccttgaccccacctttaacacggaccaagacccatatctcaacacatatcttgaccacgattcaggtcccaacccctaaccttgatatcgccctcgattagactcgactccagccaaaataaggtccaacggtgacttgggacctaatctcaacccttatcttgaatagagattcaatcccgagccaggactggaccttgatctcgagtcggggtcgggtctcgattcgaggttagggtccagtcttggatcaaaattggggtgagtcttggatcgaaattgggaaaagtctcagattgaaattgggcatgagagtcatgaagttagatcccgagtcatgaagttagatcccaagtcaaggtcagaagttggggctcagggttgaggttgaggttaaggttgggagttaggtattgagtgagggtcaggatcgaaagtcggttccgaatggggtaagtggtgaggttgaaagttagtagcgcaaaatatttcttttacttctgcgtagaaaaaatatcttttcttgaaaaaatatttttttaaacatttaagccaataaaaaatatcaaaaaattgaaaaatattttatagaaaatgttaaccttggtgccaaacacacctgcgcgcgcagaacttcacagttataaagctcggatttaccaattttcaaacaacgtaaacctgcagagggaagagaaaatggagggaaagcgttcaaacacgcagccactaacactcataaggaaaatcaaaggtagatagcgcttccattaaacttcaattgttttctgaaaattcattgcgattctcgcgttcaatacattgattctcaacgaatcgtcttcgcgtttgagccatatatactttgattttgttttgcaggatttactcgttccattgttgaggatctcgctcgaggtagggcaccgttgatctacatcgatcggttcagaaattactgtactgacacttctggaaattggtaagaagcagcggtagcttgaatatatgaaattatcaatcatagttgagcttagtggattggtttttgctgctgtttgaaatttcattgcaattagtgttttggaataatacgaaaactaacactggattaaactgtcgattttctataaataataaatgaaactacactgatcggttcagaatttactgtactgagcgaagtgtttcccattatctgttccattctgctaattggaagatctggttgaaaacagttaatgtgtgttgcagtttgaaatttcattgcaattagtgttttaaaattccaactcgaaaactaacactgaattaaactgttgatttcctatgaattaataaaacactacctcgattggttcagaaatttctctactgacactttcggaaattagtaagacgcctatgtgtgtgaggattttatttggtagcttgagtatatgattatcaattcaagttaagcttagaaatgtttttttttcttttccttcttttcgaagatctagttgaaaacaatgaatgtgctgcagtctgaaatgtcattgcaatcagtattttagaattctaacacgaaaaattacactgaattactgttgatttcctatcaataaacacaacgatgtttggttcctttctatattacaaggcctccaaagagattatccttgacgtaattgaactgaaaattgcaactgatgaagattcacataggtttaaaacggtgctttaagaatgttgctagcactgggcttggtagattattctgtggaattccagatggtatgctcctgctccccctcaacacaaccccttccaaaacgtaaaatgtagagaagaaacgaatggttattttaagtgccctgctcagaagaagaatgagcacagtctatactgagagatttgttcatagaagccattgcctatactgagacactaataagtactagtggtaattgttatgttgaatggagttataaaaacaatgaaatttactgaagttggagtttgaatggctaataaagaccatccaaatgtcgtggtagtattaatggtctttgtttaatttatgtagctcttgcagctctggtttgtctactggcaaggaagctatatccctgaagagggaatgccatgcacgtaggcttggtgagtctagggagagtaaacaatacttgtatattgtatctgctgatcttcatcacatagttggacaagaaatgatatgatagtgaaaagggtaggaatgataattaaaagttgctatcctccctgaaaaatgacaaaattaccaggagaactatttccccgttaagttgacttttctgttcttctgttttcctatatgagcctccctttccttgaagttacacaggatgcaccatggggggaaggtggagtggggtggggcccgtgggggtggggtagtacaaggtttctctctcagtttccttttctgtttggtcaaaccaacttgaaggccttttttgctctccaatctgcttaacatcctagaaccttgctgggttacttcatctctatgtttttgtttcagatgttttgttgagagttcttgtgatagttcaacaacttctgcaagaaaacaggcatggatcaaaaagagacatatattacatgcatcctactgtttttaaaggtaaatctggatcgacctctggtgttccaacgaatcctcttttcagaagaaaaatttggatgaatgctaggtgttccagtgtagttacttccctgttaatttcataggaaatggttggacattatgtactctagaatcagttttgaattattcttgtgattggttatgaagtttttcttccatggaaaatgcttatgtgctgttgtatagttcagcttactcagttgctagagatgtgccatgattttagatctctaacgcaaaatgtatatattcagaaggcttcttcctcctatatgctcatcactctcttttgcactctataatgcagaacaatctgttgttgatcgggcaattaatgacatctgcatcctcttgcaatgcagtcggcataaccttaatgtggtatgccaacctactttcctctctgtatcaaaatagactcattttagatgtatatccacatgtcgttcactgttaagttgggaaccttttaacagagcgggttcacagtctcttctatatttatttagttacatgttcattttttacagtggaggattcaattagggttcagaatattgattgatattagaaatggtcattctgctttacttatacatgcttttgacatgcaaaacagtagatcacaagtatctgaccctgcctttgccataccatgaggagtggggaggggtttgctagtgtatttgattagagggatgtgaatattgttcttgtatagaacttgaatacgacttcagagaatgtaaaggatattgctagactagggtatacccatcattcaaatgattattttattctcttttattgctaatcttgtaagaaacttgaccttttatattcttttgatgcttgccttttacaggtgtctgttggaaatgggtgcgtgcctctatacagtttatattgccttgcaggagtgtgcttctagacatgtacattttgggttcattatatgcaatgttctttctcatacttgacataatatttgcaatcttttcttcttgaaaatttcaaatgtttcttcttcagttgattatgcttatacctcctgcatttgtctcaatgtcgcttcgtatgtgtctaaattcctctttggggagcaaagttacttcatgattgagagatttgatattgtccatcatgttacaataaacttttgtactttgagcaaggtaaaatttcattataacccggagaaagcatgtcactctctaaggagtattactgcatcatcatttttggcctacttttgaagatattggtagcatatgtagatctagtttaaactgctaaccaatgaagttcccaataaatgtactgctgttgcattttcctcatgacagttttgtccgttcctttagatcgatatatagttggttctctcctttgtttatattgtaatagttccttgcaattctcagtcataaaattcttcttccaactatttatggtctagattggtgatggggtggctgcggtatgtggaatctgggaggaaaattaactgcattggcaatcctcacactgtaagaatgatagttataagctaagatgggtttctgtagttgtgtaacaatctaattatgatggttcctgcaggcatacccgattccggtccttgttgaagaggttgatggtatccttatgagtctaagcgtttgaattgtgaatttaacatggttaaacatgaacatgagtttgcggactccatacatgtgcaagttcagttattgctaaacataaagttaaatgtacactttgttgttgaatacatcctgtaatttgactttatggattgctttctcagactatggctgtagttgttactcccttaatgcttgaacaagatattattagtgttgctcaatacgttttagttgtggaaaaggaatcaggtaaaactatttataagcatatcaagcctataacagtcatgaaaaggtattcctagttcataaataaggccactatttattgttcatcatgcagttttccagcgactagcaaatgatcagttttgcaagaggaaccgttgcattgtgataacagtacgcatcttttgttttctgagaatttccacacatacttggctccataatttctttttaacagggaaggggttatcctgatgttcccacaaggaggttagacccatgttgctcaccttgccaaacttgttgcagatgaattctacttcaattaatcatatttctgtcttttcatgttgcttgcctgtggtaggtttctgcgtctcctcattgacaagctgcatttgcctgtgtacggcctggtagattgtgatccatatggctttgacatcttaactacatacaaatttggttctttggtaaggataattcagtgtggtgctattatgatgtgaacaagttgctaacgttcctccttttcactgtaacagtctatgcttctattgttagttagtccaaacttatgttcacatttctaaaagaaaagtcatacattcatcatcgttttcctatcacaagctatcaagcattgaacgcgagacactttaagttgaagtgtatagagtagttagattagatggattgatagaatgatgtgttcttcggtaacacatatctttctatgatttttgaagcaaatggcttatgacgcaacatttctacgagtctctgagatacaatggcttggagtatttgtccaggattgtgacaattatagcattccacaacaatgtctcctgcctttaactactgaaggtaacattcacacaatcatgtctcgtttcattatagctttttctcaaaacaactcgtcacaaatgactgattgtgcaatcttgtcagataagaggaaagtcgaagcaatgttaccgagatgttatttgcaaagagaagtaccacaatggaggtaaaatttcatactactaactaatgttaatggcaagacttagggttctgaaaaatattcatatgactcttctccacgtcctaaggtttgaactggagctgctgttgcacaaaggagttaagtttgagattgaagcattgtctgtacattcactcactttcttgtcccatgagtatctaccatcaaagatccacaatggagggtatatctgaatctttcctatctttgtttggttctttagcacgagaagttcaaagtatttttcatgtgctcacgtaattatcatttgaaagaacaacctaactagtcacttgtgtcaaattcatcatgttccgccattttggctattaagtttttcacgacaacggttgtggatatcgagctacaaatgagcagtgacattaagcagattgatgcagattgaaatttgtcactgtatctcgtcttaaatgatacatcagaatagattgaagaccccaaaaagcctaattcttaaaattatttgtgatgtaagttgaaattttcgcatctaacgtgttatgacactatattggttgttgttttgcccaggaaagtagaatcatgataaagtagacaataagaaatacggacttttaaaaaggattcaagttatatatattggtatagtgatatcatgtttgtgaatcgttttaccaagttactgattattatttatcacaggatttacatgtaaatactttattaatcatttgattgtatgcatttttttacacgaagagattatgcacgtagtaattggctaagatgcaagaacctagtagtttgagattgaacaatgattatatttcttcttcatgcaaaaaaaagaaaaccaacacatacatactcaaactcatttatgaattatgataacagactcaacttgtctaatgcaaagtcactttttacctatacgattgaattgctaaagtaatttatttttattacaaaccaaaattagatcactttgaaaaatatttatttgttttgatctagttttataaaacttcctcaacctaggttgattcatctttaggaatgaattaattttgttgcaatcattatattccttaaataatgacgtcatttactaatgaatatttggacaattaatgtgcaaattatggatcaagcttgacaccaatacaacatgtgataaaggattaattaaattaaaagaaaataaagaccaagcagaatagattcagagtattctactgaaaatctttaaaagtaataacaatagaaatatagaataataataataaatatctccgtgacataaataataagtacaaaatctttgtaaagatttgatttataaattacttaaacatgacaaaaataaaaaccaaatgcagagaatttagtacttggttaccattatatgaaaatggtaataaaatctttgatataattatctgattttctttctccttttaatcaatgagggagtatcttcataaacaaacaataattcaacctctacttacattgcactcgttaatttgtcctccattttttttctcatcaactctattagctctttcatttgattcaatggaaccctttgctgaattggtatgattcactttcataaaaaaaatcataattttctcctttagttagttaaaagttgtaatttttcttttatcaattatgtcttttttagggctgtattttgaaagtggacgttcattgtgatgcatgcaagatgaagatggtggacgttttgagttctatatgcggtaatatgttctatatgcttttatttcttagtagaacttgttttttctttttaataatcgtagtgtatgagcctgtttgtttgtacctcggctaattccacctctacttggtggataacttgtctgccaaaagttggacagataagaagaaatcacctagtttatgaaatttaaacacacatggtttatggctctttgaagttgaagaaatatggaagttaaatataattaagcgcaatttttaggtcacctttaccactaaactaaaaccttcacttttgtttagacaacctttttaaaattttctggtgcaatgaggggttatggaagggtacgggaaaggggatagcaagaattgaacctacatatattgtgtcgaagactcctgctttcgcgcacctagactaattccatgtgatacctattactctatccaccaaaactaggatagatgggaagaatcacctagtgttttttgtctcctgatatctcatggttctcaaccactaggtcacaagtgaaatttttacccttttgtatactgtaattctctaacaaagatgatcaaatcctcttcaaaacatgtaactccgtccatgaactctcgataagggacttaaagaagagaagacaactatggtttatttgtttttaacacattttaatttattttataggtgtttattctgtaacaatagactctgaagatgggacggccaagatttctggtgaagttgatccgaacctcctcttgagggcgttgtcaagatcaggccttggcaaccatgcagaggtgaaatgggtgagacttaagcacccaatgttgagtaatagtcatatgactgatggatatggttcctataatcatggatatggctctcataatcatggatatggttcttataatcaaggctatggttataacagttatggccac

SEQ ID NO: 29 - DNA, 1991 bp, Solanum tuberosum
  source 1..1991: mol_type = other DNA
gcgcgcgcagaacttcacagttataaagctcggatttaccaattttcaaacaacgtaaacctgcagagggaagagaaaatggagggaaagcgttcaaacacgcagccactaacactcataaggaaaatcaaaggatttactcgttccattgttgaggatctcgctcgaggtagggcaccgttgatctacatcgatcggttcagaaattactgtactgacacttctggaaattgctcttgcagctctggtttgtctactggcaaggaagctatatccctgaagagggaatgccatgcacgtaggcttgatgttttgttgagagttcttgtgatagttcaacaacttctgcaagaaaacaggcatggatcaaaaagagacatatattacatgcatcctactgtttttaaagaacaatctgttgttgatcgggcaattaatgacatctgcatcctcttgcaatgcagtcggcataaccttaatgtggtgtctgttggaaatggattggtgatggggtggctgcggtatgtggaatctgggaggaaaattaactgcattggcaatcctcacactgcatacccgattccggtccttgttgaagaggttgatgatattattagtgttgctcaatacgttttagttgtggaaaaggaatcagttttccagcgactagcaaatgatcagttttgcaagaggaaccgttgcattgtgataacaggaaggggttatcctgatgttcccacaaggaggtttctgcgtctcctcattgacaagctgcatttgcctgtgtacggcctggtagattgtgatccatatggctttgacatcttaactacatacaaatttggttctttgcaaatggcttatgacgcaacatttctacgagtctctgagatacaatggcttggagtatttgtccaggattgtgacaattatagcattccacaacaatgtctcctgcctttaactactgaagataagaggaaagtcgaagcaatgttaccgagatgttatttgcaaagagaagtaccacaatggaggtttgaactggagctgctgttgcacaaaggagttaagtttgagattgaagcattgtctgtacattcactcactttcttgtcccatgagtatctaccatcaaagatccacaatggaggggctgtattttgaaagtggacgttcattgtgatgcatgcaagatgaagatggtggacgttttgagttctatatgcggtgtttattctgtaacaatagactctgaagatgggacggccaagatttctggtgaagttgatccgaacctcctcttgagggcgttgtcaagatcaggccttggcaaccatgcagaggtgaaatgggtgagacttaagcacccaatgttgagtaatagtcatatgactgatggatatggttcctataatcatggatatggctctcataatcatggatatggttcttataatcaaggctatggttataacagttatggccacggtcatggccatggctatagttctattggtggtccttttatgcaaagaagatcgttgcccgaatataactatggttatgagggacaccacaattaccaatatcctttcagggggactgcacaagactcctacgccaccaactattaccccggtgctctgccatcacctaggccgtacaacagctattatatgtagagaaccggagagattttaatggctcgttggctttcaccgtgacaacaagaagttgtttgcgtgaatttttcttcttaattttgtttacaaaacgaatattattatatatttatagggtagttattattgaatatgtttactttttgttcaaagttaaacagctttcatctgcactcaagtaaatttacttgttggattttcatcaaggtagctgatgctttactttggtaagtatatttgttgctgctgaagtactatgccttttattttccaatatttgaaatgaataagcagccttgcaatttc

SEQ ID NO: 30 - protein, 362 aa, Solanum tuberosum
MEGKRSNTQPLTLIRKIKGFTRSIVEDLARGRAPLIYIDRFRNYCTDTSGNCSCSSGLSTGKEAISLKRECHARRLDVLLRVLVIVQQLLQENRHGSKRDIYYMHPTVFKEQSVVDRAINDICILLQCSRHNLNVVSVGNGLVMGWLRYVESGRKINCIGNPHTAYPIPVLVEEVDDIISVAQYVLVVEKESVFQRLANDQFCKRNRCIVITGRGYPDVPTRRFLRLLIDKLHLPVYGLVDCDPYGFDILTTYKFGSLQMAYDATFLRVSEIQWLGVFVQDCDNYSIPQQCLLPLTTEDKRKVEAMLPRCYLQREVPQWRFELELLLHKGVKFEIEALSVHSLTFLSHEYLPSKIHNGGAVF

SEQ ID NO: 31 - DNA, 6684 bp, Solanum tuberosum
  source 1..6684: mol_type = genomic DNA
tcttttatggttcagtgtaatcacttaaactttatttgtaacaattaaattaagcctcttgaacaagaacactaggggacacgtggaagccattcaggaacgatagcacataaattccatcacttgagctgtgacttgagttcatcaaacattcattcttcaataggtgcgggccccacaatatactctgcaaaatgcaatcgaaatcgcatctgttatggcgggtatactctatagtctgtacagacgcacaggcacaaaacacacactttcacctttctcactttgcatgtgatctctctctctccaactatatatacaaaaccctctagcttcatgtactctgcaaaatcagtgctgaaatctccttctccacgacggcaatatgttctactctcatcagcttcttgctcgcaaagctccgctcggccaaatatggtgaaaattgtcgattactacttgtcatttcgattttttcctttcgaaattcgttattttcatatgcatacgttacatttttggagtttctgcgtttttacttgcatatgttgtaaatcctgagctagatttatgtttccttctttagtcgctgtttaatgatactcagtagcttcttcacgcgatttctcgtaatctgaagttatgagttatatgttaagttgtcactgttgaattggatccgtttctgttcggaaaatgcttaaattcaaattgtttatgaatgtattgatccagtttactacaacttttgttttgattttctattctaaattcgtttaatacatatagataagctacatgttttgcgttttaaactttcatatatcgcaattcctgtagtggatcatcttttggtcttttgcttttctgtatctaatgtaatgtattcgttgaagttccttcataggattttcggtatacgttaagttttcacatttcaatttgactacgaagaatgtttaaattgatgctgtttatatctctctctttgctgtgaaggatggcggccactctacactcgaaactcaataggaaaaagcttagtaaactcaatattattaacatctggtgaggcgttgtcttccactactacgttgaactgcctttattccttgttgattttgagtaatcatcttctgcaatttcttttgtcacagtgaacaaatcttaaatccatcagtcccgatggctctgaggctctctggaattctcatgggtatgcttcgaaaaccaccgactgtccgcaattgctgctttcggtttagatatctaatcgtcagttctatctcaggtggagtagtcattgtttacgaacgcaaagtgaaactcctctacggtatgaattgccatgacgacttcatcatttctatttgaatttcgcgtcaatttctttgaattttactcctactttccccttccttattgcttcaatttttgttttctttatgttttcttaaatgcagaggatgtgactcgtctcatggtagtaacactggtcttcgatcccaatcaacttaatctctttctttgctctgttttcattaaattcagcatttatgatttggtattttcaggtgcaaattaatgaagcttggaaggtcaaagcagctaccgatcctacgttacttcccaagggtaaatcgcaagccaagtgagtaactcctctccaattcgacgtcacagtattttgccgagaagcagagagggcgaatgttaccaactgtttaatagtttcagttacttcgatagtgcttcagtaaattaacaacttaagtatgaactgccaccaatcatttgaattattaactcaatttattatggtttatttcactcaatgtttgggtcagtttcatcaatgggttatttaaggccagcttatgctgtgaatcctctagttgtttttcctaaggttgatacttaacttttcattcctcatttcaattcctgtaggtatgcagctgttactctgccagagaatcgggaggaagaactccctgagattgaacagacgttacgaaatccagacacagtcacaatgatggatttcgaacaaacctcatatttcacgatggtacattatggaaagcactgagacctcctcaatccacgaaataacttcaaaagcagaaacaaaaattgttaggaaaaataggaatttgttggaactgatctaattagactattgagcttgctttagattgttcaataagttgtgtttcattgttcagcaagtttgcaagttcaacaatagaaagttaacaatgataaagtggtttgatttcccttcgctttcttttggttactccatatgttttgtaatttgttctatgttatttccactcttgagttgtttaagctttttgagagactatcaaaagttacttgggttttgtcagtgttcatgaccttgttgcgtaggcaatcttatctgataccacttggattagagtaggaaatattagtgaaaataagatcataattgataatttctacatgagagtgcagctaaactcgcggatgttcaatgtgcagagactagataatgctgatctctatgataaacccaatgcacagaaggaacctgccaaggacttgcatcaaggtatacctagatcccactatcagcatagattatgctaatttcaccatcacagtagaatatataactatatcctagtcaatgctactttgttttccagttttgtcttgttgtgcccatctctaaacaatcctgaaaccctttttgcagttgatccagataatatcaccctcgctgaacactttgaatcccatcatacagatatgttcaatcattttgagaggtaccacgatgaacagttagtaggctctgtatttctaagtttatatggtcagttagcataaagacttcacgtgaaccaaactatccatcattaaatcacaggaggctaattagcctcattttcatttaactgcaaagctttccttctattatcctcctattaatttttaagcatgaattactctgcaggtttgatattgaaggggatgaagaaacacaaatgaattatacccagccagaggatgctcaaatcccaagtactcctgtgccatctccacctcgagaacaagcccatcaacgtaagaatgtgttactatcttctacgttagataaatgaagttttttgatatgtaaatagtagatggacttaatatgtttcactatttcacttggtgcgctttaagggagacttttctgatagagacattatggcaataaacccttcctctcaaagaggaacatggatgcaagtcgtacttacctactatcagatcagttaaaatactctgtggctacctggctgcttaacattaaacttccagtttacatatgtagttccttcaagcacagaactctattggattgagttgagctcgtaaaagtctttagatttccttaggtaattaattatttctgaaaattggttgaatggagcgaaacattattgcagctgatgagatccctgacagacatccagaggaccaagtgaagcaacaatctgatgaagttgaagaagcttttgaggtagaaactccacaagcaaccgagctagaaaataatgtaaagaaaaactgtcagcactaatcatacgtcttgacatgatattgtagcagcggcaggatcaacaaaggccaaagccagctcgacgaagagcaagaaaggccacaggtcttgcaattgatcatgagcaaactattatttctggtgacatatatcaatcctggcttcagagttcttcagatattgcatcaagaaaaaggaaaaagagaaaggtactcccatacctcccaagtctagatcttccccatctcaatttttccattctgtgcaccttagcaattaaaatttgactagggtctaatcctacaatagagcatgtttaacctttgacatcaatgactagtctttgagtatcctaagaatagcaagtacatctctctctggaaggtaaccttaactaaactaagatgcagcgtcatttattagtaaccttaagttcctgctctgtgcagactttgagagtcttacattctatgaagatagccagaatgatggaaatgcctcctattgcactacttgaaggattgttcacaaatggaaataaggaagttcactatccagcaccactcctaaaattatggatgaggaatacccaacctccgcatgattcaccttctggtctggtttttcatccatgatattagactcttagttgccaaaactacaaacagatggtaattacgtttgacttgcaggaaagacctctccaccctatcctcctgaaccatcctatacatctccaggtgaaaggatgggtaatttggaaccgcctttcgaatatttccaaagcggtgtaggctccccagcagtaggaatctctatagaaaaacaaagggcaaatctcaacaataacaagattccacctgaaattctcatggaggacctcagaaccaatcttacaaacatgggactgcatccaacagtggctaatggagtgaaagagactgatcacatggccacacctggctctggtatatctatattttttatgaatttcccaatctccatgatttgttcggcgatctgttatggtggtataactaacatttttgtgaatctataggtgatgagcctagatccattccaagctcaggatctggtcatggtttactatcacagaattctgtaaccaattcaagccggttagtactactagtagatataggttgagggatatttgtctaaagatgaaccacttgaatcatacagacaataacagaaggaaataatgaatatcatggatctcggtaccataggaaactttaaaaactttgcttctttttaaaattacgaaggtctcaccatatagcagcatctggttacattgatcaaaattgttaactcttcaggtccaacaagaaaagaccccattcttcatcgaagcacagtggcaatggtcttcaaccagtagcagaagagaacccatggcacgaccccactccaaatttcaagttgactagattatctgaactatctgaaaatggttttacacaagacaacggtttgtgaatagtcaataactttcccattttagttctggtcattttctttaatgtggtttagtttgttatgaacctccctttactcttttggcagagatattgatggaaaccggaccaacacaaacccaacatccatttattactcaacctcttgacatgatgactgactctatcaggatgtaaatccttttccattagttcctaaaatttcctccagcttcattatatatcatctgactaattgatttttcacatgataaactgatgcctacaggcagctaaagagtcattttgacactcccggatcagccgaagcagaatgtttgaatgaactaactcttgggatgacaaagaaacaagcagcatgtcttttttatcagacttgtggtgtgcatatttctttcatatcttttactctgcattgcagcacagagaaaatttatagtttccagctcatctcattagagagaattaatgtttgctccattctatgtgcagttctggccactcgagacttcataaaagtcgaacaggagcttccatatggaaacatcctcatttccagaggtgcaaagatgtgacaacggataaatagagaagatgctaatccctcacaagtcttataggttcatttattgttatagctgatacaaatttgtttttcggttaaggtattggagagttcaggcacagatttatagctcgatttatcaggagaaagtatttttattgttaacctgtctagtgtttaatcgtagaagcatagttgtctccaagagaatacagataggagtacatgattggtcattctgaaactagcgaattgcatattttgtactagcatttggtgacagctatttgttttaaaaagtgtatgaaggtcaaatgttgagaagctaaaaagatagtaacacatggaagtgctatgtatacttccagtcagacaaaacagaaatcataacagttcacgaagtcattggacaacttctctgcaatgttatcaactttcttttcttttgcttttggtataacgacatcatgctgcaatgataagatgggttaactcatagtacattgttggttttgaagtgatgtcccgaaatctattttatttgaataaaactatgtagtgcagtaataactgtgcactacaaaccatgttcagttataggccagtcttatatcgaagcctctttactcgatcaaaacacccaatagaaacataatacacctttctacaaatgcagtgtgtacactgtcatactaagaacaatattcaatagttggctcatctacagtcacctacaactttaacatgattgaatacaaacatctcaacagattaagcacatccaatccaggtttacattctgtcttccctccaccatggggcatatgtgacgatttcatcaaccttagtatcatctcagcagcctcggttgcagatagtaacacagcctgtttgactttgaatgcctccgatattcctagttctgccatatctccaacctgtcataaaagccagataagatgattagattctagcaaaatcctaactcccaataagcagcaggaatcaat

SEQ ID NO: 32 - DNA, 2016 bp, Solanum tuberosum
  source 1..2016: mol_type = other DNA
atggcggccactctacactcgaaactcaataggaaaaagcttagtaaactcaatattattaacatctgtgaacaaatcttaaatccatcagtcccgatggctctgaggctctctggaattctcatgggtatgcttcgaaaaccaccgactgtccgcaattgctgctttcggtttagatatctaatcgtcagttctatctcaggtggagtagtcattgtttacgaacgcaaagtgaaactcctctacgaggatgtgactcgtctcatggtgcaaattaatgaagcttggaaggtcaaagcagctaccgatcctacgttacttcccaagggtaaatcgcaagccaagtatgcagctgttactctgccagagaatcgggaggaagaactccctgagattgaacagacgttacgaaatccagacacagtcacaatgatggatttcgaacaaacctcatatttcacgatgagactagataatgctgatctctatgataaacccaatgcacagaaggaacctgccaaggacttgcatcaagttgatccagataatatcaccctcgctgaacactttgaatcccatcatacagatatgttcaatcattttgagaggtttgatattgaaggggatgaagaaacacaaatgaattatacccagccagaggatgctcaaatcccaagtactcctgtgccatctccacctcgagaacaagcccatcaacctgatgagatccctgacagacatccagaggaccaagtgaagcaacaatctgatgaagttgaagaagcttttgagcggcaggatcaacaaaggccaaagccagctcgacgaagagcaagaaaggccacaggtcttgcaattgatcatgagcaaactattatttctggtgacatatatcaatcctggcttcagagttcttcagatattgcatcaagaaaaaggaaaaagagaaagactttgagagtcttacattctatgaagatagccagaatgatggaaatgcctcctattgcactacttgaaggattgttcacaaatggaaataaggaagttcactatccagcaccactcctaaaattatggatgaggaatacccaacctccgcatgattcaccttctggaaagacctctccaccctatcctcctgaaccatcctatacatctccaggtgaaaggatgggtaatttggaaccgcctttcgaatatttccaaagcggtgtaggctccccagcagtaggaatctctatagaaaaacaaagggcaaatctcaacaataacaagattccacctgaaattctcatggaggacctcagaaccaatcttacaaacatgggactgcatccaacagtggctaatggagtgaaagagactgatcacatggccacacctggctctggtgatgagcctagatccattccaagctcaggatctggtcatggtttactatcacagaattctgtaaccaattcaagccggtccaacaagaaaagaccccattcttcatcgaagcacagtggcaatggtcttcaaccagtagcagaagagaacccatggcacgaccccactccaaatttcaagttgactagattatctgaactatctgaaaatggttttacacaagacaacgagatattgatggaaaccggaccaacacaaacccaacatccatttattactcaacctcttgacatgatgactgactctatcaggatgcagctaaagagtcattttgacactcccggatcagccgaagcagaatgtttgaatgaactaactcttgggatgacaaagaaacaagcagcatgtcttttttatcagacttgtggtgtgcatatttctttcatatcttttactctgcattgcagcacagagaaaatttatagtttccagctcatctcattagagagaattaatgtttgctccattctatgtgcagttctggccactcgagacttcataaaagtcgaacaggagcttccatatggaaacatcctcatttccagaggtgcaaagatgtga

SEQ ID NO: 33 - protein, 671 aa, Solanum tuberosum
MAATLHSKLNRKKLSKLNIINICEQILNPSVPMALRLSGILMGMLRKPPTVRNCCFRFRYLIVSSISGGVVIVYERKVKLLYEDVTRLMVQINEAWKVKAATDPTLLPKGKSQAKYAAVTLPENREEELPEIEQTLRNPDTVTMMDFEQTSYFTMRLDNADLYDKPNAQKEPAKDLHQVDPDNITLAEHFESHHTDMFNHFERFDIEGDEETQMNYTQPEDAQIPSTPVPSPPREQAHQPDEIPDRHPEDQVKQQSDEVEEAFERQDQQRPKPARRRARKATGLAIDHEQTIISGDIYQSWLQSSSDIASRKRKKRKTLRVLHSMKIARMMEMPPIALLEGLFTNGNKEVHYPAPLLKLWMRNTQPPHDSPSGKTSPPYPPEPSYTSPGERMGNLEPPFEYFQSGVGSPAVGISIEKQRANLNNNKIPPEILMEDLRTNLTNMGLHPTVANGVKETDHMATPGSGDEPRSIPSSGSGHGLLSQNSVTNSSRSNKKRPHSSSKHSGNGLQPVAEENPWHDPTPNFKLTRLSELSENGFTQDNEILMETGPTQTQHPFITQPLDMMTDSIRMQLKSHFDTPGSAEAECLNELTLGMTKKQAACLFYQTCGVHISFISFTLHCSTEKIYSFQLISLERINVCSILCAVLATRDFIKVEQELPYGNILISRGAKM

SEQ ID NO: 34 - DNA, 5995 bp, Solanum tuberosum
  source 1..5995: mol_type = genomic DNA
taaatactttttcattttagtttgaatttatggatgagttaaaaatagtcgtgcttagttatattttttacaaaaatatttaaaacaataacattcatataaaattataaataataattgaatgtacttaaatacaattcaaaaagggaaatgtgagatggaaaacatgtcataacctattttcaaatttgaaatacaacttttagttgaatttaaaaaatttcatagccaaatttaagttttcactttataaataaaaaaattatcttcttacaaaatttcacaattaaacatgaccaaacgcccacgaaactatctaacatatactttttttaaaaaattattataataaatttctttttctgactttaaattcaaacattactttcaaattcaactcaatgcatatgtactaaacatagtataaaagctcacttatttcattccttattaccaaaattcatttctatttatataatctgtcaattaccatataattaggacttataatttgaaaattttattttttcccaaaaaaaataaaatcttttttctgtttgtatttggctttattagagtgaattaaaaaacaaaggggctttttttctgggtgcactaaagtcaagaacgaatccgcttcaaatttgaattcaaaaaaattacacactaaactcacagcaccttcatcacccgcagtacaattaccatacgtgtcttcatatgattggtccgtcacttttttattctcaactctaattaaacagatgatttttagtgggcccaactttgtccgctcctaacgaatacctaaatcaaatggacggttcagattaaatcaatttaaatgtattatttatttattgcttttatatattaacttcacatttttcacaatttgagagtaaacacagctttcttcttcttcttcgtttttcttgaagaggaggattgatgaaaaattgttaatttttttgatcgtttttttgatttgaaggagaaaatgatgacgacccagaataggcgttcgtctgtttcgagtgcggtagcgaagagacaagcaatggcagcgaattcatcagggttagagaataatcagaccggaaaattgaatgctggagcggccaagaaacgaccggcattgtctaatatctcgaatcatacaactgtttctgctcggaactcgatttctcattcctccaaacttgtgagtgtttctctgtttttggtctctgtttttgtatgaaatggcttgattatgtgtattttactgtaggaaggtgattagcgtactggggttttctttctttgcgttgtttggttactggttcgacgatttactttttcgtatgttggttatggcctatggggtttcttgcgtaaattagagtactgggtttttctcttttgtatggtggtaatgggttttttttgttgccggttctaaggaggaaaatgcagagtactgggttttgtgatttattttttggcgtttttctttcttggagtttcataaacattagaactttcttaaaaaatgatcaagatactgggtaaaaatcagtttgagaaaatcatgttaagtgattttcgagggtttttgatatgaggggatttgtgggttttcattttttttgtcaagatttgttaattggaagttaatttttttgttaattgacttgtctttttttgaacaagttcactgttttgtgcaggaaatgcattagttatcaagggatttgttttatcttattataaattatgtttgagttaaagtatttttttaatggttaaaaagtattatgaatggaatatttgaaacatcttcccccaattcctgccttttgtttatctgttcactttgttttttgaacatttgaagaaagttctaatgtttatgttattaggttgaacaaaagttcttgctttttttcaaatggacatagtatcattggacaatcatgaagtggaccagtggcattctagattatttatttcagtgttaacctgaattgtttagcatatcattactgtggaccagtggaccaattcctgctttttgtctccttaaatgattatattactgttcttaatttgattatcattacacaaatgagcagaagaagttaagcaacttttgatattttttagttttcacagttgggattaaccttttatttaatatactgttttgcaatgtgtgtaaattgaaaaaagattgcttcttgtatctgaagttgtgactaacttggaatcatttttgactttggaaggcaccatgtacgtccaagattgtaagcattaagaagaacatttcctcagggactgctgttctgccagcatcctcctctgtcagaccaagcagcaaacctgtttctattcaaagaagtgatgcagttgtgcctaagatcactgccattcctcttcctgccacctgcagcatggacatttctccatctcactcagatggatcattagtctccatggatgaatctatgtcaacttctgacacagtgagaagtccggaggtcgaatacatagatgaccttgaatcggctgcagttgattccatcgagaagaaggcgtgtagcaccctctacatctcagaacatatcaaagccgcaggttttgatcttttcagcagagaatagtccttgttctagcatttcattttaactataacatctatttaatacaatttatctattttttattccagcagcagatatatgcaagagagatgtacttgtggacttggaatcaggggacaaaattgtcaacattgataacaatcttgttgacccacagttatgtgctacaatggcctgtgacatatatacacacttgagagcctctgaggtataaaaatgctgctaactttaactgaattgcagttttacaaacatttgttatcaaacatgttttaatgtcatctttgatcactgtactaggcaaagaaaaggccttccacagatttcatggcgaaagtacagaaagacatcaatcctagcatgcgcgctatcttaattgactggcttgttgaggtaaatttctaatatctttcttctctaaagctgtgtccctgatgaaatgtcagcctgcccaacttacgacttaattaataatgtggatgagctcagaaattgacagtttgatatggaacttgtttgatgggtataggttgccgaggagtacaggcttgtcccagacacgctgcatttgacaattaactacattgatcgatatctttcgggcaacttgatggacagacaacgactacagttgcttggagtagcttgcatgatgatcgcatcgtaagaaactaccttctgacctctactgcatatgttttcgccatgatctttacaaaattttccttgagtgcttttcatattcttgtgtccttgaatattacaagcatatctgtaagaaaatgctttaagacattaatatgggaaatgctttattgcagaaaatatgaggagatctgtgcacctcaagtcgaagagttctgctacataacagacaacacttacttcaaggaggaggtatatgatcttgattcacagaacctgcagtggttgaactttgcagtggcactaagacttaacgtattatgcaggtgttgcaaatggagtctactgttttaaattacttgaagtttgaaatgacagctccaacagccaaatgttttctgaggttaatattcttaccatgatctagtagttgcttttgagtatgatgattaggaacttattgttgagtatactgcaggaggtttgttcgagctgctcaaggacttaatgaggtaacctcttcacttaaggttgataattctccaattatataagaaacaagagttgattaaaattttataatcatctacaggttctgtcactgcagttggaacacttggctagctacattgcagaactctctcttttagaatacaacatgctttcttatgctccatcactcattgctgcttctgcaattttcttggccaaatatattcttcttccttcagtgaaaccttgggtatgtacgaattagcattgtgacaatcatataagctgttacaatgcatttttgcttcttactctcctttcgacaaatatattcttataaaatttgacttttggaaactcctaacagaactctaccttgaggcattatactttgtaccaaccctctgatttacaagactgtgtcatggcactacacagcctttgctgcaacaacaacaattctagcttaccagcagtcagggaaaaatacagccaacacaaggtaatttatcctagccccttctgacaataaagattagtggaatgaagtcctaacatatgtatactttctagatataggtttgcatagttctcttttcaattcatcccaagcctgtatactggagtctggactgcacttaaacattctattatattggaaaattaatatttcttctgaatcttcttggataaacgatcaacctttctgggagataaatgatcaaccttctctcaacactagtcaaatgatgttaactgaataatgacttgatagacatatatgtttatgtacatacagagtcatgtaggcatctgcatacatttcctatcgagtttctaacatatgtatactttctagttataggtttgcataattctcttttcaattcatcccaagcatgtatactggagtctggactgcacttaaacattctattatattggaaaattaatatgtcttctgaatcttcttggataaacgattaacctttccgggggataaatgatcaaccttctctcgacactagtcaaatgatattaactgaatgacttgatagacatgtatgttcatgtacatacagagtcatgtaggcaggcatctatcgagtttattctaatgtttggttttctgaaacagtacaaatttgttgcaaagaagtattgccctccaactgtacctgtagagttcttccagaacataagcagctaagccagggagatgtgagaagaggcatcaacttcagtatttccaattgtctgttggattaactcatggcattcaatcttatatagcctttaacttgcaatgtccatggcagagcttcattcttggtttttctctccttgaggggccttagcagagtatcttcgtttgtagtcattaacattgacattgcaggattagtctcttgtactcatactgtttttctctggcttagttagtctagtcagtttgtgtacagaagaagcgctattggctgtttcattaactcagaaactattcagtaatgattccttggtggaactattgcagtttgtgccaattagtattgagaagaacattacaactgatcaaagccttgatttctcgtcctgtcaaatgagcaactggtgcaactcaatttagagttgtacagaagttgggtgaagaaaaaaggttgagcaccaacacattgttattctatgttttgcatctatgaatttgctcataatttatatcgattaaggattcaaccgtatacattggcaaaaatattttacaccatcacaatagacgttgagttgtatcaacagatacattgttattctataatttactacatatagcacagaaacacaagccctataagagaagttcattgagcacactcaatcttggcagaacctaagccaaaggatgcatccattacactggcattaggcctaacattcagccagtgacaatcttcaaaggaacagggatgtccaccgttaggccattctacatccacaggttttatgaaagtagggccccaagcaggcgtaccatcctcgtacgaattgtgtgttaatcttcggatgtccgagccgtctgatttgatcacatatatatcaccatatggctgataatgatgagggttcgagatgggctcagctgatacagccgcgtaatctgaagtgaaaactatatacttcccatccgggctgaaataggggtggttagtcctccc

SEQ ID NO: 35 - DNA, 2036 bp, Solanum tuberosum
  source 1..2036: mol_type = other DNA
tcacaatttgagagtaaacacagctttcttcttcttcttcgtttttcttgaagaggaggattgatgaaaaattgttaatttttttgatcgtttttttgatttgaaggagaaaatgatgacgacccagaataggcgttcgtctgtttcgagtgcggtagcgaagagacaagcaatggcagcgaattcatcagggttagagaataatcagaccggaaaattgaatgctggagcggccaagaaacgaccggcattgtctaatatctcgaatcatacaactgtttctgctcggaactcgatttctcattcctccaaacttgcaccatgtacgtccaagattgtaagcattaagaagaacatttcctcagggactgctgttctgccagcatcctcctctgtcagaccaagcagcaaacctgtttctattcaaagaagtgatgcagttgtgcctaagatcactgccattcctcttcctgccacctgcagcatggacatttctccatctcactcagatggatcattagtctccatggatgaatctatgtcaacttctgacacagtgagaagtccggaggtcgaatacatagatgaccttgaatcggctgcagttgattccatcgagaagaaggcgtgtagcaccctctacatctcagaacatatcaaagccgcagcagcagatatatgcaagagagatgtacttgtggacttggaatcaggggacaaaattgtcaacattgataacaatcttgttgacccacagttatgtgctacaatggcctgtgacatatatacacacttgagagcctctgaggcaaagaaaaggccttccacagatttcatggcgaaagtacagaaagacatcaatcctagcatgcgcgctatcttaattgactggcttgttgaggttgccgaggagtacaggcttgtcccagacacgctgcatttgacaattaactacattgatcgatatctttcgggcaacttgatggacagacaacgactacagttgcttggagtagcttgcatgatgatcgcatcaaaatatgaggagatctgtgcacctcaagtcgaagagttctgctacataacagacaacacttacttcaaggaggaggtgttgcaaatggagtctactgttttaaattacttgaagtttgaaatgacagctccaacagccaaatgttttctgaggaggtttgttcgagctgctcaaggacttaatgaggttctgtcactgcagttggaacacttggctagctacattgcagaactctctcttttagaatacaacatgctttcttatgctccatcactcattgctgcttctgcaattttcttggccaaatatattcttcttccttcagtgaaaccttggaactctaccttgaggcattatactttgtaccaaccctctgatttacaagactgtgtcatggcactacacagcctttgctgcaacaacaacaattctagcttaccagcagtcagggaaaaatacagccaacacaagtacaaatttgttgcaaagaagtattgccctccaactgtacctgtagagttcttccagaacataagcagctaagccagggagatgtgagaagaggcatcaacttcagtatttccaattgtctgttggattaactcatggcattcaatcttatatagcctttaacttgcaatgtccatggcagagcttcattcttggtttttctctccttgaggggccttagcagagtatcttcgtttgtagtcattaacattgacattgcaggattagtctcttgtactcatactgtttttctctggcttagttagtctagtcagtttgtgtacagaagaagcgctattggctgtttcattaactcagaaactattcagtaatgattccttggtggaactattgcagtttgtgccaattagtattgagaagaacattacaactgatcaaagccttgatttctcgtcctgtcaaatgagcaactggtgcaactcaatttagagttgtacagaagttgggtgaagaaaaaaggttgagcacc

SEQ ID NO: 36 - protein, 488 aa, Solanum tuberosum
MMTTQNRRSSVSSAVAKRQAMAANSSGLENNQTGKLNAGAAKKRPALSNISNHTTVSARNSISHSSKLAPCTSKIVSIKKNISSGTAVLPASSSVRPSSKPVSIQRSDAVVPKITAIPLPATCSMDISPSHSDGSLVSMDESMSTSDTVRSPEVEYIDDLESAAVDSIEKKACSTLYISEHIKAAAADICKRDVLVDLESGDKIVNIDNNLVDPQLCATMACDIYTHLRASEAKKRPSTDFMAKVQKDINPSMRAILIDWLVEVAEEYRLVPDTLHLTINYIDRYLSGNLMDRQRLQLLGVACMMIASKYEEICAPQVEEFCYITDNTYFKEEVLQMESTVLNYLKFEMTAPTAKCFLRRFVRAAQGLNEVLSLQLEHLASYIAELSLLEYNMLSYAPSLIAASAIFLAKYILLPSVKPWNSTLRHYTLYQPSDLQDCVMALHSLCCNNNNSSLPAVREKYSQHKYKFVAKKYCPPTVPVEFFQNISS

SEQ ID NO: 37 - DNA, 4889 bp, Solanum tuberosum
  source 1..4889: mol_type = genomic DNA
cgtatttcctctcacatcttctgcattgaacttcaccggttatcgttgtaatctgattcaatcgtagcatgttaagactgtgaacctttgctcgatgattagtcgcccatggataaggcggtggaatcgtttcacttttcaatgtgcgctttcgcttacgtggacggcgagaagatggtggtggtggcggtggaggtggcggtgctacgacgggaggaggaggaaaagatagagacaatgtaagcaagttattgtcgatttcattgctgtttgttgccatttttttgttgtttgtctacagagaaatggttatataaggaagagaaaaatggaaatgggaagagtttgttatgaatagtactgtaaaatgtacgagaagataaagacgaaacagaaacagagcaggtagtaattccatttggtttagacttcttttttttttaatttcgaaatttttttggccttttcagattctgtttaagtgggaatggatttatgatgtgtttttatctacaaataaaatctttaatactccaagattttaaaaaaataaaaattcacggattatttttagttttaagttattggatagacgtctatttaagttaattcttcttgaattttttatttgatggaaacaagtcatttgcacttatgtccctagtttgttggtctttaatttctatctgataaggcaaataactttctcgcgagacataacttgatatttttgaattataatactccaaaagttatgccgcacacccttaaagttggatttttaggacaaaaattaaaaatttaagaccaattcatttaaacgataaactatgcaattaaatcaactgaaatttgtcccatcgccggccccaattttgcttatcatatagcccaagtgaagtgttataaattcagcccatatccaaaagtgggccaaatcaaacactatataattacttagcctccgaattcaaattgtagatttaccgccatttgaagcatgggagagttttgcagatcaaccattttcttctccgatcaacacctctgctacgccgatatccttcctccttcacaggtaactctccgtcacaaaaacaatcgcagatttgtagcagtgttgaatgtatgaattgcttcatttagaagttcaattaaattaaatcggatcgataattgttagtccatgtgaaaagttgaacggttagattcaaaattcaaaccgtattgcgatttcagcatgtctttgttttctcatctaatcgaatttatctattcaggttcgagctagaatcgaagttgcggtcctgaattttctcaaagctctaagttcaaactctccgtcaatttccgatctatcactggtttgaaattttacctcttcatcttttcgaaacaaaatccctctataatttgcacttttagcctactttatatgcgtgctgtaagtatcagtagcttctgtgcatactataatgaaatcccaaaaaggttgataaactccatcttatttatgctttcttaattgatcagaatgcttattgttcatatcagaagaggaatttaagaaaaacgtagatttggaacaaaatttagcaattttaggagatttatatgtgaacctctctgtcacctcagagaacaaatgatttaccagttctgggatgaattaggcctgaatataaatggatacagatgattcatatagtggacgtcaacaacaggcatagttgataatttatatatatggctgatacagatcagtaggaactccaacaatatcagagtgtgccgtgggttacttaccggtgattcatggatcttcctgtcccattctttttgcacgcgatctttgacgagagagaatagtgccaagtcatttataagaggtaaaagactacaagtttcttaccattgaattacttatggacaaatcaataatgctggctatgtttttgtgatcaagtttggaaggttatggagatgtgctaccaaattctggttcaggaaaagagggtgacacagagagagctatactacaagctgctctgtgattcaccagattatttcacttctcaattgcaggttaataggaccatccaaggtcattgttgtttcttctttcttcatcatttctgaatatgatctgagtgttcggttgattttgttaacacgaggtccttcatttactatctatgaggaacagacttggtggctttgcttcgatgcagccgttacagccttggaataatggcatcaagcagaggggcaatagcaggccgtttattgttacaggtactattatcaaccctttggttgtaatttcaaatgtttatactttaatttagtcaaacgcgtagcagtattagtaccttgacttggccactaacatgatctgtcatattggaatgaaataggccatgtacaacaaatggatatagagaattcatatagcccatctcaactagtttataattgaggcacagctgattgattgatttcaatatgagccaccctagtcaaactttcaatgtttccaagtttctatagttggtaaaagctagctgctggtagctgtctatgatcaactattttgctttgtatcttgattttgtgagaaaactcaaggaacctaatacttacatgatgtacaagtcttaaagttcccatttgaagcttgttcaagaatttgaaataggcagtaaataaatcagtttatccaacatttagaacttggtatttctttcttctaaagatggatatatgactttaagttttttctttaaaccactgagataggagccagacaaggaagttgttgactgctctacttgtggatcttcgggttatgctatatcaggagacctggaattgttggaaaaattaaccatggaaacagatgcacgatacatcatcatggtggaaaaggtaatttatcacttgttggaaactctagtcaatcattttttgcaagaaactaaaactagttccactttttagcatgctatattccagcgactagcagaggatcgtgtattcaatcagattccatgcattctgattactgccaaaggatttcctgatattgccaccaggtgaggtgaagagttctaaacatcttcaaagaaaattcgtttattctgacgttctagcttacagaatagctgctagaagattgttcattcaattattacctcattacatattctaatctctaaaaacatattcaggtttctgcttcatcgaatgtgtcggatgttccctaatttgccagtcttggggctggttgactggtataactgacttcactagtattgccaccacatagttgctgagcaaagttcttacaaatcaaattgtgattattaaggaatccagctggattagcaattctctgcaccttcaagtttggaagcatagggatgggacttgaagcatacagatatggtgctcttttctcttaaaagttatgttgaatcatatatccttgttgtcttcttaacttcacttataggagtctgttcctctacatgttttttaagcttgtaatgtcaagtggttaggactgcgaaaggatgatattaatcaacttatacctgaagaatgtttggtccctttgaaacctcgagatctccagattgccaagagcttgatgtcatcagagattctgcaggtataattccagttactacgtaaacgtcatttattcctctattatttggtttggaaaatcttattcacctatttttaccaggatagctacaaagaagaggtggcagcaatggttcaaagtggtcgaagggctgagattgaagctctttattgtcatggatatgattacttggttaagttccttgcgacaaaaatagtacaagccaactacctctaataattcgaccgctcatcgaaaacagtactgagaaaatattgcattttccagaattgaatgccatctgaacgacgtaggaagttcaaaatttaaaaattaattttcgtattagaaattgaaaccattacggcttactcatgcagtgatatgttatgaacttctgatataactccaaaacaccacgtcttacattgagagataagattagggcattcgaatgaagtttgcatcgctgaccagtagggcaaaagatgcaaatctcaaacaaattcccaaaataaacttaacacatccaggctagggttaaactgaacaacatccaggatagtgttatgattgtgtatcaatttagtgctcacagggtccgggctgactgggcgagcctgcaaggtgactacacaatcaaccatatagagacgaaccgaattgaccactctataataaagaaaaaaatatggccattcagctgggaaaggggggttaaatctctcatctcatttgtgcaataacaaaattataaatgtgtaacaatcaaataattatgcatctgttaaataaataatacaacttataccgacctctattccttggccaaaaacacacaaatcatcacccaaaaaaaagattaaaacaaaacagcggggagggtagtagaagaggaggagaagaaaaagaacaagggcagatcactggatgaagaaatgactgcctaaatgctgtactcccctaaacgcaatgctgtgctccttgatatactcagcaaaacaaaataaaattgatttactgtgaacctagtctcggtggccatctacatttcgttactacagttaatctcagcaacggcaaaattctttcagttctctttaagaaagagacaccctctttccctccactgagaacttgtcactgccttcaagctgcatacaaggagagacatcatcagcatgctaaaagaacaatccaaaaagatgattgcaaagacagagaacaatatgtcctg

SEQ ID NO: 38 - DNA, 1233 bp, Solanum tuberosum
  source 1..1233: mol_type = other DNA
atgggagagttttgcagatcaaccattttcttctccgatcaacacctctgctacgccgatatccttcctccttcacaggttcgagctagaatcgaagttgcggtcctgaattttctcaaagctctaagttcaaactctccgtcaatttccgatctatcactgatcagtaggaactccaacaatatcagagtgtgccgtgggttacttaccggtgattcatggatcttcctgtcccattctttttgcacgcgatctttgacgagagagaatagtgccaagtcatttataagagtttggaaggttatggagatgtgctaccaaattctggttcaggaaaagagggtgacacagagagagctatactacaagctgctctgtgattcaccagattatttcacttctcaattgcaggttaataggaccatccaagacttggtggctttgcttcgatgcagccgttacagccttggaataatggcatcaagcagaggggcaatagcaggccgtttattgttacaggagccagacaaggaagttgttgactgctctacttgtggatcttcgggttatgctatatcaggagacctggaattgttggaaaaattaaccatggaaacagatgcacgatacatcatcatggtggaaaagcatgctatattccagcgactagcagaggatcgtgtattcaatcagattccatgcattctgattactgccaaaggatttcctgatattgccaccaggtttctgcttcatcgaatgtgtcggatgttccctaatttgccagtcttggggctggttgactggaatccagctggattagcaattctctgcaccttcaagtttggaagcatagggatgggacttgaagcatacagatatgcttgtaatgtcaagtggttaggactgcgaaaggatgatattaatcaacttatacctgaagaatgtttggtccctttgaaacctcgagatctccagattgccaagagcttgatgtcatcagagattctgcaggatagctacaaagaagaggtggcagcaatggttcaaagtggtcgaagggctgagattgaagctctttattgtcatggatatgattacttggttaagttccttgcgacaaaaatagtacaagccaactacctctaataattcgaccgctcatcgaaaacagtactgagaaaatattgcattttccagaattgaatgccatctgaacgacgtaggaagttc

SEQ ID NO: 39 - protein, 382 aa, Solanum tuberosum
MGEFCRSTIFFSDQHLCYADILPPSQVRARIEVAVLNFLKALSSNSPSISDLSLISRNSNNIRVCRGLLTGDSWIFLSHSFCTRSLTRENSAKSFIRVWKVMEMCYQILVQEKRVTQRELYYKLLCDSPDYFTSQLQVNRTIQDLVALLRCSRYSLGIMASSRGAIAGRLLLQEPDKEVVDCSTCGSSGYAISGDLELLEKLTMETDARYIIMVEKHAIFQRLAEDRVFNQIPCILITAKGFPDIATRFLLHRMCRMFPNLPVLGLVDWNPAGLAILCTFKFGSIGMGLEAYRYACNVKWLGLRKDDINQLIPEECLVPLKPRDLQIAKSLMSSEILQDSYKEEVAAMVQSGRRAEIEALYCHGYDYLVKFLATKIVQANYL

SEQ ID NO: 40 - DNA, 11093 bp, Solanum tuberosum
  source 1..11093: mol_type = genomic DNA
gagtatatgtttatgtattaccaaaaaaaagtgtttttagcaacaaaaaaaaaacaatcgcttaaacatttaccagccattaaacttttaatgacaattattttgtggcaagcatagttgctaaaatattcatacactagaaagaatctttactgttaaacaatacaacttgtacatcagaatagtaaattagtattgcaacttgatctattgtttcttttaatatacaatttaagatgttataaccagaaggtctctgcaacactactaaagaggactgtctacatcggtacgaaataatgtgcttgcctttacaaaaagaacacaatgccatgttctttatatctaagctggaagttgattagtctgagtagtgttaatgttaagataagtgacacttgaactatgtcctcctttgccaatgtaagataggtcgtcgtttttggttccataacatggatcatcccaaacctggtttttatgaatgtgaaactctggggcggcttaagcatagtagtggtttaaagtcaaaaccaaatgaagcccttatgacaagtttcttctaataattctttcattttctatgaaaactttattttttatacaaatagtattccatattatttttaaaaaataaattataatctatcattgttaagaaatgaggttctcaaatttggaggcttaaacatggatcatctcaatcctgacttcatgaacgtaaaactccgttcactaagtaccttgaatattgtccttttttcctacgatttgagtacgaaagacacagtatacatccatgaagatgtaatgttcatgaaaatataaccaacaatgaaattgaaatttataataatgtttaggttcgattcattgtcacaaaagaatgatggatatagagtattggctattcattaatttaaattaaaattctaaatttgtttttaaggctttaagcggcaatataaacacacccgaagcgaggcgcccaaagttccagatgattgcaattggcgggtatacagtgcttcttcctctgcatactgcaacttcaatggaaatcgaaatctcctctgtgaaaatgctctataaacatgtgagttttttttcccccaaacatagccactatgcatttctaatccaatttgaacttcactttcactcttcttctacttttgcagctcattttctgcgccgttcaacgatgccgcatgtccgatgatctttgcagattatccgtgaaattgacctcgttttctcgatttgcactcccgctcgttggaatatcaggcaacttctctctctatatatatgagtgtgtgtttatggtaaccgcagttccgactcttccttcagaaattcgtatctgttgtctcaatataatgccgtaattctgtatatttatgtctatgatggtataagaagatgcgtcatctgagagtgattcaatttggaagacgcattgattagtttttctggatttatgaaaatcacatttgcgagtaatttttctttctttctgatccgagacttttttatgcttgtaatagggaaatgaaattgcatttaagaaacaaaatacagagttgtactttgaagttcgaactgcagtttgatatattgtgttaatacagttagcagaaagaatctatgatgatgaatcattaaattttctcaccaacagtttctgatactggtgttgggagcaaaccggaggattaccaatatctgaaataccgaaacgaccctactctggctaatcaatggggtaagcaattggcaattacatgcttgttatattttgactctattttcccaagttatatttctcagagtcataccggatgcgcacatagctttggtttaaggttcagtagacacagagctctcatctaaacatatctgtgtgtgtacatatgaaggaaacaagacctcacactaaaaaaaatttgatcaacattttaagatatattttttcacctcattgatatgtgaagaattgcaacttatagtaattttcgtattgttttgggatatttaaattttaattctaaaatattgatttaatctaatccaatatagcttcgaagattagtcaaattgactatcaaaaagtgaaaagtgacatatattttgggacaagaggagtaatgatctattctcgtgtttaggcacaacgccgagacaattgtgcatgtggttcctagatggtgcattcccataatccatgaccagaatttattctgaccaactaaaattctgattaaattactagaaaacgtcaccgtctactccatcccttggagtgaagcataatttgatgcacaacttgagatacttggaagttggaacattgttctttagatttgagctaacagattagggagctgaaaaagaggagtatattgtgaggtgagatgaaagagaaagaaatatggtgattctaggggaaaagtaacagaatattcatcaagtgtacaggttgcataaatgcctttgttttactcccatggctgccgtacaagaaaaaatagaaaacaacataaagagaggaaaagtaagtaactaacataagaattcaatttttaattatctcacggcatttcacaggtattgcaactcaaaattatgtgtctcggcctttaatgtcgtcctgcttggaagatacaattgaaaagtcttccataactttttttctaccacctgtgagtgtgctgatgatatagtataattacattgcagatgggatgatttctcttgcaactacaagtaagtcttacccttcttggtgaataattcttttgcctagtcagatttattgttaggataaaaattgagaaattttgaaaatagtaatatttttgtgatgtatgattgaagttgtatcaataaagtactgtaactacttcaactttagaggatgaacttcttgcttgccttctgctcctctgaactttgctactttagttttctaaaactcttgtgagctgagatgtgtttgttttttccattagtctatgctttggtggcagtttatgcatgacataatctgcacgtgttactttagctagtcctgttctttcctttgtcctttgagggatttgataatgatcttaagattagaggcagctttctaaagctggagatacttagaggttaaactaactccacaacattttggttttgctattcgaacagtctcagaaccttgaaacgcttaaatcgaaaagaggcattaccaataaagcaactctacattttcttatggtaaattacaataacaactacatacccagtgtaatctcatatgtggagtctagggagggtagagtgtaatcccacaagtaaggtttggggagtatagagtgtacacggatcttactcctacctcggggaggtagagaggctgtttcttagagaccctcggatcaaatacaacaaatcaaactaattatgtaaaaggcagtggagaaaacaggtcaattaataagagaagtagtacatactgtccaaagaaagaacagttccaataacgaaataatgcggtaactgaaatacaaaaaaaatatatgatagcaactatcaaaagcaagaacaaaaacatgtataagactactactacgacatacatggtgcttccagactcccgccaagcctaatcccgctgaaaagtgagacaaaactcaactacctactaaccttctaccctaatccacgatctccatatcctcgtgtcatcgatgagctgaagttgcaccatgtcctgtctaatcacctctacccaatacttcttcggtctacctctacctttcgtcatacccactatatacaacctctcacacctccttattggggcatctgcacctctcctcttcaatgcccaaaccatctcaggcctcgcttccctcatcttgtccaccacggaggccactcccactctgtcccggataacttcatttataatcttatctctcctagaatgcctacacatccatctcaacatcctcatttttgtaacttgtatcttgtgaacatggtaaattgggatcaactgtttactcaaaacgtctcatcgctaactcttctctgaatcctggctaatcattccttgaatgatacagttccttaaccattaaattttaatgacagaatacatgttcatctgtagcatctttagaaaggttgtccccactaaaaagcagaattgatgcagtttgacagttaatcgaactttatgctgttatccaacttaacaaattccaatcaagctcacacaacttgtcttttagcttagggtgatcattatctactagtaataaattgctttggaagaatggtttctggatataattatctttcataatgacaggtttatagaagttttacatatataacatatttcttacctttgacaattacataacgttggaagtactcctatatctcataggattgagaacatttggtagtttaaactgagggatgaaagttgcaggcatatctgatagcgagatatacaatttaaacgtaaatctgaaagattctaattctgctgggagattgacaaagctaccctcaactgcaaagaatggtgccaaattcaggtatgccattttcaggggctccatccatgtgatgctacacttaaattagttttctcttgaccatacccatctagtcttttccctcctttctatgcttctgtctttccacacatggctaattagctataccttgcagtgggactgaagtatcaatatcaatatccaagacccttgatgacttattggcagagattacttgctttcttcaaaaggttcatttttcatgtctatcagctgattctagctatgatttcctaaattatatgaaaaattctctaactacagtttttcattgctgtttacgcagatgatccttctgaagattccggttagttcattacttttcttgaaatgctttatatttaaatcaaatgcaactatcttctctatagacccctcttataaatgatagctactaactgttcagacagctcaaggcgttcagtgtggacctactaaatgcaagtgtatatattttggatgagttcaccatgtcaaaaatatttcggttgttatcagattcacattaagattcgaaagttttaagcttctatatgtcattaacctacttctttggccttattatatttaaaaagttgtctttttccatatcctgttttctagtaaatagctaggagcctaggaccactacctctctgtggctgatagtttgtttctcttcttacagaaagttgtaatggaactcttagtatgtggtgatgatcctttaagttcacagattgaaagtcgtattctggcaattgagggcagctctgcatattctcctgttgaaagcatagaatgcttgaaagtgggactcaaggattatattcgtaagcaccaaacttgcttctcaattgggtgagtactagaaaggtgctaggtttttggttaatgaatgatggatgcattccatcctctagtttttgttgaagggtggataatgtgttaataggtcttacttacacatgttgaaatcataattcttaggtgctaacataaaaagataacaaagagtactgagcaatgctatttcttgtttcttcattgtacactttgacatagtttccctgaactttgtcatttccttgttttacatggactatttcatctactaactttaagttagcctttcattctgcaattttcccattaaaaagtgtaacatttgcagttcttcgctctttcttgtgtggttttgtctgtatgtctgaccgtacattaaggtacttcagtgtgatgtaaagtagtgcattattgttctgaaatatacaatttgtagattttaccttcttaaaatactggtgacaaatagttagattgagtgaagatgggaaaaagaagcttgggatgcactggaccaggtgagagaaaatcaggatcaaacatgaaagggaatgctagaactcccaccatagaagcagactgaaggaggagcagaggcaagacaattgatcacatgtagcatgcaggaagtagtacttaagtttcttaaaatctggttgacagctcaattgactccttctctgttttgatgtaggaggatttaagtttgctaacgtaatttagttaagatctatttgtggtgctaaactagaaattacaacggctcatatggtatatgtaaaattgcaacatctcatataggatctttggtgatgtaactgttgtgcagaatcaaaaacaaaacaaaaaaatcaatgtgcagtgcattgaaacaagcttgtacataaagttgtagtttcttatttcagggaaaacctgaaggttggaactggggttgctaactcttcaggtagttctcagggaaatagccaggtggtggaagctgttgtgattatcaatgagatgtcagaactagtcccttcttccagcatcagggaacaagacatgaaaacagaggtttgctttggattattaattgaagaaaactcttaaaagcgtaaaaaaagtttgcattccaatatgtgctttattaattatgttgtgaccaaatgttagataattgctcactgtatagatgccatgttgcataatctttcccaccatctattaacttgtgttttgagttcatttgttgtcctagaatgcgtggattgtgaaaactaatgataatatcacagatatgcattatttatgtctttgggatttcaactttcaggggtcttttatcacactatgaatctcttgttttcatataagcatggagcacaaggtgaagaacctcgtgcactttatggtgtgtggaggctaagatttatgcaacttcccttacatcatggtgtagatatatatgcaagtaataactgaaaaatatttttgaacttttgagggccagcaagtggacctctttctttatggccatcttgatgacattggattggataggttacattacacatacaacaactgtctcaatcccaagcaagttggggttggcaatataatcctcactgaccatgtggctccatttatgttcataaatagattacatatcaggaaacaaaattctatgtggaaagtgtgattttcatattgtaaaataacctattttctaaaatctagagtatccccagtgtacaccaaacaggatacattaattatccgatcttatctactgtggacaaatatggtctctggtattgagtctaattaaatattgcttattaaacttcgaggatatcaaaagcttttgcttagtgaactatacaagttatcggttggctgtcccagccatttctagtccttacagttgtttccaaaagtatacgaaggagggggacttaatatctaacctccaaagtaaatgaaacacaagtgaggacacaaaggaaggttttggggaaatcccacttatcagctaagctcacaaaaaaggtgcgatgaacatatgaggattccaatatgaatcctcacttactcactaaacatggccaattcctttcttctgtgtcttgattctaaagttagcaaagccagctttatccatgatataaactcctctcactgcttgagggagctcattagcagatatagaaattctgtaagattgtttgatagctccaaacttagctagcccatcttccatagcattgagttccccttccgttcatgcttgtcaaatattctggatatcaagtcagtcagctttgatggttcactgatgccattgatcatatccactactattttagagtccatttttctgtagcacattagtaattccattatctggaaacccctgcaagccagtgctagctgcaatagccttggcaacattactagaacttaaaggaagaagctctgagaaggccatgacaatttttccctgatgaccttttagaaccccctcttctccagctagtttcccttctaacattgaactgccatcagtgttgagtttgacataattttgagtaggcttgttccagtttttttttttcaatcaaagggttacttatattataatattaaagattgacagtagtaacaggttcttcgcccgttgccaaggacggatcgttgttaatagtttgggtcacatcccgaccctgaataatacaaattgagggcttgttccagttgacagtaatacaagtgagctttggcttaagttatccactaatcacaaacctccctcctgttggagtttaagttaatcaacccaagatctttttttttttttgagaaaggtaacttaacccaagatctttgaaatagcaatgttcagattaacaaaatatttaagcaattttttaaaaattaagttccatgtatctgttgatgaggttctgttgaagttttttaaaatcatctctaagcattacttgctcgtcttctttcagttaagccagtatctcgcacgcctttcagtgttgtagtttgtttgtgtttctttaatttgtattaatgatcttctatgcctgatttcagatcttatatttcaaagactttgtaccttgttctattgctcagtcatccctcgatgcattgacaagcatcaactggaaaagctatgggttggctctgcagagtgttgcagatcatgatgatagtgtaatgctggaatgggagaacctgccaccagatttccaaatttatattgccatccattgttaccatagacaatatccatcataatataatacatatccatgagaattgacatggtcatacactcttagcattaacttcaaacaatgagaattgtcttttgcttaacttgttgacaaggtgaaacagtgggttgcagaaaacagttttcctgatcgaaatctagctagaaaagctatcaagtgtgctttggatgacttgaaagaaaataatcaaggggttctcctaagtacacgtgcacttaaggtaattttctcactcttctctgcattctttctggtcattggattttctagttcctggtattggcttggtatgtacaaaatacctcccattgtttgatctattctgcattcttatacgtccatacccaaacatgaagcagaaaaagtagtttgttttttcttcttttgatacggatttttaaagagtggttgctaagcagacagtattcagtaattccagctggttaggtagttcacatacagaaactaggcatgatgtggacttaacattctttaaacaccatctgaagttctatatgactagtgctgattgaatctgaacaagggataacaattattcaaacataaattagagcagtgattggcaagaaatcttttctcattgcctcattggggatgaaagcttcctagaaaaatttctcctttttactgggagtggcttttaaagcatcatctatttagcactgctgttccagcttgtcagatatagcatttttattagctggaagtgcatatgctttcatatgtttctgcagagtccttttaaattcagtacccatatccatggtcaggagcgtacatagtatgacagtagctaatgtatctgcaacctctatcccagacattatctatatatttgattagtttgtatctctatgtgtgtatctacaacttagctataggtgcaataggattccacatgaaccaatttaaaatctcgatacaccttctagctgattatgatcttctttgagcttgaaatagccaaaatttcagttttccttcgcatacatagctaaagttctaaaacaatttctccctcagacatgtgattatgcacctgaccttgcaaaaacgcttgctcgcctgatcttatcctccaatgacttgaacttccaagaagaatgttgttctcttctcggggtacagtctcaagagggtaacacggataatgttggaaattgcatcagggagaagataatttcagtcatcagattaaatgatcgtaactcctataagcataaagaagccccaaccttcctatttgaagatgattgtttccagaaagaggatttcatggacgaggaatatcaagaaggtgaagaagcttacaactctttggatctgtagaaggttaggagcattattagatgtccaattattaatttcttctcttattatgtttatagtttacctcacaatcaaactattctagttacttctgcttggctttattattgctatggaaaagggtaaatggatttatcattctgggggcaaacaatatgtatggacttcatggtccaaagtagataaactgatactcaaccatttctacaacgttgtggtgaaaaagagaatatatatatatatatatatacttcaaaatttcattttctcagttttttccatgttactgaaatatctaaggattcatttggtcatagattttggaagtatcttgtagaattattatcttttgtcaaatatcagttcaacatagaaaatcatctagtttttgggagattagttttcaaatctcaaaagttacttcaaacttgttttttccctaaaatcttacattatatgaaagtgccccattgattacttcagatttattttgctagatttgtataattttttctttagaattattgtttgtaataataataactaaggtcattaataaatattctgtataatttggaattaatatgtttgtttgaagagaaagaatccttttcatttctgtctttcgactaatatctcattactaactcagccttgctgctttgaaaattttcacgtataatattagcctagataaattcgtttccttgaagtacttgagatataggtaagtttatttattacttcttccgttcatggttacttattcattttggtgcatgttctttaagatataattattaatgtgagtattttatcacaatactcgtataacttggtgtatagtctttggtcttcagaaataatttgaaaacaaataattaatattacatattcttgaaatactggacaaagaaaaatgaatggagaaattatttccttgcttagcccatgggccggcccaacccaacttgttattgggctagggttgggatgaaaa

SEQ ID NO: 41 - DNA, 1735 bp, Solanum tuberosum
  source 1..1735: mol_type = other DNA
cggcaatataaacacacccgaagcgaggcgcccaaagttccagatgattgcaattggcgggtatacagtgcttcttcctctgcatactgcaacttcaatggaaatcgaaatctcctctgtgaaaatgctctataaacatctcattttctgcgccgttcaacgatgccgcatgtccgatgatctttgcagattatccgtgaaattgacctcgttttctcgatttgcactcccgctcgttggaatatcagtttctgatactggtgttgggagcaaaccggaggattaccaatatctgaaataccgaaacgaccctactctggctaatcaatgggatgggatgatttctcttgcaactacaagcatatctgatagcgagatatacaatttaaacgtaaatctgaaagattctaattctgctgggagattgacaaagctaccctcaactgcaaagaatggtgccaaattcagtgggactgaagtatcaatatcaatatccaagacccttgatgacttattggcagagattacttgctttcttcaaaagatgatccttctgaagattccgaaagttgtaatggaactcttagtatgtggtgatgatcctttaagttcacagattgaaagtcgtattctggcaattgagggcagctctgcatattctcctgttgaaagcatagaatgcttgaaagtgggactcaaggattatattcgtaagcaccaaacttgcttctcaattggggaaaacctgaaggttggaactggggttgctaactcttcaggtagttctcagggaaatagccaggtggtggaagctgttgtgattatcaatgagatgtcagaactagtcccttcttccagcatcagggaacaagacatgaaaacagagatcttatatttcaaagactttgtaccttgttctattgctcagtcatccctcgatgcattgacaagcatcaactggaaaagctatgggttggctctgcagagtgttgcagatcatgatgatagtgtaatgctggaatgggagaacctgccaccagatttccaaatttatattgccatccattgttaccatagacaggtgaaacagtgggttgcagaaaacagttttcctgatcgaaatctagctagaaaagctatcaagtgtgctttggatgacttgaaagaaaataatcaaggggttctcctaagtacacgtgcacttaagacatgtgattatgcacctgaccttgcaaaaacgcttgctcgcctgatcttatcctccaatgacttgaacttccaagaagaatgttgttctcttctcggggtacagtctcaagagggtaacacggataatgttggaaattgcatcagggagaagataatttcagtcatcagattaaatgatcgtaactcctataagcataaagaagccccaaccttcctatttgaagatgattgtttccagaaagaggatttcatggacgaggaatatcaagaaggtgaagaagcttacaactctttggatctgtagaaggttaggagcattattagatgtccaattattaatttcttctcttattatgtttatagtttacctcacaatcaaactattctagttacttctgcttggctttattattgctatggaaaagggtaaatggatttatcattctgggggcaaacaatatgtatggacttcatggtccaaagtagataaactgatactcaaccatttctacaacgttgtggtgaa

SEQ ID NO: 42 - protein, 489 aa, Solanum tuberosum
MIAIGGYTVLLPLHTATSMEIEISSVKMLYKHLIFCAVQRCRMSDDLCRLSVKLTSFSRFALPLVGISVSDTGVGSKPEDYQYLKYRNDPTLANQWDGMISLATTSISDSEIYNLNVNLKDSNSAGRLTKLPSTAKNGAKFSGTEVSISISKTLDDLLAEITCFLQKMILLKIPKVVMELLVCGDDPLSSQIESRILAIEGSSAYSPVESIECLKVGLKDYIRKHQTCFSIGENLKVGTGVANSSGSSQGNSQVVEAVVIINEMSELVPSSSIREQDMKTEILYFKDFVPCSIAQSSLDALTSINWKSYGLALQSVADHDDSVMLEWENLPPDFQIYIAIHCYHRQVKQWVAENSFPDRNLARKAIKCALDDLKENNQGVLLSTRALKTCDYAPDLAKTLARLILSSNDLNFQEECCSLLGVQSQEGNTDNVGNCIREKIISVIRLNDRNSYKHKEAPTFLFEDDCFQKEDFMDEEYQEGEEAYNSLDL

SEQ ID NO: 43 - DNA, 8361 bp, Solanum tuberosum
  source 1..8361: mol_type = genomic DNA
tttgtccaaagtggaaatagaataagtataaagcattaaagtcttttaaaattttaaattgttaattcttattgtatgatttgtaatacttttacgccattttcaaataatagaggtcatttcttctttctcaatttatgtagtactaaaattgttttgagattcaatcaattttttttgtctttgaaatatttctagctgttaattactgtaatttatagtattttctaagaaattttcaaataatatatattattttatttgtcccaatttatgtgtcaccggtaaaatttgaagagtcaatcagatcttttatatatttttatatcttttaaatagttaattaattaattatcgtgattcataatattttatacaattatttagtatagtaaaataaatttaaaagaaacaaacaaaacgattcatcataggaaattaccaaagcatccttcaatacatcaataatgggttcgacttttgtttttaagaaattgcacattcgaaggatatttttgtccaaagtgaaaatattgtgtaaaaaatgtgtatttattgtgattttgaatgttttgtggggtaataggacgcacgcaaagttaaagtgtctttttgaaaatctgggacaacttcaagtatcacttaatgttttttctcaaaatctaatttactttcgtaaactatgtgtcaaatcaaaatcagattaacaaattcaaaaggaatgagtaataaatagctcatacaatgacatatttattatttaactaaataataaatatgtaactaaaaatcttgttagcttttgattgaaagctaacaagatagttacaatgatagttgcattgtgacttattatatatagaatatatatttcgaatttgaaagcgaaaaggcgtcaaagattttgtttttctcccgccttgccattcatcccacaccttctccatcgcactcgccagtctcttcactcacgcacacagtagtactacagcaacaaaatatgtatttcgccacctctcatctcccccacttaccaccgtcgccaccgccggaaccaccgttaacatgcgcccaaggccatagctcgactttgattatcccaaccgatgaaggcggatcaatttgtctgctctgcttgtccaatctcatttccaatccgagatcaccgacagttcacgtttcctatgctctctcccagttatctatcgcgctttttcaaccgagttttcgccaaaccttcttcacattccactctcatttcctaatctcgcctattgtcggtgttctatcttccttcgatgatgagcccatagccaagcaaactatggatttgattatgcagttgtgtgaagctccggactgcgatgtgcatgcagagtttgtggctcggctcgcagatcgtctttccagtggatctttagcttggagtcagagacagctccacacggtaacctttccctctgtcctaatttttaaatttccgatttatggaagtgtaatttagaatggagctgcagaaaggtatagctacatagatatagccatacatgatacaacatatactcctacatagaagtgtgtcattctaaaatggactaataaggaaataaaactggaactgagtaagtatctggttttcctaatttcctcagtgtccttcagcacagtgcaactttgtgtggtggcagacagccgactgtgatcagtaaagctttcggtactgaaaatgattttgaagatcctattaagatttataataagaacaggttttggcagtatagctttattgctcactcttcaatgcctaaaatcaaatatttcttttatagtagctttccacagttatttggcaactgctttcaatttcagtgagtcaatgacactgactaacagcttaagtttaagcacagccactgttgcagatttgattggaaaaccacagtcagaatgattcctgagaaaatattagttttagccagagcagtgagtagaaagctaaaaccagcttaggtagttatttcacgtttcaatgccagtgttcaagtccattaaaagacttgtgtaggaaaacacttgtaagatgttacaaaataagcaaataaaagatgggaggaactgtaaatgattttgaatttgtgaaattttttgagttgcattaaaatgacaccaattatatgtttcctcatgatgattcacaacctttttagagtagcttcacattctattcggttcctgtctgctgctgacctctatgagcaaattgctcactttagagatggtacactttgtatgtaattgattttctcattgagaagctagaatgaacaagaaagaggaagaagttacacttagcgtttctgtcttggtattattgacctgatatctgtcaaatacacattggattttaatgagataactcagccttcaatttgcacagagaatttgtagtttctatatttatttctgtatttgcagtgacatatgttttcctctaatacatgtaatctgatccttttttaaaaaaaaagcttcactgcttaggtcttctcttggattaccaaaaaaaccattcctattgtctcgaagaaacggatgccctcattttcaatctcgtcagcggccttcaattgtccaggtgactcttgaaactgagacagtggctatctcatttttccttaaacaaagccctgaaggtcaattccttcttaagtacagtgaagatattcaaggggaaatcctgtttgttctatacaaattattcctactcaatgtgtctcaagacggtgaagattctcccagtttatttggtcatttctcgaagctcctatacttagcactggcagttctcatgaaagctcaaagtgatgatgttcgcttaaactgtataggtaagcttctttaacattacccgtttatgcttcttgagcttttgcatctctgaatttggttttccagtgaatatcttgacagttaaccattttgttcttggattattgcaaaataagaggagtatatggtgaatagctgactaatttataatatatctgacaagtataccagggaaatatggttgctaaaaagcgagaatgcattataggaatagccatatctctccttgagaaatcatttgaatctagagattttgtggctcttgagccttatgttgtggtaaacaggctccataaatctgttcacaccttggatatactctgactgataaaaagttttgcgtgtatatttgctgctgacttgactagcgaagttctatgcactcctcaccagagctctgataatctctctcttctggcttcaaccctctcttctcccctcccttccgccaccattcccataaggaaaaggagaaagggaaaaaagaaacacaacagaataagcagctgctgatgttagagtttctgcaagataatatcatctctcacatttgtcaaatcagtgatactctttgtttatgcagcattcttaacagtattaatgcaaagaggattctttcaaactacttctataattgacacaaggagcaggagttcttatgatgttgaccacttgatggaaacaaatgagcagatatcagatgggcctctagctatcttgtttgcagaggcagtcaaaggccccctgctttcttctgataatcaagttcaaatagcagcgctagatttactttacctttatctgtcggggaaagatgtcttagaaaatgaaatccaagtatttgttgaagagaacattgcagactatgcgtttgaagtgctgagattgtcaggtaagaatatcagctatacacagtgcctgagcagttagatttatacatattagtttcgtttgaagaaatgaaagatgaaagagggcatttcagtcgcactctattttatttgttttttcgtttacaattaaactgtcttgaaatcgaccaattctctggcgattacagtgttatcctacaataaacaaattaccatggcttcaatgtttgttgtccatatggttcgacaagatctaagttctctcacgacaatgagctagagaacattctaattatattaggtcagattatgcaattaatcttgtctgtaatgactaatgaagtaactcattaatttgcaggatgcaaagatccaacaattaaatcttgtattcagcttcttgatattttagcaactgctgagcaagcatttagacagagacttgcaattgggttcatggccctgattccagttctgcatcatgttgctgaaattcctttccaccctgtacagactgagacactcaggcttatttggaactctgttgagaactgcccaggggtggtatccaagtctcaggtagaagaaataagcctttcattgacaggaatgctcaagaaaaatcttgacggagaaataggcatgcttccagagacattagctctggtctgttcaatatttgttgcacttatgaaatgttcatctacctgtgggatttcaagtttcttactatcaattcaggatgcatcaagaaattgcatcttaacttgtttaattaattatggcaaatacccgggtcaacttttgaactctctttacctactgaaagaggcatattcatatagtgttgggatgaattcctcaagctcaaccaacacagaacttagaagaagcattctagatgtatgcaaaacacatatattaccgtggtttatgaaatcccttcatgagatggaagatgaggatattccagctgcaatacttgaaaatttctattccatattgctacaagattcagaaactgaaaccaaaatatttgcaaatgttctgctcacatcttcctggttcagttttgcatatggatgtttaggctttttcccttctgaaaagatgaaaaggaaggtttatcttatctttagtgtgatgacagatatcattcttggggttgattctgcgcgatgcattagcgatgctgctccgcatcttccatctgatcctatagatttgcttttccttctgggccataaaagctcccaaaatgttgaattgtcttctcgccaactggcagttctgctgttactgtacatcagctcactgtatgacgatcggtaaatagtttctggaatcttaatcttactctttctgcattttccctgcttatgttatcagtcctcagttgatcatctcatcccttttccagaattgcagatgataagcttgtgttagcttcattggagcaatatattctacttaacagcagcaaaaacatgcacggagcttctgttttgggaatatttataaatctttatgcactatacagaggtttagccaaggtgagctaccaaatcccctacagcccagaggctgaaaggattgtgttccacctacttgcggaaaagggctgggatttgctatctacaagaatccacgtaacatctttgaaatggttgttccaacaagagaaaatctgcaacgtgttgtctgcccagattttgaaattttgcagatgcaattgctccaacgtaaaccagataaatatccatggtgaagccaatcagaagatagatgtgtatgttatgacagaacttgtagctttgggggataactttttaggtatggtcatggtgtttctattgggagaggctggagaacaatattccgagtatgacattgtttcagtggtgaataccataaaacatataatagaaatctcaccaagtgcttcagatcaattttgcatgcacgggatagctgctgcaattaagaacctttactataagtttggtcattcttcatccccagatactttcatgtccatctccaaactagtatcctgcattcttcaagcagtacactctgaatccctctccgatgatgaaccctgggttgcaattgtagtgaaagtatagtactcactcttctaaatgctgtttgcttccagttcctctgtagtaattagacttttccttaattgcagattatcgactacctgatcccctcagtagctgcagatggatggacaccaggaactcttatatcaattggcattctttctatggttttgcatcactcagtaaatcaagtgatggttgaagcttcgaaaaccataatccttagtactcatttgctatcattggttaataccactatcaccaatgcctgttccaagggaccttcactaattgaacaagacgaaggaacaagatctgtagaagctcttgtttttgtgctttcactgcttttcttctctttgagaaggtatcagttcctttaacataggttctatgctttcttttattttgtttttaattttgaatctaatagcttattttgctagtgtgcatgccattttaccggggattgtggactgtcaatatctgctggatcctaccaacataccacaaccttggccttatattagtatacagtgccacgatttgtgcaagttattgcattttggatctattcctattaagttacttagctcgcaataccttctggagttattcagcggaatagaagatgagagaagtagaaaatcagacacattagaattcagaactaattatttgttgtctataatggctgttttagaaggccaaatattctcaagtgacatgtctgtagcaatgaactgttccctctgtttgtctatgctcattgggtggcaagatgtggaaacagaagtatcagctatacaaaggaacaactggtgtcggtttatagtagaagaattagtgatgtccttggcagctccatctttggcttcaaaatctttcatgatccatcacaagcctgcaattcatattgcagttgaactgctgagaagaaagaaagttcctcaatggatgacttcaatcttcaatgaatcttgcatatttgccattattagaaacattacaaattctaatttgagcgctgagttggtgttcctcttaaggaagttgcttaattatggttttctgaatgatgaacaaattgctgctctaaatcaagtattccaggtaatagatacttaatcttcaaaagttcatgggttcctatagtgatctggcctcatgaagcttgcttttttgaaaaagaacaaaaaaaagagaacactgccaaaatgaaaaaatggaattccattattattatgtttgcctgcaggaatgcagaaaatgtatctacacagacaaacttcaacgtactggggaagaggagaagacatggaacgtagcagctgcttcagattatgtaggtaaagtttgtcagtttctcattagcctcataacgactcagccatctagtgttatggagtcttcaagatttcaaagtgggaaaagggaattgttggaagaaatagacttattttcaaaatgtttaatgagggaagattgagcttgcaccattaaagttaggtttggcagagtatcatatatagacgttctttaccaaaaacaattcagatattttcctgttttgtcactcaagggcagtggcatctgctagtatcttcagtatcattggccacatacaaagcactgccttgagtaattctactttctgtgcatcaccaagttctacatattttctttactcttttgttttgttattccaaaagaaggacaaagaaagtgggaaaaaaagctaacagttgacctccccaaattgaatggtagaagaggccctttcttccgtgagaaacatttgggctgggctgggcaggcccatcgttgtggcaaaacctgaactgtgtcaactataagcctaagatcctaggggctaggccctagcattaagcaaacaaaataagtccttgataaatgttgttggttttctggtagtgtacataggaatagttaaataattgatgggaccatattacttctagtttctcccacagacgtaatagttcctctcatctcagcatgaaaaagatagcccaccatccaataatttaatacaccttttactatatatacttgttatcctaatttgtacatatactaaggctagagagaatgatcaaagagatgggatggaggacccccactcactcgacctcaaacttggggacccttccagtacttcttatataacgaatttatcagagtttctctaagatagggataaatgcaatttttcagccatagaagtggatggacattgtcttctacttagaattattcgttctatacaaatgaacaattatgagtacaattgacaatctacattcataaaacaaaaaagcacataacatatgaagtttcgtccttcataaatcatgcatgagatgagaaacatgataaaaaaggcagtggatttgcaagagggatgtggtccctgtgaggagggagattaaatcatgaaaagcaacacccacgtccctgtgtctcct

SEQ ID NO: 44 - DNA, 4353 bp, Solanum tuberosum
  source 1..4353: mol_type = other DNA
ctcccgccttgccattcatcccacaccttctccatcgcactcgccagtctcttcactcacgcacacagtagtactacagcaacaaaatatgtatttcgccacctctcatctcccccacttaccaccgtcgccaccgccggaaccaccgttaacatgcgcccaaggccatagctcgactttgattatcccaaccgatgaaggcggatcaatttgtctgctctgcttgtccaatctcatttccaatccgagatcaccgacagttcacgtttcctatgctctctcccagttatctatcgcgctttttcaaccgagttttcgccaaaccttcttcacattccactctcatttcctaatctcgcctattgtcggtgttctatcttccttcgatgatgagcccatagccaagcaaactatggatttgattatgcagttgtgtgaagctccggactgcgatgtgcatgcagagtttgtggctcggctcgcagatcgtctttccagtggatctttagcttggagtcagagacagctccacacgcttcactgcttaggtcttctcttggattaccaaaaaaaccattcctattgtctcgaagaaacggatgccctcattttcaatctcgtcagcggccttcaattgtccagtgaagatattcaaggggaaatcctgtttgttctatacaaattattcctactcaatgtgtctcaagacggtgaagattctcccagtttatttggtcatttctcgaagctcctatacttagcactggcagttctcatgaaagctcaaagtgatgatgttcgcttaaactgtatagcattcttaacagtattaatgcaaagaggattctttcaaactacttctataattgacacaaggagcaggagttcttatgatgttgaccacttgatggaaacaaatgagcagatatcagatgggcctctagctatcttgtttgcagaggcagtcaaaggccccctgctttcttctgataatcaagttcaaatagcagcgctagatttactttacctttatctgtcggggaaagatgtcttagaaaatgaaatccaagtatttgttgaagagaacattgcagactatgcgtttgaagtgctgagattgtcaggatgcaaagatccaacaattaaatcttgtattcagcttcttgatattttagcaactgctgagcaagcatttagacagagacttgcaattgggttcatggccctgattccagttctgcatcatgttgctgaaattcctttccaccctgtacagactgagacactcaggcttatttggaactctgttgagaactgcccaggggtggtatccaagtctcaggtagaagaaataagcctttcattgacaggaatgctcaagaaaaatcttgacggagaaataggcatgcttccagagacattagctctggtctgttcaatatttgttgcacttatgaaatgttcatctacctgtgggatttcaagtttcttactatcaattcaggatgcatcaagaaattgcatcttaacttgtttaattaattatggcaaatacccgggtcaacttttgaactctctttacctactgaaagaggcatattcatatagtgttgggatgaattcctcaagctcaaccaacacagaacttagaagaagcattctagatgtatgcaaaacacatatattaccgtggtttatgaaatcccttcatgagatggaagatgaggatattccagctgcaatacttgaaaatttctattccatattgctacaagattcagaaactgaaaccaaaatatttgcaaatgttctgctcacatcttcctggttcagttttgcatatggatgtttaggctttttcccttctgaaaagatgaaaaggaaggtttatcttatctttagtgtgatgacagatatcattcttggggttgattctgcgcgatgcattagcgatgctgctccgcatcttccatctgatcctatagatttgcttttccttctgggccataaaagctcccaaaatgttgaattgtcttctcgccaactggcagttctgctgttactgtacatcagctcactgtatgacgatcgaattgcagatgataagcttgtgttagcttcattggagcaatatattctacttaacagcagcaaaaacatgcacggagcttctgttttgggaatatttataaatctttatgcactatacagaggtttagccaaggtgagctaccaaatcccctacagcccagaggctgaaaggattgtgttccacctacttgcggaaaagggctgggatttgctatctacaagaatccacgtaacatctttgaaatggttgttccaacaagagaaaatctgcaacgtgttgtctgcccagattttgaaattttgcagatgcaattgctccaacgtaaaccagataaatatccatggtgaagccaatcagaagatagatgtgtatgttatgacagaacttgtagctttgggggataactttttaggtatggtcatggtgtttctattgggagaggctggagaacaatattccgagtatgacattgtttcagtggtgaataccataaaacatataatagaaatctcaccaagtgcttcagatcaattttgcatgcacgggatagctgctgcaattaagaacctttactataagtttggtcattcttcatccccagatactttcatgtccatctccaaactagtatcctgcattcttcaagcagtacactctgaatccctctccgatgatgaaccctgggttgcaattgtagtgaaaattatcgactacctgatcccctcagtagctgcagatggatggacaccaggaactcttatatcaattggcattctttctatggttttgcatcactcagtaaatcaagtgatggttgaagcttcgaaaaccataatccttagtactcatttgctatcattggttaataccactatcaccaatgcctgttccaagggaccttcactaattgaacaagacgaaggaacaagatctgtagaagctcttgtttttgtgctttcactgcttttcttctctttgagaagtgtgcatgccattttaccggggattgtggactgtcaatatctgctggatcctaccaacataccacaaccttggccttatattagtatacagtgccacgatttgtgcaagttattgcattttggatctattcctattaagttacttagctcgcaataccttctggagttattcagcggaatagaagatgagagaagtagaaaatcagacacattagaattcagaactaattatttgttgtctataatggctgttttagaaggccaaatattctcaagtgacatgtctgtagcaatgaactgttccctctgtttgtctatgctcattgggtggcaagatgtggaaacagaagtatcagctatacaaaggaacaactggtgtcggtttatagtagaagaattagtgatgtccttggcagctccatctttggcttcaaaatctttcatgatccatcacaagcctgcaattcatattgcagttgaactgctgagaagaaagaaagttcctcaatggatgacttcaatcttcaatgaatcttgcatatttgccattattagaaacattacaaattctaatttgagcgctgagttggtgttcctcttaaggaagttgcttaattatggttttctgaatgatgaacaaattgctgctctaaatcaagtattccaggaatgcagaaaatgtatctacacagacaaacttcaacgtactggggaagaggagaagacatggaacgtagcagctgcttcagattatgtaggtaaagtttgtcagtttctcattagcctcataacgactcagccatctagtgttatggagtcttcaagatttcaaagtgggaaaagggaattgttggaagaaatagacttattttcaaaatgtttaatgagggaagattgagcttgcaccattaaagttaggtttggcagagtatcatatatagacgttctttaccaaaaacaattcagatattttcctgttttgtcactcaagggcagtggcatctgctagtatcttcagtatcattggccacatacaaagcactgccttgagtaattctactttctgtgcatcaccaagttctacatattttctttactcttttgttttgttattccaaaagaaggacaaagaaagtgggaaaaaaagctaacagttgacctccccaaattgaatggtagaagaggccctttcttccgtgagaaacatttgggctgggctgggcaggcccatcgttgtggcaaaacctgaactgtgtcaactataagcctaagatccta

SEQ ID NO: 45 - protein, 1294 aa, Solanum tuberosum
MYFATSHLPHLPPSPPPEPPLTCAQGHSSTLIIPTDEGGSICLLCLSNLISNPRSPTVHVSYALSQLSIALFQPSFRQTFFTFHSHFLISPIVGVLSSFDDEPIAKQTMDLIMQLCEAPDCDVHAEFVARLADRLSSGSLAWSQRQLHTLHCLGLLLDYQKNHSYCLEETDALIFNLVSGLQLSSEDIQGEILFVLYKLFLLNVSQDGEDSPSLFGHFSKLLYLALAVLMKAQSDDVRLNCIAFLTVLMQRGFFQTTSIIDTRSRSSYDVDHLMETNEQISDGPLAILFAEAVKGPLLSSDNQVQIAALDLLYLYLSGKDVLENEIQVFVEENIADYAFEVLRLSGCKDPTIKSCIQLLDILATAEQAFRQRLAIGFMALIPVLHHVAEIPFHPVQTETLRLIWNSVENCPGVVSKSQVEEISLSLTGMLKKNLDGEIGMLPETLALVCSIFVALMKCSSTCGISSFLLSIQDASRNCILTCLINYGKYPGQLLNSLYLLKEAYSYSVGMNSSSSTNTELRRSILDVCKTHILPWFMKSLHEMEDEDIPAAILENFYSILLQDSETETKIFANVLLTSSWFSFAYGCLGFFPSEKMKRKVYLIFSVMTDIILGVDSARCISDAAPHLPSDPIDLLFLLGHKSSQNVELSSRQLAVLLLLYISSLYDDRIADDKLVLASLEQYILLNSSKNMHGASVLGIFINLYALYRGLAKVSYQIPYSPEAERIVFHLLAEKGWDLLSTRIHVTSLKWLFQQEKICNVLSAQILKFCRCNCSNVNQINIHGEANQKIDVYVMTELVALGDNFLGMVMVFLLGEAGEQYSEYDIVSVVNTIKHIIEISPSASDQFCMHGIAAAIKNLYYKFGHSSSPDTFMSISKLVSCILQAVHSESLSDDEPWVAIVVKIIDYLIPSVAADGWTPGTLISIGILSMVLHHSVNQVMVEASKTIILSTHLLSLVNTTITNACSKGPSLIEQDEGTRSVEALVFVLSLLFFSLRSVHAILPGIVDCQYLLDPTNIPQPWPYISIQCHDLCKLLHFGSIPIKLLSSQYLLELFSGIEDERSRKSDTLEFRTNYLLSIMAVLEGQIFSSDMSVAMNCSLCLSMLIGWQDVETEVSAIQRNNWCRFIVEELVMSLAAPSLASKSFMIHHKPAIHIAVELLRRKKVPQWMTSIFNESCIFAIIRNITNSNLSAELVFLLRKLLNYGFLNDEQIAALNQVFQECRKCIYTDKLQRTGEEEKTWNVAAASDYVGKVCQFLISLITTQPSSVMESSRFQSGKRELLEEIDLFSKCLMRED

SEQ ID NO: 46 - DNA, 7149 bp, Solanum tuberosum
  source 1..7149: mol_type = genomic DNA
aaaagggttcttgaagttctactcctagtggttgaattctccatcatatctttgcttccatcagtattctatacggtcgaaaacaacatctttatctcacaaatttaaggggtaaggtttgtgtacaccaccctcttcctaccttgtaggattttactgagaacaacatctcgatctcacaaatctaaggggtaaggtttgtgtacaccaccctcttcctaccttgtaggattttactgagtctttaggtgtgtaagctcacactcaaaattccttctgagctattacctgatttcccgctctatttgacatatcgtaagaaggggggttctacttaaaatgactctattccattgagatttataagaacaatcgagtgtccttgttgtgctcctttgatatgagtacaatttaatggagataaccaatattgttatgcagtatcattttctcttgtatgattgaccaacacctaatattaatataatattgtagttttcaactcgttcaactaaatacttgtattattttgtatgttaaaatttatgctagaattattttctcaaatagagccaccatatttaacgatcgaagtgcatattactcggattattgtaccaccattcaagttatatccgttatacttaaaatattataagtacactcatttcaaaacaattttagatatgtaagcacttacaattgcttcaattatttttacttgaactttagagaaatatgactagtttaactattttgtgcttgaattacgaccatatgtacctgaagtttagtcatttttaaactccgcatgtgtaaagttattctaaaattaatagacatttaaatttcgtttaaatatgacctacggaatatgggaaaactacataactaagcaaacatatttaataaaaatactttttagtccaaaatccaaaaaactcacgcgagtaacgttttataaacaagctaactcccgccatttaccactgtgagagaaatggagattttgagagagcaaccgaagagccactcagatgaatcgttcaaactcgcgatcgcaatggcactcgtccgatcaaagcttctccacaagcctccggcagcaacaccggctccgccttcttcctccaccgccgccgttcctcaacctgccgccgcagcttcttcttcctgcgcgcctctttctcattccgatgatgctgttaaatggaaacaaaaagttcgatcaatttcctttaattccttcgatttcctatttctattatcagttacttaactttcattttttaggcaaaagagcgtaaacgagaaattctcaggctcaaggaggatctcaaagtagccgaaggttagtattttaaattttcgttatagtttaagctagattgtttaagtttatttctatttaaatgtttatattgaaattttttgatgatcactgcaatttccttaggatctattattatgtgatggattcgattggaaaataacaatgtgtagttatgaccatctaggctttacatatctgattatcttgctatattttgacctcgaaattttgtgagtatgtatgtatggtaatcaaaattgaatgataagaagaataacctgaagattttttgttatgtgtttgattttgatttactattgtgttgtttgtataggtagattcacattgatcggctattttgttttgattatttgtacttttttttttcctggagtaagatggttcacagtgtgatatatttccaaaaagtgcatcatgcaagtgttatttctttgataagttgggattattgagtcctaagaaaattggagctggttctgaccaacggttcagtgatgtgttgcggagaagatttctcagacaaggtttgcattttaggaatgctgttgtacttattggtctaaagttgtcaattcagccttcatatacattagctgaattcatttacttgtatatttttccagtaaggattaaggagagaaagaggagaagaccagatgattccttacttcaccgcatttcaggtgaaagttcagttagagatctttttatggatataattttgtctttacttttgatggttaacttgcaaagtgatgatttttagaagttacactgagttgagatcttatcatacgtcagccatgctgtgataaatgtcatatcttacatgtgccataattttatctctggaaaactctaggtcatgtttggcaaaattttctaaacatgagttttcagctatagatgagaagtatgaatattgctttttcttatatggcagaacatgacaatgaaaataatgttgagcaactgagtgcttcagttgattttcttttggagctttgtgacactatttctcctcaaagtgtatgttgtttcaattagccccagctagtgatgctttgttttatgctatgaatatcgtttgtctcatctcacttggcttttgtaccaaatgtgttacagttggaggaaggtaattttaagaactggtgccaccaagccgtggactttattcttggtaatgatacaatattttcatttccttttgccttcacatgtacaattttttcatgagcaacatctggaaattttaaactttaattcctgatatgcttttctgtttgtaatacacccacgtttaataatttcacagatgtactgtttatattctaatttctagtgttgaggattgtgatagaagctgaaatcaaggggttaataagtgaatgtattatctgttctgaaacttaaatggaaaaaaactgtctagtgaagcttcatcctaagatttgagttttcaaggaaagattgctctttgagaaccatcttcatgatttgtgctgccattttaaatgaagctttctaatttttactcgaaaatgcaaaaggttcacgatttacccttctttgtcaacacctttttccaagtaccgaaccatttcactgcatagaatgcctaaatttctgagatttcagttgtaatattaagatagcaccagatgggttcattactgtctactcttctttctttagtgacttccaaattcagcagtatctgtattttactactttaaaggtacactggctacaatgtcaccaactgaaagaaacagagaacccgtggaaggcattatcaacagtttaatcatgcgtttattgagaagaatgtgcagtgctttgcatagagatggtaataatgtgatctttttattcatactaggtttttgaagactatcttcaccttagcagattgcggaagtatattttctcctaccttaataatggtagaatcagcatgttcaattaattataaagattttggtagatatgtcccagtatatgcatataaagaactaagaaatggtttcagcatgatactgataaaagttctttggtttgatacgtattaaatggaaacaaatcagttactcctattatataataatggatgtttgatttattatactctgatcgtcccatttatgcatcattgttaatttgacttacaaattctaaatagtagcaatataacagtaaagcagtggacaaatcattaaacaaatttgaattcttaaagtttattgaggttatataaaagataatattggtagagtattgtagaaagtttttcgacatatcaaaataaatatagtatcataaatttggacagagggaagcaatatttgtgatgaaactatctcatagtgtagaaagacaccttaaatttttttgcagaagaaacaaaaaaattggtgtttccacacgacatagatcatgtaaaatgcttctattcttttggatggatgctgaataatatttatgaataaattatttatatatgaaggaacaaactattgtgatgatgattctgaaagattcattgaatctaattcttattagtttaaaaatatggattatattgaatagttagaagcaaagaccagtgaaatcaaaagaggacagacccttgtgaccctgttatcgttggactgattattagtttagttggatcatgagtctgaatttcacagcgatttaaagtgatttttgctcttggaccgcagcattttcattattaaattcctcaatgtaacttacttatatttccttctatatggcttcttaactcttgattccataatgatatgattcagactctcatcactttgacgctgatgttcagttctatattcaacatttgatgcgtaaggtcggaaatgaggcttttgtcggccagcgtctaatatttgcagtttctcaaaggatttctgcaatggcagaaagtttgcttttcatggatccatttgatgatgcctttccaagtatgcataattctatgtacatgatgtaagtcccaccagcttgtataaagttgtctttaattatctggctttattgttcttttatgcttctgttttgtagttgtttctaactttcttatcacataatagagggctgcagaagggaaagagaagggagaagggggcagtgggagtcaaacccatacatattgtgggagatcccaactggtacctctaggctataagcctggcttcttgtttgttaaatgctgtcttccttcagtcattgaaatttgtttctatgctggtaataatgggatgtacaatctgacttctctataactatcctctataacgacatttcactataacaaccatttgttacgtgaaactaatctttcatgttatgttatattgtttattctctataacaatatttcactatagctgccaaaaaatgtcggaacaagtgtcctgttataaagaggctcgactgtccattatttttgtccttactcttgacgaaatttcttttcctttgtgtatgataacatattttcctttctggtcattgacatctttccatatactatttttttattttgtgtttcttgtttagaggtttgaaaacactgtaatttttatatcagaccgcttgtccctccagacttcccgatttgaaggtgtttttaatctgaggattggaatttgttccttgaaatttggagttcctatggggagtatgacatttacttcgagttggctgttccgttctttcttttgtcagttaagctaacataaagtttgaaatggttgtctgtatgtggtactgtcatcatttgcttctagtatcctctagtggagtgatcactactatatttttcgatcatcttcacaatctctttttttattttaaatggcggttttagtggtgtgctccccttttctttagtgtaaatagttattcattgcttgaaacgctgcaatgattaagtgatcagaagctgtgcctgcttcagacacaaaaagtaaattatgctgcctgaattgccagattacttagttaacttggggatgttcatgtacctcaaggtttatcaccggagttgtgtttaaacttcacatttggaaccatagcttaagcttgctagatttctgtctggaaggggctgtaggaataacgtggcatacagtttactgcctagtatttgctttttactgcatccacaatttacttcttttaatttcttcatttctttatgaatcttcttgaaactataacccataaaaaggagactaaaattgtctaatatacgttctcaattgcaggattcagcttattgaatttctggtttcagattatttgttaacctggtcaaaaggtggagatttcgacataagtgagcttcttctaatcacttggatacataacacatttgctctctctataacctatttcctctccttctatcgggtctgaggagttctgcctccgtctgagggaaattactgcatgtgatatatattcccacaaggataattagcaggctcccataaatgacctatctggtgaaggttatttttaatactgttaatgatggaaatggacctgacaatatccatacgtttgtatttactctgtagggctttttgaagaatgggttgtatcaattctcctcggaagaaaagcattggaacttctagaaaacaggaattctctttatgtcctgtacatagatcgtgtaatcggagttgtggccaagcaagtgggacagttgtcatttctgcaaaagctaagcccacagattcttgagaacttgtttagctaagcactgatctgcagcttttcccttgtgaactgtaagtaacttgctttcaacacaaatcttcttttcttgtgcatagaaaattcagctgtcatcgcaaatgctttgttacttaaaattcaagagttcttggttaattaattaattcccagagtatcaaagatcaaagttcttttaaagtgaaagatgctctttaaatatgaaaatatgaaacagcatgtaaatagtaaaatccacttattgaacaaaatctacatgacattagcacaccatcatgtgccgaaagttagaacaaaatcccacatctctttttgtggaaccagattcctggttgaaatatgttccaccaaattgtaggcttaagcaaatctttgacttccagtggcatcactatttttcatattccttgtcgtcgtagttgagatcttgcataaatgaggttgttggatggtttgacttctagctcttcgtagtttaatccaaacatgttcttttctcattttcttcacttttctttgtgatattgagggtggcgggaatctgaatctgataagtttacttataaacaaagaattcctattttagtactacctattgtctttcccaactttagagttgtccctgtccccaccttgttcatttttcaaactacattttgaagggtgattactcagcccttaaaactttcttctttttttgatggattactaataccaaaaagttcgttatatatttgaaagatgcaaaaaaggtgtattgtattggatacacttctgctttttgctagatatatagcgtccttctcgacttgcatttaaccaaacttgctcctagctactacattgtacatcatctctctatctaattcttgcatagtagacatgattcaagccaaaaccatactggttctctcattattagcaactcttttattgtcccaatactgcaaaacctctgcttctactgacattccaccatccactttcaagcctccaagccaaac

SEQ ID NO: 47 - DNA, 1269 bp, Solanum tuberosum
  source 1..1269: mol_type = other DNA
atggagattttgagagagcaaccgaagagccactcagatgaatcgttcaaactcgcgatcgcaatggcactcgtccgatcaaagcttctccacaagcctccggcagcaacaccggctccgccttcttcctccaccgccgccgttcctcaacctgccgccgcagcttcttcttcctgcgcgcctctttctcattccgatgatgctgttaaatggaaacaaaaagcaaaagagcgtaaacgagaaattctcaggctcaaggaggatctcaaagtagccgaagatggttcacagtgtgatatatttccaaaaagtgcatcatgcaagtgttatttctttgataagttgggattattgagtcctaagaaaattggagctggttctgaccaacggttcagtgatgtgttgcggagaagatttctcagacaagtaaggattaaggagagaaagaggagaagaccagatgattccttacttcaccgcatttcagaacatgacaatgaaaataatgttgagcaactgagtgcttcagttgattttcttttggagctttgtgacactatttctcctcaaagtttggaggaaggtaattttaagaactggtgccaccaagccgtggactttattcttggtacactggctacaatgtcaccaactgaaagaaacagagaacccgtggaaggcattatcaacagtttaatcatgcgtttattgagaagaatgtgcagtgctttgcatagagatgactctcatcactttgacgctgatgttcagttctatattcaacatttgatgcgtaaggtcggaaatgaggcttttgtcggccagcgtctaatatttgcagtttctcaaaggatttctgcaatggcagaaagtttgcttttcatggatccatttgatgatgcctttccaagtatgcataattctatgtacatgatagggctgcagaagggaaagagaagggagaagggggcagtgggagtcaaacccatacatattgtgggagatcccaactggattcagcttattgaatttctggtttcagattatttgttaacctggtcaaaaggtggagatttcgacataaggctttttgaagaatgggttgtatcaattctcctcggaagaaaagcattggaacttctagaaaacaggaattctctttatgtcctgtacatagatcgtgtaatcggagttgtggccaagcaagtgggacagttgtcatttctgcaaaagctaagcccacagattcttgagaacttgtttagctaa

SEQ ID NO: 48 - protein, 422 aa, Solanum tuberosum
MEILREQPKSHSDESFKLAIAMALVRSKLLHKPPAATPAPPSSSTAAVPQPAAAASSSCAPLSHSDDAVKWKQKAKERKREILRLKEDLKVAEDGSQCDIFPKSASCKCYFFDKLGLLSPKKIGAGSDQRFSDVLRRRFLRQVRIKERKRRRPDDSLLHRISEHDNENNVEQLSASVDFLLELCDTISPQSLEEGNFKNWCHQAVDFILGTLATMSPTERNREPVEGIINSLIMRLLRRMCSALHRDDSHHFDADVQFYIQHLMRKVGNEAFVGQRLIFAVSQRISAMAESLLFMDPFDDAFPSMHNSMYMIGLQKGKRREKGAVGVKPIHIVGDPNWIQLIEFLVSDYLLTWSKGGDFDIRLFEEWVVSILLGRKALELLENRNSLYVLYIDRVIGVVAKQVGQLSFLQKLSPQILENLFS

SEQ ID NO: 49 - DNA, 7076 bp, Solanum tuberosum
  source 1..7076: mol_type = genomic DNA
agatgtaatgccacacacaagataaaataatttcatataatatctcgaaataattattctttatcctgctaatcaaacaagtcatagtaccatttactgataatatggtcatggaatttgctcaaacatcacatcatttttatttaaaaggcaaagccgattaatcaccagacccattgacactgtatattaacccgtttgtctaaatttatgtgacatttttttttcttcgagaatcaaatagtttaaatttgatcgagaatttgcgcataaaatttcaattttaaaaaaaagtactataagtcacaataattgacaattcaaaatattttaaaagatatatgagaaatttaccatcaaagatagaattatttgaatctcaaaatttaaaaagtgtcatataaattgagacggagaaactagttagtttgtatatgatagtgtatatgttattttgagtttatctgttgttactccacatttgaaaccaatatagttctaagaataatctaaacatatcaggtaaagggactaaagcatagatttgaattaattgaagattaaatttattgattcatatattgcaaggatggaaatcaaaatttatcaataattagtaaccaaaaagtacgaatatcctattttaatttttaaatcgtctgaactaaatgggcctagtgtcagatgaaatgactgggccatagttattgggcccaaattaatcagtagaggtccataacagcccaaaagtcacatgataggccatatgtaccattttccccaaaagatttgaaatttccctgtatataaacccacactctcccgctgaataatcaacgcaaatcacacttccaagttccaactgttcgacggagcaaaatcacagagagaattcaaatgtatttacaaatttgattataccttcatctgttagggttctgtaattgttcaaattgaagttttaatttctcgaagatttcaatttttatagtatctgcaaatgaagttgaagatgaacaaagcatcggatcttagctctatctctgttcttcctcctcatgcaaggtaaaattctatctcagtttcacgatttcatctctttgcattgtatagcatgaaattgcgtagctctctgtgtttctgcgttttgttcgcatgcattctaatttgaatgttttgtgtgcgatacacatagcgagttggagtgagatagagagaattttactgtaaatttcagcttcttcgtgaaaatttaaggaggaactaagcgcgcatctctctgttttgccttttcttcgaatgtatattgaagatattttgatgttttgtgttctatacacacatatgcatttgtatacatgttacatgtatgtttatatggataagagggagaggtagacttttttctgtaatattgagctttatttttgtgtgatgatgatatgagaagaacgccaagtgcggagccgctctgtgttttcgcctacttctccgtgtttgtgcgatttttctcatacattatacaggtattttagatgtttttgtgtccgatatacacaaactgtatatatacatatatatatgtctatgaatgcatgaacagagatagtgagattttgaaataatattaatcctattttgatgatatgagaaggaggccaagtgtggtaccaagtgcagcagagtcttccgttttcgggaaaagccaaccatcacaggttcggtcacagcagcaatcgcaacaatccttctcacagggattttcatctcagcaagcaatctactctcagttatcacagagctctctggatgattttgtccctaatgagcaagtaattcctccatctcgctcctatctcttatttattcaaagagaagttgttgatgagatgtcattttggtatactatacaaaggaactgattcatttggtgtggaattgataatgatagacctctaaaaatcatttttgttagcaacttctgaagaatgctttagattgtctaaaatgtattttgatgcttagcaatacttgaatatgttatattgtagataattgttgcctaggttacttttgagtgtaattttgaattagtatgctttatgatgcttgaaatagatgaattaagcttctgacaatgatttactttgttaaatgttgtgtcaacacacaacactcactttatatgacgtatttgatttaagtgttatattagcgaggcttgaaaaaatattgaaatttaagtatatttgaatagctttgaaagttatgaaagttgcataaaagatgaatgatgccaatattttgcaaggtccttaaatggaaagagtgtcaaacaaattgggatggagggtgaagtagatattatttatcatctttactgtactggacagtgaatcataaattctgttgccgcatctggcagaatgtttcttattggtatatgacaaaacaggagattgtcacaatgcagtttgaagtggttgtcggcagttagcgtagatcttcttagtgttcatctacaattagttaactgatggactcttgacttttaaattgatcatatgccttcttgttttcaactctgccctgtgccagggcacatagttccatcaaacttcccactttatacattggaacttttcctcatcgcaaacaatatgctgttatgggaattttacatcttaaagcaaacaaatgttgtaactgttaataattttaatgcagagattgggttctcaagaaagagaaaattcagcaaaaaggatgagctgtttgcctcatatcaactacacacgagaagagactcaaatgcagttatcaaaaccttcgaccaattatttgcgcaaatggtcagttcctgaaagcaaatgtaagccataatccaccaccagaagctacatgctctcaacttctgtttaaaagttaggaaaatgtactccagttcagcgcttatttgcagctggaatcatcggactaaacatgtttatctaatttttctggacagaccagattgaagaacttgaacacaaaattggaatggtagagacttcattaagcaggcaaggaatgatcttagattctattcagagtgatattatgcaagttaaccggggaacaaaagagatattgatggagagtgagtattcactgcccttttaatttacgtgatgtggcaaataattaggaactccaaagagcccatatcattagtcgacgagtgtggagttttgtcttgagaagactgctggtccgattaaaacttttacttgcaaatattctggtgggtgtaaaaaaaatggcaacaaaatctaaacacatttgtttttcttctgaattttctttcagtggaaagcttacgaccgaagttagtttctcatgatgaactgttgcaattgatggtaactacagcttagcttctctgcctacatccaggaattaagtgcctgtttgttttatcacatttcctaatccatgtggcatacaatattagaacaaggagagggaagatctgaaagctagcctggaggggaccttcaaatccatgtttgaagagcttagggagaacaaatatcaagagaacatcagagatctcttatcactgcttagagctatgcccaacaaacttgagatgtgcattttgcaacttcaaactgatttgagcaagaccttggctaaagagattcaggcatgttgcatattgaaactgactttttaaattcatatttaggctaccctatgtggttggattaatgctgcttcatctatattcctattgcttgcagataatttccccccgcccagattgtcatggaaaaaaacatgaaaccgctccagtcgatccaccaaaagtacgttttcaagaacttttttctccaaattccatatgatttgtatgagtattgagtgtaatgaagaacgcaatcagaagtcttagtgcatttgaacatttgtaggtcatcaatgattgtagccttccccgtgaagtgaagtttctaaagaagtaagttctcaaacttccttctcatcgccatcactgcagccttagttttgaaaattttaagtagcaattagtgatcagtagctctccagtatgcaaagttcatagtcacttgatggatctcttattatttgcatcatttgtgtgcaatatgcataagcggtagtcatttcacaatgcctcttgagatgtgtgcattgacatttgagaacacttgcggctgggatacactctctgtcatcaggaactacttaggtgacaaatagatgtgaagattcacagcatagtgtcttttgatccatatcataaccagaaagtgagtatccccatttctcacattagctatgtgaaggaagaaagggaaaacaaaggaaagcactccccttattcctcgaaagctagccttcatgataaaccaaatgaaataagaaaaatttaagaaatttgctatagcttcaacagaaatcttgtagatacttgttaacagagttttgctgatatttctaacattgagcgacttaattcttcattgctgtgcaattacaaatcaccaaacatttcttttcacttctggttcaactatgaatctcagagatcagaaaacaactacgccgccgaagattgaaatgggaagctggactacagtaaaaattaatcaaacttgtatgaagcagaaaaatcccatcagaagtcacacacagaatgaagcatttcaaaaggtaactctctcattgtccttaagcaagcaaatgtttgttgagttatgagcaacagttgcttcctttgtatgaaatgggaagctggactacagtaaaaaataaccaaacttgtatgaagcagaaaattcccatcagaagtctcacacagaatgaagcatttcaacaggtaactccctcattgtccttatgcaaacaaatgtttgttgagttacgagaaacagttgcttcctttgtatgaaatgcgaagcctggactacagtaaaaaaaataaccaaacttgtatgatgcagaaaattcccatcagaagtcacacacagaatggagcatttcaacaggtaactccctcattgtccttaattgttgagttatgagcaacagttgcttcctttgtggcatgaaacatccaaaaaagaaacaatggagtttttagatgttgtatttatgatatgtcatagtccaccatctctgaggccttcaagttgaagtaacaaaaactactttgttcagcacaccacattttttgataacttgaaactgtgtcatccttattctcagactgagaactggctatccatttcaggaaaggggacatagaattaccattgaatctgatgaggatattgacgcgggcttttcctgcttgcttgaagaaaatggaacaggtaatttgcactccttgcttgcatcattcatttttgagaatttcatgataagcaaagtgattctacatcctgtaattgatcaatgtgcttattgacccatgcatgttgaacttatctaatgaattcaagttctatttagatgtatatcaaattatatcctatatctcaagactgactactgacaagaatgacttttccatacttctagtcaagcagaacgcctaagatatattatatgaaatcaaatacattaggtaacaagtcagaacatgtctaaaatcctgaagaatctgttacactccatactatgaagtttttctcaaaccaaagagaaactgatagctctctcttccctttgcctgttggggtacagtagggaatttgaacctgttctcaggtttagtgtcccgagggatcttgtttattttctctggaatagtctcatttcgagtctgtctaaaataagaaattttgagcatcataactgcagcaacaagtgttcttttacacagactgaaacaatcaatcgtatattttttttgtcatttgcaaagatttgcgtgcttaaacttgtctttcccttagaaaacccagggatttatccactagatgatgcaaaggaagagagtgcacgcatattaaggaaagcaaggaggcgaaagagaaagcattttaacactatcattatagattgaaggtacacagtgaatttataatctgctgaatcaaggtcctgtgatttgataagcagtaaaaaatgtattattgattcttctgtctttctttagccgattataggacatgtttgctatttgacttttcattattattagaaaatccacgactgaccattacatagcaagcaaaatctgtgttgctgctgcaatactcagtcttaggtgattgtataacgagatgtcaacagactcagcaccataagaatatgtaatgcactgggattatataagcaaaatgattacgatgttttaaattttgaattgcataaagttggctggttagatcattgcatcttctgtatacaatgttttattagctaatgagagtaaatattatgctagtaaatttttcagcgtgtgatattataccatgatagaagtatataatatggaaaagagaatccttttcaactgtgctagagaacttagaaacacctagttgagaatgaaagcatttctaccaagggaaaaaaggaaggtcggagaggttttacttattcctggacttggatggtcagtatttattcttgtttgctcataagaatctatagatcatccgtcatgttccttgcctgttgcgtttggtgtatgttaggttccttattgacttagttaaagttcagcctaaaaaatattcaaaaagagaaacaaaaaaatggcttagtctaagtagcataggcattactagccacatcgaattgcactcgtggtgtatttttattaatgtaattaagaagcatgctcaatacaaattctctacaagagtcatgcgtgggttgcttcttctttttgaataccatccaaaagtccaaacaaactttcgttggctgtaataggaagtttcccttcctgcagtcacctactatgcctccatacatgactgtagtcacttttgtaagttgaactaattttcaggacccacattttaattgagacaaattaaacttttaagcatcct

SEQ ID NO: 50 - DNA, 1779 bp, Solanum tuberosum
  source 1..1779: mol_type = other DNA
tccaactgttcgacggagcaaaatcacagagagaattcaaatgtatttacaaatttgattataccttcatctgttagggttctgtaattgttcaaattgaagttttaatttctcgaagatttcaatttttatagtatctgcaaatgaagttgaagatgaacaaagcatcggatcttagctctatctctgttcttcctcctcatgcaaggaggccaagtgtggtaccaagtgcagcagagtcttccgttttcgggaaaagccaaccatcacaggttcggtcacagcagcaatcgcaacaatccttctcacagggattttcatctcagcaagcaatctactctcagttatcacagagctctctggatgattttgtccctaatgagcaaagattgggttctcaagaaagagaaaattcagcaaaaaggatgagctgtttgcctcatatcaactacacacgagaagagactcaaatgcagttatcaaaaccttcgaccaattatttgcgcaaatggtcagttcctgaaagcaaataccagattgaagaacttgaacacaaaattggaatggtagagacttcattaagcaggcaaggaatgatcttagattctattcagagtgatattatgcaagttaaccggggaacaaaagagatattgatggagatggaaagcttacgaccgaagttagtttctcatgatgaactgttgcaattgatgaacaaggagagggaagatctgaaagctagcctggaggggaccttcaaatccatgtttgaagagcttagggagaacaaatatcaagagaacatcagagatctcttatcactgcttagagctatgcccaacaaacttgagatgtgcattttgcaacttcaaactgatttgagcaagaccttggctaaagagattcagataatttccccccgcccagattgtcatggaaaaaaacatgaaaccgctccagtcgatccaccaaaagtcatcaatgattgtagccttccccgtgaagtgaagtttctaaagaaagatcagaaaacaactacgccgccgaagattgaaatgggaagctggactacagtaaaaattaatcaaacttgtatgaagcagaaaaatcccatcagaagtcacacacagaatgaagcatttcaaaagttgcttcctttgtatgaaatgggaagctggactacagtaaaaaataaccaaacttgtatgaagcagaaaattcccatcagaagtctcacacagaatgaagcatttcaacagaaaattcccatcagaagtcacacacagaatggagcatttcaacaggaaaggggacatagaattaccattgaatctgatgaggatattgacgcgggcttttcctgcttgcttgaagaaaatggaacagaaaacccagggatttatccactagatgatgcaaaggaagagagtgcacgcatattaaggaaagcaaggaggcgaaagagaaagcattttaacactatcattatagattgaaggtacacagtgaatttataatctgctgaatcaaggtcctgtgatttgataagcagtaaaaaatgtattattgattcttctgtctttctttagccgattataggacatgtttgctatttgacttttcattattattagaaaatccacgactgaccattacatagcaagcaaaatctgtgttgctgctgcaatactcagtcttaggtgattgtataacgagatgtcaacagactcagcaccataagaatatgtaatgcactgggattatataagcaaaatg

SEQ ID NO: 51 - protein, 451 aa, Solanum tuberosum
MKLKMNKASDLSSISVLPPHARRPSVVPSAAESSVFGKSQPSQVRSQQQSQQSFSQGFSSQQAIYSQLSQSSLDDFVPNEQRLGSQERENSAKRMSCLPHINYTREETQMQLSKPSTNYLRKWSVPESKYQIEELEHKIGMVETSLSRQGMILDSIQSDIMQVNRGTKEILMEMESLRPKLVSHDELLQLMNKEREDLKASLEGTFKSMFEELRENKYQENIRDLLSLLRAMPNKLEMCILQLQTDLSKTLAKEIQIISPRPDCHGKKHETAPVDPPKVINDCSLPREVKFLKKDQKTTTPPKIEMGSWTTVKINQTCMKQKNPIRSHTQNEAFQKLLPLYEMGSWTTVKNNQTCMKQKIPIRSLTQNEAFQQKIPIRSHTQNGAFQQERGHRITIESDEDIDAGFSCLLEENGTENPGIYPLDDAKEESARILRKARRRKRKHFNTIIID

SEQ ID NO: 52 - DNA, 4800 bp, Solanum tuberosum
  source 1..4800: mol_type = genomic DNA
aaatgtagtagaaaagggagaaaagctttgtttagtaacattaagttgtggtcctatttgctccctcttgatcaacgtatacgttgctcacaataacattgatgatgatctgagtaacttaaattcatggaagaaagagttcactgtgacagctccgagtattgcatatcaattagatctagatgataatgtgtacaccataattgttaccgatgagatcgtggtgattcaacttggtgactataactctggatttttccatgttgcaactggaaagctgttgggactattttcgacaacgcgcgctactttgatcccttacaagtcaagtttggtagctttttgccatcgaccactacttccttccttctcttgagctattcttttttatgacaagggaacccgcaaaatcacacaaggagaggtaaacataccaaggcaagtcacctgtgacgggctctaccaacctaagacccctattgggaaaatccctttgactcggcaactctgtgggtcataactgttctattagagttgtttttcttaaagtcagaaatcaacttttatgtcatgtcttaaattgtttttaccatttcaatttcactgtaattcatccatctacatcatttttgatggcttgtaatttcaatacaaagttcaaaaaaatattaatattaatttactttgttagaccaacactttgacgactcattcataatcataatgttactgattatattaaagtaagcatccctcatgttaaataaaattagcatgaaatttaatgatttagttctcgtcgctaagtccagtttcttgtaacgatctttgaacgtcatcaacatcacagggaggaaagtgtagtttatgtaacaagaaggagctctttgaaattaacccaaaataaaattaaaaagggaacgcggaaaatacaaaattcgaacagactataaattagggcagtttgaaatctgcagctcctcatttccttctcgtgaagatgtcaactacagtttcgcagcaaatctccctattcagattccaagtcgagagccgtaggtttgttttcgattaatcaaaaattttattctgattcaataaaatgcacttgtgagcatgaattttgtgcagactggacgaaggaactcttcgaattctcgaatccgttttagcttgggacgattacaaatctctggacggagtggtatgtactttgaaacagttcatgagacacgaatctctccgaattattgaggaaatcgctggaaaagctgcagagcataagcttctgatcgtagattttctagttcgcgtttttgctctcatcggagatactgaggtatacagctttgactctatcaatttcaaattggtacatttcactttgacttagtcatttggaaacacatagttagtagaagatagagttaatcggaaagaacagtagtttttttttttttgatgacaaaaagaacagtagttttcagtaggatgatgttgaagacactgaaaaaatgcatacagtggaagagtgtctgctgtattaaaccatgtattttggtggaatttgtgataagttgaagcgctgcttgaaattttgtagcctgttgtgttcggtaattgtattatcttcaaaagataaatctcatgctaatattgttttgctaaggaagttatttctttactttagttttagtgttggaatgcatttcaataagtattaatagtagacacagataacttatatttctgtacaagtggcggtggtggcaggtggtaatgtgagtagcaaaagatgtaaataatgactgctgtgtggcagagaaattggtatctgtaaaggaaatatatccttccttatgtatatacaaaaactcttttcggttaaagtttgtgaaaatgaagtaatcaatagaagtgatatttaggaacacgagaacctgtctatactctatccaataagtgtaatgattggatagctttcatggtatattacttcagatacacctcgttcttttcttatatgtgaaacaatttgacagagcatgaggttaagagttagctgtagtcttcaacagaatgtcgatgtagttgtcgagaattcatctgattttaaacatcacatcatgctttaaattatctttttgaaatttgtgaaagctgcatacaaaatttatcagagttaaagtgtgtcgaactttttgggagatccaaagtgtaggcatatcctatgttgtgaaagctttaagaaaccacaactgatgatgattttattcttctattatagaaattctggttttgcctttttattttcggttccaaacacgtgatttttaacaattgggtattcacagagttgcttggcgttgagatatgaggcattgcttatgagagagcagaaagctatcagtgatcagaggcttcttgtttcatatagcgagtggctcacttttgctgagcattcacttgaaagtggcttttgttccattgcaaagaaggtaaatttctgacaaaattttgggcacttgtaagcattttacatgtgcaaatgagcaaggaacaaaattcttagtatatgctgtccattgaaaatttatggtcaggtcagagttaatgctaaatgctactgcttctactgttacgtttctatacttctgtgatcgtagcttgaaggttcttatcctgtcatattgtgttccccttttggatgtgtttgtaggttctatctctgttagtttacctgaataatttgatctgacactcagatgctattgtgaaaatcactaaactttgttatctttatgcctcttgttggaaatttgttagatgtagatttacggttcttttgcattctgaattaggaattagactcactgctgaaaacgtctcgttctaattagcctcctctacctcagcaatgagtcctcctttgtctacttcagaaatacagtatggacagtttgtcatgggcttatgtgtagtgaacttatgctaggaattagatcaatctagctgtgcaactattgcatgtttaacatcttaccgacactaagggcatatgtatttcacttgatgctatctattttgttcatttattttgagcctggtaccttatggcttcataaatattgtgaagttacaacgtcctactgcttatagtaagtgtatcccaatatctgcctctgacttgtacttttcaggcatgtgaaaaggcgctcttatgtttagacatgaacatcgtagatgaccctgaaaattatttcgtaattgaaaaaattaagaagcttaaagacgttgctgtgatctcagcgtcttcaaaatctggtatgttcaagtatttcattaaatccctcctttgtttcatagttaatgctttgccgttatatgttcctaacatgaaagtgaaatgaatttggtggaatgacatcaaagtcttctattaaatcatatgtaactagaagggtggtgaagggaaagctaattgttatctgttcattactgctaaagctttcttgtggtacaatagttcaggcgcaggcagtaacgtacttcaagaacaaaaatattcagcagaactcacaagaatcctacattcctgtggaagttaaaagttcaggaagcactctgtttagagatggaatcaaaagacgacacagacgccaattggatgaataccgacatctgaaactgaggggaataactgatggaaacacgcaaaatattttggtaggtcattatgctaagtaaaaaagatcttatttaatttcgtcatttgattacagttgatagtgcaggaatgatttttctctgaagtattactattatggagtcaccaatatgatcaaagatcaacttcccttcttttggttagtatcttggaaggtaattactttgattaatataccacgatatcattgctatgatatgtttaaaacttatataagaaatatggtcttataaaaaaatattgtgctgtggtaagaacgaacctcttgtttcatctattgactcttttctttcttgtctaattgaagagaatttgttccatcaattgaaaactcttcaaaatttatttttgcaccataataagcaatttttggcattttaaattactgataatgagacaaggtcgactgcttgccttgtctcttctcgaccttggtcctgcaataggaacctagcatgctggtgataagccttcaataaaatatgtttcttagggaatctgtaattaagtctaagcaacaaacaaagagtacatttgcagcaagatattagcttcagcccctctccatgcaatcacgtgcctatccagttgagtgttttgtcaattttcagaccttcaccaaattggataggtgtaacttactagttaaaatcaaagagttggattagtaagaaattttgactataacaattactacttttaattttcatgttgcacttttcgaaagtcaatttgactaatctttaaagttaaattagattacattaatttgatatattaaacaaaaaaattagatattcaaaaactatacaaaaagtattataaattgcaattttttgcatatcaatatgatgaaaaaatatatcgtaaaatgttggtcaaagttcttattgtttgactctaaaaaaaactatgacaattaaaaatggacgaaagaagtaggaatttgtataacttttaagaaatccaatgaacgaggacataagggaaaaaaaatcttctttctttaattgtatcacttaagaatccatgtgaaatgaaaatatcatgcacgattttgaatatgaagaatt

SEQ ID NO: 53 - DNA, 1067 bp, Solanum tuberosum
  source 1..1067: mol_type = other DNA
gaacagactataaattagggcagtttgaaatctgcagctcctcatttccttctcgtgaagatgtcaactacagtttcgcagcaaatctccctattcagattccaagtcgagagccgtagactggacgaaggaactcttcgaattctcgaatccgttttagcttgggacgattacaaatctctggacggagtggtatgtactttgaaacagttcatgagacacgaatctctccgaattattgaggaaatcgctggaaaagctgcagagcataagcttctgatcgtagattttctagttcgcgtttttgctctcatcggagatactgagagttgcttggcgttgagatatgaggcattgcttatgagagagcagaaagctatcagtgatcagaggcttcttgtttcatatagcgagtggctcacttttgctgagcattcacttgaaagtggcttttgttccattgcaaagaaggcatgtgaaaaggcgctcttatgtttagacatgaacatcgtagatgaccctgaaaattatttcgtaattgaaaaaattaagaagcttaaagacgttgctgtgatctcagcgtcttcaaaatctgttcaggcgcaggcagtaacgtacttcaagaacaaaaatattcagcagaactcacaagaatcctacattcctgtggaagttaaaagttcaggaagcactctgtttagagatggaatcaaaagacgacacagacgccaattggatgaataccgacatctgaaactgaggggaataactgatggaaacacgcaaaatattttggaatgatttttctctgaagtattactattatggagtcaccaatatgatcaaagatcaacttcccttcttttggttagtatcttggaaggtaattactttgattaatataccacgatatcattgctatgatatgtttaaaacttatataagaaatatggtcttataaaaaaatattgtgctgtggtaagaacgaacctcttgtttcatctattgactcttttctttcttgtctaattgaagagaatttgttccatcaattgaaaactcttcaa

SEQ ID NO: 54 - protein, 246 aa, Solanum tuberosum
MSTTVSQQISLFRFQVESRRLDEGTLRILESVLAWDDYKSLDGVVCTLKQFMRHESLRIIEEIAGKAAEHKLLIVDFLVRVFALIGDTESCLALRYEALLMREQKAISDQRLLVSYSEWLTFAEHSLESGFCSIAKKACEKALLCLDMNIVDDPENYFVIEKIKKLKDVAVISASSKSVQAQAVTYFKNKNIQQNSQESYIPVEVKSSGSTLFRDGIKRRHRRQLDEYRHLKLRGITDGNTQNILE

SEQ ID NO: 55 - DNA, 7182 bp, Solanum melongena
  source 1..7182: mol_type = genomic DNA
aacatgactatatttgttgcaaattaattaatttattgtatacatttgaaatgatccctttttaatattggactatcgagtaaaccaacccattaggatataataatttattactttacccttatataaatgtacatattgattgtacctttcaattcatacttcacaatgattttgcactcacaaaaataaattattttatttgtgatgcacttgtatagttcctttcatgttagttataattatttctattttatgagcattttataaaattatattattgttccgtctcgccaaaatattggagaagtcatatatttatattataagcattttttattggataaatgaaaatcgaatcattaagtgcctgataaataaaaaattgataaagaaaaatgtctcattgattgattattggtttccgcatatttaaaaaaattgaaaattaattaaatcaaacaaataatgtataaaattgaactgaacttactgatgcacacccttaatcagagcccttattctaaggtagactcaaaccttgatcttgagtaaaaaattaatatcaaattgagatttgcattaaaattagacacaaatctccaatcaaagtcaggagcggagtcagagaattagatcctaggttggggttaggacctaagagttgatcttaaggtcgggagtcgaggattgagtaagggccgagttgagagttgagtctcagatcaaggtcgaaagtgaattttaaaaaatatatttcttacttttatataggaaagtaattgttttaaaattgaacaaaacagaaaaaaaactttttcataataattaaaccaattaaatataacaaaattaacaacattttctagaaaatgttaaccttccatgccaaacacacccttgtgtgctaacttgcgcgcgcgcgcaaaacttcacatttataaagctggagttttaccagttttcagaaaacgtgaacctgcagagcaagagaaagaaaatggagggaaagcgctcgaacacgcagccactaacactcataaggaaaatcaaaggtcgatagcgcttccattacacttcaattgtttcctgaaatattcattgcgattctcgcattcaacgcattgtttctgaacgaatcatcttcacgtttgagccatatataatttaattttgttttgcaggatttactcgttccattgttgaggatctcgctcgaggtagggcaccattgatctacatcgatcggttcagaaattactgcactgacacttctggaaattggtaagaagcagcagtagcttgaatatgtgaaattatcagtcgaagttaagcttagtgaagtgtttttgcttttccttttcttctttttggtagatctagttgcaaacagtgaatgcatgctgctgtttgaaatttcgttgcaattagtgttttggaataacacagaaaagtaacagtgaattgaactggtaatttcctattaattttaaaagaactacatcgatcagttcagtaattgctgtactgacacttctggaaattggtaagacgcagtgtatgagtgagtatatgaaattgttaatcaagttaagcttagcaaagtgttttttttcctttcttcatatgggatgatctagttgaaaacagcgaatgtgtgttgcagtttgaaatttcattgcaattactattttagaatttgtgcacgaaaactaatattgaattaaactgttgatttcttatgaactactaataatacctcgattggttcagaaatttctctactaacacttctgctaattggtaagatgtgtatgtgtgtgaggatgttacttggtagcttgagtttatgaaattatcagtcaatttaagcttagcaaagtctgtttcttctttaccatcgttttagaagatctagttgtaaactatgaatatgtgcagtggtctgaaattatgttgcaaatagtgtttcagaattctgcctcagaaaatgagacttaattattgttgatttcctatctcctaattgaaacacaacagtatttggttcctttctatattacaaggcctccaaagagattatccttgatgtaattgaactgaaaattgcaactgatgaagatccatataggttttaatgctgctttaagatattgctagaactgggcttggtagattattctgtggaacttcagatggtatgcccctaagccccctcaacacaaccccttccaaaaaataaaatgtagagaggaaacgaattgttttttttaaaatgcccttctcttaagaagaatgagtgcagtctatactgcgagatttgttcgtagaagccatatcctattctgagagactaacaagtactggtagtaatggttttgttgaacagagttctaaaaacattgaagtttactgaagtgggagtttgaatggttaattacaccatccaaatgttctgatggtattaatggtctttgtttattttatgtagctcttgcagctctggtttgtcgaccggcaaggaagctatatccttgaagagggaatgccatgcacataggcttggtgagtctagggagagtaaacagtacttgtattttcatctactagtcctcatcacgtagttggacaagaaattatatgatcgataagagggtaggaatgataattaaaagttgctatccttcctgaaaaacaacaaaattaccaggagaactatttccccatttagttgacttctctgtacttttgttttcctatatcagcctccctttacttgaagttacacaggatgcaccatgggtggagggtggggtgaagtacagatttctctctcaattttcttttctgtttggtcgaatcaacttgaaggccatttgctctccaatctccttgacatcctagaaacttgctagattacttcctctctatgtttttttttttcagatgttctgttgagagttcttctgatagttcaacaacttctgcaagaaaacaggcatggatcaaaaagagacatatattacatgcatcctactgtttttaaaggtaaatgtggattgacctctggtgttacaatgaatcctcttttcagaagaaaaattcaattctaggtgccccagtgtagttaattccctgttaactttgtcggaaatggttggactttatgtactctagaatcagttttgaaatattcatatgattggttatgaattttttcttccatggaaaatacttatgtgctgttgtataatcaactttctcagtcgctggaaatctgctatgatttagatctctaacacaaaatttatatattcaaaggccacctcctccttatatgcttcatcgttttctcttgcactctgtaatgcagagcaatctgtagttgatcgggcaattaatgacatctgcatccttttgcaatgcagtcggcataaccttaatgtggtatgtcaatctactttcctctccattcaaaatagactcattttttttttatgtatatccacatgtccccactgttcagctgagaactttttcacggagtgctttcacagtctcttctatttttatttagttacatgttcatttttcacagtggaggattcaattagggttcaaaatattgattaatttagaaatggtcattctgctttacttatatatgcttttgacacgtgaaacagtagatcacaagtatctgaccccgcctcctccataccatggggagtcggggaggggtttacttgtatagttaactagtcgtgaatactgttctcgtatagaacttgaatatcgatttcagagaatgaaaaggatattgctggactagggtaagcacatcattcaaacgattagtattctcctttcattgctattttttttaagaaacttgacctttttatatttttttctaatgcttgcctctgcaggtgtctgttggaaatgggtgcgtacctctacacagttattgccttgcaggagtgtgcttctagacacatacagtttgagttcattatatcctatattctctctcatacttcacatttaatatttgcaatcttttcttcttcagttgattatgtttatacctcctgcatttgtctgaatgtgccttcatatgtgtctacattcctctttggggagcaaagttacttcatgcttgagggatttgacatagtctgtcatgtgacaataaacttttgtactttgagcaaggtaaaattttataataacccagagaaagcatgttaactctcaaggagtactattgcatcatcatctttggcctactttttaaattattggcagcacgtgtaggtctagtttaaactgctcgccagtgaaagtcacaataaatgaatctactgctgttgcattttgctcatgacaattttctgttccttaagattgatatatagttggttttcttctttgtttatattataatagagtcgtgcaattcttggtcttgaaattcttcttccaactatttctggtctagattggtgatgggttggctgcggtatgtggaatctgggaggaaaattgactgcattagcaatcctaacactgtaagaatgataattagaagctaagatgggtttctgtagttgtgtaacaatctaattatgatggttcatgcaggcacacccgattccggtccttgttgaagaagttgatggtatccttatgagtataagcatccgaattatgaccacaacatggttaaatatgaccatgagtttgtggactccattcatgtgcatgtccaagttattgctaatcataaagttgaattgatgctttgttattgaatatatcctgctatttggctgtatggattgctttctcagactatggctctagttgttactcccttaatgcttgagcaagttattattagtgttgctcaatacgttttagttgtggaaaaggaatcaggtaaaactatttattagtggatcaaggctataatagagtcatgaaaggtatttctagttgataagtgagaccactatttgttgttcatcgtgcagttttccagcgactagcaaatgatcagttttgcaagaggaaccgttgcattgtgataacagtacgcatcttttgttttctgagagtctccacatatatttggctccataatttctttttaacagggaaggggttatcctgatgtccccacaaggaggttaggcccatgttgctcaccttgttagactcgttgtagttgaatcaattagtcatatttctgtctttgcatgttgcttgcctgtggcaggtttctgcgtctcctggttgacaagctgcatttgcctgtgtactgcctggtagattgtgatccatatggctttgacatcttaactacatacaaattcggttctttggtaaggactattcaatgtggtgttatatgatatgaacacatttgcaaatcttcctccttttcactgtagcagtttacacttccatttttaattagtccaaactctaatattcgcatttctgaaagaaaattctgatacattcttcaactgttttcctatcaaaagctatcaagcatttattcttttcttgatagtaatctacgtgagacactaaggttgaagtttatatagcttttagattagatggattgataattggatgttttattcagtaacatttgtctgtgtatgatttttgaagcaaatggcttatgatgcaacatttttacgagtccctgagatacaatggcttggagtatttgtacaggattgcgacaattatagaattccacagcaatgtctcctgccattgactgtagaaggtaaaactcacacatttattatctcatttcattatagcttttaagaaacaactcctcagaaatgactggttgtgtaatcttgtcagataagaggaaagtcaaagcaatgttacctagatgttatttgcaaagagaagtaccaaaatggaggtacaattttatactactaagtaatgttaatgccagtatatacttatggtcgggttctcaagatattcatatgactgttctccacgccctaaggtttgaactggagctgctgttgcacaaaggagttaagtttgagattgaagcattgtctgtgcattcagtcactttcttgtcccacgagtatctaccatcaaagatccacaatggagggtatatctgaatcttttctatctttgttcggtattttagcacgagaagttcaaatcttttttcgtatgctcacttatatcatttgaaagaacaaccttagcaataacttttgtcaaaatttacgacaatggttgtggatatctaactacaaatgtgtattgacattaaagcaattggatctaaagtagttatataatctaaaattttgcatttagcctgttatgacactacctgttggccgttgcttttaccgtgaaagtagagccacgataaaggtgtagaaataactatatagacaataaggaatacaaatttctatgaaggatttaagttatatgtaccataaagcgataacatgtttgtcactctttttttccaagttaccaattattgtttatccatgaattacatgtaaatactttattagtgatttaattgcatgaatggtttctttaaatagtgtatttcaatttacgattagaagaatctgagttatatgcataaaaaagcaccatttgactttgagatgagaaagaaggtgcttcttgccccacctgcacaaatcctctaaggcggaatataaacctagagtggttcaatgactcaaatgtagtcaatcaagaaggccataagacccttgcagagtttcccaacaacatagagcttgggaagcttggatggtatttgatttgccaaatatatcattattgtatactctttcatatatagcgcaacccaattttattttttaccttaactttaggcataatatatagataaacatttttatttggatttaatccacaactatatactccaactttgaaatacgcaagacactttaacatggtctaaagttggccttacaaaatcccatctttgagaatgcacatctagatgcactcccttaaaaatgtcgagatatacaaggttaaggtgcttgtgagacgcaactatctcaagttgaagcctcttgatggtcttaaactcgcaatgaaaattgggagtgt

SEQ ID NO: 56 - DNA, 1182 bp, Solanum melongena
  source 1..1182: mol_type = other DNA
atggagggaaagcgctcgaacacgcagccactaacactcataaggaaaatcaaaggatttactcgttccattgttgaggatctcgctcgaggtagggcaccattgatctacatcgatcggttcagaaattactgcactgacacttctggaaattgctcttgcagctctggtttgtcgaccggcaaggaagctatatccttgaagagggaatgccatgcacataggcttgatgttctgttgagagttcttctgatagttcaacaacttctgcaagaaaacaggcatggatcaaaaagagacatatattacatgcatcctactgtttttaaagagcaatctgtagttgatcgggcaattaatgacatctgcatccttttgcaatgcagtcggcataaccttaatgtggtgtctgttggaaatggattggtgatgggttggctgcggtatgtggaatctgggaggaaaattgactgcattagcaatcctaacactactatggctctagttgttactcccttaatgcttgagcaagttattattagtgttgctcaatacgttttagttgtggaaaaggaatcagttttccagcgactagcaaatgatcagttttgcaagaggaaccgttgcattgtgataacaggaaggggttatcctgatgtccccacaaggaggtttctgcgtctcctggttgacaagctgcatttgcctgtgtactgcctggtagattgtgatccatatggctttgacatcttaactacatacaaattcggttctttgcaaatggcttatgatgcaacatttttacgagtccctgagatacaatggcttggagtatttgtacaggattgcgacaattatagaattccacagcaatgtctcctgccattgactgtagaagataagaggaaagtcaaagcaatgttacctagatgttatttgcaaagagaagtaccaaaatggaggtacaattttatactactaagtaatgttaatgccagtatatacttatggtcgggttctcaagatattcatatgactgttctccacgccctaaggtttgaactggagctgctgttgcacaaaggagttaagtttgagattgaagcattgtctgtgcattcagtcactttcttgtcccacgagtatctaccatcaaagatccacaatggagggtatatctga

SEQ ID NO: 57 - protein, 393 aa, Solanum melongena
MEGKRSNTQPLTLIRKIKGFTRSIVEDLARGRAPLIYIDRFRNYCTDTSGNCSCSSGLSTGKEAISLKRECHAHRLDVLLRVLLIVQQLLQENRHGSKRDIYYMHPTVFKEQSVVDRAINDICILLQCSRHNLNVVSVGNGLVMGWLRYVESGRKIDCISNPNTTMALVVTPLMLEQVIISVAQYVLVVEKESVFQRLANDQFCKRNRCIVITGRGYPDVPTRRFLRLLVDKLHLPVYCLVDCDPYGFDILTTYKFGSLQMAYDATFLRVPEIQWLGVFVQDCDNYRIPQQCLLPLTVEDKRKVKAMLPRCYLQREVPKWRYNFILLSNVNASIYLWSGSQDIHMTVLHALRFELELLLHKGVKFEIEALSVHSVTFLSHEYLPSKIHNGGYI

SEQ ID NO: 58 - DNA, 6752 bp, Solanum melongena
  source 1..6752: mol_type = genomic DNA
ttcgtttttttcctttctaaattcgttaagttcatattcagcaaagcaccgctcggccaaatatggtgaaaattatcgattgctacttgccatttcgtttttttcctttcgaaattcgttaagttcatattcatacgctacatttttggagttcctgtgtttttactagtacatactgtaaatcctgagctagatttttatttccttctttggtcgctgtctaatgatatccagtagctccttcacacgatttctcctaatttgaagttccagatgagttatatgttaagttttcacagttcaaattggatttgttgctgttcggaaatgcttaaattcatattgtttatgaatgtatcgatccagtttcttgctcgtaaagcttcgctccagatatgatgaaactttttaactacttctatttcgaattattcccttcaaaattcgttaaattcatatgcataagctaacattatatgagtttctgcgtttttacttgcatatattgtaaattctgtagtggatcttcttttccttttctgctttctgtatgataatgtttagaattctctgaacctcattcaccgctatttcgtttacgaagttgaacttcgagttatatatttagtagtcacagttcaattggatctgattctgttctaaaaatgcttaaattcaaattgtttatgaatgtaatgatccagcttctcgtaaagctctgttcagatgtggtgatttttttttaattacaacttctattttaattttctattctaaattcgtttgatacaaattgatgagctacatgttttgagtttctgtgtttttaactttcgtatatggcaattcctgtagtggatcttcttttgtcttttgctttctgtatttgttgaagctcctcaataggatttttcgtatatgttcagatatctcatttcaatttggcaacgaagaatgtttaaactgaaattgtttatgatgtttctctttgctgtgaaggatggcggccactcggcactcgaacctcaatcggaaaaagcttagcaaactcaatattattgacatctggtaacgcgttttcttccattactatgttgcactgcactttattcctcgttgattctgagtaatcatcttctgcaattttttgttacagtgaacaaatcttaaatccatcggtcccgatggctctgaggctctctggaattctaatgggtatgcttcaaaaaccaatgatgggtagaaattgttttgcttcttccatttagatatctaagcgtcagttttatctcaggtggagtagtcattgtttatgaacgcaaagtaaaactcctctacggtatgaattgccatgacttcttcaacatttctatttgaatttcacctcaatttcttcgaattttacaattaattcccttcccttatttcttcaaccttttattctttgtttttttctatattgcagaggatgtgactcgtttcatggtagtaacattggttttcgatccctatcaacttaatctctttctttactctgtatccattaaattcagcatttctttgtcctttaattggtgatgattacataatgtaagatttggtatttcaggtgcaaataaatgaagcttggaaggtcaaaacagctactgatcctacattacttcccaagggtaaatcacaagccaagtgagtaacttatctccaccgcgacgtcacagtattttgccgagaagcagagattgtaatggcaaattttagcaactgtctaacagtttcagttacctcgatagtgcttcagtaaattaacaactaaagtatgaaccaccaccaattagttgagttattaactcaattattatgtttagttgactcaatgtttggttaagtttcatcaatggataattcaaggccagcttattgagtcctttatactaaagagtttggtacttaaaatagctagtttactgatgaattggttgcaagttaagacttagcttttcatcctccatctcaattcctgtaggtatgcagctattactctgccagagaatcaggaacaagaactccctgagattgaacagacatcacgaaatccagacactgtaacaatgatggatttcgaacaaacctcctatttcgcaatggtacattatggaaagcactctcacctcctcaatccatggaataacttcaaaagcagaaacaataattcttaggaaaatcggaatttgttggaaggttggaactgatctaattagactattgagcttgctgtagattgttgaataagtcgcatgttgatcattcagcaaaattgcaagctaaatcaatagaaagttaacaataataaaaatggtttgatttcccttagttttctattggttactcgacatgttttgtcatttgttttttaaactttttgagagactatctaaagttatttgggttttgacagtgttcatgaccttgttgagcaggcaatcttatctgttaccaattacataatgaaaataaggtcataataagtaatttctacataagagtgcagctaaactcatggatgttcaatgtgcagagactagataatgctgagctctatgataaacccaatgcacaggagaaaccagacccggacttgcatcaaggtatacccagatcccactatcagcacagattagcataatttcactaccatagtagaatatagaactatatccttgtcaatgctactatagtttccagattctcttgttgtgcccgtatctaaacaatcctgaaatccttgatgcagttgatccagataatatcaccctggctgaacaatttgaatcccatcatacagatatgttcaatcattatgagaggtatcatgatgaacaattaataggctctgtatttctaagtttatctggtcagttaacataaagacttcacgtcaaccagactatccatcattaaatcaagggagactaattatcctcatttcaatataactgcaaagttttccttccattatcctcgtattaatttttaagctcaaattactctgcaggtttgatattgaaggggatgatgaaacacaaatgaattttagccagccagaggatgcccaaatcccaaatactcttgtgccttctccacctcaagaacaagcccatcagcgtaagttttgagttattagacttgccgctacaaaaatagggtactatcttctactttagataaatgaaaatttttgagatgtaaatagtgtatggacttcagatgattcacttggtgctttaagagagaatttactgataaagacattatggcaataaacccatcctctcaaataggaacatggatgcaagtcgtacttaggtgctatcagatcagctaaaatacttggtaacaatgtgcaattccttcaagaacaaagctcaatcctcataagagtctagatttccttgggtaattacttatattcgcaaattggttgactggagcgaaatttcgttgcagctgatgagatccctgacagacatccagaggaccaagtgaagcagcaatctgatgaagctgaagaagttttcgaggtagaaactccacaagtaactgagctagaaaataaagtaaagaactgtcagcattaatctaatgtcttaacgtgattttgtagcagcagcgggaccaaccgaggccaaagccagctcgacgaagaacaagaaaggccgcaggtcttgcaattgatcatgagcaaactattatttctggtgacatatatcaatcctggcttcagaattcttccgatattgcatcaagaaaaaggaaaaagagagaggtatggaacatacctaccaagtctagatcttccccacctcaaattttctattagcaattaaaatttgactagggtcttaacctaaaataaagcatgtttatgtttgacatcaatggcttgtgtttgaatatcctaagaatagtaagttcatctctctttggaacgtaaccttaactaaactaagctgcagcgtcatttattagtaaccttaagttcctgctatgtgcagactttgagtgtcttatcttctacgaagatagccagaatcatggaggtacctcctattgctttactggaaggattgctcacaaatgaaaataaggaagttcactatccagcaccactcctaaaattgtggacgagaagtacccaacctccgccttctggtctggtttttcatccatgattttagactcttagacgcaaaaactatgaacagatggtgattccatttgacatgcaggaaagacctctccaccctgtcctcctgaaccatcttacacatctccaggtgaaaggatggttaatttggaacctgtcagatatgtaaggaacttatgattctcaattagatttaaataagaaccacctttatttgcttctgattgagcatttgaatgtgaagcctttcgaacatttccaaagtggtgtaggctccccatcaatcagaatctctatagagaaacaaagagcaaatctcaacaataaccagattccacctgaaattctcatggagggcctcagaaccaatcttacaaacatggaactgcatccaacagaagctaatggagtgaaagagactgatcacatggccacacctggctctggtatatcaaagttttatgaatatcccaatctctgtcttgttgggaggtctgctattgcggtacaactaatatttttgtgaatctataggtgatgagcctagatccattccaagctcagggtctggtcatggtttactatcacagaactctgttaccaattcaagccggttagtattgctagtagatatatgttaagcgggtatctgtctaaagatgtcacttgaatcatacatacattaacagaaggaaataaagaacatcatgggtctcggtaccatagggaactttaaatctttgcttaatctttttaaaattatgaaggtctccccatatagcagcatctggttgcattgatcaaaattgtcaactcttcaggtccaacaagaaaagagcccattcttcatcaaagcacagtggcaatggccttcaaccggtagaagaggagaatccatggcacgatcccgctccaaatatcaagttaactagattatctgaactatctgataatggttttacacaagataacggtttgtgaatagtcaataactttcccattttagttctggtaattctcttttatgtggtttagtttgttgttaaccaccctttactccttttgcagagatattgatggaaactggaccaacacaaacccaacacccattcatgactcaacctcttgacatcatgaccgactctatcaggatgtaaatcatttttcattagttcctaaaacttcaagtttcattatgaatcatctgacttgttgttttttcacatggtacattgatgcctacagacagctaaagagccattttgacactcctggatcggcagaagcagaatgtttgaatgaactaactcttgggatgacaaagaaacaagcagcatgtctcttttatcagacttgtggtatgcttattcttccaattctttgacactgcattgcagctcagagatacttcttaattccagcttttctcattagagatgttaatgtttgcttattcgatgtgcagttctggccactcgagacttcataaaagttgaacaggagatgccatatggaaacattctcatttccagaggtgctaagatgtgaccacggataaatggagaagatgctaagccctcacaagtcttgtcggttcattcattgttatagctgatgcaaatttgtttttcagtaaggtattggagggttcaggcacagatttatagtttgaattattaggatagagggttttcattgttaacctaagtagtgtttaatcatataaacatagttatttccacgagattatagatagtaaagattggtcatattctaagaccagctaaagtatcaattcgactactgaaactgtcggaacaagcttgttggaaaatgttttaggaagtgtatgaaggtcaactgttgaagcttaaacaagacaccacttaaataagcattcaaattgtaacacaaagaagtgatatctagttccaatgaaaaggaaaagaaatcaataccgttcacagagccattggacaacttttctgcagtgttatcaactttctttgttttgctttttgtataacgccacatcatgctgcaatgatacgatggtttcactcagagtacactgttggttttgaagtgacagtccctaaatctatttcatctgaataaaactatgtagtgcagcagtaactgcccagtacaaaacatgttcagttataggcaaatctaagatcgaaacctctttacccgattaaaacttccaacagaaacacaagacaagtttctttgaacttctcatatgcagtgtccacgctgacacaactaagaacaatattcaatagtttggctcatctacagtccacctaaaatcttacctacatgattgaatacaaacatctcaacagacttttaacacataatccaggtttacatcctctcttccctcctccgtggggcacatgtgatgatttcatcaactcgtagtatcatctcagcagcctcggttgcagagagcaacactgcctgtttgactttgaatgcctccgatattcccagctctgccatatctccaacctgtcataaaagacagataacgatg

SEQ ID NO: 59 - DNA, 2292 bp, Solanum melongena
  source 1..2292: mol_type = other DNA
atggcggccactcggcactcgaacctcaatcggaaaaagcttagcaaactcaatattattgacatctgtgaacaaatcttaaatccatcggtcccgatggctctgaggctctctggaattctaatgggtggagtagtcattgtttatgaacgcaaagtaaaactcctctacgaggatgtgactcgtttcatggtagtaacattggttttcgatccctatcaacttaatctctttctttactctgtgcaaataaatgaagcttggaaggtcaaaacagctactgatcctacattacttcccaagggtaaatcacaagccaagatggcggccactcggcactcgaacctcaatcggaaaaagcttagcaaactcaatattattgacatctgtgaacaaatcttaaatccatcggtcccgatggctctgaggctctctggaattctaatgggtggagtagtcattgtttatgaacgcaaagtaaaactcctctacgaggatgtgactcgtttcatggtagtaacattggttttcgatccctatcaacttaatctctttctttactctgtgcaaataaatgaagcttggaaggtcaaaacagctactgatcctacattacttcccaagggtaaatcacaagccaagtatgcagctattactctgccagagaatcaggaacaagaactccctgagattgaacagacatcacgaaatccagacactgtaacaatgatggatttcgaacaaacctcctatttcgcaatgagactagataatgctgagctctatgataaacccaatgcacaggagaaaccagacccggacttgcatcaagttgatccagataatatcaccctggctgaacaatttgaatcccatcatacagatatgttcaatcattatgagaggtttgatattgaaggggatgatgaaacacaaatgaattttagccagccagaggatgcccaaatcccaaatactcttgtgccttctccacctcaagaacaagcccatcagcctgatgagatccctgacagacatccagaggaccaagtgaagcagcaatctgatgaagctgaagaagttttcgaggtagaaactccacaagtaactgagctagaaaataaacagcgggaccaaccgaggccaaagccagctcgacgaagaacaagaaaggccgcaggtcttgcaattgatcatgagcaaactattatttctggtgacatatatcaatcctggcttcagaattcttccgatattgcatcaagaaaaaggaaaaagagagagactttgagtgtcttatcttctacgaagatagccagaatcatggaggtacctcctattgctttactggaaggattgctcacaaatgaaaataaggaagttcactatccagcaccactcctaaaattgtggacgagaagtacccaacctccgccttctggaaagacctctccaccctgtcctcctgaaccatcttacacatctccaggtgaaaggatggttaatttggaacctgtcagatatcctttcgaacatttccaaagtggtgtaggctccccatcaatcagaatctctatagagaaacaaagagcaaatctcaacaataaccagattccacctgaaattctcatggagggcctcagaaccaatcttacaaacatggaactgcatccaacagaagctaatggagtgaaagagactgatcacatggccacacctggctctggtgatgagcctagatccattccaagctcagggtctggtcatggtttactatcacagaactctgttaccaattcaagccggtctccccatatagcagcatctggttgcattgatcaaaattgtcaactcttcaggtccaacaagaaaagagcccattcttcatcaaagcacagtggcaatggccttcaaccggtagaagaggagaatccatggcacgatcccgctccaaatatcaagttaactagattatctgaactatctgataatggttttacacaagataacgagatattgatggaaactggaccaacacaaacccaacacccattcatgactcaacctcttgacatcatgaccgactctatcaggatacagctaaagagccattttgacactcctggatcggcagaagcagaatgtttgaatgaactaactcttgggatgacaaagaaacaagcagcatgtctcttttatcagacttgtgttctggccactcgagacttcataaaagttgaacaggagatgccatatggaaacattctcatttccagaggtgctaagatgtga

SEQ ID NO: 60 - protein, 763 aa, Solanum melongena
MAATRHSNLNRKKLSKLNIIDICEQILNPSVPMALRLSGILMGGVVIVYERKVKLLYEDVTRFMVVTLVFDPYQLNLFLYSVQINEAWKVKTATDPTLLPKGKSQAKMAATRHSNLNRKKLSKLNIIDICEQILNPSVPMALRLSGILMGGVVIVYERKVKLLYEDVTRFMVVTLVFDPYQLNLFLYSVQINEAWKVKTATDPTLLPKGKSQAKYAAITLPENQEQELPEIEQTSRNPDTVTMMDFEQTSYFAMRLDNAELYDKPNAQEKPDPDLHQVDPDNITLAEQFESHHTDMFNHYERFDIEGDDETQMNFSQPEDAQIPNTLVPSPPQEQAHQPDEIPDRHPEDQVKQQSDEAEEVFEVETPQVTELENKQRDQPRPKPARRRTRKAAGLAIDHEQTIISGDIYQSWLQNSSDIASRKRKKRETLSVLSSTKIARIMEVPPIALLEGLLTNENKEVHYPAPLLKLWTRSTQPPPSGKTSPPCPPEPSYTSPGERMVNLEPVRYPFEHFQSGVGSPSIRISIEKQRANLNNNQIPPEILMEGLRTNLTNMELHPTEANGVKETDHMATPGSGDEPRSIPSSGSGHGLLSQNSVTNSSRSPHIAASGCIDQNCQLFRSNKKRAHSSSKHSGNGLQPVEEENPWHDPAPNIKLTRLSELSDNGFTQDNEILMETGPTQTQHPFMTQPLDIMTDSIRIQLKSHFDTPGSAEAECLNELTLGMTKKQAACLFYQTCVLATRDFIKVEQEMPYGNILISRGAKM

SEQ ID NO: 61 - DNA, 5583 bp, Solanum melongena
  source 1..5583: mol_type = genomic DNA
gaaatagtttgttttttgaaagttattacaactttagtttaaaagaaaaactccatatttattcaatagagtagtcttgttagattttatttgtgaaattttactaaatatactattatttttgttgttttaatacctagctcgttattcttcaaattttacaatcacatcatgacaaaaaagctatttgaaattttaaaattaggttggagttaaagatgtatttgattatatattttaaaaaaaatatttgaaatttaaatgtacgtataaaaaatatacctaatcctcttcattattttatttcatacctaaattattatgatcctaaattccatttttaactttaaattcaaataagattgctttcatgttcaactcaattcaaagctaagtgaacctttggatactaacacaatttcattccttattaccaaaatttatttccattaatataatctgtcattagcatgtaatcaggacttattattttaatttgtttttccaaaaaaaaaaatctctttttctgtttgtatttggctttattggtggaaaaaaaacacaaaggggaagcgtgagcttttttctgggtgcactaaagtcaagacgaatcccttcaaattcgaattcaaaaaattactcactaaactcacagccctttcatcaccgcagtaaatatgtcctcatctgattggtccttggtgttttaactatcacgtccaattcaaacaagtgatttttagtgggcccatcccttgtccgctcctaacgaatacctaaaactaatcggacggcccagatcttctttcaattcaaatcagccctttttccccgcctatgcatcatagtttaatcatttatttattgcttttatataacagctctcttcttcgttttcttgaagagaagttgtttacaggaatgagaagttgctgataggaggaggaatttttttcgatttttcgtctagtgattgaagggttctttttaggaggagggaatgacgacgacccagaataggcgttcgtcagtttcgagtgcggtggctaagaggcaagcgatggtggctacttcatcgtcgttggagaatcatcatgccggaaaattgaatgcaggagcgcccaagaaaagaccagcactatctaatatctcaaatcatacaactcggaactcgctctctcattcctccaaacttgtgagtatttctctttgtttttttgttctctgtttgaataaattgcatgtgtaccctttttttactctaggaagataattggggtttatggggttatcctttttttttaatctttctctgtgatttttttcctttgggttttttttattactggtttgatgattcactttttcgtatgttgtttatgtgatttcttgatcaaaatttgtattccaaggaaaatgcaggtgggttctgtgatttatttttggggtttttctttgttggattaaataagtactaaaatggttaatgttacgtggggtttcatgaaaaattgattgaagatactgggtaaaaataaatttgattaaaatcaagtgaagctatttgataggagaggatttgagggatttcgtttttttatcaagattttgatattaggaagttgttatcttggtttattgacttcccttataaaaatagttcactatttttagcaggaaatgcgtcagttatcaagggaactgaattgagttttgggtggagttttttctctttttgaaaagcttatgtttgagttagatattcttttattgtaaaaaaaagtattatggatggaaaatttgaaacatcttcccccaattcctgctttttgtttttttttttttttttttggctgtcactttgctttttgaacatttgaaagttctaatgtttatgttattaggctaaagaaaagtttttgctttttcaaattggatatatcattggacaatcatgaagtggaccagtggcattctagattatagttgtcagctttaacatgaatttgtttaaatgattttactactgttcttaattttgttaaggacaaaatttgtttttacacaaatgagcagaagtcaagcaacttttgttaattgtgttttcacagttggatgaaccttgtatttaaattaataagctgttttgcactgtgagtaaattgaaagagattgtttcttgtatctgaagctgtgactaacttcaaattatttttggcattggaaggcaccatgtacatccaagattgtaagcattaagaagaacatttctacttgcaacagtaatgcagtttcctcggggactgctgttctgccagcatcctcctctatcagaccaagcagcaaaactgtttctaatcaaagaaatgatgcagttatacctaagatcactgcaattcctcttcctgccacttgcagtatggacatatctccaactcactcagacggatcattagtctccatggatgaatctatgtcaacttctgacacagtgagaagtccagaggtcgaatacatagatgaccatgaaacggctgcagttgattccattgagaagaagacgtgtagcaccctctacatctcagaaaatatcaaagcagcaggttttgatcttttcagcagagagtagtccttgttctagcatttcattttaactataagatctttttattcaatttatctattttttcttccagcagcagatatatgcaagagagatgtacttgtagacttggaatcaggggataaaattgtcaacattgacaacaatcttgttgacccacagttatgtgctacaatggcctgtgacatatacaaacacttgagagcctcggaggtataaaaatgtttaccttctatctcttttcagttatttgaattggatgctgctgctaattttttaaccaaattgcagtgtaactaacatttgctgccagttgtcaaatatgttttaatgttatctttggtcattgtaccaggcaaagaaacggccttccacagatttcatggcgaaagtacagaaagacataaatcctagcatgcgtgctatcttaattgactggcttgttgaggtaaacttctaccagtatctttcttctctaaagttgtgtccctcacagaatatcagcgtgctggaaattatgacttaacaaatttcgatgagctcagcaattcattagtttgatgtggaatttgtttgatgtataggttgccgaggagtacaggcttgtcccagacacattgtatctaacaattaactacattgatcgatatctttcgggtaatttgatggacaggcagcgactacagttgcttggagtagcttgcatgatgatagcatcgtaagaaactaccctctgacctttactgcatttgtttttgcaatgatatttataaaaatttccttgagtgcttttcatattcttacttcctcaaatattacaagcatatctgtaagaaaatgctccaagacattaattaatatgggaaatgctataatgctatattgcagcaaatatgaggagatctgtgcacctcaagtagaagagttctgctacataacagacaacacttacttcaaggaggaggtatatgatctttattcacagaacctgctgttgtcaaactttgcagtggcactaagaactatgtattattatgcaggtcttgcaaatggagtctgctattttaaattacttgaagtttgaaatgacagctccaacggtcaaatgttttctgaggtaatatcttacccttatctagtagttgcttttaagtatatgatgatttaagaaacttattgttgagatatactgcaggaggtttgttcgtgctgctcaaggacttaatgaggtaacctctacattcaaagttgattattctccaacatattttatacaggaaacagagttgataaactttttataatcatctacaggttctgtcactgcagttagaacacttggctagctacatcgcagaactctcccttttagaatacgacatgctttgttatgctccatcactcattgctgcttctgcaattttcttggccaaatatattcttctccctgcaatgaaaccttgggtatgtatgaattagcattgtgacaatcatacaaacggttgtaatgtattttcccttcttattctccttttcacaaatatattcttataaaatttgacttttggaaactcctaatacagaactctaccttgaggcattatactcagtatgaaccctctgatttacgcgactgtgtcatggcactacatagcctttgctgcaacaataaaaattctagcttaccagcagtcagggaaaaatacagccaacacaaggtaaacatcttctgaatcttcttgtataaatgatcaaccttctgaaggaatcccctggggacaaatgaccatccttctcaacactaatcaaatcatgttaactgaatagacatttatgtttatgtacataggcatccgagtttattttaatgtttggttttttgaaacagtacaaatttgttgcaaagaagtattgccctccaactatacctgtagagttcttccagaacacaagctgctaagccagggagacatgagaagaggcatcaacttcagttttccaattgttggttggactaattcatgtcatttgaacgcgaaggaatacaatctaatagtcataaacttgcagtgtcccaggaagagttcattcttggttcttctcccctcgtgcggccttagcagagtatcttcatttgtagtcattagcattgacattgcaggattagttttgtactctactgttcttctctagtttagttgcttctaagtttgtgtacagaagaagagcaagctgttggctgcttcatttaactcggaaactattcagtgataattccttttgtgccaactgttcaaagtcatcatttttcgtcgtcatatgagcaactggtacaactcaacttagagctgtacagaagttgggtgaaaagaaaagttaagcattgtgattgtatattttacatctattaatttactcttaattaatatcgatcaaggattcaaccaaccatatatacattgataatgctaaaaatattttacaccgtcagcatagacgttaagttgtatcaacagatacattgttattctatgatataacatataaaacaaaaataccagccccataatacaagctcattgagcacactctatcttagtagaacctaagccgaaggatgcatccattacactggcattaggcctaatattcagccagtgacaatcttcaaaagagcagggggttccaccattaggccattccacatccacaggttttatgaacgttgggccccaagcgggggttccatcctcatatgaattgtgggttaatcttcggatgtccgagccatctgttttgatcacatatatatcaccatatggctgataatgatgagggtttgatatgggctcagctgataccgcggcgtaatctgaagtgaacacgatatacttcccatccgggctgaaatacgggtggttagtccttccacccgtaccactctgtatcagcttcttgat

SEQ ID NO: 62 - DNA, 1482 bp, Solanum melongena
  source 1..1482: mol_type = other DNA
atgacgacgacccagaataggcgttcgtcagtttcgagtgcggtggctaagaggcaagcgatggtggctacttcatcgtcgttggagaatcatcatgccggaaaattgaatgcaggagcgcccaagaaaagaccagcactatctaatatctcaaatcatacaactcggaactcgctctctcattcctccaaacttgcaccatgtacatccaagattgtaagcattaagaagaacatttctacttgcaacagtaatgcagtttcctcggggactgctgttctgccagcatcctcctctatcagaccaagcagcaaaactgtttctaatcaaagaaatgatgcagttatacctaagatcactgcaattcctcttcctgccacttgcagtatggacatatctccaactcactcagacggatcattagtctccatggatgaatctatgtcaacttctgacacagtgagaagtccagaggtcgaatacatagatgaccatgaaacggctgcagttgattccattgagaagaagacgtgtagcaccctctacatctcagaaaatatcaaagcagcagcagcagatatatgcaagagagatgtacttgtagacttggaatcaggggataaaattgtcaacattgacaacaatcttgttgacccacagttatgtgctacaatggcctgtgacatatacaaacacttgagagcctcggaggcaaagaaacggccttccacagatttcatggcgaaagtacagaaagacataaatcctagcatgcgtgctatcttaattgactggcttgttgaggttgccgaggagtacaggcttgtcccagacacattgtatctaacaattaactacattgatcgatatctttcgggtaatttgatggacaggcagcgactacagttgcttggagtagcttgcatgatgatagcatccaaatatgaggagatctgtgcacctcaagtagaagagttctgctacataacagacaacacttacttcaaggaggaggtcttgcaaatggagtctgctattttaaattacttgaagtttgaaatgacagctccaacggtcaaatgttttctgaggaggtttgttcgtgctgctcaaggacttaatgaggttctgtcactgcagttagaacacttggctagctacatcgcagaactctcccttttagaatacgacatgctttgttatgctccatcactcattgctgcttctgcaattttcttggccaaatatattcttctccctgcaatgaaaccttggaactctaccttgaggcattatactcagtatgaaccctctgatttacgcgactgtgtcatggcactacatagcctttgctgcaacaataaaaattctagcttaccagcagtcagggaaaaatacagccaacacaagtacaaatttgttgcaaagaagtattgccctccaactatacctgtagagttcttccagaacacaagctgctaa

SEQ ID NO: 63 - protein, 493 aa, Solanum melongena
MTTTQNRRSSVSSAVAKRQAMVATSSSLENHHAGKLNAGAPKKRPALSNISNHTTRNSLSHSSKLAPCTSKIVSIKKNISTCNSNAVSSGTAVLPASSSIRPSSKTVSNQRNDAVIPKITAIPLPATCSMDISPTHSDGSLVSMDESMSTSDTVRSPEVEYIDDHETAAVDSIEKKTCSTLYISENIKAAAADICKRDVLVDLESGDKIVNIDNNLVDPQLCATMACDIYKHLRASEAKKRPSTDFMAKVQKDINPSMRAILIDWLVEVAEEYRLVPDTLYLTINYIDRYLSGNLMDRQRLQLLGVACMMIASKYEEICAPQVEEFCYITDNTYFKEEVLQMESAILNYLKFEMTAPTVKCFLRRFVRAAQGLNEVLSLQLEHLASYIAELSLLEYDMLCYAPSLIAASAIFLAKYILLPAMKPWNSTLRHYTQYEPSDLRDCVMALHSLCCNNKNSSLPAVREKYSQHKYKFVAKKYCPPTIPVEFFQNTSC

SEQ ID NO: 64 - DNA, 4591 bp, Solanum melongena
  source 1..4591: mol_type = genomic DNA
acttcttttttttgaatttcgaaaaaaaatggccttttcaaattctgttttaaagtgggaaataggaatgaatttatgatgtttttatctacaattatttctaaagaaatctttaatactctccgaattcattattccaaaaataaatttttatttcgtatcaattaatattatttataaaatacttatattaaatccgttctcattgtttaaccaaggaagagatcaattattggtctatattaagtgaattttaaaacataaattaaatgttcattttcagtacttatgcttaaactatatattctgctagaaaatataatttagttgagaacattactaaaaagaaggataaaaatcgggaaaaagaagtctaaatttatatttttatatcatgatattttataagttttggggaaatttttataaatagcctaagtttaaaacttaatatggtcaaatagctagaggggggcatgattgagagagggggagagaaacgaaattgtatatgtatatttgtcaaactgactatgtatatctgtcaaaataattgtatatatgaagctggtatacatatgtaattatatatccgacaaaaaattgcaaagagagaggcgagagaggagagagaaaatagcaacaaatctctaactataacaataaaactctaactataaattataatttttttcaaactataattatataatataaatacatatatcatatgtttgcctagtcatgttattttttctaagtttaaccacttccttaaagttcgacttttggcgacaaaaattaaagattcaactcatttaaacgacaaaaaatgcagaattaaatccactcaaatttgtcccattgccggccccaattttgcttatcatagcccaagtaaaatgttataaattcagcccatatccaaaagtgggccgaatcaaaccccatataaatactcaccctccgaattcttgcagatttaccgccatttgaagctatgggagaattctgcagatcaaccattttcttctccgatcaactcctctcctacgccgaaatccttcctccttcacaggtaaatctccgtcactgaagtattcgcagatttgtagcagtgtaaaatgtgtgaatcgcttcatttagaagttcaattaaatcggatgcatagtttttttgcaatatccagaataatttgtctcagtgaaaagttgaagtgttagattcaaaattcaaatgaacaattgatgaaccacaaattaactgttaacattaaaaaaaaaaaaaaaacatatctatagctaagtcttaatacccaaaatatcttaaagccctaagttcgaactctccgtcaatttccgatctatcactggttcgaaattttacctcatcatcttttcaaaaaggaattctactataatttgcacttttagcctacttcaaatgcttgctgtaagcttcgaaatgaaatccaaaaaagttgataaatccattgtgtttatgctctcttaattgttcagaataatacaaatttggatatcacaattttaggagatttatgtgtgaacctctcggtcgcctcaaagaacaaatgatttaccgttattgggatatattatgcttgaacataaatcgatatagatgattcatatagtagacgccaactagaggcatttgatagtttctatatatgacatatgtgagacagatcagtaggaactccagcaatagtagagtgagccgggggctacttaccggtgattcatggatcttcctatcccattctttttgcacgcgatctttaaccagagagaatagtgccaaatcatttataagaggtaaaaggctacaagcttcttaccatcagattacttattggacaaattcatatttaataatgttgggaatgtttttgtgatcaagtttggaaggttatggagatgtgctacaagattctggttcaggaaaagagggtgacacagagagagctatactacaagctgctctgtgattcaccagattatttcacttctcaattgcaggttaatagaactatccaaggtcattgttgtttctcctttcttcatcacttctgaataatgatctgtgcgtttggttggttttgttaacgggatctcatttaaattctatgaagaacagatttggtatccctgcttcgatgcagccgttatagccttggaataatggcatcaagcagaggggcaatagctggccgtttactgttgcaggtactagtcttaatcctttagttgtaataacaggtgtttataatgtgaagcagtattagtagcttgacttggctagtaacatgatcagtcatatatatggaatgaaataggccctgtacaacaaatggatatagagaattcatatagccatctcaagtagtttataattgaggcacaactgattgactgatttcaatatgagagccaacccagtcaaacttttaatgtttctaagttcctatagttggtaaaattaactgctagtagccgtctatgatcaactactctacttgtggatcttcaggttatgctaaaaactcaagagaactggaatacttggaaaaattaacaagtcgaaacagatgcacaattaaagcatgatcagggatttgaaataggaattttatccaacatgttagaaacttggtatttcaatcacccaaaaagaaactaaaactagttccacattttagcatgctatattccagagactagctgaggatcgtgtgttcaataaaatcccatgcattctgatcaccgccaagggattccctgatatagccactaggtgaggtgaatagttagacctcctttattccgacgttccagttcatagaatagctgctaaaagattgtccattctcttattaactcaacatattctgctctctaaaatcttattcaggtttctgcttcatcgaatgtgtcaaacattccctaatttcccagtcttggggctggttgactggtataaatgatttcactagtattgccaccacatagttgcagagcaaagttcttacaaatcaaattgtgacttttaaggaatccagctggattagcaattctttgcaccttcaagtttggaagcatagggatgggacttgaagcatatagatatggtgctcttttctcgtaaaacttatgtttgaatcatgtccttgttatcttaacttcacttataggagtcttttaccttacatgtttttttaagcttgcaacgtcaagtggctagggctgcgtaaggatgatacttatcaacttatacctgaagaatgtttggtccctttgaaacctcgagatctccagattgccaagagcttgatgtcatcagagattctgcaggtatgattacatttgttatgggaacgtcattctttcttcatggttggtttggaaaaccataagatcactgatttttaccaggatagctacaaagaagaggtggcagcaatggttcagagtggtcgaagggcagagattgaagctctttattgtcatggatatgattacttggtgaagttccttgcgacaaaaaatagtacaagccaattacctctgaaattcactccctcattgaatacaagtactcagaaaatattgcatttaaaagaattgaatgatatgcggacgatgcaggaagtgtagaatttaaaaatcagtttgtactagaaattgaatccattacgcgtttcttatgcagtagtgtgctattctcctgccgccctcttgtatttactctgtagcctgaaccaaacactaacaaggcttattcacccaaaaataccagggtgccttgtacagagaaaacctatgattagagcatacaaatgaagtttgcctcgacgacaagtagggtggaagatgcaatccccaacttaacaaagcaaattctcaaagcaacccaacaatcctgaaaagaaactgaacacatccagactaatattatgattttgaggcaacttacagttcacagggtccgtactgattggttgatcctgcaaggtagttcccacaatcaaccatatgtcgagttgactaactggatactcaataataaaggaaaaaattttggccattcggctggggaaagaggggttgaaacctgctcatcccatctgtgcaataacaaattatgtgtaacaccaaataattgtgcatctgttcataagacaacttatactgacctctattccttggcctataagagagatacaacaacaacaacatacccagtggaatcccacaagtggggtctggggagggtaggatgtacgcagaccttaccactacctaagtagagaggctgtttcctgggaaccctcatctcaaaaacccatccgcagaatgacctagatatgatcaaaagtaaaagtcaaaaggtaaagaaaactcaaaaatttggataactcaaaatttagggttaaagaagaatacaatctaaacataagagacatatcaacccgaaaaaaaaaaaaaaaaaaagagaaccagggcagatcactaggtgaagacacgactgcctaatgttgtaatcccaaaaatgcaatgctgtgctcctt

SEQ ID NO: 65 - DNA, 1215 bp, Solanum melongena
  source 1..1215: mol_type = other DNA
atgggagaattctgcagatcaaccattttcttctccgatcaactcctctcctacgccgaaatccttcctccttcacaggtccgagctcgaattgaagttgcagtcctgaattttcttaaagccctaagttcgaactctccgtcaatttccgatctatcactggttatggagatgtgctacaagattctggttcaggaaaagagggtgacacagagagagctatactacaagctgctctgtgattcaccagattatttcacttctcaattgcaggttaatagaactatccaagatttggtatccctgcttcgatgcagccgttatagccttggaataatggcatcaagcagaggggcaatagctggccgtttactgttgcaggttatggagatgtgctacaagattctggttcaggaaaagagggtgacacagagagagctatactacaagctgctctgtgattcaccagattatttcacttctcaattgcaggttaatagaactatccaagatttggtatccctgcttcgatgcagccgttatagccttggaataatggcatcaagcagaggggcaatagctggccgtttactgttgcaggagccagacagggaagttattgactgctctacttgtggatcttctggttatgctatatcaggagacctggaattgttggaaaaattaaccatggaaacagatgcacgatatatcattatagtggaaaagagactagctgaggatcgtgtgttcaataaaatcccatgcattctgatcaccgccaagggattccctgatatagccactaggtttctgcttcatcgaatgtgtcaaacattccctaatttcccagtcttggggctggttgactggaatccagctggattagcaattctttgcaccttcaagtttggaagcatagggatgggacttgaagcatatagatatgcttgcaacgtcaagtggctagggctgcgtaaggatgatacttatcaacttatacctgaagaatgtttggtccctttgaaacctcgagatctccagattgccaagagcttgatgtcatcagagattctgcaggatagctacaaagaagaggtggcagcaatggttcagagtggtcgaagggcagagattgaagctctttattgtcatggatatgattacttggtgaagttccttgcgacaaaaatagtacaagccaattacctctga

SEQ ID NO: 66 - protein, 404 aa, Solanum melongena
MGEFCRSTIFFSDQLLSYAEILPPSQVRARIEVAVLNFLKALSSNSPSISDLSLVMEMCYKILVQEKRVTQRELYYKLLCDSPDYFTSQLQVNRTIQDLVSLLRCSRYSLGIMASSRGAIAGRLLLQVMEMCYKILVQEKRVTQRELYYKLLCDSPDYFTSQLQVNRTIQDLVSLLRCSRYSLGIMASSRGAIAGRLLLQEPDREVIDCSTCGSSGYAISGDLELLEKLTMETDARYIIIVEKRLAEDRVFNKIPCILITAKGFPDIATRFLLHRMCQTFPNFPVLGLVDWNPAGLAILCTFKFGSIGMGLEAYRYACNVKWLGLRKDDTYQLIPEECLVPLKPRDLQIAKSLMSSEILQDSYKEEVAAMVQSGRRAEIEALYCHGYDYLVKFLATKIVQANYL

SEQ ID NO: 67 - DNA, 7525 bp, Solanum melongena
  source 1..7525: mol_type = genomic DNA
aaatgccaactaataagaaaagcagtaatccatagaaagtacagtaacagtaataaaataatgcggcaactgaaaaccagaagacaataggtggtaacagtgatcaaaaacaagaaattacatgtataagactaatactacgtcatacacggtgcgtccagactccaatcaagcctaataccaccgaaaagcaagacaaaactcaactacctactaaacttctaccctaatccacgacctccatacccttgtgtccttggtagttgaaattgtgtcaagtcccgtctaatcacatttcccaatacttgtttagcttacttctatctttcatcgtgtccactatatccaacgtctcatacctcctcattggggcatgtaaaccttttctcttcacatacccaaaccatctcaacctcgtttctctcgtcttgttcaccatggaggccactccaaccttgtgttggatatcctcatttataatcttatctttcctaatatgcccacacatctatgttagcatcttcatttttgcaacttgcaccttctgaacatcataaattgggatcagttgttcactaaaaatgtctcattgctaattctgcaccgagtcctaactaatcacgtcttgaatgatacagttccttaacctttagcttttaatgaatagaatacatgttcacctgtaaaatcttctgaaaggatctatccacaggggaattgatgcagtttgacaattcatgaactttatgttgttatccaacttaagaaattccaatcaagctcacacaacttgtcatttagcttagggtcatcattatctaccagtaataaactgttggtattgtttcggaagaatggtttttgaatagaattatctttcataatggcaggtttatataattcacatatataacatattttttactttgacacttacataacgttggaagtactcctatatctcatagggttgagaatatttggtagtttaaactgagggatgaaagttgcaggcatttgtgatagtgagatacacaatttaaatgtaaatctaaaagaatctaattctgctgggagactgacaaagctaccctcgactgcaaagaatggtgccaaattcaggtatgccattttcaggggctccaactatatgatgctactcttaaattagttttctcttgactgtgcccatctagtctttcccccctttctatgattctgtctttctgcacatggttaattagttataccttgcagtgggactgaagtatcagtatcaatatccaagagccttgatgacttattggcagaggttacttgctttcttcaaaaggttcaattttcatgtctatcagctgaagctagctatgatttcctacattatatgaaatttctattaactacagtttttcatggctgtttccgcagatgatccctctgaagattccagttagtttgttacttctcttgaaatgctttatattcaaatcaaatgcagctatctcctctatagactcttctcatagttcaaacgtgacttggttggttgatttagatgatagctactaactgctcagacagctcaagatgttcactatataggatacaatatcaacgacggacctactaaatctaagtgtttatcttttggatgggttcaccatttcaaaaatatttctgtcaatatcagattcgcattaagatttttgaaaattttaagattttatatgtcattttaaccaaattctttggccttatatattaaaaagttatcttttgacttatcctctttcctagaaaataggtaggatcccaggaccactacctctctttggctgatagtttgtttttcatcttacagaaaattgtaatggaactcttagtatgtgatgaggaccttttgggagcacagattgaaaatcacattttggcaattgagggaagctctgtatattctcctgttgaaagcatagaatgcttgaaagtgggactcaaggattatatttgtaagcaccaaacttgcttcttgactgggtgagtactataaaggtgctaagtgatggctaataaatgatccgttccaacatctactttctgttgaaagatagatatattgtgttaataggtcttacttccgcatgttgaaatcatatatcttaggtgcgactatacaaagataacgaagagtgcttagcaatgctatttcttgcttcttgattgtacattttgacagtttccctgacctttatcatttctttgctttacttggatttttgcatctagtaacttagtgttgggcctttcattctgcagttttcccattaaaaagtgtaattgctgttcttgtgtggtttgtctatatgtctgactgttcattaaggtacttcagtttgatgtcaagcagtgcatcatttttctgaaatgtataatttgtaggttttatcttctcaaaatactggtctcgaaaaatagtttagattgaatgaagatggaaaaaagaagctagggatgcactggatcaggtgagagaaaatcaggatcaaacataaaaaaggaatgcctgagctcccgctatagaatcacacatagcatgcaagaagtagcaactcaaactcaagtcttatatgatctggttgacagttcatttgactcctcctatattttgatgtaggataatttaaatttgctagcacttttcaattaagatctataggtagcactaaactagaaattgtgacggctcatctggtagttataaaattgcaacatctcatataagatttttgcagagtcaactgttttgcgaagcctaaaacaaaaaaaatcaatgtgcagtgcattgaaacaagtttttaggtaaagttgtagattcttatttcagggaaaatctgaaggttggaactggggttgctaactcttcaggtagttctcggggcgatagccaagtggtggaagctgtggtgattatcagtgagatgtcagaacaagtcccttcttcctgcatcagggaacaagacatgaaaacagaggtttgctttggattattaattgaagaaagctcttaaaaccataaaagaatgtttgccttccaatatgtgctttattaattatgttttgaccatatgtagattatagttcactgtatagatgttttgttgcatattctttcccaacttctatctacttgtattttgagttcatttgttgtcctagaatgtgtggattatgaaagctactactaatatccctgatatgcattatttaattgggatttcaacttttagggttattttatcattataatgaatctcttgtttttatatgaaccatggagcacaaggtgaagaacctcgtgcactcgatggtgtatggaggctacgacgtatgcatctacccctacatcaggagtaagctatttatgagagtaatgactgaaaatatttttgaatttttgagggccagtaagtggacctttttctttatggccatcttgatgacattggattggataggttacattacatacacaagagctatgtctcaattccaagcaagttggggttgataatataatcctcaatgaccctgtggctccatttatgttcatagataagattacatatcaggaaacaaaattctatgtggaaagtgtaattttcatattgtaataaaaaataaagtattttctaaaatctagagtatccccattgtacgccaagcaggatacaataattatctgatcttatctatgtaaagaaatatggtctctggtattgcgtctaattaagtattgctttataaactttgaggatatcaaaagcttatgccaagtgaatcgttcatgttatcagttggttgtcccaggtatttctagtacaattgtttcttcatagtctggacatatgttggaagctcaacataaccaagacatgtttaaaggcgctctttgtgccttagcatcaatctggagttgtcatatggtatcaagaagatgtttggtctgctaaaatcgtagctttggttgaaatcccactatcagttaagctcacagaaaaggtgtatgaacatatgagcattccaatatgaatcctcacttattcactaaccttaacctattcctttcttccatgtcttgattcttaggttagcaaggccagttttgtccatgatatgaactcctcttactgcttgagagagctccttagcagatacaaaaattctgtaagattgtttggtagctccaaactcagccagcccatcttccatagtattaacctctataacattgagttgcccttcctttcatgcttgttaaatgattctggattctggatttccactcagtcagctttcaagatggtttaccgaggccattgatcatatgaactattattttagagttcatctccagtagaacattagcaattgcattatttgcaagccagtgctagctgcaatagccttggcagcattactagaactagaaggaagagcctctgagaaggccatgatgattttgccctgatgacctcttagaaccacaaccaccttttctccagctaggttcccttataatgttgaactgccatagcgttgagtttgatataattttgactaggcttgttccagcagacaattgatacaagtgagctttggcttaaagttatccactaatcacaaacctcccccctgttggagtttatttaagttaatcaatccaaaatcttttgaaatggcaacttgaggttatcaaaatattttgaccatttttaaaaaaattaagttccctgtatctttgatgaggtgctgttgaagatttttaaaatcgtctctgagcattacttactcgtcttctttaagttaagccagtatgttgcttgccttcactttcttttcagtattactgtttttttgtgtttctttaattggtattaatggttttctatgccttattccagatcttatatttcaaagattttgtaccctgttctattgctcagtcatccctcgatgcattgacaagtatcaactggaaaagctatgggttggatctgcggagtgtttcagatcatgatggttgtgtaatgctggaatgggagaacctgccaccagatttccaaattcatattgccatccattgttaccatagtcaatatccatcataacctaatacatatccatgataattgacatgatcatacaatcttagcattaacttcaaacaatgagaaattgcatgtgtgttttgcttaacttgctgacaaggtgaaacagtgggttgcagaaaacagcttacctgatcgaaatcttgctagaaaagccgtcaagtgtgctttggatgaattgaaggaaaataatcaaggggttctcctaagtacacgtgcacttaaggtgaaattttctcacccttctttgcattctatctggtcattggattttctagttcctggtattggcttagctatgaacaaaatactccccccattgtttgatctattctgcattcttatacgtccatagccaaacatgaagcagcaaaagtagtttgtattttgttttcctgttgatacggattgttaaagattggtcgctaagcagatagcattcagtaattccagctggctaggtagttcacacatagaaactagtcatgcattggactttacattctttaagcaccatctgaagttctatatgactagtgctgattggatctgacaagggatgacagttattcaaacgcaaacaagaacagtaggttggcgagaaatctactctcattgcctcattggagatgaaagcttcctagaaaattttcttctttttactgggagtggctttttgcactgctgttccagcttttgtcagatatagcatttttattggctggaagtgcacatgctttcatatgtttctgcagacctttaaattcagtacctatattcatggtcaggggagtgtaagtatggcagtagctgatgttctggcaccctctaagccagacagttgctatatattcaaatagtttgtatctgggtatatataaattaatccactgctacaatttagcactagacgcaatcggattccacatgcaccaatttaaaatctcgatacactctctagctgaatatgatatttctttgagcttgaaatggcagaatttcagtttgcttttacatatatagctaattaaggttctatttttttctctcacagacgtgtgtttatgcacctgaccttgctaaaacgcttgctcgcctaatcttttcctccaatgacttaaacttccaagaagaatgttgttctcttctcgggatacagtctcaagaggttgacacagatagtgttggaaattgcatcagggagaagataatttcagtcatcagattaaatgatcgtagctcccaaaagcataaagaagcaccaaccttcctctttgaagatgattattatcagaaagaggatttcatggacgaggaatatcaagaaggtgaagaagcttacaactctttggatctgtagaaggctaggagccgtgttagatgtccaactattattttcttattatgtttatgattttatctcacaatcaaactatcctagttacttccgttaggttttgttattgctatagaagggtaaatggattaatcattttgggggaaacaatctgtatgaacttgatggtattccaatatatcagacaattatttcgttttcctcgaattacttgagaaaacaactagaaattacataatgttactatttcctcacaccaaaattagttttcttactatagcgcctagcttaatgggaatggctagtaacgatcagaatttctatattgacagcaaattatacaaacgaatttgtatattggaagcaaactacttatcttgtttgtatattggcaacaaattatacaaatggattttgtacattcgcagcaaactacttatcttgtttgtatactattagcgaattatacaaacagatttgttatatcgacaacgaactacttaccctatttgtatattgccaaagaattacacaaataaatttgtatattggtaacgaattatacaaacagaaatacttataccaaacgaaagtatggctacaacaacaacaacatacccagtgaaacctacagggtctgcggagagcaaagtatactcagactttaccactacctcagagagatagagaagttgtttccaaaagattctcggctcaaatgtatttgccccaaataaaagaaaaaaattagatacagaataactattaaaacgaagagaaatgtcaattctacaaagaaaaaaaaagaataaaagtagcaaaataatcgaagagcaataacaagacaatcataatagcatgaccaattctatgataaacctaaaaccgtcacaaggcaatacaacattctaccctaatacatgttctccaatcctttcaatccaaggcacatcctcgatgaaatgaagttgcatcatatcctgtctaattatttctcccaata

SEQ ID NO: 68 - DNA, 1368 bp, Solanum melongena
  source 1..1368: mol_type = other DNA
atgaaagttgcaggcatttgtgatagtgagatacacaatttaaatgtaaatctaaaagaatctaattctgctgggagactgacaaagctaccctcgactgcaaagaatggtgccaaattcagtgggactgaagtatcagtatcaatatccaagagccttgatgacttattggcagaggttacttgctttcttcaaaagatgatccctctgaagattccagttagtttgttacttctcttgaaatgctttatattcaaatcaaatgcagctatctcctctatagactcttctcatagttcaaacaaaattgtaatggaactcttagtatgtgatgaggaccttttgggagcacagattgaaaatcacattttggcaattgagggaagctctgtatattctcctgttgaaagcatagaatgcttgaaagtgggactcaaggattatatttttttcccattaaaaagtgtaattgctgttcttgtgtggtttgtctatatgtctgactgttcattaagggaaaatctgaaggttggaactggggttgctaactcttcaggtagttctcggggcgatagccaagtggtggaagctgtggtgattatcagtgagatgtcagaacaagtcccttcttcctgcatcagggaacaagacatgaaaacagagcatcaatctggagttgtcatatggtatcaagaagatgtttggtctgctaaaatcgtagctttggttgaaatcccactatcagttagcaaggccagttttgtccatgatatgaactcctcttactgcttgagagagctccttagcagatacaaaaattctatcttatatttcaaagattttgtaccctgttctattgctcagtcatccctcgatgcattgacaagtatcaactggaaaagctatgggttggatctgcggagtgtttcagatcatgatggttgttgggttgcagaaaacagcttacctgatcgaaatcttgctagaaaagccgtcaagtgtgctttggatgaattgaaggaaaataatcaaggggttctcctaagtacacgtgcacttaagacgtgtgtttatgcacctgaccttgctaaaacgcttgctcgcctaatcttttcctccaatgacttaaacttccaagaagaatgttgttctcttctcgggatacagtctcaagaggttgacacagatagtgttggaaattgcatcagggagaagataatttcagtcatcagattaaatgatcgtagctcccaaaagcataaagaagcaccaaccttcctctttgaagatgattattatcagaaagaggatttcatggacgaggaatatcaagaaggtgaagaagcttacaactctttggatctgtag

SEQ ID NO: 69 - protein, 455 aa, Solanum melongena
MKVAGICDSEIHNLNVNLKESNSAGRLTKLPSTAKNGAKFSGTEVSVSISKSLDDLLAEVTCFLQKMIPLKIPVSLLLLLKCFIFKSNAAISSIDSSHSSNKIVMELLVCDEDLLGAQIENHILAIEGSSVYSPVESIECLKVGLKDYIFFPLKSVIAVLVWFVYMSDCSLRENLKVGTGVANSSGSSRGDSQVVEAVVIISEMSEQVPSSCIREQDMKTEHQSGVVIWYQEDVWSAKIVALVEIPLSVSKASFVHDMNSSYCLRELLSRYKNSILYFKDFVPCSIAQSSLDALTSINWKSYGLDLRSVSDHDGCWVAENSLPDRNLARKAVKCALDELKENNQGVLLSTRALKTCVYAPDLAKTLARLIFSSNDLNFQEECCSLLGIQSQEVDTDSVGNCIREKIISVIRLNDRSSQKHKEAPTFLFEDDYYQKEDFMDEEYQEGEEAYNSLDL

SEQ ID NO: 70 - DNA, 8393 bp, Solanum melongena
  source 1..8393: mol_type = genomic DNA
tgttcaactagagaaggtcccttggaacaggcattggtgatggtggtatttactaatgatagcaaaggaacactaaggattatggtttttgaagcttcaaccatcacatgatttactgagtggtgcaaaaccatagacagaatggcaattgatataagagttcctggtgtccatccatctgcagctactgagggaattaggtaatcgattatctgcaattaagggaaaagtctatttactacagagcaactggaagcaaacagtattcagaagagtgagtacattactttcaccacaactgcaacccagggttcatcatctgagagggattcagagtgtacggcttgaagaatgcaggatactagtttggagatggccatgaaagtatctggggctgaagaatgaccaaacttatagtacaggttcttaattgcaccagcaatcccgtggatgcaaaactgatctgaagcacttggtgatatctctattatatgttttatggtattcaccactgaaataatgtcatactcggaatgttgttctccagcttctcccaacttgatgtggcttcatgcctaacaaatgaatgacccttctatttatactacttcctaggagccaatgtgtaaataatatttacactataagtccctatatatttacaacttagtccctctctggattcttccacacaagtctagagaggaccaatgcctacaagacacttcctaacattctaccactctctgaaacctttcaagcctctctagtcttctcttcaatcttctacatgattctagagagttccggagccttccggagtcttccagagccttccggaacatgctgaacacgttcttgcactattttggctcaaaactgtggcaggagcaggacgtgtcagtaaggagttttatttttctcccgccctttcaaaattttacaccttctatcgcattcgccggtcacttcgctcacgtaaacagtacagcaacaaaatatgtatttcgccacctctcacctccaccatttaccaccgtcatcacctccggaaccaccgttaacatgtgcccaaggtcatagctcgactttgattattccaactgatgaaggcggatcaatttgtctgctctgcttgtccaatctcgtttctaatccgagatcgccgaccgttcacgtttcctatgctctctcccagttatctatcgcgctttctcaaccgaggtttcgccaaaccttcttcacattccactctcatttcctaatctcgcctctcgtcggtattctatcgtccttcgatgatgagccaatcgccaagcaaactatagatttgattatgcagttgtgtgaagctccagactgcgatgtgcatgcagagtttgtggctcggctcgcagatcgtctttccagtggcgctttagcttggagtcagagacagctccacacggtaaccctttccctctgtcctaatttgtaaatttccgatttctggaagtgtaattgaaaacggagctgtagaaaggtgtagctacagcacagagatacagccatacatgatacgacatatactactacaatgaagtgatttataaatttgcacaggaagtgtgtcactctaaaatggactaataaggaaataaaaatgaagctgagtaagtatctggttttccgaatttcctcagtgtgcttcagtattatgcaactttgtgtggtgacggacagccggctgtgatcagtaaagcttttggttggaacctttcaattgcagtgagtccatcaaattgaccaacagcagaagtttaagcttagccactgttgcagattggattggaaaattagagtcagaatgattccaaagcatattagttttagccagagcggctagtagaaagctaaaacctgcttgggtagttatttcaaggttcaatgtcagtgttcacgtccataagaagtttgttgtggaagaaaacacataaagatgttatgaaataagaaaataaaagatgggaggaactataaatgattttgaaacttgtgaaaaatgttgcataaaaaatggcacaaaatatatgtttccgcatgataactcacaaccttttcagagtagcttcacactctattcggtgcttgcctgctgctgccctatatgggccaattgcccattttagagaattactctttgtatgtgattaatttcttcattgagaagctagaatgaaccagaaagaggaagaaggacactaagtgtttctgtcttggagttatttgcctgatatcagtccaaaacacattggattttagtgagataactcagcctttagtttgcacagagaatttgtagtttctacgtttgcagtgacatatgttttcctctaatatgtgtaatctgaccttctgttctctctcaaaaaaaaaaaagcttcattgcttaggtcttctcttggattatcaaaaaaaccattcctattgtcttgaagaaacagatgccctcattttcaatctcgtcagtggccttcaattgtccaggtgactcttgaaattgagatagcggctatcttatttttgccttaaattaagcccgagggccaattccttcttgagtacagtgaagatattcaaggggaaatcctgtttgttctatacaaattattcctactcaatgtgtctcaagacggggatgatgctcccagtttatttggccattcctcgaagctcctacacttggcactggcagttctcatgaaagctcaaagtgatgatgttcgcttgaactgtataggtaagtttctttaacattactcgtttaccagtttctgctgcttgaaccttagtatctctgaaattggttttccagtgaatatgttgacagttaacaattttgttcctggattattgcaaagaggagtatatggtaataatatctgacttattttttattctatctgagaagtgaactagtgatgtatggttgataaaaagcgagaacacattataggaatagccatatacctccctgagagatcatttgaagctggagattttgtggctcgtaagcctaatgttgtggtaaacaggctccacaaacaactaattgttggttgttaattctgttttcacactttgaatataatctgactgataaatggttttgcatgtatatttgctactgacttgactagcaaagttctatgcactcttcaccagacctctgataatctctctcttctggcttctaacctaccttctcccctcccttccttaaccattcccataaggaaaaggaaaaatagaaaaaacaaacacaacagaacaaccagcttctgatgttagagtttctgcaagataatctcctctcacatttgtcaaattagatactcatcgtctatgcagcattcttaacagtaataacacaacgaggaatgttagagtttctgcaagacaatctccttgctcacatttgtccaattagatactctttgtctatgcagcattcttaacagtaatactgcaaagaggattctttcaagctacttctataattggcacaaggagcaggagttcttatgatgttgaccacttgatggaaacaaatgagcagatatcagatagacctctagctatcttgtttgcagaggcagtcaaaggccccctgctttcttctgataatcaagttcaaatagcagcactagatttactttacctttatctgtcagggaaacatgtcttagaaaatgaaatccaggtatttgttgaagagaacattgcagactatgcgtttgaagtgctgagattgtcaggtaagaaagtcagcaatacacaatgcctgagcagttagacgtatatgtattagtttcatttgaagaaataaaagatgaagagggcatttcagtcgcactctaatttcatttgtttgtttttttacaactaaactatcttgaaatcgacctattctctggtgatcacagtgttttcctacgattaacaaattaccacggcttcaacctttgttgtccgtatggtttgacaagatctaagttctctaacgacaatgagctcgagaaattctaattattttacgtcagattatgcaattaatgttgtctgtaatgactaaagaagtaatttattaattttcaggatgcaaagatccaacaattaaatcttgtattcagcttcttgatattttagcaactgctgagcaagcatttagacagagacttgcgattgggttcatggccctgattccagttctgcatcatgttgctgaaattcctttccaccctgtacagactgagacactcaggcttatttggaactccgttgagaactgcccaggggtggtatccaagtctcaggtagaagaaataagcctttctttgacgaggatgctcaagaaaaatcttgacggagaaataggcatgcttccagagacattagctctggtctgttcaatatttgttgcacttatgaaatgttcatcttcctgtgagatttcaagtttcttactatcaattcaggatgcatcaagaacctgcatcttaacttgtttaattaattatggcaaatacccgggtcaacttttgaactctctttacctactgaaagaggcatattcatatagttgtgggatgcatccctcaagctcaatcaacacagaacttagaagaagcattatagatgtatgcaaaacacatgtattaccttggtttatgaaatcgctacatgaaatggaagatgaggatattccagctgcaatactcgaaaatttgtattccatattgctacaagattcagatactgaaaccaaaatatttgcaaatgttctgttcacgtcttcctggttcagttttgcatatggatgtttaggcttttttccttctgaaaagatgaaaaggaaggtttatcttatctttagtctgatggcagatatcatacttggggttgattctgcacgatgcataagcgatactgctccacatcttccatctgatcctatagatttgcttttccttctgggccataaaagctcccaaaatgttgaattgtcttctcgccaaatggcagttctgctgttactgtacatcagttcactgtatgacgatcggtaaatagtttctggaatctcaatcttactctttcagcatcttccttccttatgttatcagtcttcagttgatcatcacaaccttttccaggattgcagatgacaaacttgtgttagcttcactggagcaatatattctacttaacagcagtgaaaacatgcacggagcttctgttttgggaatatttataaatctttatgcactctacagaggtttagccaaggtgagctaccaaatcccctatagcccagaggcagaaaggattgtgttccacctacttgctgaaaaggactgggatttgctatctacaagaatccacataacatctttgaaatggttgttgcaacaagagaaaatctgcaatgtgttgtctgcccagattttgaaattctgcagatgcaattgctctgatgtaaaccagacaaatatccatggtgaagccaatcagaatatagatgtgtatgttatggcagaacttgtagcttcaggggacaactttttaagtatgctcatggtgttcttattgggagaagctggagaacaacattccgagtatgacattatttcagtggtgaataccataaaacatataatagagatatcaccaagtgcttcagatcagttttgcatccacgggattgctggtgcaattaagaacctgtactataagtttggtcattcttcagccccagatactttcatggccatctccaaactagtatcctgcattcttcaagccgtacactctgaatccctctcagatgatgaaccctgggttgcagttgtggtgaaagtaatgtactcactcttctgaatactgtttgcttccagttgctctgtagtaaatagacttttcccttaattgcagataatcgattacctaattccctcagtagctgcagatggatggacaccaggaactcttatatcaattgccattctgtctatggttttgcaccactcagtaaatcatgtgatggttgaagcttcaaaaaccataatccttagtgttcctttgctatcattagtaaataccaccatcaccaatgcctgttccaagggaccttctctagttgaacaagacgaaggaataagatctggagaagctcttgtttttgtgctttcactgcttttcttctctttgagaaggtagatccgttcctttaacacagtttccatgctttctttaattttggttttaatttagactaacagcttattttgctagcgtgcatgccattttaccagggattatggactgccaatatctgctggatcctatcaaaatctcacaaccctggccctatatcagtatacagtgccatgatttgtgcaagttattgcattttggatctattcctataaagttactaagctcgcaatacctgctagagttattcagcggaatagaagacgagagaattagaaaatcagacacattagaattcagaactaattatttgttgtctgtaatggctgttttagaaggccaaatattctcaagtgacaggtctgtagcaatgaactgttccctctgtttgtctatgctcattgggtggcaagatgtggaaacagaagtatcagctatacaaaggaacaactggtgtcggtttatagtagaagaattagtgatgtctttggcagcaccatctttggcttcaaaatctttcatgatccatcacaagcctgcaattcatattgcagttgaactgctgaaaagaaagaaaattcctcaatggatgacttcaatattcgatgaatcttgcatatttgccattactagaaacattacaaattataatttgagtgctgagctggtgttcctcttaaggaagttgcttaattatggttttctgaatgatgaacaaattgctactctaaatcaagtattccaggtattagatactttatctttgaaagttcattggttcctattgtgatctggcctctcaaagattgcttttattacaaagaaaatttgcaaagaaataaaagatgaaaagagaacattaccaaatttccctgcaaggatcatgatcaaagaagtttggctgcaggactgcagaaaatgtatctacacagacaaacttcaacatgctggggcagaggagatggcattgaacgtagcagccgcttcagattatgtaggtaaagttgggcagtttctcattagcctcataacgactcaatcatctggttgtatggagtctacaagatttcaaagtgggaaaagggagttgttggaagaaatagacttattttcaaaatgtctaatgagggataattgagactaaaattctaaaaagatctttatagcaatactttttggatagaagggcaagtatgtttttgcagaatgacaatcaattaagcaagcatggattttgctgatggatcatttcattctttcttaagagttaaatagactcttgcaccattaaagttaggtttggcagagtatcatatacgttctttaccgagaacaattcagatattttctgttttgtcactcataaactcaaagggcaatcacatctgctagtataatcctaaacctgtcaccaaaataaaattagaagtcttcagtgtcatcagccacatgcaaaccactgcctcagcaattctacttttgttcatcaagttgtacagattttcttcatcacttcatttcgtattccaaaagagggacaaagaaatttggggggaaaagctaacagttgacctccccaagttgaacagtaacagaggccctttctttcttatttgagaaacggttgggcctggaaggcccatcgttgtgacaaagcctgaactgggtcaacataagcccaagaccgtcagcccacacaatcctcccaagactcgactggtagcattagggaaagctaaataattgatgggaccatattacttctagtttctcccacggacgtaatagttcctctcgtctcagcactaaaattcccttgcatgaaaaagatagcccaccaataatataatatagttgtaataacctttcactatacatcttatcctaatttgtatatatactaaggccatagaaaattatcaaagagatggagagatgggaggacccccaccaactcgtcctcaaactcggggacccttccagtacttcgttgtataaaccacttatccgaatttctcgaggatagcgatgaatgcaatttgtcttctatttagaattatatgtcatatacaaatgaacaattataaatacagtgataatctacattcataaaaccaaaaagcacacaacatagaggt

SEQ ID NO: 71 - DNA, 4029 bp, Solanum melongena
  source 1..4029: mol_type = other DNA
atgtatttcgccacctctcacctccaccatttaccaccgtcatcacctccggaaccaccgttaacatgtgcccaaggtcatagctcgactttgattattccaactgatgaaggcggatcaatttgtctgctctgcttgtccaatctcgtttctaatccgagatcgccgaccgttcacgtttcctatgctctctcccagttatctatcgcgctttctcaaccgaggtttcgccaaaccttcttcacattccactctcatttcctaatctcgcctctcgtcggtattctatcgtccttcgatgatgagccaatcgccaagcaaactatagatttgattatgcagttgtgtgaagctccagactgcgatgtgcatgcagagtttgtggctcggctcgcagatcgtctttccagtggcgctttagcttggagtcagagacagctccacacgtattatgcaactttgtgtggtgacggacagccggctgtgatcagtaaagcttttggttggaacctttcaattgcacccgagggccaattccttcttgagtacagtgaagatattcaaggggaaatcctgtttgttctatacaaattattcctactcaatgtgtctcaagacggggatgatgctcccagtttatttggccattcctcgaagctcctacacttggcactggcagttctcatgaaagctcaaagtgatgatgttcgcttgaactgtatagtgaatatgttgacagttaacaattttgttcctggattattgcaaagaggagtatatggaatagccatatacctccctgagagatcatttgaagctggagattttgtggctcgtaagcctaatgttgtgatactctttgtctatgcagcattcttaacagtaatactgcaaagaggattctttcaagctacttctataattggcacaaggagcaggagttcttatgatgttgaccacttgatggaaacaaatgagcagatatcagatagacctctagctatcttgtttgcagaggcagtcaaaggccccctgctttcttctgataatcaagttcaaatagcagcactagatttactttacctttatctgtcagggaaacatgtcttagaaaatgaaatccaggtatttgttgaagagaacattgcagactatgcgtttgaagtgctgagattgtcaggatgcaaagatccaacaattaaatcttgtattcagcttcttgatattttagcaactgctgagcaagcatttagacagagacttgcgattgggttcatggccctgattccagttctgcatcatgttgctgaaattcctttccaccctgtacagactgagacactcaggcttatttggaactccgttgagaactgcccaggggtggtatccaagtctcaggtagaagaaataagcctttctttgacgaggatgctcaagaaaaatcttgacggagaaataggcatgcttccagagacattagctctggtctgttcaatatttgttgcacttatgaaatgttcatcttcctgtgagatttcaagtttcttactatcaattcaggatgcatcaagaacctgcatcttaacttgtttaattaattatggcaaatacccgggtcaacttttgaactctctttacctactgaaagaggcatattcatatagttgtgggatgcatccctcaagctcaatcaacacagaacttagaagaagcattatagatgtatgcaaaacacatgtattaccttggtttatgaaatcgctacatgaaatggaagatgaggatattccagctgcaatactcgaaaatttgtattccatattgctacaagattcagatactgaaaccaaaatatttgcaaatgttctgttcacgtcttcctggttcagttttgcatatggatgtttaggcttttttccttctgaaaagatgaaaaggaaggtttatcttatctttagtctgatggcagatatcatacttggggttgattctgcacgatgcataagcgatactgctccacatcttccatctgatcctatagatttgcttttccttctgggccataaaagctcccaaaatgttgaattgtcttctcgccaaatggcagttctgctgttactgtacatcagttcactgtatgacgatcggattgcagatgacaaacttgtgttagcttcactggagcaatatattctacttaacagcagtgaaaacatgcacggagcttctgttttgggaatatttataaatctttatgcactctacagaggtttagccaaggtgagctaccaaatcccctatagcccagaggcagaaaggattgtgttccacctacttgctgaaaaggactgggatttgctatctacaagaatccacataacatctttgaaatggttgttgcaacaagagaaaatctgcaatgtgttgtctgcccagattttgaaattctgcagatgcaattgctctgatgtaaaccagacaaatatccatggtgaagccaatcagaatatagatgtgtatgttatggcagaacttgtagcttcaggggacaactttttaagtatgctcatggtgttcttattgggagaagctggagaacaacattccgagtatgacattatttcagtggtgaataccataaaacatataatagagatatcaccaagtgcttcagatcagttttgcatccacgggattgctggtgcaattaagaacctgtactataagtttggtcattcttcagccccagatactttcatggccatctccaaactagtatcctgcattcttcaagccgtacactctgaatccctctcagatgatgaaccctgggttgcagttgtggtgaaaataatcgattacctaattccctcagtagctgcagatggatggacaccaggaactcttatatcaattgccattctgtctatggttttgcaccactcagtaaatcatgtgatggttgaagcttcaaaaaccataatccttagtgttcctttgctatcattagtaaataccaccatcaccaatgcctgttccaagggaccttctctagttgaacaagacgaaggaataagatctggagaagctcttgtttttgtgctttcactgcttttcttctctttgagaagcgtgcatgccattttaccagggattatggactgccaatatctgctggatcctatcaaaatctcacaaccctggccctatatcagtatacagtgccatgatttgtgcaagttattgcattttggatctattcctataaagttactaagctcgcaatacctgctagagttattcagcggaatagaagacgagagaattagaaaatcagacacattagaattcagaactaattatttgttgtctgtaatggctgttttagaaggccaaatattctcaagtgacaggtctgtagcaatgaactgttccctctgtttgtctatgctcattgggtggcaagatgtggaaacagaagtatcagctatacaaaggaacaactggtgtcggtttatagtagaagaattagtgatgtctttggcagcaccatctttggcttcaaaatctttcatgatccatcacaagcctgcaattcatattgcagttgaactgctgaaaagaaagaaaattcctcaatggatgacttcaatattcgatgaatcttgcatatttgccattactagaaacattacaaattataatttgagtgctgagctggtgttcctcttaaggaagttgcttaattatggttttctgaatgatgaacaaattgctactctaaatcaagtattccaggactgcagaaaatgtatctacacagacaaacttcaacatgctggggcagaggagatggcattgaacgtagcagccgcttcagattatgtaggtaaagttgggcagtttctcattagcctcataacgactcaatcatctggttgtatggagtctacaagatttcaaagtgggaaaagggagttgttggaagaaatagacttattttcaaaatgtctaatgagggataattga

SEQ ID NO: 72 - protein, 1342 aa, Solanum melongena
MYFATSHLHHLPPSSPPEPPLTCAQGHSSTLIIPTDEGGSICLLCLSNLVSNPRSPTVHVSYALSQLSIALSQPRFRQTFFTFHSHFLISPLVGILSSFDDEPIAKQTIDLIMQLCEAPDCDVHAEFVARLADRLSSGALAWSQRQLHTYYATLCGDGQPAVISKAFGWNLSIAPEGQFLLEYSEDIQGEILFVLYKLFLLNVSQDGDDAPSLFGHSSKLLHLALAVLMKAQSDDVRLNCIVNMLTVNNFVPGLLQRGVYGIAIYLPERSFEAGDFVARKPNVVILFVYAAFLTVILQRGFFQATSIIGTRSRSSYDVDHLMETNEQISDRPLAILFAEAVKGPLLSSDNQVQIAALDLLYLYLSGKHVLENEIQVFVEENIADYAFEVLRLSGCKDPTIKSCIQLLDILATAEQAFRQRLAIGFMALIPVLHHVAEIPFHPVQTETLRLIWNSVENCPGVVSKSQVEEISLSLTRMLKKNLDGEIGMLPETLALVCSIFVALMKCSSSCEISSFLLSIQDASRTCILTCLINYGKYPGQLLNSLYLLKEAYSYSCGMHPSSSINTELRRSIIDVCKTHVLPWFMKSLHEMEDEDIPAAILENLYSILLQDSDTETKIFANVLFTSSWFSFAYGCLGFFPSEKMKRKVYLIFSLMADIILGVDSARCISDTAPHLPSDPIDLLFLLGHKSSQNVELSSRQMAVLLLLYISSLYDDRIADDKLVLASLEQYILLNSSENMHGASVLGIFINLYALYRGLAKVSYQIPYSPEAERIVFHLLAEKDWDLLSTRIHITSLKWLLQQEKICNVLSAQILKFCRCNCSDVNQTNIHGEANQNIDVYVMAELVASGDNFLSMLMVFLLGEAGEQHSEYDIISVVNTIKHIIEISPSASDQFCIHGIAGAIKNLYYKFGHSSAPDTFMAISKLVSCILQAVHSESLSDDEPWVAVVVKIIDYLIPSVAADGWTPGTLISIAILSMVLHHSVNHVMVEASKTIILSVPLLSLVNTTITNACSKGPSLVEQDEGIRSGEALVFVLSLLFFSLRSVHAILPGIMDCQYLLDPIKISQPWPYISIQCHDLCKLLHFGSIPIKLLSSQYLLELFSGIEDERIRKSDTLEFRTNYLLSVMAVLEGQIFSSDRSVAMNCSLCLSMLIGWQDVETEVSAIQRNNWCRFIVEELVMSLAAPSLASKSFMIHHKPAIHIAVELLKRKKIPQWMTSIFDESCIFAITRNITNYNLSAELVFLLRKLLNYGFLNDEQIATLNQVFQDCRKCIYTDKLQHAGAEEMALNVAAASDYVGKVGQFLISLITTQSSGCMESTRFQSGKRELLEEIDLFSKCLMRDN

SEQ ID NO: 73 - DNA, 8436 bp, Solanum melongena
  source 1..8436: mol_type = genomic DNA
aattcctttgacacaagtcttttagtgtgtagcttacactcaaagttcctttgacacgagtttttaaatgtgttagtgcacgttcaaaattccttcgatacaatccttgttattctacattctgtttcatgcatatttttgcatgtaacattgtaattactatttacgtcctaaataatattgttgtttcatttcactttttcagagtcaaattataataatgttaagatgacaaattaaatttgagtaaataaataagcaaataaaaagaatatagacccactttttaaattactaaaaattgcatacaaattatgaaatatgttctgattaatctaaagattatttggattccattagtaatgaagatttttttttgaaattaagatcttttttcctcttgaaaatgaagatggtcgaggatgacctatgatgcgtcttatccaaaggaaaagtgcttttcttatcgtcacgatatgattgttagcagtggcggagccactcttcggctagggggttcatctgaacctccttcaatgaaaaattatactatttatacatagttaaaattaatttttatctatatatatacagtagatataaaacctctttcgactagttcatgtgcttgtttttttaaattttgaacccccttaattcaaattctaactctgtcattgattattgggggtttcgaatctatcttttttctggtgacatctattccaagaatatttttgtgtcacttttcacatgaaagtcgagttctgatcttcttctaataaatatttgatttttggaccattatacaaaccatatccatttcgtatgaaaataatacaagttattcatttcaaaataacttcaaatatataatatttatttgatttatatgatattattgatattcaattctttttaaaaaaaaagcctcgcgcgtaacgttttataaacaagctaactcccgccatttaccgtaagtgctagagaaaaagagagaatggagaatttgagagagcaaccgaagagccagtccgatgaatcgctaaaacttgcgatcgcaatggcgctcgtccgatcgaagcttctccacaaacctctggcagcaccgccacctccgccttctgccgcggcagcggcggctttttcttcgtccgtgccttcttctcattccgatgatgctcttaaatggaaacgaaaagttcgatcgattaaaatctgattcttcgctattatttttgttatttctagaagttgagtggagaaatttcagttatttaacttcatttttcaggcaaaagagcgtaaacgagagattctcagactcaaggaggacctcaaaatagcggaaggttagatttcacgtttttgtaatattttaaactaaacaaattattttacttatttttttgttgattatactgaaaatctgacgatcgccgcaatttccagttatctattgtaatgtgtttgatttcgattgtccatttgctatattccgagctagaatgttgtgacttattgtgttttcgtttcaattcaaaattgcagtgataactagagtttcctgaggatcttttagctaaatgtttgatttcgattttgcaattttttgttatctgtataaattgattcgtttagaacggctaattttgattgtttttctttatttttggagtaagatggttcacagtatgatatatttccaaaaagtgcatcatgcaagtgttatttctttgataagttgggattattgagccatgaaagaactggagattgttgtgatcaacggttcagtgatgtactgcggagaagatttctcagacaaggtttgttttaaaggaattcggcatatttattaatctaaagttgtgaaacattagcttgattcattgacttgtacacttctccagtgaggattaaggagcgaaagaggagaagaccagatgattccttacttcatcgaatatcaggtgaaaatcagttatgggtgcaattttgtgtttactttctgtggttaacttgcaaagtcataggatttttaaaagttattgcatggagatcttatcatacctcagtcatgatgtgataaatctcttttttatgtgtgccataatttgatctctggaaacagtagatcctgtttggctaattttgctgaacctgaattttctgctatagatgagaagtatgaatattgtgtctttcctcaaatggcagaacgtgataatgaaaataatgttgaacagcttagcacttcagttgattttctattggagctttgtgacactatttctcctcacaatgtatgtagtttcaattaactccagctaggtgatgcattgtcttatgctatgcatatggtttttgtgtctcatctcacttggcttttgtaacaaatgtgttacagttggaggaaggtaattttaagaactggtgccaccaagctgttgactttattcttggtaaggagacaatattttcttttccttttccttcatgtatacaattttttcatgagcaacatctggaaatttcaaacttgaattcctgatatgcttttcagtttgatatgccgacgattaattatttcacagatgtactgttatattctaatttcagtgtcgaggattgtgatagaagctgaaattaaggggttaataagtgaatatattatctgttctgaaatttaaatgagaaaacagactgaatagtgaagcttcatcttaagattttgagttttcaaggaaagatttctctttgagaacaatcttaatggtctggactgccattttaaatgaagctttctaatttttattcaaaaatgcaaaaggttcacaatttacccttctttatcaacacctttccaagtactgaaccatttgactgcatagaatgcctaaatttctgaggattntaactagagtttcctgaggatcttttagctaaatgtttgatttcgattttgcaattttttgttatctgtataaattgattcgtttagaacggctaattttgattgtttttctttatttttggagtaagatggttcacagtatgatatatttccaaaaagtgcatcatgcaagtgttatttctttgataagttgggattattgagccatgaaagaactggagattgttgtgatcaacggttcagtgatgtactgcggagaagatttctcagacaaggtttgttttaaaggaattcggcatatttattaatctaaagttgtgaaacattagcttgattcattgacttgtacacttctccagtgaggattaaggagcgaaagaggagaagaccagatgattccttacttcatcgaatatcaggtgaaaatcagttatgggtgcaattttgtgtttactttctgtggttaacttgcaaagtcataggatttttaaaagttattgcatggagatcttatcatacctcagtcatgatgtgataaatctcttttttatgtgtgccataatttgatctctggaaacagtagatcctgtttggctaattttgctgaacctgaattttctgctatagatgagaagtatgaatattgtgtctttcctcaaatggcagaacgtgataatgaaaataatgttgaacagcttagcacttcagttgattttctattggagctttgtgacactatttctcctcacaatgtatgtagtttcaattaactccagctaggtgatgcattgtcttatgctatgcatatggtttttgtgtctcatctcacttggcttttgtaacaaatgtgttacagttggaggaaggtaattttaagaactggtgccaccaagctgttgactttattcttggtaaggagacaatattttcttttccttttccttcatgtatacaattttttcatgagcaacatctggaaatttcaaacttgaattcctgatatgcttttcagtttgatatgccgacgattaattatttcacagatgtactgttatattctaatttcagtgtcgaggattgtgatagaagctgaaattaaggggttaataagtgaatatattatctgttctgaaatttaaatgagaaaacagactgaatagtgaagcttcatcttaagattttgagttttcaaggaaagatttctctttgagaacaatcttaatggtctggactgccattttaaatgaagctttctaatttttattcaaaaatgcaaaaggttcacaatttacccttctttatcaacacctttccaagtactgaaccatttgactgcatagaatgcctaaatttctgaggatttatttgtaatattacaatagcaccagatgggttcattactctctagtcttcttctttaatgacttccaaattcagcatttgtattttactaatttaaaggtaccctggctacaatgtcaccaacagaaaggaacagagaacctgtggaaggcattatcaacagtttaatcatgcgtttattgagaagaatgtgcagtgccttgcaaggagacggtatttatgtgattttttaaaaattcatactaggttttcgaagaccatcttcacctcagcagattgcgaaagtattcacctatcttaataataatgttagaataagcatgttcaattaattgtacagattttggtagatttgtaccagtatatgcatatatatacataactaagaaatggtttcagcatgatactgagaaaagttctttggtttgatacgtatttaatggaaacaaatcagttttaacaatggatgtttggtttattatactctgatcttctcatttatgcagcattgctggataagatttgagtttaaaatgttaatttgatttcaaaattctaaatagtagcaataaaatggtaatgcagtgggcaaatcattaaaaaaatttgaattcttaaaatttattgaagttgtataaaagatattattggtagaataatgtagaagcttttggacatttcaaaataaatatagtattctgaatctagacagaggcaagcaatttttgtgatgaaactacctcttactgtagatagacacgtcgatagtttttccagcagaaacaaaaatattgttgtttccacatgacatagatcatgtaaaatgcttctaattattttggatggatgctgaataaaatttatgactaaattatttatccatgaaggaacaaactattgtgactgattctgaaagcttcattgaatctgattcttattagttaaaagtaatacgtatcatattgaatagttaaaagcaaagaccattgaaatcaaaagaggacagacccttgtgaccctcttgtcactggactgattattagtttagttggatcatgagcctgaagttcagagcaatttaatatgatttttgctcttggacagcagcatgttcatcattaaattcctcaatgtgacttacttatatttcattttacatggcttcttaaatcttgattccataatgatatgtttcagaattcaatcactttgacactgatgttcagttctatattcaacatttgatgcgtaaggtcggaaatgaggcttttatcggccagcgtctaatatttgcagtttctcaaagaatttctgcaatggcagaaagtttgcttttcatggatccatttgataatgcctttccaagtatgcataactctatgtacatgatgtaagtccaccagcttgtataaaattacttgtctttgtctggcttagttgttcttttaagcttctgttttgtagttctttccaactttcttataatagagggctgcagaaggggaagaagggggcagtgggagttgaacccatacatgttgtgggagattccaactggtacctctaggctataagcctcacttcttgtttgttaaatgccgtcctccttcagtcactgaaatttgtttctttgctggtgataatggatgtgcaatcagagacctcaataacaacatttcactataacaaccatttgtaacgtggaaccagtctttcatgttatgttatattgtatgttctctataacaacatttcactatagtctatagctgctaaaaaatattggaactaataatgttgttataatgaggtttggctgtccattattttggtccttactcttgatgaaatttcttttcctttacctatgataacatatttccctttctggtcattgacatctttccatatacttttttaaaaaaaattctgtttttagtttagagatttgagaacactgtaatttttttaaatctgttttggaccactagtccctccagacttcctgatttgaaggtattttaagctgaggagtgtaatttggtcctttaaatttggagttcctatggggagtgtgacatttactttgagacattgagttggctcttttgttctttcttttgtcagttaagctacataaagtctgaaatggttgtttgtacgtggtattatcatttttttattctagtatcctctagtgtagttgtcactattatattttgggatcatcttcataatttattgtaaatggtagttttagcagcaggattatgtggtgtgttgtgcccctttttttgtgtgtaaatagttattcattggttgaaacgctgcaatgatttagtgatcagaagctgcgcctgcttcagatacaaaaagtatattatggcgcctgaattgctagattacttagttagcttgggtatgttcatgtacctgaaggtttatcatcggaattgggtttaaacatcatacttggaaccatagcttaagcttgctatatttcggcctgtaagtggccgtgtgaagaatgtggcatacagtttactgcctagtatttgttttttacttcatccacaatttacttcttcttatttcttcatttctttatgaatcttcttgaaactatagccataaaaaggagactaaaattgtctaatatacgttctcaaatgcaggattcagcttgttgaatttctggtttctgatcatttgttaacctggtcaaaaggtggagatttcgacataagtgagcttcttctaatcacttggatacctaacatgttttctctatttgtaaccttctgtcgggtctgaggagttctgcctccgtctgagggaaattactgcatgtcatatatattcccacgagggtagcaggctccataaatgacctacctggtgaacaatcttttcatactgtgaatgacagaaatggactcctaacatatcaatacattttatttactctgtagggctttttgaagaatgggttgtatcaattctccacggaagaaaaacattggagctattagagaacaggaattctctttatgtactgtacatagatcgtgtaatcggagttgtggccaagcaagtgggacagttgtcatttctgcaaaagctaagaccacagatttttgaaagcttgttgaactaagcactgacctgcagcttttcctttgtgaactgtaagtaacttgctttcaacacaaatcttcttttcttgtgcatagaaaattcagctgtgtcatcgcaaatgctttttcacttaaaattcaagagtgcttgacacaaatgctttttacttaaagttcaagagtgctttgttaattaattcccagaggatcaaagattaaagttctttaaagtgaaagatgctctttaaatgtgaaaagatgaaacagcatgtcaatggtgaaatccacctatcgtataaaatctacatgacattagcacaccatcatgtgccgaaagttagaacaaaatcctacgtctctttatgctgaacctgattccaggttgaaacttccaccagattgtcgcttaagcaaatctttgatttcctgcggcatcactatttttcatattccttgatgtcgtaattgacatcttgcataaatgaggttgttggacggtttgacctttggttctttgtagtttaatctagatatgttcttttttcatttatttacttttctatgtgaaatcggggttggaagtctgaaccagattagttacctagtgctacctattgcctttcccaactttagagttgtcccatgtccccaccttgttcaactttcaaactacattttgaagggtgattactcagtcattaaaactttcttctccttttatgacagattactagtaccaaaagttcattatttttgaaagatgcaaaaaagatgtattgtattggatactcttctgctttttgcaagatatatagcgtccttcccgacttccatctaaccaaacttgctcctagctactacattttacgtcagctctctttctaattcttgcatagtagacatgattcaagccaaacctttactggttctctcattattagcaactcttgtattgtcccaatactgcaaaaccacagcttctactgacattctaccatccacttccaagcatccaactcc

SEQ ID NO: 74 - DNA, 1725 bp, Solanum melongena
  source 1..1725: mol_type = other DNA
atggagaatttgagagagcaaccgaagagccagtccgatgaatcgctaaaacttgcgatcgcaatggcgctcgtccgatcgaagcttctccacaaacctctggcagcaccgccacctccgccttctgccgcggcagcggcggctttttcttcgtccgtgccttcttctcattccgatgatgctcttaaatggaaacgaaaagcaaaagagcgtaaacgagagattctcagactcaaggaggacctcaaaatagcggaagatggttcacagtatgatatatttccaaaaagtgcatcatgcaagtgttatttctttgataagttgggattattgagccatgaaagaactggagattgttgtgatcaacggttcagtgatgtactgcggagaagatttctcagacaagtgaggattaaggagcgaaagaggagaagaccagatgattccttacttcatcgaatatcagatgagaagtatgaatattgtgtctttcctcaaatggcagaacgtgataatgaaaataatgttgaacagcttagcacttcagttgattttctattggagctttgtgacactatttctcctcacaatttggaggaaggtaattttaagaactggtgccaccaagctgttgactttattcttggtaaggagacaatattttcttttccttttccttcatatggttcacagtatgatatatttccaaaaagtgcatcatgcaagtgttatttctttgataagttgggattattgagccatgaaagaactggagattgttgtgatcaacggttcagtgatgtactgcggagaagatttctcagacaagtgaggattaaggagcgaaagaggagaagaccagatgattccttacttcatcgaatatcagatgagaagtatgaatattgtgtctttcctcaaatggcagaacgtgataatgaaaataatgttgaacagcttagcacttcagttgattttctattggagctttgtgacactatttctcctcacaatttggaggaaggtaattttaagaactggtgccaccaagctgttgactttattcttggtaccctggctacaatgtcaccaacagaaaggaacagagaacctgtggaaggcattatcaacagtttaatcatgcgtttattgagaagaatgtgcagtgccttgcaaggagacgaattcaatcactttgacactgatgttcagttctatattcaacatttgatgcgtaaggtcggaaatgaggcttttatcggccagcgtctaatatttgcagtttctcaaagaatttctgcaatggcagaaagtttgcttttcatggatccatttgataatgcctttccaagtatgcataactctatgtacatgatttctttccaactttcttataatagagggctgcagaaggggaagaagggggcagtgggagttgaacccatacatgttgtgggagattccaactggattcagcttgttgaatttctggtttctgatcatttgttaacctggtcaaaaggtggagatttcgacataaggctttttgaagaatgggttgtatcaattctccacggaagaaaaacattggagctattagagaacaggaattctctttatgtactgtacatagatcgtgtaatcggagttgtggccaagcaagtgggacagttgtcatttctgcaaaagctaagaccacagatttttgaaagcttgttgaactaa

SEQ ID NO: 75 - protein, 574 aa, Solanum melongena
MENLREQPKSQSDESLKLAIAMALVRSKLLHKPLAAPPPPPSAAAAAAFSSSVPSSHSDDALKWKRKAKERKREILRLKEDLKIAEDGSQYDIFPKSASCKCYFFDKLGLLSHERTGDCCDQRFSDVLRRRFLRQVRIKERKRRRPDDSLLHRISDEKYEYCVFPQMAERDNENNVEQLSTSVDFLLELCDTISPHNLEEGNFKNWCHQAVDFILGKETIFSFPFPSYGSQYDIFPKSASCKCYFFDKLGLLSHERTGDCCDQRFSDVLRRRFLRQVRIKERKRRRPDDSLLHRISDEKYEYCVFPQMAERDNENNVEQLSTSVDFLLELCDTISPHNLEEGNFKNWCHQAVDFILGTLATMSPTERNREPVEGIINSLIMRLLRRMCSALQGDEFNHFDTDVQFYIQHLMRKVGNEAFIGQRLIFAVSQRISAMAESLLFMDPFDNAFPSMHNSMYMISFQLSYNRGLQKGKKGAVGVEPIHVVGDSNWIQLVEFLVSDHLLTWSKGGDFDIRLFEEWVVSILHGRKTLELLENRNSLYVLYIDRVIGVVAKQVGQLSFLQKLRPQIFESLLN

SEQ ID NO: 76 - DNA, 6807 bp, Solanum melongena
  source 1..6807: mol_type = genomic DNA
atttatcttctaaaaaatataaaattttaataaaatgaaaagacaaatataaaaaaaatctaaaaaattcaattaatttaagacatacagagtatttgattcatttgttcgttaatattcacaaatgcgctatagttagtcattccatctttatattattttgagtttgtacaattgttactttacatttgaaggtaatatagttctaagaataattcaaacatattacataaagggactataacatagtttgaattaatttaagattcaatctattggttcatatatcagaagaattaaaatcaaaattcatcaatactgagtgataatttgcaattgaagaattttgcatatagccactcaaaaatatcttaattatgcttcatagctatagtttgtgtaattacatttcgtataattatagcaacatttgtatacgttgtatagttcgctacaattcacagtttttgtgtagcgtttctataattcgctatacaatttgattcgtgtataacttttgtataattgcgcgaattatataaatctcaaattgttattacaactagacatttgctacgaatcataattaatttaaattataattatgttagctaattaactaatatatatttacttatccacgtaatttttccttgtctgaaaaaatgggccctagatgacttggcccaaatttatcagtagaagtccatcacagcccagaagtcacatataggcccatttgtaccgttttccacaaaagatttgaaagttccctgtatataaacccccactctcccgctggattatcaacgcagatcacactttcaacttcaagttccaactgttcgacggagcgaaatcacagaaaaattaacttcaaagcgctcggggaattcaaattaatttacaaatttgattatttcttcatcggttagggttctgtaattgtccaaattgaagttttaattctcgaagatttcaatttttatagtatctgcaaatgaagttgaagatgaataaagcatcggatctcagttccatctctgttcttcctcctcatgcaaggttcaattctatctcaatttcacgatttcatctatttgcattgtatagcatgaaattgcctacctctctgtgtttctgcgctttctccgcatgcattccaatttgaatatttcatatgcgacacacatgaatatattgagtgaaatagagagaatattactgtaagattgagttgcttggtgaaagaggaggaactaatcgcgcatgtctctgttttgcttttttcttctaatatattgaagatatttgatgtttcgtgtgctatacacgcatatgcataggacatgttacatgtatgtgtggacgaataagagagagacaggtagaaattttgccgtgatattgagcttttttggtgtgatgatatgagtagacgccaagtgcggagccgctctgcgttttagcctacttctccatgttttcgcgatttttctcatacattacagatattttggatgttttcatgtccgatatacacaaaggcacacatatacatatacctgtctatgagtgcatgaagagatagagagattttaaaataatattgagtttattttgatgatatgtgaaggaggccaagtgtggtaccaaacgcagcagactcttcggtctacgggaaaagccaagcatcacaggttcggtctcagcagcaatcgcaacaatccttctcacagggattttcatctcagcaagcgatctactctcagctatcacagagctctctggatgagtttgtctctaatgagcaagtaagttctccatctcgctccttatctcttagttattcaaagagaagttgttaatgtgatgtcattttggcattctctgacttctaattcacaattatgtacaaaggacctgattcatttggtgggaaatgataattatggacttctaaaaattattttcattagcaacttgggaagaatgcttcagattgtcttaaccatattttgatgcttagcaagacttgaatctgtaatatcatagataattgttgcctaagtgagttttgagtgtaatttatcatttgtatgctttacgatgcttgaaattgatgaatttagcttctgactattatttaccttgttaaatgttgtgtcaatacacgacactcactttatatgaagttcaagcatatttgaacagctttgaaagttctgaaagttgcataaaagatgaatgatgccaatattttgcaaggtccttaaatggaaagagtgtcaaacaaattgggatggagagagaagtagatcttatttacgtatctttactgttttggacagtgaatcataaattctgttgccgtgtctgtcagaatgtttcttatgtatatgacaaaacaggagattgtcaaagtgcactttgaagtggttgtcggctgttaggttagtagatcttccccgtgttcatatacaactagttaactgatagattcttgacttcaattgatcatatgccttcttgttttcaactctgctcagtgtcaggacagagagttccataaaactttttactttataactttattgtaacagacaatatgctgttatgggaattttacatcttaaagcaaacaaatacttgcagagattgggttctcaagaaagagaaaattcagcaaaaaggatgagtggtttgcctcatatcaactacacacgagaagagactcaaatgcagttatcaagaccttcgaccaattatttgcgcaaatggtcagttcctgaaaacaaatgtaagccataatccaccaccagaaaatacatgctctgaacttctgttcaatagttaatgaaaatgtactccagtcagcactaatttgcagctggaataattggactaaacatgttcatgaattctaatttttctggacagaccagattgaagaacttgagcacaaacttggaatggtagagacttcattaagcagacaaggaatgatcttagattctattcagagtgatattatgcaagttaaccggggaacaaaagagatgttgatggagagtgagtattcactgcccttttaatttacatgatgtggctaaatagttaggaactccaaagagcccatatcattagttgacaatgtggaatttcgtcttgagaagcctgctggtccgattaaaatttttacttgcaaatatttctggtggatgtaaaagaaaaaggcgacatctaacacatttttttttcttctgaattttctttcagtggaaagcttacgaccgaagttagtttctcatgatgaactgttgcaattgatggtgaaacagcttagctgctctgcgtacatctagaaattaagtgcttgttcgttttatcacatttcctaatccattgtgacacaatatccagaaggagatggaagatctgaaagctagcctggaggggaccttcaaatctatgtttgaagaacttatggagaataaatatcacgagaacatcagagatcttctatcactgcttagagctatgcccaacaaacttgagatgtgcattttgcaacttcaaactgatttgagcaagaccttggctaaagagattcaggcatgttgcatgttgaaactgacttttttttttcatatattggcgaccctctgacgtgggttaatggtgcttcatctatattcctattgcttgcagataatttccctcccgccagattgtcgtggacaaaaacccgaaactgctccagtcgatccaccaaaagtacgtcttcaagaactcttttctcctaattccatatgatttttatgagtattgagtgtaataaagatggatcagaaatctttgtgcatttgaacattgtaggacatcaatgattgtagcgctccccgtgaagtgaagtttctaaagaagtaagttctcaaacttccttcacattgccatcactgcagccttagttttgaaatctttaagtaacaattattaatcagtagctctccagtatgcaaaattcataatcacttgatggattctcttattatattgcaccatttgtgtgcaatatgcacaaggggtagtcatttcacaatgccacttgagatgtgtgtattgacacttgataacacttgcagctgggatacactctctgtcatcagggactacttaggtggcaaatagatgtgatgattcacggcatagtgtcttttattccatattaaaaccagaaactgagtatccccatttctcaccttagctatatgaaggaagaaatggaaaagaaaggaagcactccccttattcctcgaaagctagccttcatgataaatcaaatgaaataagaaataagaactttgctatagtaacagaaatcttaaagatattttctttaaaagttttactgttctttctgacattgttaattcttaatttctgtgcaattgcaagtcaccaaacatttcttttttctggttcaactataatctcagagatcagaaaacaactatgccgccaaaaattgaaacgggaggctggactacagtaaaaaataaacaaacttgtatgacgcagaaaatttccatcagaagtgaaaaacagaatgaagcatttcaacaggtaactctctcattgtcctcatgcaagcaaatgtttgttgagttatgagcaacagtttcttcctttgtatgaaatgtgaagctggactacagtaaaaaataaccaaacttgtatgaagcagaaaattcccatcagaagtcacaaacagaatgaagcatttcaacaggtaactcccttattgtgcttaattgttgagttatgagcaacagttgcttccgttgtggcatgaaacatccaaaaaagaaacattggggttttagatgttgtatttatggtatgtcatagttcacgatctctgaggccttcatgttgaagtaacaaaagctactttgttcagcagaccacatttttgataacttgaaactgtgtcacccttattctcagagctgacaactggctatccattttaggaaaaggaatgtagaattaccattgaatctgatgaggatattgctgcaggcttttcctgcttgcttgaagaaaatggaacaggtcatttgcacttcttccctgcatcattcatttttgagtatttcaggataagcaaagtgatttttacatcctgtaattgatcaatgtgcttattgaccccatgtatgttgaagttatctaatgaattcagacagatctatttaggtgtatatcaaattatatcctatatctcaagattcaccattgacaagaatgacctgtccatacttctagtcaagcagaacacccaagatttataatatgaaatccaattcataaagtaacaagtcagaacacgtttaaaagcgtgaagcatctttgttgcactccatactattaagctttttctcaaaccaaagagaaactgataatcctctcttccctttgtgagttggggtgaggtagggaatttgaaccttagtgtcccgatgggtcttcttctttttctctgaaatagtcacattttgagtctgtcctaaaacaagaaattttgagcataataactgcagcaacaagtgttttttacacagactgaaacaatcattcatatattttttgtcatttgctaagatttgagtgtttaaactgtctttcccttaaaagacacagggctttgtccactagatgatgcaaaggatgagagtgcacgcatactaaggaaagcaaggaggcgaaagagaaagcattttaacactatcattatagactgaaggtacacggtgaatttataatccgctgaattaaggtcctgtgattcgataagcattaaaaaatgtattattgactcttttgcctttctgtagccaatatagaatatgtttgcaattgacttttcattattattagaaaatccacgactgatcattacatagcaagcaaaatctgtgttattgctgctatactcagtctagggtgattgcataccaagatgtctacagactccgcatataagaatatgtaatgcactggtattacataagcagaatgattatgatgttttaagttttgaattgcataaagttggctgattaggtcattgcatcgtctgtatacaatattttattagctaatgagcgtttatattatgctagtaaattttcagcctgtgatattataccatgatagaagtgtataaaatggaaaagagtgtcattttcaactggtgaagagaagttaggaacacctagtagagaatgaaagcatatcaaccctgggggggagggggggaggtggaggggaaagaaaggtccaagagattttacttatttctggacttggatggtcaagtatttttttggttacgtgctgtactactcttctgtcaagatcctgaattctaaataagagagccattctccactggtgaatctatccacataattttccttagagcataattatgtggaatttgttcttgtttgctcacaagaatctacagatcatccgtcatgtccctgcctattgcttttggggtgttaggttccttattgacttggcctaaaaaaacccaaaaagagaacaaaaaaatggcttagcagaagtagcaggcaattactagccacatcacattgcacttgtggtgtgtgtttttcatatggtaagaagcatgctcgatttctgcacaaatcctctagaaggaatgaatgcgtgggttggtgggtttcttatcctttttgaatatcatccaaaagtccaaacaaattttggttg

SEQ ID NO: 77 - DNA, 1188 bp, Solanum melongena
  source 1..1188: mol_type = other DNA
atgaagttgaagatgaataaagcatcggatctcagttccatctctgttcttcctcctcatgcaaggaggccaagtgtggtaccaaacgcagcagactcttcggtctacgggaaaagccaagcatcacaggttcggtctcagcagcaatcgcaacaatccttctcacagggattttcatctcagcaagcgatctactctcagctatcacagagctctctggatgagtttgtctctaatgagcaaagattgggttctcaagaaagagaaaattcagcaaaaaggatgagtggtttgcctcatatcaactacacacgagaagagactcaaatgcagttatcaagaccttcgaccaattatttgcgcaaatggtcagttcctgaaaacaaataccagattgaagaacttgagcacaaacttggaatggtagagacttcattaagcagacaaggaatgatcttagattctattcagagtgatattatgcaagttaaccggggaacaaaagagatgttgatggagatggaaagcttacgaccgaagttagtttctcatgatgaactgttgcaattgatgaaggagatggaagatctgaaagctagcctggaggggaccttcaaatctatgtttgaagaacttatggagaataaatatcacgagaacatcagagatcttctatcactgcttagagctatgcccaacaaacttgagatgtgcattttgcaacttcaaactgatttgagcaagaccttggctaaagagattcagataatttccctcccgccagattgtcgtggacaaaaacccgaaactgctccagtcgatccaccaaaagacatcaatgattgtagcgctccccgtgaagtgaagtttctaaagaaagatcagaaaacaactatgccgccaaaaattgaaacgggaggctggactacagtaaaaaataaacaaacttgtatgacgcagaaaatttccatcagaagtgaaaaacagaatgaagcatttcaacaggaaaaggaatgtagaattaccattgaatctgatgaggatattgctgcaggcttttcctgcttgcttgaagaaaatggaacagggctttgtccactagatgatgcaaaggatgagagtgcacgcatactaaggaaagcaaggaggcgaaagagaaagcattttaacactatcattatagactga

SEQ ID NO: 78 - protein, 395 aa, Solanum melongena
MKLKMNKASDLSSISVLPPHARRPSVVPNAADSSVYGKSQASQVRSQQQSQQSFSQGFSSQQAIYSQLSQSSLDEFVSNEQRLGSQERENSAKRMSGLPHINYTREETQMQLSRPSTNYLRKWSVPENKYQIEELEHKLGMVETSLSRQGMILDSIQSDIMQVNRGTKEMLMEMESLRPKLVSHDELLQLMKEMEDLKASLEGTFKSMFEELMENKYHENIRDLLSLLRAMPNKLEMCILQLQTDLSKTLAKEIQIISLPPDCRGQKPETAPVDPPKDINDCSAPREVKFLKKDQKTTMPPKIETGGWTTVKNKQTCMTQKISIRSEKQNEAFQQEKECRITIESDEDIAAGFSCLLEENGTGLCPLDDAKDESARILRKARRRKRKHFNTIIID

SEQ ID NO: 79 - DNA, 5050 bp, Solanum melongena
  source 1..5050: mol_type = genomic DNA
gacttattttttttaaagtcagaaaataacttatttgtcatgttgaacataccaatttcactgtaattcatctcatttattatttttgatggcttggagtttaaacacacacaaaaaaaaagttcaaataaatatttgtaatattcatttaatttgtttgagcaacactttgacgactcattcatagtcgtaatgaaattgattactttaaggtaagcacccctccatttcaattttgagattgaaaattcgagtcaaaacaaataaataatgttactgataatcatagaagttacttgtagataggacatgagagacatccttttgttccatctcgtctatgacatttgcagttcctttttgtttccaaacttaccaattcgtaaattaaaagtgattagttaacataattatagtttgaattaattacgccgcgacaaacatttaactataattacagtttgagttttctataatttttgcgattgtataccgaaatacaaacactgtgaattgtatagcgaattatacaattgttcgcataaattatataacaaaatatacaaaagttatacaaaacttgtgaattgtatagtaaattatacaaatctatacaatgttgcgcgaattatataaatgatgttataactatagttacgaaatataattatctaaactatagttatgtattataactagactttatatgtttgtcatttataaaatttgttgggccgatctaatttgcacaaaaactttgcctaatgggcctagtagtttgtctagttctcctataataatttagcaccggatttcatttgttgctaatccagtctcttgtaaataacaagggggaagtgtagtttatataacaagaaggagctctttgaaattatcccaaaataaaatttaaaaaaaggacgcggaaaatacaaaattcgaaaagactataaatttgggcagtttgaaatctgcagctcctcatttccttctcgtgaagatgtcaaacgcagtttcgcagcaaatctccctattccgattccaagtcgagcgccgtaggtttgtttttgattaatcaaaattttcattctgattcaattcagtaaaatgctgagcatgatttttcagcagattggatgaagaaactcttcgaattctccagtccgttttagcttggaacgatttcaaatctctggacggagtggtgtgtgctttgaaacagttcatgagacacgaatctctatgcattattgaggaaatcactggaaaatctgcagagaataagcttctgatcgttgattttctagttcgtgtttttgctctcatccgagatactgaggtatatactttctagtataagctttgactctatcgagttcaaattggtacatttcactttgagttagttatttggaaacaaattatttactaacagatcggaaagaacagttgtttctagtaggatgatgttgaagacactgaaacgtttgatgtattaaaccatgtattttggtgaaatttgtgataaatagaagtgctgcttgaaattttgtagcctgctgtgttcggtaattgtattatcttcaaaagatagatctcatggtaaatatttttctgctaaggaacttatgtccttgcgtggttatagtgttcacatgcacttcaattacacagataacttatatagctgtataagtggcgatgtttaggtggtggtggtaggtggtaatgtgactagcgaaagatgtaaataatggctgctgcgtgccagagaaattggtattacgcatctgtgaatgaaataaatccttccttatgtatgtacagaaactcttttaggtaaaagtttgtgaaagtgaagtaatcagtagaagtgatatttaggaacacgagaacctgacaattcaattaagtgtatgattggatagctttcatggtatattactgcagatatacctcgttcgtctcttttatgtgacacaatttaattgagcatgacgttaagagttagctgtagttttcattagaatgttgatgtaattgtcgagaatccatttgacattaaatatcacatcgtgctttaaagtgtctttctgaaatttgtgaaagatcatacgagatttatcagagttaaagttgttgattattttgggagatctaaagtgtaggcatatcctatgtttgagaaagctttaagaaaccgcacctgatgatgatggtattcttctgttataataattctggttttgctttatttttggttcctaacatgtgacttttaacaattgggtattcacagagttgtttggcgttgagatatgaggcattacttatgagagagcagaaagctaccagtgatcagaggcttcttgtttcatatagtgagtggctcacttttgctgagcattcacttgaaagtggcttttgttccattgcaaagaaggtaaacttccaacaatcttgggcacttctaagcatcttacatgtgcaaatgaacaatgaacaaaattcttagtatatgctgaccatttgaaaatttatgctcacttcataagattttgacctatgctaccagcacattaaggtcagagttaattctaaaatgatgctacttgttgtattgttatatttctttccatttgaaaatttatgctcacttcataagattttgacctatgctaccagcacattaaggtcagagttaattctaaaatgatgctacttgttgtattgttatatttctttccatttgaaaatttatgctcacttcataagattttgacctatgctaccagcacgttaaggtcagagttaattctaaaatgatgctactgcttgtactgttatatttctatactcatgtgatcataccttgaagattgttatcatgtcatgttgtgttccctttttggatgtgtttgttgatcaaccagaagtgaactttataataggttctatctctgttgggttagctgaataagtttgatctgacattcagatgctattgtgaaaataatcactcaactttgttatctctatacctcttgttggagaatttgttagatgttgcttatggttcttttgcattctgaataaggaattagactcactgctgaaaatccttctaattaaccttctgctgaccgggtcctcttttgtctacttcagaaatacagtatacggacaatttgttatgggcttatattgtagtgaaagttatgctaggagttagatcaatctagctgcgcaactatggcatggttaacatcttgccgacaccaagagcatatgtatttcacttgatgctatcgatttggaacatttattttgagcgtgatacgttatggctttcataattatagtgaagttacaatgtcctacgccttatagtaagtgtatcccaatatctgcctctgacttgtacttttcaggcatgtgaaaaggcactcttatgttttgagatgaacatcatagatgaccctgcaaatgacttagtaattgaaaaaattaagaagcttaaagatgttgctgtgatctcagcatcttcaaaatccggtatgttcaagtatttcattaaatacctcctttgtttcatcatagtttatactttgccattatatgttcctaacatgtgagtgtattgaattcaagaatttggtggaatgtcatcaaagtgttccattagagcatgtaactagaagcggttttgaaagggaatttaatagttattcattactgttaaagctttcttgtggtacatcagttcaggcacaggcagcagcgtatttcaagagcacaaatattcagaagaattcacaaaaatcctacatttctgtggaagttaaaagttcaggaagcacactgtttagagatggaatcaaaagacgacacagacgccaattggatgaataccgacatttgaaactggatggaacagctgatggagacacgcaaaatattttggtaggtcattctgccaatatcattccattccctgcctactttcatcatttgattacaattgatagtgcaggaatgatttttctctgaagtattagtattacggagttagctgggaaaaagagctgttttcctcggaatagaagataataagtttggaatcatgtggaaagcattaaatgctcaagagtgggaatcgaagcttggggttcttcaactctcattgtttatggcgtatcatttcagaaacaccacgatataattgctatgacatgtttgatacttacaagaaatttggtcttatatgtatgcctacgaaaacagtcacaaaaatttgttctgtggtaagaacctctggtttcatctattgactcttttttttttctctaattgaagactgtttaatcaagtgaaaactcttcaaaatttattttttcaccataataagcaacttttggaatttttaaattactttaaatgagacaaggtcagactgcttgccttgtctcttctcaaccttggtcctgcaataggaacctagcatgctggtgataagccttcaataaaatatgtttcttagggaatctgtaattaagtctaagcaacaaacaatgagtacatttgcagcaagatattagcttcagcccctctccatgcaatcacgtgactgcgcagttgagtattttgtcaattttcagagcttcaccaaattggataggtgtaacttactagtcaaaattcgggagttggcttagtaaggaaattttttattcaaaacaattaggaatttgtaattccttatagaaatccaatgaagagggcataaggcaaaaaaacatctttctttaattttaccacttaaccattcatgtgaaattaaagtatcatgcacattttgaataagaaaaatcaagagtggatatagggccaaactcaattgcttagtgcaaatcttgtatgtgttaaaacactcactatattgggatgaaattgttattaggtctgcatattgatcagttcggtttgattttgaaatttatagattatctatttgtagaatcgttataaaatcattaagatattaagatcg

SEQ ID NO: 80 - DNA, 825 bp, Solanum melongena
  source 1..825: mol_type = other DNA
atgtcaaacgcagtttcgcagcaaatctccctattccgattccaagtcgagcgccgtagtagattggatgaagaaactcttcgaattctccagtccgttttagcttggaacgatttcaaatctctggacggagtgatgtgtgctttgaaacagttcatgagacacgaatctctatgcattattgaggaaatcactggaaaatctgcagagaataagcttctgatcgttgattttctagttcgtgtttttgctctcatccgagatactgagagttgtttggcgttgagatatgaggcattacttatgagagagcagaaagctaccagtgatcagaggcttcttgtttcatatagtgagtggctcacttttgctgagcattcacttgaaagtggcttttgttccattgcaaagaaggcatgtgaaaaggcactcttatgttttgagatgaacatcatagatgaccctgcaaatgacttagtaattgaaaaaattaagaagcttaaagatgttgctgtgatctcagcatcttcaaaatccgttcaggcacaggcagcagcgtatttcaagagcacaaatattcagaagaattcacaaaaatcctacatttctgtggaagttaaaagttcaggaagcacactgtttagagatggaatcaaaagacgacacagacgccaattggatgaataccgacatttgaaactggatggaacagctgatggagacacgcaaaatattttggtaggtcattctgccaatatcattccattccctgcctactttcatcatttgattacaattgatagtgcaggaatgatttttctctga

SEQ ID NO: 81 - protein, 274 aa, Solanum melongena
MSNAVSQQISLFRFQVERRSRLDEETLRILQSVLAWNDFKSLDGVMCALKQFMRHESLCIIEEITGKSAENKLLIVDFLVRVFALIRDTESCLALRYEALLMREQKATSDQRLLVSYSEWLTFAEHSLESGFCSIAKKACEKALLCFEMNIIDDPANDLVIEKIKKLKDVAVISASSKSVQAQAAAYFKSTNIQKNSQKSYISVEVKSSGSTLFRDGIKRRHRRQLDEYRHLKLDGTADGDTQNILVGHSANIIPFPAYFHHLITIDSAGMIFL

SEQ ID NO: 82 - DNA, 9089 bp, Capsicum annuum
  source 1..9089: mol_type = genomic DNA
ctttgggttctgtgttgtcttattggtacttttctaaatcttacactaaattttatacatcttttatataattatacctagtatgtgtcgaatttaataggtgtcgaaacaaaaaaaatttgtctataggtccgcaccaggtgtaatcacacaattgagatccggtgagcatagagtgtacgcataccttatctctgcctcgtggaggtggagagcctatttctaaaacaccctcagctcaagtacaacaaatcaaaacattctaaatagtaactacaacgaaataatacgataatcgaagtacaataaacaacagatagtaataaaaaatcaaaggacaacaaactattgtagcaatactacgaatagtagtactcacggttaaataacgcgttacaagttatgatacacgtaatacttactacgacaaattagcataatttcacgtaagatacactaacatcacaaattaatattcaaattaactctcgaaaagtgaaataacaactaaaaaagaacggagagactaatagtaatctgaattaccaaaaaaaaaaaaagaatgtttcgatccaattgaactctgatttctgttcggaaattgctggaacgagctcaattcttcttacacaacgtagctacgtagtacatgctcctccgtgtcaatttacgtggcaccttttgaattttgtgattcaaatagatttatatttaattgtaattgcttcactcttgaaaagtgaaaagtgtcgtatatctgattttggagggaaatccaaaattcaattgttgtggtgttaaaattaaagttgtatcaaatgtcttttaattttttgatcttaaatatgctacgtgaaaagttaaaattaatatattatcaaaaaagaaaaagaatcattcttggactaaaaagaaaaatagttggttcttttttagacggagggagtatgaaatattgggtataaagaagaagaattaatcaaaaggtgaaaaatgagaaatgcatgagggacaagaaagtaaaaacacatgcaaaatgatgacggtaagcaccgcgtgttataaattattttttccctctgtttttgtttttgtgctgccccgaatttcggtttatcaattttcgaaaaacgtgaacctgcagggtgaagtggaaagaaaaatggagagaaagcgtttgaatgcgcagccattagcactcattaggaaaatcaaaggtagttagagcttcgattaaacttcaattttagctgcaaattgttagaatttcgaatgtgaggtaaatttgcatactataaacctttagtgtttggactttcccaggatccgctcatggcagaagctttagtgcatcggactatcttttttttttttgtttgaattttgaatgtgatgataaactgttagtatttggcctttccgaggacccgcgcatagcgggaggtttggtgcaatggtctgtctttttttgtttgaattttgaatgtgaagtaaatttgagtagtgttcggcctttccgatggactgtcctttgtgctgttcgaattacgaacgtgaggtgaagttgcgtatgatacaccgttgtgattcgactcttccatggacgtggcgtgtagcggggggctttagtgcaccttttttgccctttttgttgttcgaatttcgaatgtgaggtaactttgcgtatgataaaccgttgtggttcgacttttccctggacgtggcgtatagtgggagctttggtgcaccgttttttcccttttggttgttcaaattttgaatgtgtggtaaatttgcgtacgataaaccgttagtgtttgacctttccgctcacagagggaggtttagtgcatcgggctgttctttttgttgttcgtatttcgaatgtgaggtaaaggctggttatgatacactgttgtggttcaaatcttccatggacgtggcacatagcgggagttttagtacaccgggctgtccttttttaccttttttattgtttgatcgaatgtgaggtgaggcataaaccattatggttcggcccttccttggaaactgcacatagtaggagctttagtgcaccgggctgccattttccgtgcccttttcattgtccgaattttgcgttcaacacattgttttgacgaatcgtcgtcacgtttgagctgaattttgatttttttgttgcaggatttactcgttcaatcgttgagggtctagctcgaggtagtgcacctttgatctacattgatcggttcagaaattactgtacagacacttctggaaattggtaagatatgagaagcttaacgaagtgttttatttttttggtatgttagttgaaaacagtgaatgtgctgctgaattaaactgtcgatttcctatcactatctctatcggttcagaaattactgtacttaagcttatggaaattagtaagatgcagtgtatgtgtgtgcagatgttatttggtaggttgaatatatacacatgtaattatgaatcaagttaatcaagcttatggaagtgtttctttttcttattgttgtttgaaatttcattgcaattagtgtataggattacaataccaaaaattacactgaattaacctgtcgacttcctattaatttaattaaacacagcgagttttggttagtttctctattacaaaggcctccacagagatatccttgacataattgaactgaaaattgcaattgatgacgatacatatagctttaaaatgcagctttaagaaagttgtaatttatgggcttggtagatgattctgtggaattctagatggtatgcccctgctcccctcaagacaagcccttccaaacaataaaatgtagagacgaaacgaatcattattctatgtgtctttctcagaagaagaatgatcacagtttactctgagagatttgttcatagaagccatatcctattctgctacacaaataagtactagttgaacggatttctaaaaacaatggaatttactgaagttggagtttgaatggctaattaatatcatgcaactgttcagatagtattaatggtctttgtttaatttatgtagctcttgcagctctggtttgccggcaggcaaggaagctatatccttgaagagggaatgccatgcacgtaggcttggtaagtctagtaagggtaaacaatccctgtatatttcattgactagtcctcaccaaatagttggagaagaaatgattgatcgagaagggggcaggaaagataattcaaagttgttatcctccgtgaaaaatgacaaaattagcaggagaactatttccccgtttagttgactttaccgttagcctccatatccttgtaagttacaggatgcaccaggaggggtgggggtgaagggtactctcccaaattaacttgaaggccgtttttgctctctaatctccttaacatcccagaacctcgctggtttattcctttctgtgtttttcatttcagatgtcttgttgagagttcttctgatagttcaacaacttttgcaagaaaagaggcatggatcaaaaagagacatatattacatgcatcctactgtttttaaaggtaaatctggatcgatctttggtgttctagtgaatccactttccagaaaaaaaatctggacctattcttggtgtgccagtgtagctacttccctgttaatcccattggaaaaggtgagactttatgtactctagaatcagttttgaaatggtcttgtgattggttatgaagtttttttccaaggaaaatgtgtatgtgttgttgtaatgtgccacaagttagatcgctaacacaaaatgtatatatcagaaggccgcctccttctatgctcactattgtcttttgcactctataatgcagaacaatctgttgttgatcgggcaattaatgacatctgcatcctcttgcaatgcagtcgacataaccttaatgtggtacatcaattaactttcctctgtatcaaaatagactcagttaagatgtatgtccgcatgtcgtactgttaagttgggaactttttcacttcgcagtctcttctatttttatttagttacatgttctttttcacagtgaaggattcaaaaatattgcatctacatgcttttgccatgcgaaatggtagttcacaagtatctgagcgaccacgcgaaccgcataaatttcttgctttgggagtagaattttgtttgatttttctattgcacggcctttccttctccatagcatggggagtgaggtaggggttcactagtgtagttgattagaaggttgtgaatactgtttctcgtaaagaacttgaatatagaatcaaaaggatattctcagatatggtacccatcattcaaatgcttactttattctccctttattggtaattttgtaggaagcttgaccttttatattcttttgatgcttgccttctgcaggtgtctgttggaaatgggtgcgtacctctatacagttcatatttccttgcaggagtgtgcttctagacacgtatagtttgagttcactatatgcaatgttctttctcatactcaatacacatatttgcaatcttttctcttgaaaatttcaaatgcttctttcagttgattatgtttatacctcctgcatttgcttgaatgcctctccgtgtatgtctaaaatcctctttggggagaaaaatggctttatgattgagctgacatagtgtatcatgttacaataatcttttcacttctgtactttgagcaaggtaaaattttataaaaacctggagaaagcatgtcaactctcaagggggtattattgcattttgcttatgacaattttctgttccttaagatagatataatagttggttctcttctttgttcatattgtaatagtcccttgcaagtttcggtcataaaattcttcttccaactatttatggtctagattggtgatgggctggctgcggtatgtggaatctgggaggaaaattgactgcattagcaatcctaacactgtaagtccagtgtaacaatctaataaatagaagctaagatgggtttctgtagttatgtaacaatttaattatgatggttcctgcaggcttacccgattccggtccatgttgaagaggtcaatggtatccttatgtttaggcgtttcgaattatgaataaacatgagtttcatacatgtgaaagtccagttatcactaaacataaagatgaatcgatgcttttttattgaatacatcctgtttttgactatatgacttgctcattgctttttcagactgtagctgcagttgttactcccttaatgcttgaataagatattcttagtgttgctcaatatgttttagttgtggaaaaggaatcaggtaaaactattcataagcagatcaaggctataaaaggtattcctagttcataagtaaggtcactatttgttgttcgtcatgcagtgttccagcgactagcaaatgatcagttttgcaagaggaaccattgcattgtcataacagtacgcatcttttgttttctgaaaattcccacacatatttggctccataatttctttttaacagggaaggggttatcctgatgttcccacaaggaggttagacccatgttgctctcaccttgtcacacatgttgcagatgaatccttcttcagttaatcatatttctgtcttttcacgttgcttgcctgtggtaggtttctgcgtctcctcattgacaagctgcatttgcctgtgtactgcctggtagattgtgatccatatggctttgacatcttaactacatacaaattcggttctttggtaaggattattaatgtggtgttattatcatgtgatcaagttgctaatattcctccttttcactgtaacagtctacacttccttagttaattagttcaaacttacattcacatttctaaaagaaaagtctgatacattcttcaccgttttcctatcaaaagctatcaagcattcatttttatcttgatagtaatctacgcaagccacttaagttaaagtgtatagagtagttaggttcgacggattgatttacggatgttttctttctttatatgcgttttgaagcaaatggcttatgatgcaacgtttctacaagtctctgagatacaatggcttggagtatttgtccaggattccgacaattacagcattccacagcaatgtctcctgcctttgactgtagaaggtaaaacccacacattcatcgtctcatattattatagtttttcaaagaatcgaaaaaaaaaaaactgacaaatgactggttgtgtaatcttatcagataagaggaaagtcgaagcaatgttacatagatgttatttgcaacgagaagtgccaaaatggaggtagaatttcatactactaaagtaatgtcaacgccaagttgtcaaaatattcacatgaatgttctccacttcttgaggtttgaactggagctgctgttgtacaaaggagttaagttcgagattgaagcattgtccgtgcactcgctcactttcttgtcacacgagtatctaccatcaaagatcaacaacggagggtatatctgaatcttttctatctttgttcagttctctagcacaagaagttcaaagtatttttcgtgtgctcgagtaaatcatttgaaagaacaacctaactagtcactttcgtcgactacatcatgtccgttcgtgttgtcaattaagtttttcgcgataatggttgtggatatcgagctacgaatgtgcattgacattagccagtttgatagagagaatgaaattatttactgtatctcatcctaaatgatacattgaattagatcgaagaccccaattagccttaattctcatgatttaagttatatataacgacaatgaagagctttcacacagcaacaacaacaaaatacctcgtgaaatccctcaatagagcgtatgcagaaggtaccactaccttgaggatagcatttatgatgttatgttagtaactctttttaccaagttacgaatcacgtttatcgtgatctatatttaattaatttattagtgatttgattggataaatagtttttttacctcatcagtgtatatctatttaagcttagaaggatttgagatatacacataataaaagcaccatttaaaaatgtggtacaacttgtttaatttttttaaaaattatcatagcgtccaagtccgtttgcttcacctcaattagttcgaaataactttgtccatcaaggctcgaacagatgagaagacatcaacggaatttaaattaaacttccatgcatggtttataggcctttgaatttgaagaactatagaaggaaaatattattaagcgttatgcaaatatgaaagactgtacttatgcacaaagctcatggttgtacgacagatggaaactgaattcgatctgaggtctcctacatgggcaacccacctcccaaatactaaaccatgccctcgttggcaataagaactttgaattgagagaaactataacacaattcaaagcaaaaataaaagagcagctcggtgtactaaagctcccgctatgcgcaggatcgggggaagagccccaccacaagggtgtattgtacgtagtcttaccttgcatttctgcaagagactgtttccaaggcttgaacccgtaacctcttgatcacatgacaataactttaccagttactccgatcgaaagagaaaatatgaaggaaaaaaaaaggtgtgtattctatgtttaggtacttaaaatgatccatacataataatttgtataatccaaactatcataacattcattgtgcaattaacaagttgctaatgaactagctcttatggcatttagcaaaatcattttacattccaagaacaatattatcattgaaacatcgcgcagtatatgaaactcgcgtaaattaacaagtttgctcactgcaacactgtcaaatttgatattttcactaatacgggtctgatgcagatgccttcaacttcttgggtggtggattacctccagacagtatcacataagagtagaagcagaacattagagcagtgaaaagatttaagagcaaagtgaatgataatgttgtacggttgcaccaggtaatggatacttgagaaaagaagaagacgttgtaatacctaatggcagcaaagaagccggcagggaacaattttcctgtctgcataaacaaaacaaaacaaaatgttaaacctacaaacagatacagaacaattttcctgtctgcatcaactttcttctctctttacagtcgtcttccaaccccacacgatatatctatgatcacatgcatacaatgttaaacctacaaacagatacagatcaaagacattacgcccaaaagaagtgttccctgttcacaaccaataacatgctaaagagtactgtccaccagccaaaatgtgatgatttggacttttatttgaaaatagtattattgttatatatgtatttatattatagtaaatatctatcaagatctactgtgatatctattaggatttgtgtcacgacccaaatcgaggccttggctgtaacaagcatcccgaaccaagaaggcccgaacgccctcctgtatctggtaatcatgcacaatattcatactgtaaaagcagatacggaaatacatagctaaacggaaacatggtcataaatctgaaatctgtttaacactactagaataggtttttcaacataaaataacatctctatccgtctgcaaaatctctactacataagacatcaaaacttgtctgaatctgggacaaggcccccagtagaccaaaaccataataaatgataaatgtctgaaagtaaataggccttctgaaatatagaaggcacaccaactagtactcttcactcctgcctgaagaaatctactgcttatcagaccccctagactgtacctcagaacctggagggaggggggaggtcaatacagttgtactggtacataaagtaatccaaaataaagcttttatataaataaattaatggagagcaatttttcaaaacatcatgca

SEQ ID NO: 83 - DNA, 1685 bp, Capsicum annuum
  source 1..1685: mol_type = other DNA
tattgggtataaagaagaagaattaatcaaaaggtgaaaaatgagaaatgcatgagggacaagaaagtaaaaacacatgcaaaatgatgacgggtgaagtggaaagaaaaatggagagaaagcgtttgaatgcgcagccattagcactcattaggaaaatcaaaggatttactcgttcaatcgttgagggtctagctcgaggtagtgcacctttgatctacattgatcggttcagaaattactgtacagacacttctggaaattgctcttgcagctctggtttgccggcaggcaaggaagctatatccttgaagagggaatgccatgcacgtaggcttgatgtcttgttgagagttcttctgatagttcaacaacttttgcaagaaaagaggcatggatcaaaaagagacatatattacatgcatcctactgtttttaaagaacaatctgttgttgatcgggcaattaatgacatctgcatcctcttgcaatgcagtcgacataaccttaatgtggtgtctgttggaaatggattggtgatgggctggctgcggtatgtggaatctgggaggaaaattgactgcattagcaatcctaacactgcttacccgattccggtccatgttgaagaggtcaatgatattcttagtgttgctcaatatgttttagttgtggaaaaggaatcagtgttccagcgactagcaaatgatcagttttgcaagaggaaccattgcattgtcataacaggaaggggttatcctgatgttcccacaaggaggtttctgcgtctcctcattgacaagctgcatttgcctgtgtactgcctggtagattgtgatccatatggctttgacatcttaactacatacaaattcggttctttgcaaatggcttatgatgcaacgtttctacaagtctctgagatacaatggcttggagtatttgtccaggattccgacaattacagcattccacagcaatgtctcctgcctttgactgtagaagataagaggaaagtcgaagcaatgttacatagatgttatttgcaacgagaagtgccaaaatggaggtttgaactggagctgctgttgtacaaaggagttaagttcgagattgaagcattgtccgtgcactcgctcactttcttgtcacacgagtatctaccatcaaagatcaacaacggaggatgccttcaacttcttgggtggtggattacctccagacagtatcacataagagtagaagcagaacattagagcagtgaaaagatttaagagcaaagtgaatgataatgttgtacggttgcaccaggtaatggatacttgagaaaagaagaagacgttgtaatacctaatggcagcaaagaagccggcagggaacaattttcctgtctgcataaacaaaacaaaacaaaatgttaaacctacaaacagatacagaacaattttcctgtctgcatcaactttcttctctctttacagtcgtcttccaaccccacacgatatatctatgatcacatgcatacaatgttaaacctacaaacagatacagatcaaagacattacgcccaaaagaagtgttccctgttcacaaccaataacatgctaaagagtactgtccaccagccaaaatgtgatgatttggacttttatttgaaaatagtattattgttatatatgtattta

SEQ ID NO: 84 - protein, 402 aa, Capsicum annuum
MHEGQESKNTCKMMTGEVERKMERKRLNAQPLALIRKIKGFTRSIVEGLARGSAPLIYIDRFRNYCTDTSGNCSCSSGLPAGKEAISLKRECHARRLDVLLRVLLIVQQLLQEKRHGSKRDIYYMHPTVFKEQSVVDRAINDICILLQCSRHNLNVVSVGNGLVMGWLRYVESGRKIDCISNPNTAYPIPVHVEEVNDILSVAQYVLVVEKESVFQRLANDQFCKRNHCIVITGRGYPDVPTRRFLRLLIDKLHLPVYCLVDCDPYGFDILTTYKFGSLQMAYDATFLQVSEIQWLGVFVQDSDNYSIPQQCLLPLTVEDKRKVEAMLHRCYLQREVPKWRFELELLLYKGVKFEIEALSVHSLTFLSHEYLPSKINNGGCLQLLGWWITSRQYHIRVEAEH

SEQ ID NO: 85 - DNA, 8515 bp, Capsicum annuum
  source 1..8515: mol_type = genomic DNA
tgtccttcaaccaaattactcgtgtctgcatctggagatacggagtacaggttgcctctactgttacgattacgcctccaactcggatctggattcaagtacatgtttgcttggggcttttcctattttactatcttgtgttgcatttgttgttcaactatttgggtcatttgctcttaataggcctgcaaactgatgcctgcaaactgagttattgttgctagattattgagcaccaataactctgaactacggttagagggctattctgaaccatatttgactgcgcatcgagatcgccgcagctcccataataatatggaccctgttagtatcttgatcatgaaatatgccatcatattccaactagtcctttgattccactatcccaccttaatttgttccaatgatagatttcaaatatttcatataataaaggtgtaaatctcatgcttcgatttactagtgttaagtcgttcttctatgatttggtgtaatcacttaactaacaattaaattaagccctggacaaagagcactagggacacgtggcaattcaggactaatagcacaaaaaatgcatcacttaagctgtgattcaagtccatgaaacattcatattcttctaaggatggggcccacactaggcattaaattaagccctggacaaagagcactagggacacgtggcaattcaggactaatagcacaaaatatgcatcacttaagctgtgattcaaatccatgaaacattcatattcttctaaggatggggcccacactaggctctgcaaaatgcaaaatcccatctgttatatatggcgggtgtatacacaatacggttacgcattgcagacgcacaggcactaaacacacgctatttacctttttcactttgcatgtgatcattctctctctctccacctatatatacaaaactttctcacttcaaaattctctgcaatttcactactgaaatctcctttttcacgacggcaaaatgttctactctcatcagcttcttgctcgtaaagctccactcggccaaatatggtgaaaattatgaatttctacttgttattccattttttcatttttgtaatcgttaaattcttattgttaagctacaaatttttgagtttgtgcatttttacttcatatattctaagttcctgttctagatcttcgtttccgtctttgctcgctgtctaatgatattcactgttctttgaagctcctttatacgattttttttttttaatttgaagttccagttgattttatgttgagttatcatagttcaaattggatctattcgtgtttgaaaaacgtttagaatcaatttgtctatgaatgtattatccagcttgttgctcgtaaagctccgcttcaaatatggtgaaattttttaactacagcttctatttcactacagtttcagcgtttttacttccatatattgcaattcctgcgctaggtcttcgttcacttttttttatctaatgatattcagtgctctctaaagctccttcatccaattttttgcaatttgaagttccggcttagttatatgtaagtttcatatttcaaatttgatctgtttctgttcgaaaaatgcttagaatcggattgtttatgaattcattgatccagcttctagctagaaaagctccgtttggccaactatggtgagatttattaactacaactactattttgagttttcttggtttctaaattcgttttgatgcatatagataagctacaggtttcgaatttctgcgttttttactttcacatatcgcactttctgtagtggatcttcttttccgtttctgcttctctatctaatgagcttcagtattatctgaagctccttcacttttattttgtaatccgaaggtcctttatctctgaagcttcagcattcagtagacacagtttaaattgtatccgtttctgatctaaaaatgcttcaattcaaattgtttatggtgaaaatttttaactacaattttgatttttctttcctcaattcgttttaatacatataaataggctacatgctttgagcttttgctttcatatatcataatttctgctgtggatcttattttcctcttttgctctctgtatcgactgatttttagtattttcttgtgctcctccatccgtaagtttgtaatccgaaaaacacttcaagttatgtgttacgagtcacagttcaagtaggatctgtttctgttctagaaatgcttgattaaaatagtttatgaatgtaatgatccagcttcttgcatgtaaagctgtgccccaaatatggcgaaaatttcaactgcaacttctatattcgttcaacgcataaagataagctgcatatttgagtttctacgttttttatttgcatatattgtaattcatgtagcggatcatctattcctctttggctttctgtttctagtgttcagtattcgtttaagctccttcatagtattttttgtatttgttaagttttcgcagttcaatttggctacgaagaatgcttaaattgaaattgatgatctttgtgtttgctgttgaaggatggcggccactctgcactcgaaactcaataggaaaaagcttagtaaactcaatataattaacatctggtgaggcgttttcttccattactacatggaactgcacttcattccttgttgactttagtaatcaaattctgcaatttcttttgtcacagtgaacaaatattaaatccatcggtcccaatggctctgaggctctctggaattctcatgggtatgcttcgaaaacaaatggctgttctgttcgcaattgtgttgctgcttctgtttagatatctaatagttagttctatctcaggtggagtagtcattgtttatgaacgcaaagtgaaactcctctacggtatgaattgccatgactttttcatcgtttatatttgaatttcacgataacttcctcgaattttactccaaattccccttgtttcttcaactgttttagtctttgttgttttctttaatgcagaggatgtgactcgtctcatggtagtagcatcgatcttcgacccatatcagcttatctctttcttttctttgttttcgttaaattcagcacttctttgtcctttaattggtattttcaggttcaaatcaatgaagcttggaaggtgaaagcaactgttgatcctacgttgcttcccaagggtaaatctcaagccaagtgagtaactcatctccactttgacgtcacagtaatttgccgagaagcagagattatgatggccaagttttgtaactgtccaatagtttcagttatgtcgatagtgcttcagtagatttaacaactaaagtatgaaatgccaccaattagttgaattattaacttgatttattatggtttgtttcaccccatgtttgggtcagtttcatcaatggattatttaaggccagcttatgctgcaagtcctttatacctggggactttggtaattaaagagagtgtattttagtgatgaactggtagtaaaagttgaacttctgattccttttgttgttattcctaagttgatacttaagcttatcattcctctttttaatccctgcagacatgcatctgttactctgccagagaatcaggaggaagagctccctgagattgaacagacgctacgaaatccagacactgccacaatgatggatttcgaacaaacctcctattttgcaatggtacattatggaaagcactgccacctcctcaatccacgaaataacttcaaagtagacaataaaacgaagatcaaaaaaacctacagaaaaatgcagaatacatctttttgttggaagttggaactgatctaattagactattgagcttgctttagattatcgaattaagtcgtatttcattgttcagaaagattgcaagctgaatcaatagaaagttaacaatgataaggtggtttgatttcctatctctttcttttggttactcttatgtgttttgcaatttgttctttgttatttcaactcttgggttgtttaagctttttgaaagactttaaaagttatttggattttgtccatgttcatgaccttgttgagcattcaatcttatctgataccaccaagtacatagtgaaaataagatcatacttagtacaacataagagtgcagctaaactcgcggatgttcaatgtgcagagactagataatgctgacatctacgataaacccaatgcaggggaggaatgtgccccggactttcatcaaggtatgcatagattccactatcagcatagattatgctaattgcaccaccaccgtagaatatataactatatcctttgcaaatgccacttctattttcacttttctcttgttgtgcctatatcttagcaaccctgaaatttttgttgcagttgatgcagaaaatattaccctgcctgaacatttcgaatcgcgtcatacagatatgtctaatcattttgagaggtatcgtgataaacagttaaaaggctctgtatttaaaactttcaccagctatctttctaagtttatattgtcagttaacgtaaagacttcacgtgaaccaaactgtccatcattaaatcatgggagacttattttcctcatttccaattgggctgcacagctttccttctattatcctcctcttaatttttaagcatgaattgctccacaggtttgatattgaaggggacgatgatacacaaatgaattttacgcagccagaggatgctcaaatcccaagtactcctgttccatctgcacctaaagaacaagcccataaacgtaagaatgtgttactagacttgcctttgcagaaaagtacagattttctactttagataaaataagtttttttctagaggtaaataatggatggacttgagatgatttacttggttcttaatgagatacttttctgatagagacattatggcagtaagtccttcctctcaaagcagaacatggatgcaagtcgtacttacctacaatctgatcagctaaaatagtttgtgacacctggttgcctatctttaaactgcctgtttacatgtgtagttccataaagaataaagctctattggattcagttggtctcgtaaaagtctttagattcacttaggtaattccatattttcacaaattggttgaatggagtgaaattttgttgcagctgatgagatccctgacagatatccagaggaccaagcgaagcagcaatctaatgaagctgaagaagcttttgaggtagaaaatccagaagcaaccgagctagaaaatgttgtaaggaaaaactgtcagcattaatgtaccgtgttgacatgattttgcagcagcggcaggaccaacaaaggccaaagccagctcgacgaagagcaagaaaggccgtacgtcttgcaattgatcacgagcaaactgttatttctggtgacgtatatcaatcctggctaaagaattcttcagatatttcttcaagaaaaaggaaaaagagaaaggtactcccgtaacacccaagtatagatcttccccatctcaacttttccattctgtgcaccgtagcaattaaaatttgactagggtcttatcctaaaataaagcatgtttatctttgacatcaatggctagtgtttggatatccgaagaatagtaagtgcgtcactctttggaaggtaaccttaactaagatgcagcatcatttattcataacattaagttcctgatctatgcagactatgagtgtcttatcttctatgaagatagctagaatcatggaggttcctccgattgcattattagaagaattgttcacaaatggaaacaaggaagttcactatccagcaccactcctaaaattgtggatgagaagtaccctacctccgcatgattcaccttctggtctggtttttcatccatgatcttatactcttagttgcaaaaactataaacagatggtaattccatttgacatgcaggaaagacctctccaccctatcctcctgaaccatcctactcatctccaggcgaaaggatgggtaatgtggagcctggtggatatgtaaggaacttgtgattccctattagttttaactgagaacctgcctccatttgtttctgattgagcatttgaatgtgaagcctttcgaacatttccaaggtggcataggttctccatccaaaggaatctctatagagaaacaaagagcaaatctcaacaataacgagattccacctgagattctcatggagaacctcagagccaatctgacaaacatgggactgcatccaacagaggctgatggagtgaaagagactgatcacatggccacacctggctctggtatatcgaatttttatgagtatcccaatctccattgttgatgggctatctgttatggtgatattactaatatttttgtgaaactataggtgatgagcctagatccattccaagctcaggatctggtcatggtttactatcacagaactctataacgaattcaaggtacgtactaaaagtagatatgcatacattaacagaaggacacaaagatgaaccacttaaatgatacatacattaacagaaggaaataaggaggaatatcatgggtctcggtaccataggaaacttcaaatctttgcttcttcttcttcttttttaaattttgaacgtctcagccatatatgcagcatcgggttacattgatcaaaactgttaactcttcaggtccaacaagaaaagaccacattcttcatcgaagaacagtagcaatggccttcaaccggtagcagaagagaatccatggcacgatcccactccaaatttcaagttgactagattatctgaactatcagaaaatggtgttacacaagacaatggtctgtgaatagtcaataactttcccattttagttctggtcatttccttaatgtggttttgtttgttgtgggaaccaccttttgctctttttgcagagatattaatggaaaccggaccaacacaaacccaacgcccattcgttactcaacctcttgacatgatgactgaaactatcaggaagtaaatcctttttcattagttcctaaaacttcttccagtttcattatgactcctctaacttaatgatttttcacatgatacattgatgcccacaggcagctaaagagtcattttgacactcctggatcggcggagacagaatgtttgaatgaactaactcttgggttgacaaagaaacaagcagcatgtctcttttatcagacttgtggtatgcatatttctttcaactcttttatctgcattgcagctcagagaaacttcttagttttcaacttctcattatagagaatagaattaaattttgctccattctatttgcagttctggccactcgagacttcataaaagtccaacaggaggtgccatatggaaacattctcatttccagaggtgcaaagatgtgatcacggataaatcaagaagatgctaaaccctcacaagtcatgtaggttcatctattgctatggctgaatcagttcgtctttcagttaatgtattggagagctcaggcacaggtttatagctcgaattatttggaggaagtatttttattggttaacctatcttgtgtttaatcgtacaaacctagttatctccaagagaatatatttagtatatgactggtcattcagataatagctaattgcatattttgcaataactttttgtcaaaaccaagtatcaacagtgttcaccattggaaacatcgaaatggtcgcaacaactctttttggcaatgttatcaacttccttttcttttgctttttattgaacatcatgctgaaatgatagaagatcggttaactcatagtacgttgttggttttgaagtgatttcccgaaatctattcatttgaatagaggcgtagttcaataataactatccagtacacaacatgttctctataggcaaatcttggatagaaacttccttgcttgatctatcaaaactttcaacaaacacgaacattacacacatttcttcacatattcacatattcaatagtttggctcatctatcgtcacctaaaatcttaactacatgactgaatacaaacatatcaacagattaaacacatccaatcctgtttttacattctatcttccctcctccgtggggcacatgtgatgatttcatcaacccttagtatcatctcagcagcctcggttgcagagagcaacacagcctgtttaactttgaatgcctccgatattcctagctctgccatatctccaacctgtcataaaagccagataaagatgatcagatctagaaaaatactaactcccaataagaagcaagaatcgatgatttgcacgagatttgaactgtgcttggagaaaaaggaaaagtttcagccttcttccttcactatgatttgctaaaaggaagtaacaaaataaa

SEQ ID NO: 86 - DNA, 1893 bp, Capsicum annuum
  source 1..1893: mol_type = other DNA
atgttctactctcatcagcttcttgctcgtaaagctccactcggccaaatatggatggcggccactctgcactcgaaactcaataggaaaaagcttagtaaactcaatataattaacatctgtgaacaaatattaaatccatcggtcccaatggctctgaggctctctggaattctcatgggtggagtagtcattgtttatgaacgcaaagtgaaactcctctacgaggatgtgactcgtctcatggttcaaatcaatgaagcttggaaggtgaaagcaactgttgatcctacgttgcttcccaagggtaaatctcaagccaaacatgcatctgttactctgccagagaatcaggaggaagagctccctgagattgaacagacgctacgaaatccagacactgccacaatgatggatttcgaacaaacctcctattttgcaatgagactagataatgctgacatctacgataaacccaatgcaggggaggaatgtgccccggactttcatcaagttgatgcagaaaatattaccctgcctgaacatttcgaatcgcgtcatacagatatgtctaatcattttgagaggtttgatattgaaggggacgatgatacacaaatgaattttacgcagccagaggatgctcaaatcccaagtactcctgttccatctgcacctaaagaacaagcccataaacctgatgagatccctgacagatatccagaggaccaagcgaagcagcaatctaatgaagctgaagaagcttttgagcagcggcaggaccaacaaaggccaaagccagctcgacgaagagcaagaaaggccgtacgtcttgcaattgatcacgagcaaactgttatttctggtgacgtatatcaatcctggctaaagaattcttcagatatttcttcaagaaaaaggaaaaagagaaagactatgagtgtcttatcttctatgaagatagctagaatcatggaggttcctccgattgcattattagaagaattgttcacaaatggaaacaaggaagttcactatccagcaccactcctaaaattgtggatgagaagtaccctacctccgcatgattcaccttctggaaagacctctccaccctatcctcctgaaccatcctactcatctccaggcgaaaggatgggtaatgtggagcctggtggatatcctttcgaacatttccaaggtggcataggttctccatccaaaggaatctctatagagaaacaaagagcaaatctcaacaataacgagattccacctgagattctcatggagaacctcagagccaatctgacaaacatgggactgcatccaacagaggctgatggagtgaaagagactgatcacatggccacacctggctctggtgatgagcctagatccattccaagctcaggatctggtcatggtttactatcacagaactctataacgaattcaaggtccaacaagaaaagaccacattcttcatcgaagaacagtagcaatggccttcaaccggtagcagaagagaatccatggcacgatcccactccaaatttcaagttgactagattatctgaactatcagaaaatggtgttacacaagacaatgagatattaatggaaaccggaccaacacaaacccaacgcccattcgttactcaacctcttgacatgatgactgaaactatcaggaagcagctaaagagtcattttgacactcctggatcggcggagacagaatgtttgaatgaactaactcttgggttgacaaagaaacaagcagcatgtctcttttatcagacttgtgttctggccactcgagacttcataaaagtccaacaggaggtgccatatggaaacattctcatttccagaggtgcaaagatgtga

SEQ ID NO: 87 - protein, 630 aa, Capsicum annuum
MFYSHQLLARKAPLGQIWMAATLHSKLNRKKLSKLNIINICEQILNPSVPMALRLSGILMGGVVIVYERKVKLLYEDVTRLMVQINEAWKVKATVDPTLLPKGKSQAKHASVTLPENQEEELPEIEQTLRNPDTATMMDFEQTSYFAMRLDNADIYDKPNAGEECAPDFHQVDAENITLPEHFESRHTDMSNHFERFDIEGDDDTQMNFTQPEDAQIPSTPVPSAPKEQAHKPDEIPDRYPEDQAKQQSNEAEEAFEQRQDQQRPKPARRRARKAVRLAIDHEQTVISGDVYQSWLKNSSDISSRKRKKRKTMSVLSSMKIARIMEVPPIALLEELFTNGNKEVHYPAPLLKLWMRSTLPPHDSPSGKTSPPYPPEPSYSSPGERMGNVEPGGYPFEHFQGGIGSPSKGISIEKQRANLNNNEIPPEILMENLRANLTNMGLHPTEADGVKETDHMATPGSGDEPRSIPSSGSGHGLLSQNSITNSRSNKKRPHSSSKNSSNGLQPVAEENPWHDPTPNFKLTRLSELSENGVTQDNEILMETGPTQTQRPFVTQPLDMMTETIRKQLKSHFDTPGSAETECLNELTLGLTKKQAACLFYQTCVLATRDFIKVQQEVPYGNILISRGAKM

SEQ ID NO: 88 - DNA, 5853 bp, Capsicum annuum
  source 1..5853: mol_type = genomic DNA
aggtcagttttcctatataaataaaggagttttctctcattataattcatccctcaagagaagaaataagaattactctctctattctctctactcttctttttattctttattgttttatatcaatttgaagattatttcaactttaaacagttttttttcttcaatgtctactcatcattctctctaaacacaacttatgaaatttcactatgtccactcattgtttttcaactcttagaagcacttcatgtccaaaaaaactatacaaaatataattcgaacttaaaaaaaaaaaaatctactttaaattcaaataagtttgctttcaagttcaactcaattcaaatgtaataacaaagtaagtacatataagctcacatatttgagtgagtagatactaacacaatttcattccttattagcaaattcatttccactaatattatatgtcattaccatctaatcaggacttattaatatttacttactatatttttctttcaaaatatccctttttctgtttccatttggcttttattatagtgaaaaaaaacaaaggggaagcgtgagcttttttctgcttgcactaaagtcaagacgaatccccttcaaattcgaattcaaaaaattactcgctaaactcacagcttattcatcagcagcagtacacatgctttcatctcattggtccttcgcatttcaactcgtaaacccagtaatttccaattcaaacaggtgatttttagtgggcccaccctttgtccgctcctaacgaatacctaaactcaatcggacggaccagatcttccctcaattcaaatcacccctctttccccgcctatagcatcatagtttaatcatttatttattgcttttatatacttcacatttcacacacacatatacgcttgtaatagctttcttcttcgtttcttcatttacttgaagaagcgggtgatcgaatttttctattgaagggtatttttggaagaaggaaatgacgacgatgaaccagaataggcgttcgtcggtttctagtgcggtagcgaagaggcaagcaatggcagctaattcatcgtcgtcgttgttggagaataatcatgccgcaaaattgatggccaagaaacgaccggctctatcgaatatctcgaatcatacaactgcttccgctcgtaactcgctctctcattcctctaaacttgtgagtcattttcttcttcttttttttcactcttcaattgttctgtcttaattctgtaccttgtaaagcttgtttaactgtacttttttttaaactgtaagaaaatacttggagtactagggtttttcgtctttttcccgtggtctttttctttgccttttattgttgaactactacaaatcggccaactggcattcaattattatcaaactgactaaatcttttaacactatatcaatttttttcgtatgttgatactgtaaatttgtataatgcagggaaaacgtgggtgggttatgtgatattttgtgggttttctttcttttttaactagagatagttccatggttctcattttttctttttgtgtaagttttttggagggttccttcttggattacgtggggttccatgaggaatatgttaaagaaaaggactgaacaaattagctaaaaatcaatttgagagattgggtgatttctttgctgtcaagattttgatatggcgaagttgtattctttgtttattgacttcccttatataaacaagttacactgtttttatgcgtcagttatcaagggaatccacttgtggggtggatttgtttccctttttattaaaattatgttggagttaaatattattttaatgattaaaaagcattatgaaaggaaaatttgaaacatcttccctcaattttctgctttttgtctccttttgtttgtctgtccacttttctttttgaacgtttgaagaaatgtcttaatatttatgttaatcggttgaagaagactttttgctttttcaaatggacatagcatcattggacaatcatgaagtggattattattttcagatttaacatgaattgtttagcatatcataaactaatggtttttattactgttcctaatttgttaggaaaatgtttatctttgcatgaatgaacagaagaagtttaacgacttttgttaattttgagttttcacagttggatgaaccttttatgtaataagctgttttgcaatgtgagttaatgtttcttgcatctgaagttgggactaacctgaaatcatttttgactttggaaggcaccgtgtacatccaagattgtaagcgttaagaagaacatttctactagcaacagcaatgcagtttcttcaggtactgctgtactgccagcttcctcctctgtcaggccaagcagcaaaactgttgtatcaattcaaagaagtgatgcagttgcgcctaagatcactaccattcctcttcctgctacttgcagcatggacatatcaccgtctcactcagacggatcatcggtctccatggatgaatctatgtcaacttctgacacagtgagaagtccggaggtcgaatatattgatgaccatgaaacggctgcagttgattccatcgagaagaaggcgtgtagcatgctctacatctcagaacatgtcaaagcatcaggtagttttaccttgacgtttgatcttttcagcagagagtagtccttgttctagcattataacatctatttatacaatttatctattttttattccaacagcagatatatgcaagggagatgtacttgtggacttggaatcaggggataaaattgtcaacattgataacaatcttgttgacccacagctgtgtgctacaatggcctgtgatatatacaaacacttgagagcctctgaggtattaaaatgtttacacccttaatctcttttcaattcttatgatcttttaaatttgacgctgctggcaactttaaccacctaataattgacagctttgcaattgctgtttgaaatataaatcgaattgcagttttactaacatttgcgggcatttgtcaaatatgttttaatgtaagctttggtcattgtaataggcaaagaaaagaccttccacagattttatggagagagtacagaaagatataaatcctagcatgcgtgctatcttaattgactggcttgttgaggtaaatttctagtatcttacgacttaacaaatgttgatgaactcagaaattcgtcagtttgatatggatattgattgatgtttaggttgccgaggagtacaggcttgtcccagacacactgcatctgacaattaactatatcgatcgatatctttcgggcaatttgatggataggcaacggctacagttgcttggagtagcttccatgatgatcgcgtcgtaagaaactaccttctgacctctactgcatatgttttcgccatgatccttaatgaattttccttagagtgcttttcatattcttacttcctcaaatattgcaagcatttctgtaagaaagtgctccaagatattaatatgggaaatcctatatatttcagcaaatatgaagagatttgtgcacctcaagtagaagagttctgctacataacagacaacacttacttcaaggaggaggtatatgatcttgattcacagaacctgcagctgttgaactttgcattgggaataacaactgtgtatttattatgcaggtcttgcaaatggagtctgctgttttaaattacttgaagtttgaaatgacagcgccaacagccaaatgttttctgaggttaatatcttactattatctagtactagtagttgtttttaagtatgatgatttaggaacttattgttgagatatactgacaggaggtttgttcgtgctgctcaaggacttaatgaggtaacctcttcacatgtaaaaggatagttctccagcatattttagacaggagacagagttgagtgaaagagctgattacaattttataatcatctacaggtcctgtcactgcagttggaacacttggctagctacattgcagaactctctcttttagaatataacatgctttgttatgctccatcactcattgctgcttctgcaattttcttggccaaatatattcttctcccctcaatgaaaccttgggtatgtacgaattagcattgtggcaatcatacaaacggttacaatgtatttccctgcttattcttattttgacaatatatattcttataaaatctgacttttggaaactcctaaaacagaactctaccttgaggcattatactcagtatcaaccctctgatttacgagactgtgtcatggcactacataacctctgctgcaataataacaattctagtttatcagcagtcagggaaaaatacagccaacacaaggtaattttatttctgatctcttacttttagccccctccgacgatgaagaaggggaatgaaataaagtccaaacatatggtatactttctagatataggcttgcataattccttttttaattcatcccaagcctgtatactcgagtcgggactgcaattaaacattgatgaagagcgataaatgtcttttgaatctttttggataaatgatcgaccttctgaacactaatcaaatcatgttaaactgaataatgacttgatagacatatatgtttatgtacatacagaggcatatcggtatctgcttacacgtcctcccgattttattctagtgtttggttttttgaaacagtacaaatttgttgcaaagaagtattgccctccaactgtacctgtagagttcttccagaacataagcagctaagccagagagatatcagtggaggcattgacttcagttttccaattgattgttggattgattcatggcatttcaacgggaaggaacaatcttatagtttagtcagaaacttgcgatgtccctgaaagagcttcagtcttggttcttctcgccttgtgtggccttagtagagcatctttgtttgtgatcattaacattgacattgcaattagtcttgtactctactgttcttctctagattagttactctagtcagtttgtgtacagaagaagagcaattggcagtttcattaactcagaaaaactattcagtaatatttcttttgcggaaatttttcagtttgtgtcaattaggattgagaacaaacatccaattgatcaaagtcctgattttctcgtcgtcaaatgagcaactggtggactaaattagagttgtccaaaagttgggtgaagaaaacaaactaagcagtaacacattgtgattcaaattctttattttacatctattagttcgctccaactttttatatataataaggattcatcctatatacaccgacaatgttaaaatagttaatactgctactatcaaaagatacattattattctatattttacaaataacacacaagtagaaaccacaaaacagaaactcactgaccacactcaatcttggttgagcctaagccaaaagatacatccgttaaactggcattaggcttaacattcagccagtgacaatcttcaaaagaacagggatgtccaccatttggccattccacatccacaggttttatgaaagttggcccccaagcgggggtcccatcctcgtacgaattgtgggttagtctttggatttccgagccatctgatttgatcacatagatatcaccatatggctgataatgatgaggattcgagatgggttcagccgataccgcagcataatctgaagtaaacactatatacttcccatccgggctgaaatacgggtggttagtc

SEQ ID NO: 89 - DNA, 1491 bp, Capsicum annuum
  source 1..1491: mol_type = other DNA
atgacgacgatgaaccagaataggcgttcgtcggtttctagtgcggtagcgaagaggcaagcaatggcagctaattcatcgtcgtcgttgttggagaataatcatgccgcaaaattgatggccaagaaacgaccggctctatcgaatatctcgaatcatacaactgcttccgctcgtaactcgctctctcattcctctaaacttgcaccgtgtacatccaagattgtaagcgttaagaagaacatttctactagcaacagcaatgcagtttcttcaggtactgctgtactgccagcttcctcctctgtcaggccaagcagcaaaactgttgtatcaattcaaagaagtgatgcagttgcgcctaagatcactaccattcctcttcctgctacttgcagcatggacatatcaccgtctcactcagacggatcatcggtctccatggatgaatctatgtcaacttctgacacagtgagaagtccggaggtcgaatatattgatgaccatgaaacggctgcagttgattccatcgagaagaaggcgtgtagcatgctctacatctcagaacatgtcaaagcatcagcagatatatgcaagggagatgtacttgtggacttggaatcaggggataaaattgtcaacattgataacaatcttgttgacccacagctgtgtgctacaatggcctgtgatatatacaaacacttgagagcctctgaggcaaagaaaagaccttccacagattttatggagagagtacagaaagatataaatcctagcatgcgtgctatcttaattgactggcttgttgaggttgccgaggagtacaggcttgtcccagacacactgcatctgacaattaactatatcgatcgatatctttcgggcaatttgatggataggcaacggctacagttgcttggagtagcttccatgatgatcgcgtccaaatatgaagagatttgtgcacctcaagtagaagagttctgctacataacagacaacacttacttcaaggaggaggtcttgcaaatggagtctgctgttttaaattacttgaagtttgaaatgacagcgccaacagccaaatgttttctgaggaggtttgttcgtgctgctcaaggacttaatgaggtcctgtcactgcagttggaacacttggctagctacattgcagaactctctcttttagaatataacatgctttgttatgctccatcactcattgctgcttctgcaattttcttggccaaatatattcttctcccctcaatgaaaccttggaactctaccttgaggcattatactcagtatcaaccctctgatttacgagactgtgtcatggcactacataacctctgctgcaataataacaattctagtttatcagcagtcagggaaaaatacagccaacacaagtacaaatttgttgcaaagaagtattgccctccaactgtacctgtagagttcttccagaacataagcagctaa

SEQ ID NO: 90 - protein, 496 aa, Capsicum annuum
MTTMNQNRRSSVSSAVAKRQAMAANSSSSLLENNHAAKLMAKKRPALSNISNHTTASARNSLSHSSKLAPCTSKIVSVKKNISTSNSNAVSSGTAVLPASSSVRPSSKTVVSIQRSDAVAPKITTIPLPATCSMDISPSHSDGSSVSMDESMSTSDTVRSPEVEYIDDHETAAVDSIEKKACSMLYISEHVKASADICKGDVLVDLESGDKIVNIDNNLVDPQLCATMACDIYKHLRASEAKKRPSTDFMERVQKDINPSMRAILIDWLVEVAEEYRLVPDTLHLTINYIDRYLSGNLMDRQRLQLLGVASMMIASKYEEICAPQVEEFCYITDNTYFKEEVLQMESAVLNYLKFEMTAPTAKCFLRRFVRAAQGLNEVLSLQLEHLASYIAELSLLEYNMLCYAPSLIAASAIFLAKYILLPSMKPWNSTLRHYTQYQPSDLRDCVMALHNLCCNNNNSSLSAVREKYSQHKYKFVAKKYCPPTVPVEFFQNISS

SEQ ID NO: 91 - DNA, 5082 bp, Capsicum annuum
  source 1..5082: mol_type = genomic DNA
ctgctcattaatctctgtgacaatataaaagtggataagtaaaaataaataaaagaagtaactcttggatttttaaaattggacaagtaaagttagataactatttttaacataaatggataaattatattttggcgcattatccacaacccaccccacgcccttaaagaacttatgccaccctaggcataagtttgatttttagtcaggggtgaacaaaaagtgattcgaccaataacgccaaatcggaaaaaaaaaatgttactagtttatcattgtcggattgttgtgttaatgatttttaaaacaattttgtaaatgtttttatccggctatgagttcggtttgtgattttaatattttagtgaatgtttaaattgatacctcagtaagactatggtaaattatatttttatctctaatcagataatagtggtttttgattttaaatacatatcctattatttttttatattttataattgttgtcttagtgtctataatttgtcttcacgtagaacaaatgaaaattggattaaaaaaaatatagacgagcattttcttattggttaaacatcaaaactgaattattaaggactaaaaatgggttaatcgaaaaatgataacaaatatcttattaattttactttcgatttaacatactcacaaactgaaaatcaatgaattaaactatttatatataaaatcgaatcaaactgatcatacacgatgcaaaaattaaagatgagctttgaagtgcaaaagtcaaaaaccacgctgcaaataaatcgactgaaatttgtcacgttgtcggttccaaaaaattaccccatatacaaaaatgggccgaaatcaaacccgatataaatcagcccatatacaaaaagtgggcctcggtccaaaatatcagcccatatacgaaactgggccgaaatcaaacccgatataaatacttaagcctctgaaattcaaatttcaaatttaccgccatttgaaagcaatgggagaattgagcagatcaaccattttcttctccgatcaacacctctgttacgccgatattctttctccttcacaggtataacaatttcattaaatccatacaaacaatctccaacaaaaatgcaagataagattgcgtatatcgggagctttagtactccgagctgcccctaatagtagtgtagaaagtatggattgcttaatttagacatttaactaaatccagtttatatttttatttacttgcttaatatttgcaatatctgaagtaattattgcttgtgtttgatcgtctcatgtgaaagtttaaactgttagaattgaaacttaatttcattataaatatctgtatttgtttgttttcttatatgatcggatttatttgttcaggtccgagctcgaatcgaagttgccgtcctgaattttcttaaagcactaagttcgaattctccttcaatttccgatctatcactggttagaaatcttactactaagcttttttttttttaatggaatcgactataacttgcaaattagcctaatgtacgcttgttgtgaaatccaaaacggtcgattaatccactgtgtatgaacttttagttgttcaaagtatctatttttctttcggattaagagaaaactgaagaaagatgccaaaattgggaacaaaagttagcaattttgaggaatttatacaatgaaagtctatgtttgccttaaactacaaactagtcatcagtattgggatgaaatacgcctggacatacacggatatagatatttattatagtcttagttgatgatttatagtatatgtgacacagatcagtagaaactcgagcaatagcagagtgagccgggggttacttaccggtgattcatggatcttcttgtcccattcattttgcacgcgatcattaacgaaagaaaatagtgccaagtccttcataagaggtaaaataatacaatttaaccatgagattacttaatagtataagataacaatgctcactgagtttttgtgtcaagtttggaaggttatggaaatctgctaccaagttctggttcaggagaaaagggtgactcagagagagctatattacaagctgctatgtgattcaccagattatttcacttctcaattgcaggttaataggactatccaaggttaatgatgtttctgggtaatgatttgtgtgtttggtccattttgttaatgtccagacccaactgttggattatactgggtgttgttgttgttcgttgattggttaacgaggtcttcatttactatctatgaggaacagacttggtggctttgcttcgatgcagccgttatagtcttggaataatggcatctagcagaggggcaatagcaggccgtttattgttgcaggtagtactattcctaatcctttcattgtaattactgctgtccacacctatgttgctctacttactgcttttttagaatccacagtcaatttaatcaaacacttagcattgttagtagcttaacttggctcgtagcatgatctgtcatatatgaatgaaatatattgacttgtttacaattgaggcagtgttgattgcttgatatgtttatgagccaacctagtcgaactttttaatgtttccaagtttcgatagttgctaaagttagctgctggaggctgtgtatgataaactattctgctttgtttcttctgattttgtgtgaacaatcatgggacttaacactctattggaaataacctctctacctctcaggtaggggtaaggtctgcgtatactctactctgcccagaccccactgcgtgggattacactgggtatgttgttgttgttttgttgttgtaatcaaagaacttaatacttaaatgtacaagtcttacagttacccatggtcaaaaatttgaaataggtagttatccaacatttagaacttggtatttttttcttgcaaaaatggatatatgacttaaccttgcttctttaaaccactgagaaaggagccagacaaggaagttgttgactgctctacttgtggatcttcgggttatgctatatctggagacctggaattgttgggaaaattaaccatgggaacagatgcacgatacatcattatggtggaaaaggtattttatcacttgttggaaactttagtcaaatcatttttgcaagaaactaaaagtagttccactttttagcatgctgtattccagcgactagctgaggatcgtgtattcaatcaaatcccttgcattttgatcactgccaagggattccctgatattgccactaggtgaggttgaagagttatgaatgtattttctagctcacagaatagctgctagaagactgtccattcaattattaactcttaacatattctaatctctaaaaactttcaggtttctgctgcatcgaatgtgtaagatgttcccaaatttgctagtcttggggctggttgactggtataaatgaattcactagtgtaggaaccatattagatgcagagtaaagttcttattcacagcttcgaattctgatctttaaggaatccggctggattagcaattctttgcaccttcaagtttggtagcatagggatgggtcttgaagcatacagatatggtgctcttttctcttaaagagttgtgttgaatcataagtccatgctatcttaacttcacttataagaatctgttactttacatgttattttagcttgcaacatcaagtggttaggactgcgaaaggatgatattaatcaacttatacctaaagaatgtttggtccctttgaaacctcgagatctccagattgccaaaagcttgatgtcatcagagattctgcaggtataattccagttagtatggaaacatcattctttcttcattagttggtttgaaaaatcatatgatatcgatttctaccaggatagctacaaagaagaggtggcagcaatggttcagagtggtcgaagggcagagattgaagctctatattgtcatggatatgattacttggtgaagttccttgcaacaaaaatagtacaagccaattacctctgataatttgccattcatagagaacaggtactgagaaagtactgcattttctagacattcagcaatttactcggaggattcagttttcatattgatccatgctcttaatatctatcatatgttgtatatgtgtttcgattatagtactattttgtggttgattattgtctctttttggtagactttgcaccctttccttgctagttgctatattttctttacttctggatttaccatacttgagccagggtctttcgaaaaaagcagtggtaaggtttacgtacactttaccctcctcaaacctcacttgtgggatttcactgggtatggtggtgttgtattcagttttcatattatcccttttaatttctttccttgtttttttggcaaaccaatccaagtccaacttgttctaggagaaggagtagtagaagtggacgttatatataacggtaactcagtgagttttttggcaaaccaatccaggtccaacttggtctgggagaagcagaagtagaagtggacgttatatataatggcaactcagtgatccaaagtccactcaccacgcgacataattggactcactccaatattctcaatacaatacatatagccacaatcaccaaccatcaacaagacgattactttttcttatcgtgattactttgtaatttctcgaaagtactaagaatttaaagcgactaaagtatgagcacacctagcacaaccacggacatgacattgacattaaagagaagcataacagaagaagaatcagtggagaaattcgcgatggcgaattgtgtggatataatgaagaggaacgagttgtcaggacgacatgaactcttcaagtgcaagacatgtgaaaaacagtttgattcattccaagcacttggcggtcatagaacaagtcacaagaataagaagaataagctcatggcaacgagtactaacaataactcattacccgttaagcccaagaaatataagtgctcca

SEQ ID NO: 92 - DNA, 1380 bp, Capsicum annuum
  source 1..1380: mol_type = other DNA
gcaatgggagaattgagcagatcaaccattttcttctccgatcaacacctctgttacgccgatattctttctccttcacaggtccgagctcgaatcgaagttgccgtcctgaattttcttaaagcactaagttcgaattctccttcaatttccgatctatcactgatcagtagaaactcgagcaatagcagagtgagccgggggttacttaccggtgattcatggatcttcttgtcccattcattttgcacgcgatcattaacgaaagaaaatagtgccaagtccttcataagagtttggaaggttatggaaatctgctaccaagttctggttcaggagaaaagggtgactcagagagagctatattacaagctgctatgtgattcaccagattatttcacttctcaattgcaggttaataggactatccaagacttggtggctttgcttcgatgcagccgttatagtcttggaataatggcatctagcagaggggcaatagcaggccgtttattgttgcaggagccagacaaggaagttgttgactgctctacttgtggatcttcgggttatgctatatctggagacctggaattgttgggaaaattaaccatgggaacagatgcacgatacatcattatggtggaaaagcatgctgtattccagcgactagctgaggatcgtgtattcaatcaaatcccttgcattttgatcactgccaagggattccctgatattgccactaggtttctgctgcatcgaatgtgtaagatgttcccaaatttgctagtcttggggctggttgactggaatccggctggattagcaattctttgcaccttcaagtttggtagcatagggatgggtcttgaagcatacagatatgcttgcaacatcaagtggttaggactgcgaaaggatgatattaatcaacttatacctaaagaatgtttggtccctttgaaacctcgagatctccagattgccaaaagcttgatgtcatcagagattctgcaggatagctacaaagaagaggtggcagcaatggttcagagtggtcgaagggcagagattgaagctctatattgtcatggatatgattacttggtgaagttccttgcaacaaaaatagtacaagccaattacctctgataatttgccattcatagagaacaggtactgagaaagtactgcattttctagacattcagcaatttactcggaggattcagttttcatattgatccatgctcttaatatctatcatatgttgtatatgtgtttcgattatagtactattttgtggttgattattgtctctttttggtagactttgcaccctttccttgctagttgctatattttctttacttctggatt

SEQ ID NO: 93 - protein, 382 aa, Capsicum annuum
MGELSRSTIFFSDQHLCYADILSPSQVRARIEVAVLNFLKALSSNSPSISDLSLISRNSSNSRVSRGLLTGDSWIFLSHSFCTRSLTKENSAKSFIRVWKVMEICYQVLVQEKRVTQRELYYKLLCDSPDYFTSQLQVNRTIQDLVALLRCSRYSLGIMASSRGAIAGRLLLQEPDKEVVDCSTCGSSGYAISGDLELLGKLTMGTDARYIIMVEKHAVFQRLAEDRVFNQIPCILITAKGFPDIATRFLLHRMCKMFPNLLVLGLVDWNPAGLAILCTFKFGSIGMGLEAYRYACNIKWLGLRKDDINQLIPKECLVPLKPRDLQIAKSLMSSEILQDSYKEEVAAMVQSGRRAEIEALYCHGYDYLVKFLATKIVQANYL

SEQ ID NO: 94 - DNA, 13918 bp, Capsicum annuum
  source 1..13918: mol_type = genomic DNA
ctcctcccctcccctccactctattccctgttctttttcctctgtccgctgtttctcattcttgtagactctagtttatggttagatgatgggagagattgacaaaccaactgtaacatatgcggcgctgttgtctgattaactaacattttctgtgttttaggtggttctggagtctggaccttcttgataattttaatttaagttgtcttttccattaattttctctttgaactcttgctagcatagatggtcactcttttccagagttgatcatcttggtgtgcagatttctctttgttcttccttttgtgttattcatagcggcgtgcactttcttgtaaataacatcacgcgtggaattaaactgcgtatgttgttcttgtaaactctatccgctagtcttgtcaaaaaacgaggagcaactttgcaacagggtgacagtcgtttcaatatggatattcaaacaccgttaggtaattttaaaattaaccgcaaggggatcagttatggttgatgtcatttgataatcaagaagaaaattatacacaagtataaattggaagaaacaattatatatttcacaccacattacatattttcatcattttgccttttctcaatttctcacaggcttctcatattcagctcatgaaattgttaactcaaattaatatgcatacaattaacttctttctttatctctctctctttttttttttaaaaaatttatactgatggtaggttcattcattgtcacaaaggcataatgggtagtattgttttttctgatgtcaataatttaagattataaattgcttgactttgttttggaaaaccgtaaattattttcccttatttatttatttatttatttatttatttattgtttaagcgtaagcggcaagataaagcatacccctaaggcagagagctccaggttatgattgttgcaattggcggggtatagagtactctgcatactgcaactacagcagaaatggaaatggaaatctcctctgtgaaaatgctctataaacatgtgaaattttttctcatttctaatacactttttttggcttggcattacttaaaatttattcaccccagtttcacactttttgcagctcattttctgcgccgttcaacgatgccgcatggccgattatctctgcagattaaccgtgaagttgacccccgtctctcgatttggcctcccgctcgttcgaatttcaggcgatttctctctccatatgtgaactactgtgtatatgcgtgttcctaaatatgggcacgcgcgcgcgcacacacacatttctaattgactctccgtttagaaactcctatctgttgtatcaatgtatgacgtaattatggatagagtaaaggattaaaaacatacctaaagtatctcagcttttcgtgtttcatacatgaagaactatcatatcaggtctgcgagttttctaactcaactatcaccaattatcaggtaggaaaacgaaataatcaaatgttggcttgaggtgtgttataagatatttcaagtgtgatttttacctctaatggatgtctatgatggcatagaacacgtgtcacctcgaaatgattcaatttgaagacacattgactagtttttagctggatttatgaaattcacatctgtgtgcaattttttttttctccaaatataatcagtataataaattcattctcttctccagaattcaaaggattttatttaatctattttaccatggccttcaactgacagtgattctactcctttttctgggcttgggactggcttcggtttgcgtagctgtcattgtgggattaatttacaacactagctatttatagcttttagttgagagctcaaataagtcagagttgcaacttaacaagtggtttgtccatgctaatctgtgtagttcaaattttcaatgattttttttgcttggaatagggaagggaaatgatttcgcgtttaagaaacagaatacggagtagtaacttcgaattgcagtttgctatatttttttgatgcagttagcagaatctatgataatgaatcaatgaattttctcatgaacagtttctgataccggtgttgggagcaaactggaggactatcagtatttgaaatacagaaatgaccctattctagctaatcaatggggtaagcatttggcaattacatgcttgttatgttttgactattgtttcccgagttatatttgtcacattagttgtaactgaagtgcaaatagctttggttcaaggttcaatagacacagagctctcatctaaacatatttgtgtatcgtacaaatgaaagaaacaagaactcacactaaaagaattttgattaacgttttaagatatatattttttcaccacattgatatgataagaattgcaacttatagtactttttgtatagtttttgaatattgaaatgttaattctaaaatatggatttgatctaagctaatccaatttagcttcgaagattagtaagattgactattgagaagcgaagaatgacacatattttgggacaagggaagtaatgatctattctcttgtttatacacaacaccgagatcatttgttcatgtggttcctagatggtgcatgttgcatataatccatgactctggactttattctggctgactaaaatgctgattaaagcgctagaaaaagtcaccttctactccatctcttggatatgaagcataattggatgcacaacttgaggatacttggaacattgttctccagattgagctaacagagtaggaagctgaaaaagaggagagtattttggggtgagatggaagagaaagaaatatgacgattctagtggctaagtgccagaacatttcagccagtgatctggttgcataaatgtctctgtttaactcccatggttgccgaacaagaaaatggaaaacagctaaagagatgaaaaataagtgactaccattagagttcaatttttaattattctgctcacggcgtttcacaggtattgcggctcaagattttgtgtctctgccttttatgttatcctgcctggaagatacaattaaaagccttccataagttttgttctacggcctgtgagtgtgctgataatatagtgtatcttcacattgcagatgggatgctttatcttgcaactacaagtaagtgtgcccttcttgatgaataattctttttcttggtcaaattttgttttaggacaaaaattgagaagtttcgtaaatatatttttatatatgaaaatgttgccatggaggtcacgggttcgagctgtggaagcaacctcttgcagaaatgcagtgtaaggctgagcacaatagacccttgtggtccgggctttccctaaaccccgtgcatagcacaagcttaatgcccggactgccccttttttgatgtaaaaattaagttgtatcaatgaagtactgtaactacttcaacttcaaaggatgaactacttgcttgccttctgctcctctgaacttcgctactttactttagttttctaaaacttgtaggggctgagatgtggtttatttgtagtgcagttcaattagtctatgctttggtggcagtttgtaaatgacagtctgcacacacattactctagctaatactactttttcctttgtcctttgagggatgtgatactcaatgaactttacagcggaagattagagggattgttctaaagctggagatacttataggttaaactaatggcaaaacattttcggtcttcctattcaaacagtctcagaaccttgaaatctttaaatgaaaagaggcattaccaataaagcaagtccacattttctttatggcaaattgggatcagctttttactgaaagctctcatcgctaactctgcactgaatcctgtcaagtcacgtcttgaatgatacagttccttagtcattaaactttagtgagagaatacatgttcatatgtaatgtcttctgataggatgtatccacaaaaaaaggggaattgatacagtttggcagttcattgaactttatgctgtaattcaacttaagaaattccaatcaagctcgcgcagtttagcttagggtgctcactatctactagtaataatctgttggtactgctttggaagaatgatatttggatagaattatattcatgatgacaggtttatataattcacctataaagcatatttgttacttttgacaattacgttaagttcaaagtactccaatcatctcattggattgagaatatttggtattttaaactgagggatgaaagttgcaggcgtatctgatagtgagattcacaatttaaacttaaatctaaaagaatctaattctgttgggacactgacaaagctaccatcaactgcaaagaatggtgccaaattcaggtataacactttcaggggctccatccacgtaatgctaatcttatgttaattttctcttgaccgtgcccatgcttcccgttctatgcttcggtctttcagcacatggttaattagttataccttgcagtgggactgaagtatcagtatcaatatccaaaagccttgatgacttattggcagaggttacttgctttcttcaaaaggtgcagttttcatgtctatcagctgattctaccaatgatttctcaaattataaggaaatttccgttaactacagttttccatggcattttatgcagatgatccttttgaaggttccggttagtgcattacttttcttgaaatgctttatattcaaatcaaatgcaattatctcctctatagaccctctcatagttcaaaagcaaatgtgacttggttgatataatgatagctactaagtatccatgttatttcattgaaccgctacaagatcaacaattccataagcttgggcttctgttgctgacataaaaacatctctttccatatctttggatacaacccagaagggtttgcccgttcattgtacataaacccttgtgcgggtttcacgcagtttcagcagtcttccgcttctacgacacattcggttacttgtgccatataaaaaccactagcagagcaaagttcagttcatgagactgcagcgcagcgcagcggagcagccgcgacactttcttaccttagctggatctaactgctcagacagttcaaataggatacaatatcaactatggacctaccaaatgctagtgtttagtttttggatgggttcaccatgtcaagaatttttctgtcagttatcagaatcgcattaagattcaaatatgttaagcttttatatcattttacccatgctccttggccttattgtatttaaagagcttatgttttcgttatcctgtttcctaggaaatagctagaaccactacctctgtggctgatagtttgtttctttcttacagaaagttgtaatggaactcttagtaggtggtgatgactctttgggatcacagattggaagtcgtattctggtaatcgagggcagctctgtgtattctcctgttgaaagcataaaatgcttgaaattgggactcaaggattatgttcgtaagcaccaaactcgcttctcagttgggtgagtactagaaaggtgctacattttggctgatgaatgatgcattctgacatctactttttgttgaagggtggaggtaatgtgttaatagttctaacttccacatgttgaaataataattcttagttgctaaatttttttctttttttaagaaaaactaaagctactgctatgcgcggtgtccggggaaggaccccatcacaagtgtgtattgtacgcagccttaccttgcatttctgctagaggctgtttccaaggcttgaacccgtgacctcctggtcacatgacaacaactttactagttactcctaggctccccttcagttgctaaaataaaaagataacaaatattacttggcaatgctattttttgttttttcgttgtccactttgacatggtttcgctgacctttgtcctttctttgctttacatagactgttgcatctacatctttaaattagtcctttcattctgcaatttgcccattaaaaagattcaacatttgcatttcttcacgctttcttgtgtggtttgttagtatctctgactgttcattatgtttcttcagtgtcatgttaattagtgcattatttttctgaaacgtacaatttgtaaatttaccttcttaaaagactggtctagacaaatagtttaggttgagtgaagatggaaaagagaaatatgggatgcactggaccaggtgatagaaaattagagctaaacataaaagggagtgctagagctcaagccatggaagtagagtgaaggagaagtagaggcaagacgattgatcacagcaacttaaactcaagttttctataatctggttgacagttcaattggctccttctatattttgatataggaggatttaagtttgctaacattgtttagttaagatctattggtggttcaaagctagaaattgcaacggatcatatggtatgtataaaattccaacatctcatataagatctttggagaggcaactgtggtccagagccaaaaacaaaaaaattaatgtatagtgcattgagacaagcttgtatgtaaagttctagtttcttatttcagggaaaacctaaaggttggaactggggttgctaactcttcaggaagttctcagggcaatagccaggtggtggaagctgtggtgattatcagtgagatgtctgaactagttccttcttcctgcatcagggaacaagacatgaaaacagaggtatgctttagattattaattaaataaagctcttaaaactataaaaaatgtttggattccagcatgcgctttataggctatgttgtatcaaatatagataatagttttcactgtatagatgtcttgtcgcatataagttcgagttcatttgttgtcaagttcatttgttgtcctagaatgcatggattgaaagctaatgataatatcttagatatgcattgtttaatgtcttcggaattccgattttcagggttcttttatcaggaaaataaatctctggtttttacataaagcatggagcacaaggtgaagaacctcgtgcgccctgtggtgtatggaggccaagatttatgtgcaacttcctgtatatcatggagtagagagctatttatgtgagtagtaggattaatattgcgtgtgttcgggagactaagtgggtaggtactaaggccagggatgtggatggtttcaagttgtggtactcaggcggtgagaggcgtcgtaatggagtgggcatcttagtcgatgaagagctaagagggcaggtggtggaggttaagagggtcagtgataggctgatgacaattaagttgatcataggggggtttacgctgcatgtgtatagtgcgtatgcgccgcaggtgggcttgggagaggaggtgaaagcgagtttttgggaggctttggatgaggtggtgagaagcgtgcctagctcggagaagattgtcatagcgggggacttcaatgggcacattggagtttcttcgggaggttatgatgaggtgcatagagggtttggtttcggtgaacgaaatggtgagggagttgctctgttggattttgcaagggccttcaggctggtggttgtgaactcgagcttaacgaagaaggaggaccaccttattacctttcgaagcgcatcaaccaagactcagattgactttctgctgcttaggaagagggattgggttctctgtaaggattgtaaagtcattccgagtgaacatctgtcgactcagcacaggctgctggtgatagacttgtgtatcagaaagagcaagaagagtagggctggaggggcggcctagaattaggtggggtagcttgacgccagttagtgcgatggagataggggcgaaggtggtaggtttgggggtgtgggagagtagggggatgtggatgtcatgtgggataaagcggccagctgcatccgggagatggctagagaggttttgggtgtttcgaggggtcgggcaggttgacataagggggactggtggtggaatgaagaagttaagaagaaagtggagactaagaaatggcgtatgttaagttgattgagagtaaggatgaagagaagaagcgggtgaatagagaggattacaaagttgcaaggagtaaggctaagttagctgttacggctgctaaaaaagtggcgtttgagagcttatacgtggggttggaggagaaaggggggaaaataggttgtataggcttgctaaggctagggagaggaaggggcgtgacctcgatcaagtgaagtgcattaagggggagaacggtagagttttggtggaacatgagcacattaagaagagatggcaggagtattttcatagacttttaaatgaggatggggacagaggcattgtgttaggggagtcggagagctcggaggagagccgtgatttcggttactgtaaacgttttatggtagaggaggttagagaggatattcgtaagatgcggagaggtagggcgacggggcctgacgagtttccggtggaattttggaagtatgctggtggggtaggcttaaggtggttgactgatttgttcaacgccattttcaagacagggagaatgcctgaggcttggagatgaagtacgttgattccgttatataaaaacaagggtgacgtttagagttgcaataactataagggtattaagctgttgaaccacactatgaagatttgggagagggtggttgagcggaggttgaggagggtagtgtccatttcggagaatcaatttggttttacgcctggacgctcgacgacagaggcaatccacctgatgagaagattggtggagcagtttagggaaaggaagagggatttgcatatggtgttcatcaatctggagaaggcgtatgacaaagtccctagggaggttctttggagatgcttagaggtgagaggagttccggtggcgtacatcagagcaattaaggacatgtacgatggaggaaagactcgggtgaggacggcaggaggagactcagggcattttccggtcgagacaagtttgcatcagggatcgactcttagcccgttcctttttgcgttggtgatggatgtgttgacgcggagtattcaaggtaaggtaccgtggtgtatgttatttgcggatgatgtagtgctgattgatgagacacgggggtgtgtgaatgagaaattggaggtttggaggcaaactgttgaatctaaggggtttaggttgagtaggtccaagacggagtatttggaatgcaagtttagtgactcgagtcaggaggacgatgtggtgttgttgttggattctcaggatgtttgtaagaaggatagttttaagtatctggggtctgtgattcagggaaatggcgagatttatgaggatgtcactaaacgtattgacgcaggttggatgaagtggaggctcgcctcgggagtgttgtgtgatcagaaggtaccacttaagcttaaaggcaaattctacagagtggcagtccgtccggccatgctgtatggagcgtagtgttggccagtcaagaactcccatattcaaagattgaaggtggcggaaatgagaatgttgcgttggatgtgtggactaactagagaggataaagttaggaatgagattatccggaagaaggtgagagtggcttcggtggaggacaagatgcgagaagaaaggttgagatggtttggacatgtgatgaggaggggcacggatgcccctgtttggaggtgtgagaggctagctttggatggtttcaagaggagtagaggtaggcctaagaaatactggagggaggtgattaggcatgacatggaactgcttcagattactgaggacatgaccctagacaggaaagtgtggaggtcgcggattagggtagacggctagggtgagtgtgtaggtaatcgctaggtgataggggagtttgagtgtggtgggtggtttaggcctgtgagggcatgttactaccacatgggtatctatgttcttatttcatattccgtattgttcgtatttctcttatttcccatttctttgagacttagtgttcttatttttttatctcttattgctgttatgctatacaacctgtttcatgtctcattacgaccttggtatactattctctatcttgagccgagggtctattggaaacaacctctctacttcctcggaggtagtggtatggactgcatacattttaccctccccagacctcactttgtgggaatatactgggtctgttgttgtagtaactgaaatattttcaaattttgagggtcagtatgttgatctttttctttatggtcatcttgagacaacaactatgtctcaattccaagcaagttggggttatcctcactgaccatgtggctccatgtatgttcataataggcttacatatcatgaaaaaaattatgtggaaagtatgattatcatattgtaataaaaaataaagtattttctaaaatctagagtatccccattgtacaccaaacaagatacgttaattatccagtcatatctactgtaaacagatatgatctctggtattgagtttaattaagtattgcttacaattcgaagatatcaaaagttttcgctaagtgaatcatccaagtcaggttgattttttcaggaatttctagtccttacagtagtttccgcatattccgtaggtatgttggaagctcaacggaacaaagacatgttaaaaggcactgtgtgtgtcttagcatcaatccagagttgttgtatggtatcaggatgatgtttggtctgctaacattgtatgcgtcttttgcttatttcataaaaccattcccgcaggctttcaccttctgtggtggtggttgtttggttggtttggggggtgggggggtggagggggttctacatcacatattacttaagccaaaagtatacaaaggaggattccaacattcaactgccatctgttcggagtttgatatatttttgagtaggtttggtccagtagacagtgatacaagttagctttggctttaagttatctactaaccacgaacctccctccagttggagtttaagttagtcaagccaaagtcttctgaaataactatcttcaaattagcaaaatattttaagcaattttttaaaaattaagttccctgtatctgtttgatgaggtgctgttgaagtttcctagaatcatctctgagcattacttgctcgtcttcttttagttgagccagtatctcacacgcctttccattttcttttcagtactagagtttgtttgtgttttttgatttgtattaatgatatctatgcctgattccaggtcttatatttcgaagactttgtatcttgttctattgctcagtcatcccttgatgcattgacaaacatcaactggaaaagctatgggttggctctgcggagcattgcaaatcatgatggtagtgtaatgctggaatgggagaacctgctaccagatttccacattcatattgccatccattgttaccatagacaatatccatcataatctaatacacatccatgataattgacatggtcacatactcctattgtttgcaaacaatgagaattgttttgcatgtgtgttttgcttaacttgctgacaaggtaaaacagtgggttgcagaaaacagtttacctgatcgaaatcttgttagaaaagctgtcaagtgtgctttggatgacttgaaggaaaataatcaaggggttctcctaagtagacgtgcacttaaggtaattttgtttactcctctgcattctgtctggtcattgcattttctagttcctggtattagcttagctatgaacaaaatatcccccattctttgatccatattgcattctttgaatgtccatacccaaacgtgcggcagaaaagtagtttgtatgcttttcttttgatacggatcattaaatattggttgctaagcagatagtattcagtaatcccatctggctaagtagttcccttacacaaactagtcatgctttagacactaaattctttaaactccatctgaagctctatatgactagtgctgattgaatctgaacaagagatgacagttattcaaacacaactaagaacaatggttggcaagaaatatactctcattgcctcattgaggatgaatgcttcatagaaatagttcttttttactgggggtggcttttgaagcatcatccgtttagcactgctgttctcacttttgtcagagcatttttattagctggaagtgcatatgctttcctatggttctgtagagtccttgtaaattctgtacctagtccattgtcgggggttacgtagtatggcaatagctgatgttaccgcaatctctattccggacattagctatatattggaatagtttgtatctgcgtgtatatttgtattaatccactgctactacttaggataggtgctaaagtgctaacatctttttttccatcgcagatgtgtgattatgcacctgaccttgcaaaaacgcttgctcagctgatcttatcctccaatgacttgaacttccaagaagaatgttgttctcttcttggggtacagtctcaggaggttaacatggataatgttggaaattgcatcagggagaagataatttcagtgattggattaaatgatcgcaactcccagaaaaataaagaagccccaaccttcctctttgaagacgattgtttccagaaagagcatttcatggaggaggaatatcatgaaggtgaagaagcttacaactttttggatctgtagaaggttaggagatatgttagatgtccaattattttttttttttcctcttattatgtttatggtttatcaatcaacctattttcgttacttctgttgggctttattatggttttatgattttgggggggggggggggggggggggggggggggcacaatatgtatggatttcatggtctttgagttttttggtccgcagtagataaactgaagtagtttgcacgttgaactaatatactcaaccacctctacaacgctgtggaaaaacagaatataaatacttccaaatttccattaacacaaattttacaggtataaggtttgtgtatacactaccctccctagagctcactttgttaggtatgttgttactgaaatatctaaatcatcttttaccgagatattttctggtttctgaatacatcctttaaacctttcgactagtatctcctacttacttcgccttgttgcttgaaaattttcacttaaaatatcagactcgattaattcgtcttgaattaattataaattaaacaaggtttactacatttagtctaaagttttcttggtattaatttcagagagcgaaaagtgtaaagatatcaagtatgtaaatgtactgacaaaactataattgagtgagacaaatatatctatactgcatccgttcacttttacttcattttatatgttggtattttatcaaaatatttatattaattgatatatggttttaactagctatattgtacgaggcaaagtatcgaacgaggatgctgcaatgtatgtgtaggtttactatgagagataagattagaaataaggttatccgagatacggtgagagtgactttagtggaagataagatgcggaagcgaggttgagatggttgaggcatggtccagtgcgggaagttgactatggatgaatttaagcgaggtagagatagtccgaagaagtattggagggacatgaccctaaataaaaaggtgtggaggatg

SEQ ID NO: 95 - DNA, 2018 bp, Capsicum annuum
  source 1..2018: mol_type = other DNA
gactttgttttggaaaaccgtaaattattttcccttatttatttatttatttatttatttatttattgtttaagcgtaagcggcaagataaagcatacccctaaggcagagagctccaggttatgattgttgcaattggcggggtatagagtactctgcatactgcaactacagcagaaatggaaatggaaatctcctctgtgaaaatgctctataaacatctcattttctgcgccgttcaacgatgccgcatggccgattatctctgcagattaaccgtgaagttgacccccgtctctcgatttggcctcccgctcgttcgaatttcagtttctgataccggtgttgggagcaaactggaggactatcagtatttgaaatacagaaatgaccctattctagctaatcaatgggatgggatgctttatcttgcaactacaagcgtatctgatagtgagattcacaatttaaacttaaatctaaaagaatctaattctgttgggacactgacaaagctaccatcaactgcaaagaatggtgccaaattcagtgggactgaagtatcagtatcaatatccaaaagccttgatgacttattggcagaggttacttgctttcttcaaaaggtgcagttttcatgtctatcagctgattctaccaatgatttctcaaattataaggaaatttccgttaactacagttttccatggcattttatgcagatgatccttttgaaggttccgaaagttgtaatggaactcttagtaggtggtgatgactctttgggatcacagattggaagtcgtattctggtaatcgagggcagctctgtgtattctcctgttgaaagcataaaatgcttgaaattgggactcaaggattatgttcgtaagcaccaaactcgcttctcagttggggaaaacctaaaggttggaactggggttgctaactcttcaggaagttctcagggcaatagccaggtggtggaagctgtggtgattatcagtgagatgtctgaactagttccttcttcctgcatcagggaacaagacatgaaaacagaggtcttatatttcgaagactttgtatcttgttctattgctcagtcatcccttgatgcattgacaaacatcaactggaaaagctatgggttggctctgcggagcattgcaaatcatgatggtagtgtaatgctggaatgggagaacctgctaccagatttccacattcatattgccatccattgttaccatagacaggtaaaacagtgggttgcagaaaacagtttacctgatcgaaatcttgttagaaaagctgtcaagtgtgctttggatgacttgaaggaaaataatcaaggggttctcctaagtagacgtgcacttaagatgtgtgattatgcacctgaccttgcaaaaacgcttgctcagctgatcttatcctccaatgacttgaacttccaagaagaatgttgttctcttcttggggtacagtctcaggaggttaacatggataatgttggaaattgcatcagggagaagataatttcagtgattggattaaatgatcgcaactcccagaaaaataaagaagccccaaccttcctctttgaagacgattgtttccagaaagagcatttcatggaggaggaatatcatgaaggtgaagaagcttacaactttttggatctgtagaaggttaggagatatgttagatgtccaattattttttttttttcctcttattatgtttatggtttatcaatcaacctattttcgttacttctgttgggctttattatggttttatgattttgggggggggggggggggggggggggggggggcacaatatgtatggatttcatggtctttgagttttttggtccgcagtagataaactgaagtagtttgcacgttgaactaatatactcaaccacctctacaacgctgtggaaaaacagaatataaatacttccaaatttccattaacacaaattttacaggtataaggtttgtgta

SEQ ID NO: 96 - protein, 503 aa, Capsicum annuum
MEMEISSVKMLYKHLIFCAVQRCRMADYLCRLTVKLTPVSRFGLPLVRISVSDTGVGSKLEDYQYLKYRNDPILANQWDGMLYLATTSVSDSEIHNLNLNLKESNSVGTLTKLPSTAKNGAKFSGTEVSVSISKSLDDLLAEVTCFLQKVQFSCLSADSTNDFSNYKEISVNYSFPWHFMQMILLKVPKVVMELLVGGDDSLGSQIGSRILVIEGSSVYSPVESIKCLKLGLKDYVRKHQTRFSVGENLKVGTGVANSSGSSQGNSQVVEAVVIISEMSELVPSSCIREQDMKTEVLYFEDFVSCSIAQSSLDALTNINWKSYGLALRSIANHDGSVMLEWENLLPDFHIHIAIHCYHRQVKQWVAENSLPDRNLVRKAVKCALDDLKENNQGVLLSRRALKMCDYAPDLAKTLAQLILSSNDLNFQEECCSLLGVQSQEVNMDNVGNCIREKIISVIGLNDRNSQKNKEAPTFLFEDDCFQKEHFMEEEYHEGEEAYNFLDL

SEQ ID NO: 97 - DNA, 8721 bp, Capsicum annuum
  source 1..8721: mol_type = genomic DNA
gtggtaatataaatatcatattttgaatatatcaaaattaacagaaaattatttctgataaaacttttattatataataatagtattttaacatttttaaatttactatttctgtttaaaatattaataaatcattaaagtaatataaatatatcatcacttacacaactttatctatattaaaaatattttagaagagtactaaattatatttctaccaaatatcaaactaaattaaataatccataatatatttagatattactaaaattttcaaacgaacagcttaggaactgatctatcggtcccagtaaatgataaataagttgaggtaattataaaaaaatttagacaccaaaaatatgtgaaaacacagaaaatgatcgtgaagtttattacaataagttaatcacaattacatatatgtctcctcctttaattgtcacctgcgtctacataaattgaaacaaacatgaggttttactcttaaattgaggccaatgttaataattaaagaattttacaatatactcgctccatttcgttttagttggcctttttttaaaaaatatttatttcaatctaattgttcctttaatgaaattaagaagattttattatgttcttctaatactattcttaacattaaatgactaaataaaatgtatttactcaaatttatattttcaaaatatagggctaatttaataaaataaattcctaattaatatttttttaataggtgtgtggatcaactaatatgaaacggagtaatagtttgctaagttcaataaccatgcctaaaattaatgaacatgaatttaggccctctccttcacatataaattacgggaagtatgacctaaattcagattagaaattagaactaaagggacctcttggttgtcagtgtatatatatttcgaattcctaggcaaaaagggtagccttagcatctttgtttttcgctcttcactcacgcacacagtacagcaaacaaatgtatttcgccacgcctcacctccaccacttgccaccgtctccaccggtaacatgcgctcaaggccatagctcgactttgattattctaaccgatgaaggcggatcaatatgcctgctctgtttgtccaatctcatttctaatccgatatcgccgactgttcacgtttcatacgtgctttcacagttatctatcgcgctttctcaaccgagttttcgccaaaccttcttcacatttcactctcatttcctaatttcgcctttagtcggagttctatcttccttcgatgatgagcctattgccaagcaaactatggatttgattatgcagttgtgtgaacctccggattgtgatgtgcatgcggagtttgtggctcggcttgcagatcgtctttctagtggctctttagcttggagtcggagacagcttcacacggtaacctttccttctgtaataatttttgaatttccaatttatggaactgtaaaattgagaatggatctgttgaaaggtatagatactcgtactgattcaatttgtttggcatagtttgacttgacacaaaatttaagaaatgaagtaagacttttaaaacttgtgattttttaaacattcactattatttgagtgactagagaacttttggagcttgtgctcttaatcatgacaaaatatctgtgtggcaacaaaaacttatcattaaagaaatatagaatttgtgtcagtctaaaatggactaataaggaaataaaagtggaatggaggaggtatctggttttcctaatttcctcagtgtgcctgtgcaacttcttgtggtggtggacaactgattgtgatcagtaaagttttcggtaatcaaaatgattttgaatttgatgatcctgttaagatttctattaaaaccggtgttggcagtatagctttattacaattagctcttcttcaatcccgaagataaaatacagcttttatccaggagtagcttttccacggtgatttggcactgctatcaatttcagtgagtcactgacattgactaacagcagaagtttaagcgcagacattgttgcagatttgattggaaaatcacagtcaggatgaatccaaagaatattagttttagcattagcggctagtggaaagaaaaaacctgtttaggtagttagttcaaggttcagtgtcagtgttcatgtccatagaaaagtctgttgttgatgaaaatacgaatgttaccttctcaaaataaaataaaatatataagatgttacgaaataagcaaataaaagatgggagaaactataaataatgttgaacttgtgaaaattttgagtggactttaaaatggcaccattcatagtagcttcacactctatttggtgcctgccagctgctgacctcgatgtgcaaactgctcatttttgagacggtaccctttgtatgtgattgatttcctcattgagaagctagatgaacaagaaagaggaagaagttacacttggtctttttctgtcttggaattatttgcctgatatctgtacaatatacattggattttagtgagataacttagccttcactttgcacagcaaatttgtagtttctatatttgcagaaatatgtcttccactaacgtgtgctatctgacctttttattaatagcttcactgcttaggtcttctcttggattatcaaaaagaccattcctattgtctcgaagaaacggatgccctcattttcaatctcgtcagcggtcttcacttgcccaggtgactcttgaaactgagtcagtggctatctcattttaccttaaacagagccctgaaggtcaattccatcttgagtacagtgaagatattcaaggagaaatcctgttcgttctttacaaattattcctactcaacgtgtctcaagatagtgaagatcctcccagtttatttggccatttcccgaagctcctacactctgcactggcagttctcatgaaagctcaaagggatgatgttcgcttgaactgtataggtaagctttaacattgcccttttcttcttctcaaactttagcatctgtgaaattggttttccagtgaatatcgtgacagttttagcatttctgttcttgggttattgcaaagaaagaggggtatatggtaataatatctgacttttttgtaattatattagaagggaactagtgaagtatggatgataaaaagcgagaatgcatgataggaataaccatatgtctccccaagcgatcatttgaagctagagatttgtggctcgtgagcctaatgtcgggataaacaggctccacaaacaactaattgtttgttgttaattctgttcacaccttgaatatactctggctgataaaaagtttttcgtgtatatttgctgctgattcgactatcaaagttctatgcactcttcaccagagctatgataatctctcttttctggcttctaaagcccccttctcccctgtattccccccacccccaactctcataaggaaaaggaaaaagagaaaaaagaaacacaacagaataaccagctgctgatgttggagtttcagcaagataatatcatctctcacattcatcaagtcagtaatactgtttgtctatgcagctttcttaacagtaataatgcaaagaggattatttcaaactacttctataattggctcaaggagcaggagttcttatgatgctgaccacttgatggaaacaaatgagcagataccagatggacctctagctatcttgtttgcagaggcagtcaagggccccctgctttcttctgataatcaagttcaaatagcagtgctagatttactttacctttatctgtcgaggaaagatgtcttagaaaatgaaatccaagtatttgttgaagagaacattgcagactatgcgtttgaagtgttgagattgtcaggtaagaatatcagcgatacacagtgcctaagcagttagatttatatgtatcagtttcatttgaagaaatgaaggatgagggcattgcggtcgcactctatttttgtttttgtttttttcttttcaactaaacgatctttgaattgaccaattctctggtgattacaacgtcttcctacaatcaacaaattaccatgccttcaatgtttgttgtccatatggttcgacagtatctagttctccgacgataatgtgctagagaacattctaattattttaggtcagattatgcaattaatgttgtttttaatgcctaatgaagtaatttataaatttgcaggatgcaaagattcaacaattaaatcttgtattcagcttcttgatattttagcaactgctgagcaagcatttagacagagacttgcaattgggttcatggccctggttccagttcttcatcatgttgctgaaattcctttccaccctgtacagactgagacactcaagcttatttggaactctgttgagaactgcccaggggtggtatccaagtctcaggtagaggaaataagcctttccttgactgggatgctcaagaaaaatcttgacggagaaataggcatgcttccagagacattagctctggtctgctcaatatttgttgcacttatgaaatgttcatcttcctgtgggatttcaagtttcttactatcaattcaggatgcatcaagaaattgcatcttaacttgtttaattaattatggcaaatatcctggtcaacttttgaactctctttaccttctgaaagaggcatattcatatggttgtgggatgaacccctcaagctcaatcaacacagaactcagaagaagcattatagatgtatgcaaaacacatatattaccttggtttatgaaatccctacatgagatggaagatgaggatattccagctgcaatactcgagaacttctattccatattgctacacgattcagacactgaaaccaaaatatttgcaaatgttctgttcacatcttcctggttctgttttgcgtatggatgtttgggtttttttccttctgaaaagatgaaaaacaaggtttatcttatttttggtgtgatggcagatatcattcttggggttgattctgggcgatgcattagcgatgctgctccacatcttccatctgatcctatagatttgcttttccttctgggccataaaagctcccaaaatgttgaattggcttcttgtcaactggcagttctgctgttactatacatcagctcgctgtacgacgatcggtaaatggttgtcttactcttctgcattttcctgcttatgttatcatccctcatttgaaatctcaactcctttccagaattgcagatgataagcttgtgttggcttcactggagcaatatattctacttaacggcagcgaaaacatgcacggagcttcggtgttgggaatattgataaatctctatgcactctacagaggtttagccaaggtgagctaccaaatcccctatagcccagaggctgaaaggattgtgttccacctacttgctgagaaggactgggatttgctatctacaagaatccacataacatctatgaaatggttgttccaacaagagaaaatctgcaatgtgctgtcagcccagcttttgaaattttgcagatgcaattgctccaatgcaagccagataaatatccatggtgaagccaatcagacgatagatgtgtatgttatgacagaacttgtagcttcaggggataactttttaggtatgctcatggtgttcctattgggagaggctggagaacaatattccaagtgtgacattgtttcggtggtgaataccataaaacatataatagaaatctcaccaagtgcttcagatcagttctgcatgcatgggatagctggtgcaattaagaacctgtactataagtttggtcattcttcatcctcagatactttcatggccacctccgaactagtatcctgcattcttcaagcagtacaatctgaatccctctccgatgatgaaccctgggtttcaattgtggtgaaagtatagtactaactcttctaaaatactgtttgcttccagttcctcttagtaaatagacctttcccttaattacagattgttgactacttcatcccctcaatagctgtagatggatggaccccaggaactcttatatcaattggcattctttctatggttttgcaccactcagtaaatcaagtgatggttgaagcttcaaaaaccataatccttagtactcctttgctatcattggttaataccactatcgccgatgcctgttccaagggaccttctctagttgaccaggatgaaggaacaagatctggagaagctcttgtctttgtgctttcactggttttcttctctttgagaaggtagatccgttcctttaacacacagtttctatgctttcttttattttgtttttaatttagaaactaatagcttattttgctagcctacctgccattttaccggggattatggactgccaatatctgttggatcctaccaacgtcccacaacccttgtcccatattagtatacaatgccacgacttgtgcaagttattgcattttggatctattcccataaagttacttagctcccaatgcctgctggagttattcagcagaatagaagatgagagaagtagaaaatcagacacactagaattcagagctgattatttgttgtctataatggctgttttagaagggcaaatattctcaagtgacatgtccgtagcaatgaactgttccctctgtttgtgtatgctcattggatggcaagacgtggaaacggaagtatcagctatacaaaggaacaactggtgtcggtttataatagaagaattagtgatgtctttggcagcaccatctttgatttcacaatctttcatgatccatcacaagcctgcaattcatattgcagttgcactgctgagtgggaagaaagttcctcaatggatgacgtcaatcttcgatgaatcttgcatatttgccattactagaaacatcacaaattctaatttgagcgctgagctggtgttcctctttagaaagttgcttaattatggtgttctgaatgatgaacatatttctgcactaaatcaactattccaggtaatagattctttatcttagaaagatcattggttcctattgtgacctagcctcacgaattgcttttaaaaaaaaacaagaaaaatagcaaagaacgaaaaatgaaaagagaacatagttctgaattctgattgccaaaattctctccaaggattacgatcaaagaaataatggaattccataattatgttcgcctgcaggaatgcagaaaatgtatctacacagacaaacttcaacatgctgaggcagaggagaagacattgaatgtagcagctgcttcagattatttaggtaaagtttgtcagtttctcattagcctcataacgactcaaccatctaatggtatggagtctacaagatttcaaagtgggaaatgggaattgttggaagaaatagacttgttttcaaaatgtctacagagggatgatgtaacaaatctgcaagaccacggggcaacactacgccacagcaacagggacaaacagacccctaaatacttggagcactatgtggtcccaaatgccaagcaatggccaactgtgccagtaccattagcaccaggtagtgctgccaggagctctgcaacataacacctatctatataatcaaaagggatgctaccaaagaggatcatggatgaagttgtcttttaatttcttagctatgtaatagtctggaatctccctcaattcttggtttttttctctttttttagcttggctacagctttcaataattgtaagttgttctctatctttcaatacaagttagttttttccagatgattaagattataattcttgagccgggggtctttcggaaacagcctttctacttcatcagaggtagaggtatggactgcgtacatcttaccccccagaccccactaagtgggaatacactgggtttgttgtttgtttgtttgattaagattataattctaaaaagatcttcatagcaatactttttggatagatggacaatctgtttttgcagaatgacagccaattaagataacatggattttgcttacggatcattcattgcattctttcttaagagttaagtgacttcttgccccattaagttagttttttctcggagtgcacaactgcacatacatctttagaaagaacaattgttatttcctgttttatcacttctaaacctaacgggtaatggcatctgctaaaactattcctatagctgtcgctggaataaagctaaaaaatcttccctacaatacaggccacatggagaagtgcagcgtaaaaaatccatctgcatttcttccaaagatgataatgaaaactactacttccgtttccattaattcgactctattttctttttgaatgcctcaaattgtttgacatcattttatttcaattcaattcttacagagtacaagaaattctgattcctagatccttttggggtttttatctttctgaatgtgatgttttatctatctaattaatcttttgattgctactttaatatgttcttatacttatcaccataatactgataacatcttaaactcggaaggccattcacgtcatgttcacagaaagagtaattaattgt

SEQ ID NO: 98 - DNA, 4382 bp, Capsicum annuum
  source 1..4382: mol_type = other DNA
cctaaattcagattagaaattagaactaaagggacctcttggttgtcagtgtatatatatttcgaattcctaggcaaaaagggtagccttagcatctttgtttttcgctcttcactcacgcacacagtacagcaaacaaatgtatttcgccacgcctcacctccaccacttgccaccgtctccaccggtaacatgcgctcaaggccatagctcgactttgattattctaaccgatgaaggcggatcaatatgcctgctctgtttgtccaatctcatttctaatccgatatcgccgactgttcacgtttcatacgtgctttcacagttatctatcgcgctttctcaaccgagttttcgccaaaccttcttcacatttcactctcatttcctaatttcgcctttagtcggagttctatcttccttcgatgatgagcctattgccaagcaaactatggatttgattatgcagttgtgtgaacctccggattgtgatgtgcatgcggagtttgtggctcggcttgcagatcgtctttctagtggctctttagcttggagtcggagacagcttcacacgcttcactgcttaggtcttctcttggattatcaaaaagaccattcctattgtctcgaagaaacggatgccctcattttcaatctcgtcagcggtcttcacttgcccagtgaagatattcaaggagaaatcctgttcgttctttacaaattattcctactcaacgtgtctcaagatagtgaagatcctcccagtttatttggccatttcccgaagctcctacactctgcactggcagttctcatgaaagctcaaagggatgatgttcgcttgaactgtatagctttcttaacagtaataatgcaaagaggattatttcaaactacttctataattggctcaaggagcaggagttcttatgatgctgaccacttgatggaaacaaatgagcagataccagatggacctctagctatcttgtttgcagaggcagtcaagggccccctgctttcttctgataatcaagttcaaatagcagtgctagatttactttacctttatctgtcgaggaaagatgtcttagaaaatgaaatccaagtatttgttgaagagaacattgcagactatgcgtttgaagtgttgagattgtcaggatgcaaagattcaacaattaaatcttgtattcagcttcttgatattttagcaactgctgagcaagcatttagacagagacttgcaattgggttcatggccctggttccagttcttcatcatgttgctgaaattcctttccaccctgtacagactgagacactcaagcttatttggaactctgttgagaactgcccaggggtggtatccaagtctcaggtagaggaaataagcctttccttgactgggatgctcaagaaaaatcttgacggagaaataggcatgcttccagagacattagctctggtctgctcaatatttgttgcacttatgaaatgttcatcttcctgtgggatttcaagtttcttactatcaattcaggatgcatcaagaaattgcatcttaacttgtttaattaattatggcaaatatcctggtcaacttttgaactctctttaccttctgaaagaggcatattcatatggttgtgggatgaacccctcaagctcaatcaacacagaactcagaagaagcattatagatgtatgcaaaacacatatattaccttggtttatgaaatccctacatgagatggaagatgaggatattccagctgcaatactcgagaacttctattccatattgctacacgattcagacactgaaaccaaaatatttgcaaatgttctgttcacatcttcctggttctgttttgcgtatggatgtttgggtttttttccttctgaaaagatgaaaaacaaggtttatcttatttttggtgtgatggcagatatcattcttggggttgattctgggcgatgcattagcgatgctgctccacatcttccatctgatcctatagatttgcttttccttctgggccataaaagctcccaaaatgttgaattggcttcttgtcaactggcagttctgctgttactatacatcagctcgctgtacgacgatcgaattgcagatgataagcttgtgttggcttcactggagcaatatattctacttaacggcagcgaaaacatgcacggagcttcggtgttgggaatattgataaatctctatgcactctacagaggtttagccaaggtgagctaccaaatcccctatagcccagaggctgaaaggattgtgttccacctacttgctgagaaggactgggatttgctatctacaagaatccacataacatctatgaaatggttgttccaacaagagaaaatctgcaatgtgctgtcagcccagcttttgaaattttgcagatgcaattgctccaatgcaagccagataaatatccatggtgaagccaatcagacgatagatgtgtatgttatgacagaacttgtagcttcaggggataactttttaggtatgctcatggtgttcctattgggagaggctggagaacaatattccaagtgtgacattgtttcggtggtgaataccataaaacatataatagaaatctcaccaagtgcttcagatcagttctgcatgcatgggatagctggtgcaattaagaacctgtactataagtttggtcattcttcatcctcagatactttcatggccacctccgaactagtatcctgcattcttcaagcagtacaatctgaatccctctccgatgatgaaccctgggtttcaattgtggtgaaaattgttgactacttcatcccctcaatagctgtagatggatggaccccaggaactcttatatcaattggcattctttctatggttttgcaccactcagtaaatcaagtgatggttgaagcttcaaaaaccataatccttagtactcctttgctatcattggttaataccactatcgccgatgcctgttccaagggaccttctctagttgaccaggatgaaggaacaagatctggagaagctcttgtctttgtgctttcactggttttcttctctttgagaagcctacctgccattttaccggggattatggactgccaatatctgttggatcctaccaacgtcccacaacccttgtcccatattagtatacaatgccacgacttgtgcaagttattgcattttggatctattcccataaagttacttagctcccaatgcctgctggagttattcagcagaatagaagatgagagaagtagaaaatcagacacactagaattcagagctgattatttgttgtctataatggctgttttagaagggcaaatattctcaagtgacatgtccgtagcaatgaactgttccctctgtttgtgtatgctcattggatggcaagacgtggaaacggaagtatcagctatacaaaggaacaactggtgtcggtttataatagaagaattagtgatgtctttggcagcaccatctttgatttcacaatctttcatgatccatcacaagcctgcaattcatattgcagttgcactgctgagtgggaagaaagttcctcaatggatgacgtcaatcttcgatgaatcttgcatatttgccattactagaaacatcacaaattctaatttgagcgctgagctggtgttcctctttagaaagttgcttaattatggtgttctgaatgatgaacatatttctgcactaaatcaactattccaggaatgcagaaaatgtatctacacagacaaacttcaacatgctgaggcagaggagaagacattgaatgtagcagctgcttcagattatttaggtaaagtttgtcagtttctcattagcctcataacgactcaaccatctaatggtatggagtctacaagatttcaaagtgggaaatgggaattgttggaagaaatagacttgttttcaaaatgtctacagagggatgatgtaacaaatctgcaagaccacggggcaacactacgccacagcaacagggacaaacagacccctaaatacttggagcactatgtggtcccaaatgccaagcaatggccaactgtgccagtaccattagcaccaggtagtgctgccaggagctctgcaacataacacctatctatataatcaaaagggatgctaccaaagaggatcatggatgaagttgtcttttaatttcttagctatgtaatagtctggaatctccctcaattcttggtttttttctctttttttagcttggctacagctttcaataattgtaagttgttctctatctttcaatacaagttagttttttccagatgattaagattataattct

SEQ ID NO: 99 - protein, 1343 aa, Capsicum annuum
MYFATPHLHHLPPSPPVTCAQGHSSTLIILTDEGGSICLLCLSNLISNPISPTVHVSYVLSQLSIALSQPSFRQTFFTFHSHFLISPLVGVLSSFDDEPIAKQTMDLIMQLCEPPDCDVHAEFVARLADRLSSGSLAWSRRQLHTLHCLGLLLDYQKDHSYCLEETDALIFNLVSGLHLPSEDIQGEILFVLYKLFLLNVSQDSEDPPSLFGHFPKLLHSALAVLMKAQRDDVRLNCIAFLTVIMQRGLFQTTSIIGSRSRSSYDADHLMETNEQIPDGPLAILFAEAVKGPLLSSDNQVQIAVLDLLYLYLSRKDVLENEIQVFVEENIADYAFEVLRLSGCKDSTIKSCIQLLDILATAEQAFRQRLAIGFMALVPVLHHVAEIPFHPVQTETLKLIWNSVENCPGVVSKSQVEEISLSLTGMLKKNLDGEIGMLPETLALVCSIFVALMKCSSSCGISSFLLSIQDASRNCILTCLINYGKYPGQLLNSLYLLKEAYSYGCGMNPSSSINTELRRSIIDVCKTHILPWFMKSLHEMEDEDIPAAILENFYSILLHDSDTETKIFANVLFTSSWFCFAYGCLGFFPSEKMKNKVYLIFGVMADIILGVDSGRCISDAAPHLPSDPIDLLFLLGHKSSQNVELASCQLAVLLLLYISSLYDDRIADDKLVLASLEQYILLNGSENMHGASVLGILINLYALYRGLAKVSYQIPYSPEAERIVFHLLAEKDWDLLSTRIHITSMKWLFQQEKICNVLSAQLLKFCRCNCSNASQINIHGEANQTIDVYVMTELVASGDNFLGMLMVFLLGEAGEQYSKCDIVSVVNTIKHIIEISPSASDQFCMHGIAGAIKNLYYKFGHSSSSDTFMATSELVSCILQAVQSESLSDDEPWVSIVVKIVDYFIPSIAVDGWTPGTLISIGILSMVLHHSVNQVMVEASKTIILSTPLLSLVNTTIADACSKGPSLVDQDEGTRSGEALVFVLSLVFFSLRSLPAILPGIMDCQYLLDPTNVPQPLSHISIQCHDLCKLLHFGSIPIKLLSSQCLLELFSRIEDERSRKSDTLEFRADYLLSIMAVLEGQIFSSDMSVAMNCSLCLCMLIGWQDVETEVSAIQRNNWCRFIIEELVMSLAAPSLISQSFMIHHKPAIHIAVALLSGKKVPQWMTSIFDESCIFAITRNITNSNLSAELVFLFRKLLNYGVLNDEHISALNQLFQECRKCIYTDKLQHAEAEEKTLNVAAASDYLGKVCQFLISLITTQPSNGMESTRFQSGKWELLEEIDLFSKCLQRDDVTNLQDHGATLRHSNRDKQTPKYLEHYVVPNAKQWPTVPVPLAPGSAARSSAT

SEQ ID NO: 100 - DNA, 8175 bp, Capsicum annuum
  source 1..8175: mol_type = genomic DNA
ggccaacgtgctgaatgacacgatttttgaatcactgtttaagccatacatacactcagtggcagagccagaagttcggatgaactcctgaattgactgtggctccggcactgcatacacttgaagtatatacacatatgactaaagttaaccagttttactcgaacttccatcattttcccctatacgtcaaacgcttttgctgacttaaagtcatttttacttaaaacttcaatcatatttgaagtctattcagttcattttctcgtgaagttcaaggatttttgcttaaattaaatcatttttgtctaaatttcaatcatatagaacttaaaatatttttatacccaattttagataccgcatatctaaagttattctgaattaggagtgtgcatcgttcggttcgattcggttttatgtattatcgatttggtttattagttttcgatttttaaatatgctaaaccaataaaatattttttatcgattttcgatttatcgatttttagtccttaatagttcgatttcagtttaaccgataagaaaatactcacgaaatagaaaaatagtaactaacatgaaaagaaatcgaatcttagttacagccaaaatcattcatgatttgttttaatttacaagaatctcatgtttgaactaaatgttatttagaagaaattaagagaaaatatacatacatatatataggtgtaaaatagtaatttaatatattcttattggattatcaatttatccagtaaccgaataagaaaaaattatatcaaaccaataacccaataattttcttttataaaatcattacaaaatcgttaaatcaataacaataaatcaataatacctttatcagttcgattcattaatcagtttgatttttgcacacccctaatacatatccattttttttttctttttaaataacgatgctcaaatacgtataaataccgtactcccgccatttctctccacatagagaaatcaaatggaaattgtgagagaacaagcgaagagtaactccgatgaatcactcaaactcgcagtcgcaatggcgattctccgatcaaagctcctccacaaacctccgtcagcaccgccgccgcctcctccgccttactcctccactgccgctgctgccactgccgctgcagcttcttcctccgatgatgacgctcttaaatggaaacgaaaagtgagtttcctggactatcactgtgtgcgttttcaaaatttagctcacttttcatacttgaaagtgaacaattaataattgaagtgtattttgataaataattggtgataattgctcactctagttcactattctattatctcgtgaagttgttgcgcggatgaatttctgtttattttagagtcaaaaggtgaaaaacaacatgtaaactatttattttttttgagtttcgtgcctgaactatcaccgtgtgtgttttcaactatctcgaactatttatcgaaatatacctcacttttcatacctgaaatatcgcgatagttcaagtagaaaaagtaaacaattagtacctgaagtgtgttttgacgttatctgcatatgacgaatttcaattagtttaatttaatttttttaaaaaaaaaattgaaggctaaagagcgtaaacaagagattgtcagacttaaggaagatctcaaagtagcggaaggttagtttttttcacgttcattattatttaatttaaataaatttattttacttctatttttttaatgtgaatattgaaaattttggcaattgcagcaattttagtgtgtatctgttgttatgtatttgattccaattgtcaagttgtgtagttatgaattccgacctcagaactttgtggcagcttaattgtgtttttcgattttaaatcggaattgcaatgatatggagagttccctgaggattttgttaaatgtttgattttggttttgcaatgataagcagagttttttgaggatattgctaaatgtttgattttgattttgcaatgataatcagagttttctgatgactttgcgaaatgtttcatttcgattttgcaatgatagccagagtttctgaggattttgctaaatgtttgatttcgattttgcaatgataaccagaggtttcagagtttttgaggattttgctaaatgtttgatttcgattttgcaatgataactagaggtttcagagtttctgaggattttgctaaatgtttgattttgattttgcaataataatctgtagtgttttgagtatagtctgtataaatagattcattttgaacaactaatttttaatgtttaatttattttattttttatttttgaataagatggttcacagtaccatatatttaaaaaaagtgcatcatgcaagtgttatttcttcgatagctcgggattgtgatccctaagagaattgatcctccagctattttcttgagtatatgttgttatgtgttcaatttccatttcaaatgtcaactgtgtatttctgaaattctaggttctaagtatctgattggtttgctatatttcaacctcaaaaaatttgtaacttattgtgtttttcattttaaaatcaaaatcgaaatgataacaagagttttctgtggtatttttctctatgtttgatttctctgtactaatctgctatctgtatagctagattcatattgatctgctataatcttttgataatttaccttttctttctggaataagatggttcacagtatgatttatttccaaaaagtgcatcatgcaagtgttatttctttgatgagttgggattattgagccctaagagaactggagattgttctgatcaacagttcagtgatgtgttgcggagaaggtttctcagacaaggttttgtttctatggaattctgctgtatttattagtcttaagttgtgaatttctccctcagtaattctgtgcacattagcttaatccgatgacttgttgtatatttttccagtgaggattaaggaaagaaagaggagaagaacaaatgattccctgcttcaccgaatttcaggtgaaaatccggttagagttcttcttatggatgtaaatttatctttccttttgatgattaacttgcaaagtgatgattcttagaaagttacactgagttgagatcttatcatacctcagccattctgtgataaatgtcatttactatgtgtgctgtaatttgatctctggaaaacactaggccctgtttggaaattttgctgaacatgaattttcagatatcgatgagaagtatgaatattgtcttttcttaaatggcagaacgtgacaatgaaactaatgtcgagcaactgagcacttcagttgattttctcttggagctttgtgacactctttctcctcaaagtgtatgttgcttctattaacccaagctactgatgcgttgtcttatgttatgaatatgatttcgatgtctcatctcacttggattttgcactaaatatgttgcagttggaggagggtaattttaaaaactggtgccaccaagctgtggactttattcttggtaatgacacaatgttcacttccttttgccttcctgtgtacaaattttcatgtgcaacatctcgaaatataaacttgaattcctgatatatttttttgtttctaatacaccaacaattaattttttcacagaagtactgttattttctaattttttagtgttgagcattgtgatagaagctgaaatcaaggggttaataagtgaatgtattatctgttctgaaacttaaatgaaaaaaagattgtctagtgaagcttcgtcctaagatttaagttttcaaggaaagattgctcttaaagactgcaatttgagaaccatcttcatggtttgtactgccattttaattgaactttactcaaatatgcaaacagttcacggtttactcttctttgtcaacaccttaatgcaagtactggaccatttcactgcatagcttactgaaatttcagttgtaatattaagatagcaccagatgggttgatctattactatctagtcttcttcccttgatgacttccaaattctactgcatttgtattatactattttaaaggtacactggctacaatgtcaccaaccgaaaagaacagagaacccgtggaaggcattatcaacagcttaatcatgcgtttgttgagaagaatgtgcagtgccttgcaaggagatggtaattatgtagtcttgtttttattcatactaggttttcgaagaccatcttcaccatagcagattgcgaaagtatatttttatctacctttactaatggtagaatcagcatgttcaatcaattacgctgcttatattatgtactctgaaaacttatcaatccttgcctactgtaacatgtagaagtagaagtactatttaggttgaagaagagaatatagcttcttgatgctacgcaaacctattagatcttcatttctatggacttccatgaacgttatatgtcagagcaagcagacttcaaatgtaaacattctcagcagaaaagatttcagaatcatactgctctgtagctatgaaagatttagtaattttatacccataaattctctaagtgttcatacttaagaaatgacaccgtgaagttcttaactgagttccgagattcctgcagcaagcaattataagattttggtagatatgccctggaatatgcatatacagaactaagaaatggtttcagcatgatactgagaaaagttctttggtttgatacatatttaatggaagcaaatcagttttctataataatggatgttttttttattatactctgatcttcctgtttgtacatcattattagatggaatctgagtttaagatgttaatttaacttacccgttaccatagtagcaataacttagtaaagcagtggcaaaatcgttaaacaaagctgaactcttaaaatttatggaagttgtataaagatattattggtagaacagtgtagatagtttttggacatttcaaaacaattatagtatggaaaattttggcagaggcaattaacatttgtgatgaaactatctgcttagtgtagaaagtcaccctgataacttttccagcagaaacaaaaaaatggttgttttcacgtctattaaatcccccaatgtaacttacttatatttccttctacatagcttcttaactattgattttataacacgtctattaaaattccagtgtaacttacttatatttcattctacatagcttcttaactcgtgattttataatgacatgttacagaatctcatcactttgacacagctgttcagttctatattcaacatttgatgcgtaagatcggaaatgaggcttttgtcggccagcgtctaatatttgcagtttctcaaagaatttctgcaattgcagaaagtttgcttttcatggatccatttgatgctgcctttccaagtatgaataactctatgtacatgatgtaagtcccaccagcttgtatatacttactcgtctttattgttcttttatgcttctttgtagctgcttcttactttcttatcacataattgagggctgcataattggaaggaaggagaaaggggcagtgggagtcatgcccgcaaatttgtatgggagattcccactgctgcctctaggctataagcctgtcttcttgtttgttaaatgccgtcttccttcactcgttgaaatttgtttctttgctcgtgatagtggatgtacattattttggtccttactcttgacgaaatttcttgtcctctatctatgacatatattttcctttctggtcattgacatctttccatgtgcttttttttcctgtttctagcttggagtttgaaaacaatatgatttttatatctgttttggactgcttgttcctacagacttccccatttgaaggtatttttaagctgagaagttggaatttgttccttcaaatttggagttcctacggggagtttgatatttactttgagttggctgtgtcgttctttcttttgttagttaagctgacataaagtttgcaatggttgtgtattgcggtattagtataatcatctttttcttctagtatccggtagtggattgatcgctactgtatttttcggtcatcttcacaatcttattgattgtaaatggtggttttagctgcaggattacttggtgtgtgctctccttgttttgtctatatagttattcattgcttgaaacactgcaacgattaagttatcagaggctgtgcccttcagatattatattatgctttttacatgaacaaagcactatattctgcctgaattgctagactacttagttaacttggggatgttcatacacctcaaggtttatcatcagaatcgtgtttaaacttcacactttgaaccatagcttaagcttgcaaaattttgttctataagaggctgtaataataatgtggcatacagtttgttgtctagtatttgatcttttactgcatccacgtttgcttcttcactccctcgcttccttcccaaatgaattttcttggaactgtaacacaattaaaggagatttaaaaagttttttcttgatatgtgttctccatggcaggatccagcttattgaatttctggttacagattatttgttaacctggtcaaacactggagatttcgaaataagtgagcttcttttaatcatcttgatccagtaatgcttttctttcttcataatctatatcctctccatccgcctggtctgaggcagttctgcctccggctgaggaaatttcaaattgataggctatgggtcgtaaacatactgtatctgagatatatgcccacaaggataactagaagttacgacaaatggcctattgaaggatcattttcatactgttaatgacggaagtgtacctaacatatccatacgtcatatttactttgtagggctttttgaagaatggtttgtatcagttctccaaggaagaaaagcattggaactactagaaaacaggaattctctttatgtactgtacatagatcgtgtaattggagttgtggccaagcaagtggggcagttgtcatttctgcaaaagctaagtccgcagattcttgagaacttgtatagctaagctcttacctggacctttcccttgtgaactgtaagtaacttgctttcaacacaattcttcttttattgtccattgaaaattcagccgtgtcatcgtaaattcttttttactgttcaagagtctttttaaaattgattcacagagcaccaaagatcaaagttctattaaagtgaaagatgctctttaaatgtgaaaagattaaccagcatgtaaatagttaatccacctctacatgacattagcacagcatcatgtgccgaaagccagaacaaaatcccacatctctttatgctgaacccgattccaagttgaaatatgctccaccaaattaccggctttaagttaatctttgacttccctatggcttcactacttttcattacacataaactgctcaagttattggtattactgaacatactacgttgttgagatcatctagcataaaggaggttgttggacggtttgacttttgtctctttgtaatccagacatgttcctttctcattttctttactttctttgtgaaatctgggggtggggatctgaatcagattagtttacttacaaacaaagaattcctgttctagtactttctattgtctttccattccaccttttgagttgtccgtccccaccttgttcatatttctaactacatcttgaagggtgattacacagtcatccaagcatttcatccttttatgacagataactactaccaaaaagttcattatgtttaaaaggtggaaaaaaggtgtatagtattggatacactttctgctttttgcttgatatatatgtatatgtccttcccaacttccatctaatcaaattaacttgctcctagctactacattttacgtaatctctctatcgaattcgtgcttagtagacatgattctagtgaaagccgtactgttcctctcattattcgcaactctcttactgtcccattactacaaagcctcagcttctaatgacattccgccatccactt

SEQ ID NO: 101 - DNA, 1752 bp, Capsicum annuum
  source 1..1752: mol_type = other DNA
ttcattaatcagtttgatttttgcacacccctaatacatatccattttttttttctttttaaataacgatgctcaaatacgtataaataccgtactcccgccatttctctccacatagagaaatcaaatggaaattgtgagagaacaagcgaagagtaactccgatgaatcactcaaactcgcagtcgcaatggcgattctccgatcaaagctcctccacaaacctccgtcagcaccgccgccgcctcctccgccttactcctccactgccgctgctgccactgccgctgcagcttcttcctccgatgatgacgctcttaaatggaaacgaaaagctaaagagcgtaaacaagagattgtcagacttaaggaagatctcaaagtagcggaagatggttcacagtatgatttatttccaaaaagtgcatcatgcaagtgttatttctttgatgagttgggattattgagccctaagagaactggagattgttctgatcaacagttcagtgatgtgttgcggagaaggtttctcagacaagtgaggattaaggaaagaaagaggagaagaacaaatgattccctgcttcaccgaatttcagaacgtgacaatgaaactaatgtcgagcaactgagcacttcagttgattttctcttggagctttgtgacactctttctcctcaaagtttggaggagggtaattttaaaaactggtgccaccaagctgtggactttattcttggtacactggctacaatgtcaccaaccgaaaagaacagagaacccgtggaaggcattatcaacagcttaatcatgcgtttgttgagaagaatgtgcagtgccttgcaaggagatgaatctcatcactttgacacagctgttcagttctatattcaacatttgatgcgtaagatcggaaatgaggcttttgtcggccagcgtctaatatttgcagtttctcaaagaatttctgcaattgcagaaagtttgcttttcatggatccatttgatgctgcctttccaagtatgaataactctatgtacatgatgatccagcttattgaatttctggttacagattatttgttaacctggtcaaacactggagatttcgaaataaggctttttgaagaatggtttgtatcagttctccaaggaagaaaagcattggaactactagaaaacaggaattctctttatgtactgtacatagatcgtgtaattggagttgtggccaagcaagtggggcagttgtcatttctgcaaaagctaagtccgcagattcttgagaacttgtatagctaagctcttacctggacctttcccttgtgaactgtgaaattccagtgacattgacactgttggactttctcgcgtatctcaacttgtcttataacaatttgagcggactgattccaaccaatccacattttgacactttgtatcaagacggaacagcatatatcgggaacaaatacttatgtggtgctcctgatgggatgagctgcagcaacagcaacggaccctctaccaacgaaacagctgagaacagatacgatcaagaaaatgtcctttttgttgtagttatattctcgggttttgtaacaggaacatctggtgtatttctgctgttatatttgatagatgacaactggaggaataggtattggagggcagtacacgaaattgtgttgaaaatagtgaactgtaagctatgatatgtgcatatactaaatactgcatattccaatgca

SEQ ID NO: 102 - protein, 391 aa, Capsicum annuum
MEIVREQAKSNSDESLKLAVAMAILRSKLLHKPPSAPPPPPPPYSSTAAAATAAAASSSDDDALKWKRKAKERKQEIVRLKEDLKVAEDGSQYDLFPKSASCKCYFFDELGLLSPKRTGDCSDQQFSDVLRRRFLRQVRIKERKRRRTNDSLLHRISERDNETNVEQLSTSVDFLLELCDTLSPQSLEEGNFKNWCHQAVDFILGTLATMSPTEKNREPVEGIINSLIMRLLRRMCSALQGDESHHFDTAVQFYIQHLMRKIGNEAFVGQRLIFAVSQRISAIAESLLFMDPFDAAFPSMNNSMYMMIQLIEFLVTDYLLTWSNTGDFEIRLFEEWFVSVLQGRKALELLENRNSLYVLYIDRVIGVVAKQVGQLSFLQKLSPQILENLYS

SEQ ID NO: 103 - DNA, 7188 bp, Capsicum annuum
  source 1..7188: mol_type = genomic DNA
cagaaaaattcaaatcaacaataaatgcccccttttctttaaacacacacaaaaaaaaaaaaatctaatccgcgtccatccgacccgactcacaaaaatgacacaaacaaatatgtctctatattccacttggaacaggagcagatttgtttgtgtcttttttgtaagtcgggtcaggtgggacggattagatgaacgtgtgttttctttttagaaaatgaagcatttaacattgatttgatcctaaagtgtgatagcgaggaaaatttgacctaaaagtacgacgaatgatatatttagctaatttttcaaaataaaagggtaaattggtacatgcaaataggagtaggaatgacaattttcgaaccttcaataaacaaaatatattcatgcatgcattctttctcttcattaggtatgttgttgtcattattaattaatctctgtattattattaagtttctactgttgttactccacatttgaaggcaatataattccaaaaataaaataaattttaattaataaaaaattagatgtgctaagtcattaaaatataaaataagttttaattaattaaaaattagatatgctaagtcatatatcacaatgaccgaactcagaattatgaataacagagtgatgagacactttcaaattgtgtgaactaggcgggcctaatgatcagatgaaatgaatgggccttaattattcagtacaggtccatcacagcccatttataccgttatacccgaaagatttgaaactcccatatataaacccccacactctcccgccggaatatcaatgcaaatcacacttgcaagttccaaccgttggattcgccggagcaaaatcacagtaaagtaacctcaaagatctgtgaatattcaaatgtgttaacaattttgatcgatatactcataatctagggttccgtaattgtgccaaattggaggtttagattctcgaagatttcgaattttccagtaatcggaaaatgaagctgaagatcaataaagcatcggatctcagttctatatccgttcttcctcctcatgcaaggttcagttctatctcaattttattcatttcatctctttgcattttgtctaccctgaaattgcctgtatatctgtgttcctgcgttttctgagagagtagagagaatgttactgtaattttgagattttttgtgaagatttaaggaggaataaagcgccaacttctctgttttgcttttttactctaatacgttacagatgtttcgatgcatgttacgtgtactgtttgtgtgagtaagagagtaaggtagaaaatttgctgtaattttgaggttttctgtatgatgatgtgagaagaacgccaagtgcggagccgctctgtgcatttttttctcatatattgcagctatttcgatgttgttgtgtgctatacaatacacataactcatgcatatgtatgcatgctagatgcatgtttgaatgaataagagagaggtagaaaaatttctgtaactttgagcttttctttgtgcgatgatgtgagaagaacgccaagtacggagccgctctctgcgttttttttatacattacagctatttcgatcttcttttttgtccaatatacacaaacttcacatacctatctatgcatgtatggagagagacagtgagagagatttaccataatattgagcttattgatgatatttgaaggaggcctagtgtggtaccaagtgcagcagagtcttctgtatttgggaaaggccaagcgtcacaggttcggtcacagcagcaatcacaacaatccttctcacagggattttcatctcagcaaatgacctactctcagccatctcagagctctctggatgaatttgtcacacatgaacatgtaattcctctttctcactcctgtttctcagtcattcgaattatagttgttaatgaaatgtcattttggtatatttcaactgctaactaacagtaatatgcaaaggaactcattcatttggtgcggaaatgataatgattgatttctaaaggtcattttggttagcaacttctcaagattgctttagattgtctaaaatgtattttgatgctttgcaaaacttgaatctgttagatctttgataattgttccctaggttaggttacttttgagtgtaattttgcattagtattgctttatgattcttgaaatagatgaattttgcttcaaactatgatttactttgttaaatgctgtgtcaatacgcaacactcactttatatgagatatttgtttaagtattatattagtggtggttgaaaagatattaaagtgaaagttttatatttgaacagtctgaaaattgcataaaagatgagtgatgtcaaaattttgcaaggtccttagacggaatgagtgtcatacaaattgggatggagggagaagtagatactagttatcatctccactgtattggaaagtgaatcataaatttctgttcccgtgtctatcagaatttttcttattgctatatgacaaaacaggggattgccacagtgcactttgaagtggttgtcagcaggttgtagagcttctcagagttcatatacaactggttatctgatggaatcttgaattttaaattgagtagacgccttattgtttcaactctgcccagtgcccagggctcaagttccctaaaacttccccactttatacatttgaaatttagctcatctcatagcaaacaaaatgctcttatgagaattttacatcttaaagcaaacaaatgctgtaactgttaataattttaatgcagagattaggttctcaagaaagagaaaattcagcaaaaaggctgagctctttgcctcatatcaactacacacgagaagagaatcaactgcagttatcaaaaccttcggccaattatatacgcaaatggtcagttcctgaaaacaaatgtaagccacagtccaccaccagaaatctctctacttctgattaatatctaaggaaaatgtattccagttcggcagactaatttgctgctggaatcattggaataaacatgttcatgaattctaattttgctggacagaccagatcactgaagaacttgaccacaaaattggaatggtagagacttcattaagcaggcagggaatgatcttagattctattcagagtgatataatgcaagttaatcggggaacaaaagagatactgatggagagtgagtattcattgccattttaatttacgtgatgtggctaaataattatgaactccaaagagtgctatcattagttgacgattatagaattttgtctttagatgcctgctggtccaagtaaaatctttacttgcaaatatttctggtggattagacagacaataaatggcaacaaaatctaacacatttggtttcttctgaaattcttttcagtggaaagcttacggccaaagatagtttctcatgatgaactattgcaattgatggtaactatagcttagctgctctgcgtacgtccagaaattaagtgcctgtttgttttatcatatttcctaatccatgtgacatacaatatccagaacaaggggatggaagatctgaaagctagcctggaggggaccatcaaatccatgtttgaagagctgagggagaatacatatcaagaggacatcagggatcttttatcactggttagagctattcccaacaaacttgagatgtgcattttgcgacttcaaactgatttgagcaagaccttggctaaagagattcaggcatgttgcattttgaaactgacttttttagatcacatttaggctatgggttaatgcttcttcttctatattcccattgcttgcagataattgccacccacccagattgtcatggacaaaaacatgatagtgctccagtcgatccaccaaaagtacgttaccatttttttttttctaaaagatggcctggaactggtctgtcttcacagcccctaaaggtaggctaccctctatggttcggttaatgctgcttcttgtctattcctattgcttgcagataattgccctccgtccagattgtcatggacaaaaacatgaaactgctccagtcgatccaccaaaagtaatgttttcaagaactcttttctccgaattccataagatttttatgagtattgagtataatgaagaacatgatcagaaatcttagtgcatttgaacatttgtagggcatcaatgattgtaaccctccacgtgaagtgaagtttctaaataagtaagttctcaaacttccgtccatttcatccttctcatcgccatcgctgctgccccatttttgaaatgtttaagtagcaatgattaaccatagctctccactatgcaaagttcataagcacttgatggttctcttactatttgctgcatcatttgtgtgcaatatgcataagcaccaatcatttcgcaatgcccctagagatgtgtgtattgacacgcaactgggagacactctctgtccacaggaactacttaggtggcaaacagatgtgaagattcacagcgtagtgtcttttgatccatatcatcataaccagaaagtgagtatccccatttcttacattagctgtatgaaggaagaaatggtaaacacaggaaagaactctcgttatacctcaaaagctttaatgcaagttagccttcatgataaaccaaatgaaataagaaaaattctaagaactttgctatagcttcaacagaaatcttaaagatattttgtttacaaagttttgctgatctttttaacattgaacaacctaatgcttaattgctgtgcaattgcacgtctccaagcatttcttttcacttctggttcaactatgaatctcagagatcagaaaacgactatgctgccgaagattgaaatgggaggctggactacagtaaaaaataaccaaacttgtatgaagcaagcaattcccgacagaagtcgcaaacagaatgaaacatttcaacaggtaactctctcattgtccttacgtgaacaaatgtttattgagttataagcaccagttgcttcctttgtatgaaatgggagctggactacattaaaaagtaaccaaatttgtatgaagcagaaaattcccatcagaagtcacaaacagaaagaagcatttcaacaggtaactccctcgttctccttatgcaaacaaatgttgaattatgtgcaacaattgcttcctttgtggcatgcaaacatccataaaagaaacaatggggttttagatgttgtacatatgatatgttttagtccaccatttctgagtccttcacgttgaagtaacaaaaactactttgttcagcacaccacatttttgataacttgaaaccgcgtcacccgtattctcagagcagacaactggctatccatttcagggaagggaatgtagaattaccattgaatctgatgaggatattggtgcagccttttcctgcttgcttgaagaaaatggaaaaggtaatttgcattacttgcccgcatcattcatatttgaggatttaatgataagcagagtgatttctacatcctgtaattgatgaatgtgcttattgaaccatgtatgttgaacttatctaatggatttagatagatctatttagatgtatatcaaattatgtcctatatctcaagactcacctctgacaagaatgacgacttagatttataatatgaaacaaaataataaataaaggaaaaaaagtcagaacatgtctaaaagcctgaagcatctttgttacactccatataagtttttctcaaagcaaagacaaactgatagccctctcctccctttgtcagtcggcgtatggaagggaatttgaactggttctcaggtttagtgtccccaggggtctttttctctgaaataatcacatttcgagtgtgtcctgaaatgggaatttttgagtatcaaaactgcagcaacaagtgtcttttttccacagactgaaacaaacattcatatttttttttggtcgtttgctatagattggagtgcttaaactgtctttcccttaacgacacagggatttgtccactagatgatgcaaaggaagagagtgcacgcatattaaggaaagcaaggaggcgaaagagaaagcattttaacactatcattatagattgaaggtactcaacgacaatttataatccgctcaaggttctgtgatttgataagcagtaaaaaatgtattattttttcatccgtctttccttagccgatacaggacatgttgtttgtaattctgtgctccattattattagaaaatcccccactggtcattacatagcaagcataatctatgctgttgctgcaatgcgcagtcttgagtgattgtatatctttccaatgcccataataataagtaaaataccagattagtaaataattacaagcaatatgagtgatgttttattttttgaattgcataaatttggctagttattagttcattgcatcttttgcgtacaatgttatatgttgtaaattttcagcatgtgatactaaaaccatatgatataatgatagaagtatataatatgataaaaaggatccttttcaatgggtggaagatagcttagaaacaccaacttgtatcactttgatgagagaataaaagcatatcaaacagggagaaaatggaacattgaagagtctttactaattctttgatttggataatcactatctttttcagcttcatcttatgctcctcttttaccaagagccattgtcccctggtgaatctatttacataactttctttagagcataaatattgtgtggattttgtgcttgtttgctcataagaaatccatacatcatctgtcgtgtttcttgcctgttgcttttggggtgttaagttccttattgacttagtagaagtttagccttaaacaaaatggcttaatagaatagcaggcaattactagccacaccgcattgctctcgtggtgtgtatattgtatgatcctaataacttaagaagcatgctcactcttcaggacaaatccctctagaaaggatgaatgcgtgggctggtgggtttcctctccttttgaatatcatccaataatccgaacaaaccttagttggctgtcacatgaaatttcccttcccatgctt

SEQ ID NO: 104 - DNA, 1817 bp, Capsicum annuum
  source 1..1817: mol_type = other DNA
aaacccccacactctcccgccggaatatcaatgcaaatcacacttgcaagttccaaccgttggattcgccggagcaaaatcacagtaaagtaacctcaaagatctgtgaatattcaaatgtgttaacaattttgatcgatatactcataatctagggttccgtaattgtgccaaattggaggtttagattctcgaagatttcgaattttccagtaatcggaaaatgaagctgaagatcaataaagcatcggatctcagttctatatccgttcttcctcctcatgcaaggaggcctagtgtggtaccaagtgcagcagagtcttctgtatttgggaaaggccaagcgtcacaggttcggtcacagcagcaatcacaacaatccttctcacagggattttcatctcagcaaatgacctactctcagccatctcagagctctctggatgaatttgtcacacatgaacatagattaggttctcaagaaagagaaaattcagcaaaaaggctgagctctttgcctcatatcaactacacacgagaagagaatcaactgcagttatcaaaaccttcggccaattatatacgcaaatggtcagttcctgaaaacaaataccagatcactgaagaacttgaccacaaaattggaatggtagagacttcattaagcaggcagggaatgatcttagattctattcagagtgatataatgcaagttaatcggggaacaaaagagatactgatggagatggaaagcttacggccaaagatagtttctcatgatgaactattgcaattgatgaacaaggggatggaagatctgaaagctagcctggaggggaccatcaaatccatgtttgaagagctgagggagaatacatatcaagaggacatcagggatcttttatcactggttagagctattcccaacaaacttgagatgtgcattttgcgacttcaaactgatttgagcaagaccttggctaaagagattcagataattgccacccacccagattgtcatggacaaaaacatgatagtgctccagtcgatccaccaaaaataattgccctccgtccagattgtcatggacaaaaacatgaaactgctccagtcgatccaccaaaaggcatcaatgattgtaaccctccacgtgaagtgaagtttctaaataaagatcagaaaacgactatgctgccgaagattgaaatgggaggctggactacagtaaaaaataaccaaacttgtatgaagcaagcaattcccgacagaagtcgcaaacagaatgaaacatttcaacagaaaattcccatcagaagtcacaaacagaaagaagcatttcaacagggaagggaatgtagaattaccattgaatctgatgaggatattggtgcagccttttcctgcttgcttgaagaaaatggaaaagggatttgtccactagatgatgcaaaggaagagagtgcacgcatattaaggaaagcaaggaggcgaaagagaaagcattttaacactatcattatagattgaaggtactcaacgacaatttataatccgctcaaggttctgtgatttgataagcagtaaaaaatgtattattttttcatccgtctttccttagccgatacaggacatgttgtttgtaattctgtgctccattattattagaaaatcccccactggtcattacatagcaagcataatctatgctgttgctgcaatgcgcagtcttgagtgattgtatatctttccaatgcccataataataagtaaaataccagattagtaaataattacaagcaatatgagtgatgtttta

SEQ ID NO: 105 - protein, 434 aa, Capsicum annuum
MKLKINKASDLSSISVLPPHARRPSVVPSAAESSVFGKGQASQVRSQQQSQQSFSQGFSSQQMTYSQPSQSSLDEFVTHEHRLGSQERENSAKRLSSLPHINYTREENQLQLSKPSANYIRKWSVPENKYQITEELDHKIGMVETSLSRQGMILDSIQSDIMQVNRGTKEILMEMESLRPKIVSHDELLQLMNKGMEDLKASLEGTIKSMFEELRENTYQEDIRDLLSLVRAIPNKLEMCILRLQTDLSKTLAKEIQIIATHPDCHGQKHDSAPVDPPKIIALRPDCHGQKHETAPVDPPKGINDCNPPREVKFLNKDQKTTMLPKIEMGGWTTVKNNQTCMKQAIPDRSRKQNETFQQKIPIRSHKQKEAFQQGRECRITIESDEDIGAAFSCLLEENGKGICPLDDAKEESARILRKARRRKRKHFNTIIID

SEQ ID NO: 106 - DNA, 10948 bp, Capsicum annuum
  source 1..10948: mol_type = genomic DNA
aacccacagacactactctttagatgtgcaaaggaaaaattctgctccagtacaatggtctacaaaccacacaagtgacgtaaaccgcatcagacaagtccagtgcgacaagctcgactaagaaaagatgcatgcagtttcaagcctaagagaacccccaccccccacaatttggaagatcacttagtcaagcaattcgaccacattgcgggctcctcttgcactatttaattaattttttttcctgactgtcccaccccaacagcccacactaggccactcccaagcctccctgacacgcctcggtcggtttttggccaaaaaaagcccgagccacgggcaagttagaaaccaacttatttgtagtgtttcaaattgtttttactatgtcaatttcgttcatgtgatttataacttttgatggctcggagtttcaacacacacaaaaaaaggttcaaagaaaaaattaatttactttgtttgagcaacattttttattatctaacgatttatcgtaatttactgatcaatttatttctctaggccgggagtacacatatatatatttttttcttattttttatattgattcattagaagttctatctaacaaagagagagaaaatttagcaggaaatatatatatagtaaattttgcttttaaaaaaaaaaaaaaaagaatgaatcatcacaatcaatattcatcattaaataaattttgcaggaaatgtaatgatttagcactagatttcactcgttgctaaatctagttttttgtaacgacctttaaacgccattttaacaattttagtaaagcttccatttaaaacgggatcaggataaggatagtaattaacagggagcaaagtgtagtttattaaacaagaagacctcttagaaatttacccaaaattaagaaaacgcgggaaatacaaaattcgataagcctataaattagggcaatttgaaatctccagttcctcatttccttctcgtgaggatgtcaattgcagtttggcagcaaatctccttattccgattcgaagtcgaaagctgtaggtatgtttccgattcatcaaaatttgcattctgattcagtaaaatgcatttgtgagcatgatttttgtgcagatttgatgaacgaactcttcgaattctcgagtctattttagcttcgattgatttcaaatctgtggaaggagtagtgtgcactttgaaacagttcatgagacatgaatctcttcgcattattgaggaaatcgctggaaaatctgtagagcataagcttctgatcgtcgattttctggttcacgtttttgctctcattggagatactgaggtataccgtacatacaactttgattttattgagtttaaattggcagatttcactttgatttcgttatttggaaacaaatagttaatagcagttagatttaatcgggaagaacagtaattttcagtaggataatgttgatgacactagaaatgcatatagtgaaagagcgtctgatgtattaaactgtgtattttggtgataagtagaagttctgcttgaaattttgtagccttttgtgttcagtaattgtattatctttgaaggatatatctcgtgttaatgtttttctaaagaagttgttgtattatgtagtttaagtgttcaaatgcacttcaataagtataagtagtagaagagataacttatatagctgtagaagtggcgcacgcgcttctggtggcggcagcaggtggtaatgtgagtagcaaaagacgtaaacaatgactgctgagcactggagaaactgtattaagtatatctaagggaaatttatccttccttatgtatacacaaactgttttaggtaatcagtatatgcaacattttggaacacgagaacctgactatccagaaaatgtaatgaaggaatgatgttaatttgatacttagagccaatgacaggaaaaatcagtttgattactcacggccatagtcattttaattgttgcctagatttcatggtggatcattgcagcttgttgaatacaaaagaaacaggtctcaagtgtggaaaattctaggagaaacaataatagactagttgtttttctattataactgttttcagttagttacactagtgctaacggctagttagttagttagttagttagcgtaatctctagcctataaatgtatatgactatacacattgaagtacaatgaatacaggcagttactcttatctctcatcttcttcctctctcagttctcttccttcctttcttctacaaacactatcaaactctgtacttccttcattgatgaattaacaagaagcttactgctatcttgtataattacatggtatcagagccaggttggctagatcaaaactagctaccttagtcgattctgaagattgaaaaaagtgctcaatcacagattcagatttttttcaagttcttaaaggatttcttgagtcaagatttgaaggttcaagtaatgacaaatggtgtcgaaatgggtggtggatcaatcagcagtgcaagagcagttactgcaatggattacaatcatgctctctttctcagtccctcagatgttagtggaacacagatcatctccttccaattgacaggtgtggaaaatttctctatctggttcaggtctatgcgtgtagctctgttaggaaggaataaattaggacttgttgatggttcttgcacaaaagaaaagttttcttccaatctgggaaaccactaggaaagagtaaatgctattgtattatcatggattatgaactctgtgtctaaagagttataggtggaatcatgtatgcatcagttgcaagtgttgtgtggaatgagttgcttgaaagattcaataaagtagatggtgctagaactttcaatctgcacaaggaaattgcaacactatctcaaagaacagcttctgtgtcctgctatttctcaaaactgaaggatctatgggaagaatttgaggcacttgtgcctgctcctggttgtgattgtgaaaagtccaaggagtttgttctacatctacaaaaactaaagttgtttcagttcctcatgggactaaatgaaacatatacacaggctagaagtcagatactacttatggctcctttgcctactgtcaatcaggcatatgccatgataatgagtgatgaaagccaaaaatctatagctactaatgcaggtgtgctaagatctggtcctacaggcattggtagaagtcttgacttagccatgtttacaagaaatgggacacagaaattcaagaaaaactacaatttgcaatgtgacttctgtaagctaaaaggtcatactaaggaaaattgttggaagttagttggatatcctcaaaatcacaagttcaaaaagaggttcagtccaaaggatctaatgcagtatacaaggtgactagtgattctcaagatactacagaaatgactacaaggcaaggttcacattcaaggtctatccaaagtaactggttcaatgatggatgccatcaagaagagtctgaaatgcagttggatcaactaggtcagatgggaataacagcctttactaaggaacaatatgatcaaatcctgaagttgatcaacaaaaatagtggtgctagcacttctactgagacaacaaatgctgcaaatgcaggtattagtgtatttctagcttcatatgagtcaagaaattggataattgacactagtgccacaaatcacatggttggaaagttagatctactagtgaatgagtccatagcaaaactaggtaagccaagaagggtgcatttacctaatggtgatctgactgaagttacacatgtaggatctagttatgtgtctgctgaaaatagtataataaatgtgtatcatattcctcagtttacatgcagcttgctttcagtatcttaactgaccaaggaatggaaatgttcagtgaacttctttcctgatttttgtgctttcctttgtactagaaaggtgagggggattggtaagcttgatggaggtctgtatctcttagtgaatactcaagaaaggaaggttgcagcagcaacaaaagtctctactaaagctaatgaaagtaaagcccaagctgaggttgatctgtggcataaaagattaggacatgcctcctctaatatacttctaaagttgctacgtactaaatttcatgtagtaaaagatagagtaaagaaatgtactatctgtccttgtgccaagcaaaccagacttccttttcctacaagtaatactcagtctgcatgttgttttgatctaatacatatggatctatggggaccttatagaattcctactacgaatggtaataagttcttcttaatagtggttgatgattgttcaaggtttacttggttgttcttattgaaactcaagtcagatgtgtatgtgcagatataacaatttcttgagtatgttaagatacagtttggcaaaactgtgaaagtaattagaactgacaatggaactgagtttgtgaactcattatgcagtagtttatttgcaaccaaaggtattgtacatcacacctcatgttcttattcacctcaacagaatggtgtggctgaaagaaagcacagacacatcctagaagtcacaagagcattgaggtttcaagcaacaatacctgttaagttttggggatattgtgttttagctgctgtgtatctcataaataggttacctagttcaagtattgattattatactccatatgagaaattatatggtactaaaccatcttgtgagcacctaagagtaataggttgcctctgttatgctaaggtgctaaatgagtctgacaagctcatgccaagatcaagagcagctgtgttgatgggatattctagtactaagaagggatatgtcttatatgacatatctactaatgttttctttgttagcagggatgtgtctttcagggaagatatgtttcctttcaagcttgaagcagctaatgatcagattccctatcatgtgtttccattagaagatcaatattcagcagcaagtgatgttatggcacccttgcaggctcctataaatgtctcatctcaagaggtttcgaacattgtgaaccagcaagaacacctacagcctcatgtacctactactagacagaccataaccaaggtgtatcaaagaaaatcaagcaaacatcaagaggttactcagcaagaacatcaactacaaagggttcctaatactacagaacctgcaactcaaccatctgcagctcaagatcaaaggaaatcaactaaagaaaggaagtcaccagcatggataaatgattttgactcttagaatacaaagaaggtacgtcatgctcttgctaatcatgtatcatatgataaactatctcagccctataagagttttgtggtgaaactgagcctacaagctactctgaggcctgcaaagatcctagatggatagatgcaatgaagactgaaatagaggccttaaattccaaccacacttgggaggttgttcccttgtctaaaggtaaaaaagccattggttgcaggtggatatataaggtgaagtataaggcttcaggtgaagtggaaagacttaaagccagacttgtagcaaaggttatggacaaagagaagggattgactataaagaaaccttctcaccagttgtgaagatgaaaatagtaagaactattcttgctactgctgcaaagaagaattggtttgttcatcagatggatgtctacaatgcatttctaaatggtgacctcactgatgaaatatacatgaagttgcctaagggatttgccagtcaggggagaattcagtatgcaaactgaccaaatctctatatggcataaagcaagcacctagacaatggaacatgaagctatcagaagtcttactaaggtctcagtttgttcaaagtcaatataatccatctctgtatataagaaggacacaagaaggaatcactttggtacttgtgtatgttgatgatatgctaatcactggtgatagcttgaaactgatagaagatgcaaaagttatgctacaacaaagcttcaaaatgaaggatctaggtgagttaaggttcttccttggtatagaatttgcaaggtcaagcaaagggatactaatgcaccagagaaagtacactctagagttactatcagagttgggattgacagcagctaaaccagtggttactcctatggactacaatgccaaactgacctcaaaacaatttgatgatcgtgtcaaacagctacaacctactgatgatcctcctgcagatcaaggtgtatatcaaagattgattggcaagttactatagttaaccatgactagacctgatattgcatttagtgtacagacactaagtcagtttctacaagagccaaagaagtctcatatggatgctgcaatcagagttgtgagatatgttaaaaatcaacctggtcagggtgtgttactatctagtgaaccaagtgatcaggtgagtgcctactgtgatgcagattgggcatcatgtcctcaaactcggagatcagtgactggttactttgtaaaaattgggaagtcagttatatgctggaagtcaaagaaacaagctactgtttccagaagttcagctgaggctgaattcagaagcttagcagctgtaacagctgagttggtttggatactaggcttgctaaaggaaattggaatggaagtaaagctgccagtcaaagtgtttagtgacagcaaatcagctattcaaatagctgccaatccagtttaccatgagagaactaaacacattgacattgattgcttcttcataagagaaaagataagccaggggatgatcactacaaactatatttctacacaagatcaacttgcagatatgctgaccaaaggcctcaccaaggctcaacaagtgcatctaaatcacaagctaggaatgtgtgacattttttcaacttcctagcttgagggggagtgttgaatacaaaagaaagaggtctcaagtgtggaagattcagaagaagcaataatagactagttgtttttctgttataactgttttcagttagttacactagtgctaacggctagttagttagttagttagttagttagttagcgtaatctctagcctataaatgtatatgactatacacattgaagtacaatgaatacaggcagttactcttctctgtcatcttcttcctctctcagttctcttccttcctttcttctacaaacactatcaaactctgtacttccttcattgacgaattaacaagaagcttactgctatcttgtataattacacagctacacctcattttttattttatgtgacacaatttgactaagcatgaggttaatagttaactgtagtcttcaacagaatgtcgatgtagttgtcgaaaatatatttgatatcagatacatcacggcatgctttaaattatctttttgcaacttgtgaaagatgcatgtctttacgggaaacatatccttctctatgttaatatacaacctgttttaggtaaaagtttgataaaatgaagtactcagtatatatttaggaatatgagaacctgactatccacttaaggggtcgttcggttggaaaacaagctatcctgcaattagttatcccaccctcaagaagggataaaaataacactacaatcccgggataactaattccgagatgagttatcccatgcattttgaattaatcctgagattagttatccctcatccctcctaccaaacgaccactagatgtaatgaaggaatgatgttaatttgacacttatgtccaatggcaggaaaaatcagtttgattactcactgtcatattcatttaatttttgcgtagctttagcctttaacagtagatagctgcagctgcacctcgttcttttcttttatgtgacacagtttgagtgagtaagaggtcaagagttacctgaagttttcaactgaatggcgatgtagttctcgagagtttatttgaatattagatacagcacagcatgtttaaattatctgtttgaaacttgtggaagatgcgcacaaaatttatcagatttaagagtgtgtcaaaacattttgggagatccaaagtgttggcatatcctatgatgtgaaagctttagaaaacataactaatgatgatggcattcttctatattagcaattttggttgtctttttgttttcgttccaaactcgtgaatctcttaacactttggtattatagagttgcttggccttgagatatgaggcactgcttatgagagagcagaaagcttcctgtgatcagagatttcttgtttcatatagcgagtggctcacttttgcggagcattcacttgaaagtggctattgttccgttgcaaagaaggtaaatttctgacaaaattttgggcccttgtgagcatattagatatacaaatgtcaaatgagcacggaataaagttcttagtatgtgctgtcttttgcaaatttatgctcacttcgtaacatttttgacctatgctaccattacgttaaggtgagagttaaattctaaaatgacctactactagtactgttatgtttccttagttatcataacttgtggttcttatcatgtcatattgtgttccccttttggatgtggttgtatatcaaacagaaatgatctttataataggttatatctgggttgggttaactggaagactgatctgatctgacattcagatgatatttgtgagatcagtaaactttgtcatctctatgcctcttgttggaggaatttgctggatgtaggttaaatttggttcgtttgcattctgaattaggaattacactcactgctgaaaacatctcttataattggttggcctcctctgcctcagcaattgtcctccttgtctactgtcagaatatagtatggacaacttgatagacatcagaaagggttgtggccaccgtgcaaggacactaaatgtgtcttagttccaaaatcaatactgtaattattaagtaattttttcttttgaatatcagtttccaacttccaatcaacaatgggtaaatctataggatgaaagttatggtaagaattagatcaatctagcaatgtaactattgcatcttcaacatcctgccaatactaagagcatatgtatttcacttgattctgtctattttgtacatttatctttgtgccttgtatgttatggtttcataaatgtagtgaagttacaatgtcctacaacttatagcaagtgtatccaatacttgcctctgacctgtaattttcaggcatgtgaaaaggcgcttttatgttttgagatgaacatcatagatgaccctgcaaatgatttcgtaattgaaaaaattaagaagcttaaagatgttgctgtgatctcagcgtcttcaaaatctggtatgttcaagtatttcattaaatccctcctttgtttcatcattaatgctctgccactatacgttcctcacatgaatgtgaattgaattcaagaacttggtggaatgacatcgaagtgttcctttagcccatgtaattagaagggagtggtgaagggaaaggtaatagttatcagttcattactgctaaagacttcttgtgatacattagttcaggcgcaggcagcagcatacttcaataacaaaagtattcagcagagctcacaaggatcctacatttctgtggaacctaaaagttcaggaagcactctgtttaaagatggaatcaaaagacgacacaaacgccaattggatgaataccgacatttgaaactggataaaataacttctggaggcgcgcaaaatattttggtatggtcattctgccaatatcattccttctccagcccccaaagtaaaaaagatcttatttagtttaattgttaaacaataattgattgtgcaggaatgatttttctctgatgtattactattagggagtaccaatatgatcaaaagatcaaatgctcttcttatggttagtatttcagcaggtaatttactctggttaatgttgtacgatatcattgctacagtatgtttaaaacttacaagaaaattggtcctatacgtatgccggtgggaagacaacaacataccagtggtctcataaagtgggatctggggagggtagagcataaaatgttcagaaagaaaaataatagaagtaatagaagtacaagaaacaacatatagtaacaaaacgtctgcctatggaaagagtcagaaaaaacttatgttgtcgtaagaacctcttgtttcattattgactctttttttttttaatctctaagagaatttgtttcagctattgacttttctcttcaatatttgcttttgcaccataataagcaatttttggcattttaaattacagttaataagacaagggtagaatacttgccttgtctcttctcaaccttggtcctgcaataggaacctagcatgctggtgataagtcttcaataaaatatgttggttagggaatctgtaattaagtctaagcaacaaacaatgagtacatttgcagcaagatattagcttcagcccctctccatgtaatcacgtgcctatgcagttgagtcttttgtcagttttcatatttcagcaaattggataggtgtaacttttactagtcaaaatcagaaagttggcttagaaattttgaatcaaacaattaggaatttgtaaatctttttagaaatctaatgaagaggacataatgaaaaaaaaatcttctcttgagtaatcatgtgagatgaaagtatcgtgcatggttttcaatgggaagaatcagggatggatataggttaatggatacaatttcatttgaattcaatagcttaattgagattttttatgtgttaaaaattcg

SEQ ID NO: 107 - DNA, 1640 bp, Capsicum annuum
  source 1..1640: mol_type = other DNA
cgtgaggatgtcaattgcagtttggcagcaaatctccttattccgattcgaagtcgaaagctgtagatttgatgaacgaactcttcgaattctcgagtctattttagcttcgattgatttcaaatctgtggaaggagtagtgtgcactttgaaacagttcatgagacatgaatctcttcgcattattgaggaaatcgctggaaaatctgtagagcataagcttctgatcgtcgattttctggttcacgtttttgctctcattggagatactgagagttgcttggccttgagatatgaggcactgcttatgagagagcagaaagcttcctgtgatcagagatttcttgtttcatatagcgagtggctcacttttgcggagcattcacttgaaagtggctattgttccgttgcaaagaaggcatgtgaaaaggcgcttttatgttttgagatgaacatcatagatgaccctgcaaatgatttcgtaattgaaaaaattaagaagcttaaagatgttgctgtgatctcagcgtcttcaaaatctgttcaggcgcaggcagcagcatacttcaataacaaaagtattcagcagagctcacaaggatcctacatttctgtggaacctaaaagttcaggaagcactctgtttaaagatggaatcaaaagacgacacaaacgccaattggatgaataccgacatttgaaactggataaaataacttctggaggcgcgcaaaatattttggtatggtcattctgccaatatcattccttctccagcccccaaagtaaaaaagatcttatttagtttaattgttaaacaataattgattgtgcaggaatgatttttctctgatgtattactattagggagtaccaatatgatcaaaagatcaaatgctcttcttatggttagtatttcagcaggtaatttactctggttaatgttgtacgatatcattgctacagtatgtttaaaacttacaagaaaattggtcctatacgtatgccggtgggaagacaacaacataccagtggtctcataaagtgggatctggggagggtagagcataaaatgttcagaaagaaaaataatagaagtaatagaagtacaagaaacaacatatagtaacaaaacgtctgcctatggaaagagtcagaaaaaacttatgttgtcgtaagaacctcttgtttcattattgactctttttttttttaatctctaagagaatttgtttcagctattgacttttctcttcaatatttgcttttgcaccataataagcaatttttggcattttaaattacagttaataagacaagggtagaatacttgccttgtctcttctcaaccttggtcctgcaataggaacctagcatgctggtgataagtcttcaataaaatatgttggttagggaatctgtaattaagtctaagcaacaaacaatgagtacatttgcagcaagatattagcttcagcccctctccatgtaatcacgtgcctatgcagttgagtcttttgtcagttttcatatttcagcaaattggataggtgtaacttttactagtcaaaatcagaaagttggcttagaaattttgaatcaaacaattaggaatttgtaaatctttttagaaatctaat

SEQ ID NO: 108 - protein, 265 aa, Capsicum annuum
MSIAVWQQISLFRFEVESCRFDERTLRILESILASIDFKSVEGVVCTLKQFMRHESLRIIEEIAGKSVEHKLLIVDFLVHVFALIGDTESCLALRYEALLMREQKASCDQRFLVSYSEWLTFAEHSLESGYCSVAKKACEKALLCFEMNIIDDPANDFVIEKIKKLKDVAVISASSKSVQAQAAAYFNNKSIQQSSQGSYISVEPKSSGSTLFKDGIKRRHKRQLDEYRHLKLDKITSGGAQNILVWSFCQYHSFSSPQSKKDLI

SEQ ID NO: 109 - DNA, 20 bp, synthetic construct
  source 1..20: mol_type = other DNA
acactcttaaggaaaatcaa

SEQ ID NO: 110 - DNA, 20 bp, synthetic construct
  source 1..20: mol_type = other DNA
aaccgttcgatgtagatcag

SEQ ID NO: 111 - DNA, 20 bp, synthetic construct
  source 1..20: mol_type = other DNA
ccggaaggtgaatcatgcgg

SEQ ID NO: 112 - DNA, 20 bp, synthetic construct
  source 1..20: mol_type = other DNA
ccgcctttcgaatatttcca

SEQ ID NO: 113 - DNA, 20 bp, synthetic construct
  source 1..20: mol_type = other DNA
aacagtaatgcagtttcctc

SEQ ID NO: 114 - DNA, 20 bp, synthetic construct
  source 1..20: mol_type = other DNA
cgacacagtgagaagtccgg

SEQ ID NO: 115 - DNA, 20 bp, synthetic construct
  source 1..20: mol_type = other DNA
atagtacctgtaacaataaa

SEQ ID NO: 116 - DNA, 20 bp, synthetic construct
  source 1..20: mol_type = other DNA
agtgatagatcagaaattga

SEQ ID NO: 117 - DNA, 20 bp, synthetic construct
  source 1..20: mol_type = other DNA
ggacatgcggcatcgttgaa

SEQ ID NO: 118 - DNA, 20 bp, synthetic construct
  source 1..20: mol_type = other DNA
gagtgcaaatcgagaaaacg

SEQ ID NO: 119 - DNA, 20 bp, synthetic construct
  source 1..20: mol_type = other DNA
gagagcataggacacgtgaa

SEQ ID NO: 120 - DNA, 20 bp, synthetic construct
  source 1..20: mol_type = other DNA
ctagcagatcgcctttccag

SEQ ID NO: 121 - DNA, 20 bp, synthetic construct
  source 1..20: mol_type = other DNA
gttcaaactcgccatcgcaa

SEQ ID NO: 122 - DNA, 20 bp, synthetic construct
  source 1..20: mol_type = other DNA
agaaattctcaggctcaagg

SEQ ID NO: 123 - DNA, 20 bp, synthetic construct
  source 1..20: mol_type = other DNA
tccaagttccaactgttcga

SEQ ID NO: 124 - DNA, 20 bp, synthetic construct
  source 1..20: mol_type = other DNA
gttgaagatgaacaaagcat

SEQ ID NO: 125 - DNA, 20 bp, synthetic construct
  source 1..20: mol_type = other DNA
gtaatcgtcccaagctaaaa

SEQ ID NO: 126 - DNA, 20 bp, synthetic construct
  source 1..20: mol_type = other DNA
gattatcgaaaacaaaccta

SEQ ID NO: 127 - DNA, 20 bp, synthetic construct
  source 1..20: mol_type = other DNA
tggaaattggtaagaagcag

SEQ ID NO: 128 - DNA, 20 bp, synthetic construct
  source 1..20: mol_type = other DNA
acactcataaggaaaatcaa

SEQ ID NO: 129 - DNA, 20 bp, synthetic construct
  source 1..20: mol_type = other DNA
acaaacctcatatttcacga

SEQ ID NO: 130 - DNA, 20 bp, synthetic construct
  source 1..20: mol_type = other DNA
gatcctacgttacttcccaa

SEQ ID NO: 131 - DNA, 20 bp, synthetic construct
  source 1..20: mol_type = other DNA
ggtagcgaagagacaagcaa

SEQ ID NO: 132 - DNA, 20 bp, synthetic construct
  source 1..20: mol_type = other DNA
ttaagaagaacatttcctca

SEQ ID NO: 133 - DNA, 20 bp, synthetic construct
  source 1..20: mol_type = other DNA
ggcgtagcagaggtgttgat

SEQ ID NO: 134 - DNA, 20 bp, synthetic construct
  source 1..20: mol_type = other DNA
ctaaaagtgcaaattataga

SEQ ID NO: 135 - DNA, 20 bp, synthetic construct
  source 1..20: mol_type = other DNA
ggacatgcggcatcgttgaa

SEQ ID NO: 136 - DNA, 20 bp, synthetic construct
  source 1..20: mol_type = other DNA
gagtgcaaatcgagaaaacg

SEQ ID NO: 137 - DNA, 20 bp, synthetic construct
  source 1..20: mol_type = other DNA
tttccttatgggaatggtgg

SEQ ID NO: 138 - DNA, 20 bp, synthetic construct
  source 1..20: mol_type = other DNA
ttaacagtattaatgcaaag

SEQ ID NO: 139 - DNA, 20 bp, synthetic construct
  source 1..20: mol_type = other DNA
gcggcggtggaggaagaagg

SEQ ID NO: 140 - DNA, 20 bp, synthetic construct
  source 1..20: mol_type = other DNA
agaaattctcaggctcaagg

SEQ ID NO: 141 - DNA, 20 bp, synthetic construct
  source 1..20: mol_type = other DNA
tccaagttccaactgttcga

SEQ ID NO: 142 - DNA, 20 bp, synthetic construct
  source 1..20: mol_type = other DNA
gttgaagatgaacaaagcat

SEQ ID NO: 143 - DNA, 20 bp, synthetic construct
  source 1..20: mol_type = other DNA
attaatcgaaaacaaaccta

SEQ ID NO: 144 - DNA, 20 bp, synthetic construct
  source 1..20: mol_type = other DNA
gtaatcgtcccaagctaaaa

SEQ ID NO: 145 - DNA, 3366 bp, Solanum lycopersicum
  source 1..3366: mol_type = genomic DNA
cccttgatcacaggaagcagcggaacgtgttggtgagaaactagtgcaggcttgtgttgacctcaacatcgatgaaatttcatgttatgatcgaaatggttttgctcgaggagacagaatgcaagcctttgagattgccatttctcgacatggtttcatgttcaaatagttcatccttcttttctatgtgcattttgtatagccttttaagactctgaagctcttaccttttacaaaactgttgcgaaataattcagaatttagacgttgtgtgttttgaaatacctgagtggattatgatgtatatctaacttctatctaaacttggtatttggcacatgttatatacatttcaatctcaaaaagtttggattctatagaatcgcgctactaatcatgtgtgtgaatacgacctagcggtctataaaatttcaagtcttagaagggacaaaatcactagatttttttttttccatacgtctagctttgatggacagagttatcgatacttatccttatttggtttagtatagtcaaattcgaggttctattttcttttgtctgatcaattttgaaaataattcattatctgaataagaatagagggaaaagaaaatcaatagcctgttttcaataaaacagtaatttttactagcctttttttaacacagaaaaattgtttctgctacaacttaaaaacctttttttatttattgaccaaaaaccacatattttcaaaatataaatatttcttttattttaaaaaaatgcttttcggttgacatttttaaaactgcttatttttatttattatttaaactgcttaggatattaactgaccctatgaagaatacagttataaagtagttataatgaatgataaatgatttactatctatctgtctacacatttcaaatgtaaaaactataaataaaccaaaaaaaccacatcaaaacttcattcaaactttcacaattttctcaaccaaaaaccacaaaaatggagcaaactagtgaaggaattggaataaaaatgtatagtacatcgaaacgcgtcgataattcatcgtctatgtatcctactaatttaccacaaggtgaaataatcccagaattaccaataccaattggtggtaaaaaaagaagagcaatggcaaatggtgtacaaaaaacactttcaaaaacttcattacttgttaattttctcccaacgggaacccttttaacatttgaaatgttacttccctcagtatttggtaaaggagattgttcaccaattactacatttatgattttaacgttacttggactttgtactttgtcatgttttttctttcattttaccgatagttttcgaggtcctgatggtaaaatttactatggttttgttacaccaagaggtttgaaagttttcaagactggacttggtgtcgatgtgccaaaagatgaaaggtaaatttaatttaatcgcgcttagccatgaacactgttttgtatttaaaaaaaaattgatatttgtgttggaatatttttgtaaatcgcccttggttatgaacattattcttctatgagttattttttagtagagagttttcattttgtgaaattttttatgataggtaacttttagtgatgattcttttgatgttttaatgtgtgagagatgtaaaatcgcctttaggtgtgaatactattttctacgagtaaagagaaaatatacagatttgtgacgggagtatttttttacgaaagatttttatttactaaaattgtgaaaattttatgattactgacaatagtttcggtaacaaaaattatgatagttttatggttgtaacaaaatagaaagattttttcaaaattttgacagttttatttcagaatttatcaatatacatgaaaattgtgacagttttaatccagaatttgttaatttgtgactgattcttactgctttttaaatataattagtcgatttcgcaacttattagtcgatttcatgcctcaaagtcattgtttcaccatgagatgttatagttatataggaaaatcttcaacattatggacgaaatttacgatgttttttattttctttgatttagggtgttgacatcgttttgttttggtttgttgtgactaggtacattgtgggagtgacagattttgtacatgcaatgatgtctgttttggtgtttgtggcaattgcattttctgatcacagagtaacactttgtctatttcctggacatgctaaagaacttgatgaaattatgaggagttttccattaatggttggagttatttgtagtggactttttcttgtttttcctaattcgagatatggtgttggatgtatgtctgcttagatatctacgtttacattctttcatgtattgtaatatacgttggttgatatttatttaaaatctatctatcttgtattgaactacgatgatctgtaacatatgtacttttactttgcatttctctaagagaccttacatagtagtaactttagtggtgttatgttgtattaactttactggtcaattcaagactccccttcgtgaaggaaagcaaaaatactttactggtcatcattttttcaaaaaaatactttgtatcttatcaaactatcctacataaattgaaattccttaataatatggattgaaacatgattatatgaagagaatggacgtaagaattcatatattataatcaaacataacttgtttggagttgaaacatagataattattgttatttttattgttacaaactcaatacacatgcatcaaatttatactgaatcatgaatctctttctttttgggtactcaatcatgaatattaagataggagtaagatatgtcgtacatttgaatttgtaggaggctaagaatggattacttggacttataccatatacattggccagtgaggatgaagaatggtgatgaccaagcaataaagttggtaaatgaggatgtaattccatttgacataagaggaacatggcaagctatggaagaatgttacaaataaattgtttgatatttgtaggtggcattgagatgggtatatgagcaaggagttagtgtattagtgaagagtttttaacaaggatagaatgaaagagaatcttcaaattttggattggtatttaagcaatgaagaaaatggtaagattcaagagattcttcaaaggtgaactttttgtacatccagatggaccgtacacatccccagatgaattctgggatggtgaactataaaatgatactgcgaaattgttcaatccttttttcatcattgggtcgatttaggctccttcccttccactgcatatccaggttccacacag

SEQ ID NO: 146 - DNA, 838 bp, Solanum lycopersicum
  source 1..838: mol_type = other DNA
tataaataaaccaaaaaaaccacatcaaaacttcattcaaactttcacaattttctcaaccaaaaaccacaaaaatggagcaaactagtgaaggaattggaataaaaatgtatagtacatcgaaacgcgtcgataattcatcgtctatgtatcctactaatttaccacaaggtgaaataatcccagaattaccaataccaattggtggtaaaaaaagaagagcaatggcaaatggtgtacaaaaaacactttcaaaaacttcattacttgttaattttctcccaacgggaacccttttaacatttgaaatgttacttccctcagtatttggtaaaggagattgttcaccaattactacatttatgattttaacgttacttggactttgtactttgtcatgttttttctttcattttaccgatagttttcgaggtcctgatggtaaaatttactatggttttgttacaccaagaggtttgaaagttttcaagactggacttggtgtcgatgtgccaaaagatgaaaggtacattgtgggagtgacagattttgtacatgcaatgatgtctgttttggtgtttgtggcaattgcattttctgatcacagagtaacactttgtctatttcctggacatgctaaagaacttgatgaaattatgaggagttttccattaatggttggagttatttgtagtggactttttcttgtttttcctaattcgagatatggtgttggatgtatgtctgcttagatatctacgtttacattctttcatgtattgtaatatacgttggttgatatttatttaaaatctatctatcttgtattgaactacga

SEQ ID NO: 147 - protein, 225 aa, Solanum lycopersicum
MEQTSEGIGIKMYSTSKRVDNSSSMYPTNLPQGEIIPELPIPIGGKKRRAMANGVQKTLSKTSLLVNFLPTGTLLTFEMLLPSVFGKGDCSPITTFMILTLLGLCTLSCFFFHFTDSFRGPDGKIYYGFVTPRGLKVFKTGLGVDVPKDERYIVGVTDFVHAMMSVLVFVAIAFSDHRVTLCLFPGHAKELDEIMRSFPLMVGVICSGLFLVFPNSRYGVGCMSA

SEQ ID NO: 148 - DNA, 3448 bp, Solanum tuberosum
  source 1..3448: mol_type = genomic DNA
gttaaatgggctcaattattgggcttgtgattgtggcccaaaattatcgatcaagtaaaatatctgtatttgaatgaatttttagattatgcaaaatatcagtattaacaaatgtaacaaataaaatgaattaaaataaatataatgaacgtaattaatgacatgtaaatatgcaattttaaaattaactgataaaaaatcctaaattttgataaataaggatagttatcgataaacttatttaaaattataaaaaaaaatattttgaaccattagataaataaaccttaaaagttgcgaattttcaaaaatgttaggccaaaattgggtgtcaacaagtatcattcttatctatatttaaaacggcttatttaaagttaaattgtcattgataaattttactctagtttaaaaacatgaaaatacttagttggtaactcaatttttatattcacgacaattttaaaaaatattttaagaatacattttactcatgttgaaaaattaggtgtatttactaaatagatattttaaaaattgtcatcagttcaaagataaaactaataattcacgagtttaagggaaattttcagtacttctcactaatcgaaaagatttagaggtaaaatcaacatgggacgtttttttttttgtttatttaattttcttaaaaggaaaagttaataaatggagttaagtattgaaggatccattcaaatattttcacattttttttataaaaaaataaaataaaaattaattattgaaaagctttatagatcgtgcagaagtgggtgtgtattgggtagtttttaaacaaccatttaaattaaattaaaatagtaataattaatattaaaaaaatatagaatttttttgtatatagagatagaagattcaaaacatttgtaagtgcatttacgtaaccaaaactataaataaaccaacaaaacttcattcaaaactttctctaccattttctcaatcaaaaaccacaaaaatggagcaaactagtgaaggaattggaataaaaatgtacagtacatcgaaacgcgtcgataattcatcttctatgtatcctactaatttaccacaagatgatacaatcccagaattatctcaacctgcattaccaattggtgggaaaaaaagaagagcaatggcaaatggtgtacaaaaaacactttcaaaaacttcattacttgttaattttctaccaacaggcacacttttaacatttgaaatgttacttccatcagtatttggtaaaggagattgttcaccaattactacatttatgattttaacattacttggactttgtactttgtcatgttttttcttccattttaccgatagttttcgaggtcctgatggcaaagtttactatggttttgttacaccaagaggtttgaaagttttcaagactggacttggtgttgatgtgccaaaagatgaaaggtaattttttatgttggtaatcgcccttagccacgaacactattttctataaaaaagagaaaaatagagatttgtgataggaatatttttgactaaagagtttcatacatatatgattgtgacaaaagatgaaaggtaacttttagggatggtttttgtaatatttgtgtgtgtgagagacgtacatcgcccttggctatgaacactatttttctatgagaaaagagaaaaatattaatttgtgatggaatgaatattttttactagagagttttcatttatgtaaattttatgattgtgacaaaagatagaaaggtaactttttagtgatgattttttcaatgtttatgtgtgtgagatgtaaattcgcccttggctatgaacactattttctatgagaaaagagaaaatatacagatttgtgatggaatatttttgactaaagattttcatccacataattataaaaaatttatgattgtgacaaaaggttttccgtcacaaaaattgtgtgttttttttaaaaatatagttatttgcttaaagtcattgtttcaccataaaagatgacagtttttagataaattatcaatttcacccctcaaaatcattgtttcaccataaatcgtgacagttgtatagcaaaatcttcaatattgtggacgaaatttgcaatgctttctttattactaatattgtgttttttcccccttaatttagtgtgttgacatcattacctttttgttggttggttgtactaggtacattgtgggattgacagattttgtacatgcaatgatgtctgttttggtgtttgtggcaattgcattttctgatcatagagtgacactttgtctatttcctggacatgctaaagaacttgatgaaattatgaggagttttccattaatggttggagttatttgtagtggactttttcttgtttttcctaattctagatatggtgttggatgtatgtctgcttagctatttttattttattctacactagactacatttcttttctagttttatactgtttcatatatattgtaatttaagttggtcgatatttatttaaaattatctatatgatatattgttttcttttctttttcaaatttatatttcaaaatttaaatatattggtattttgctagctgttctaaatatgtcccatatccctcctatttattgcacaaaaataacagctataactaaatatttatattgcttggactttttaaatatatcacgtggagtatttcaaattttcaataataccccctctattccaaatgtaattgtccttttcaagagtcgtgaattttcctaattttcaaaactaaatttaattagataagataactatgtacaagttacaacctctgccacacacatcaataaatctatcacttcaaccagataaggtaactacttaaaatttgtacatccaaatctctacacatttcaaaattgccactatccagctgtaatcttctttgtatcgttccaattaagtacgtacttaatcatatggctatgttagtcccaaaaattatgttgaattctggtcatgaaatgcctctaataggcatgggaacagcaccaacggcaccaacattaccaccaattgaccaattagtctccatttttatcgatgctatcgaagctggttatcgacactttgacaccgctgcggcctatggctccgaggaagcactaggtcgagccgtggctgacgcgatacaacgcggactcatagagagccgtgaagatgtttttattacatctaagttatggtgcaccgaaacacatcatgaccttgttcttcctgctctcaaaagatctctcgcgtaagtttgctcatactattgattttaaattcgaataaaataaaaagttgtgatagattaacatcttatacatgtttctacggggtgggggtttggttcaacccctaccatgtagtaatatatatatata

SEQ ID NO: 149 - DNA, 687 bp, Solanum tuberosum
  source 1..687: mol_type = other DNA
atggagcaaactagtgaaggaattggaataaaaatgtacagtacatcgaaacgcgtcgataattcatcttctatgtatcctactaatttaccacaagatgatacaatcccagaattatctcaacctgcattaccaattggtgggaaaaaaagaagagcaatggcaaatggtgtacaaaaaacactttcaaaaacttcattacttgttaattttctaccaacaggcacacttttaacatttgaaatgttacttccatcagtatttggtaaaggagattgttcaccaattactacatttatgattttaacattacttggactttgtactttgtcatgttttttcttccattttaccgatagttttcgaggtcctgatggcaaagtttactatggttttgttacaccaagaggtttgaaagttttcaagactggacttggtgttgatgtgccaaaagatgaaaggtacattgtgggattgacagattttgtacatgcaatgatgtctgttttggtgtttgtggcaattgcattttctgatcatagagtgacactttgtctatttcctggacatgctaaagaacttgatgaaattatgaggagttttccattaatggttggagttatttgtagtggactttttcttgtttttcctaattctagatatggtgttggatgtatgtctgcttag

SEQ ID NO: 150 - protein, 228 aa, Solanum tuberosum
MEQTSEGIGIKMYSTSKRVDNSSSMYPTNLPQDDTIPELSQPALPIGGKKRRAMANGVQKTLSKTSLLVNFLPTGTLLTFEMLLPSVFGKGDCSPITTFMILTLLGLCTLSCFFFHFTDSFRGPDGKVYYGFVTPRGLKVFKTGLGVDVPKDERYIVGLTDFVHAMMSVLVFVAIAFSDHRVTLCLFPGHAKELDEIMRSFPLMVGVICSGLFLVFPNSRYGVGCMSA

SEQ ID NO: 151 - DNA, 3503 bp, Solanum melongena
  source 1..3503: mol_type = genomic DNA
ttcttccttattttaccttttacaaaagtagtatatcattgcagtcgcgaaagaactcagaatttagacgttgggggttttgacatacacaagtgtaagttatatctatacttggtttttggcacatgtatatacatttcaatcttgaaaaaattgggttcaatcgaatcgtgaacataatgttggatccgctactaatcatttatacttcaaatagacgatatacatgagcattcatggatataacctagtggtcaacaaagtaggttgagaatctgaaatttcgagttcaagtcttgtaagagacaaaacctcgaatgatcatggacaaagttatccgatacttattgttgttcacattaaaatatccctatttgctctttgtgtattcaaaattcgaggttctattttcctttatctaatcaattttgaataattcattatctgaataagaaaatagagggaaaaaaatcaattcaaaaagcagaaaattttagttttttttttccaataataaaaaaattgtttctactactcactgtcagaatttaaaagtttgtaaccaccttatctctaaaaaaaattgtagttaagttttaattcaaattttgaacttaaaagtttaattaaatttatatttaaaaagttacttaaaatctgcaaattaattaacgggggtggggctacgtgcatagattagtgtagttaattgaagattaatttttattataaatgaatatttttttaaaactactttcattttaattttaaaacactgttttaaatttcagttttgttttttcaaattgtaatttattatagataattattaattaatactacaaaaaattaagaaactttttatggtgacacgtggcagtttttggttcaggatgtttaccattgtttagaagatccaaaaaattgtaagtgcatctacgtaaccaaaactataaatagaccaacaaaacttcatttcttcagatctttcaaaaaaaaaatggaggaacgtagcgatggaattggaattaaaatgtacagtgcatcgaaacgcgtcgataattcttcatcgtaccctactgatgtaccaatttcagaattagtggaaccatcaatggttgttggtaaaaaacgaagagctatggcaaatggtgttcaaaaaacactttcaaaaacatcattgcttgttaattttttaccaacaggcacacttttaacatttgaaatgttacttccatcagtatttggtaaaggggattgttcaccaattactacttttatgatgttgacacttcttggactttgcactttgtcatgttttttctttcattttaccgatagttttcgcagtcccgatgggaaggtttactatggtttcgttacaccaacaggtttgaaagttttcaagactggacttgggattgatgtgccaaaagaccaaaggtatgtctgctttataatttgtgtcattgcgtgtcacccattttttaattttatcagaaaatagaaaaatacaaatttgtgacagttgtatctatggttttctgattaaattttaatttgtgtgtgagatgtaaatcgccctcggtgaccaacactattttgagaagcagaaaaatataaatttgtgactaaagatttttttgttgtgacagttttatagtatatggtttgtgactaaactttaatttgcaatatttttgtgcatgagatgtaaattgcccttggccacgaacactattaacttatgagaagaaaaagatacaaatttgtgatggaatatttttcactttaacatttttccatcacaaatttgtatatggtttgtgactaaatatttttgaaaaaccataaagttgtgatagttttattctggaatttatcaatatagacgaaattcatggcagttgatagatttttctttggtcgcaaatataatatttttatatagtcagtcgatttcacgtttcaaagtcatttcttcaccttaaaatatgataattttatggaaaaatctttcatattttagacctaaggtatgtgtagttcttaatttgcaatatttgtttatgtatgagacataaatcgcccttggccgccaacactattacttatgagaaaagagaaaaatacaaatttatgacaaaatatttttcacaaatttgtgacaagattctctttttgatcacaaatatcttttttttttcgatttcacgcctcaaagtcatttcttcaccataaaacgtaacaattaattttttttttttgttgtactaggtacattgtggggttgacagattttgtacatgcaatgatgtctgttttggtgtttgtggcaatagcattttcagatcatagagtgacactttgtctatttcctggacatgcaaaagaacttgatgaaattatgaggagttttccattaatggtgggagttatttgtagtggactttttcttgtttttcctaatactagatatggtgtcggatgtatgtctgcttagaaactttcattataattctacattctagactagactactttttttttgtttgaaaaaattatgttcttatggtacggtttgatcagttgtaataaaagtttattacatttttattattggatcaataagtatgactatggttgatgtttgattagatatatttatatttagtgtcagagtcagaattttgtttagggagggacacaatttaaagaaacgattataattaatgtttaattagatctatatccaatgatggaatgagaattttgtttagggagtgtcacaattttaaaaagtaaaattatgtcaagaaataataatcacataagaccactaaagcaacataaaaccaactacattaaaaataatagcaaaaatatagtgaactttatgaaatcaagatataattttatacttaatttttaatttatccatatcgttaattataattattattctattgtatttttcaagatattatacttattgtattcaaacgatgatttaataatttttatgtcaattaatagtgaacaactattattgaacgaattaagggagtacagcatccaacttggggtgaaagtgacaattccaaagaatagtcatttatattaaaattaaaaatttccacatttcaaaatcactttttaaatatatatatttaaatatgttgatgcagaaataaatagactacagtagaaaagtcttaacattacttcacccttcaattattttactttgccctatgtttttcagactccttaaaaatatcatataatctattttaaattttttaaaaatacatttttcttataaaatgattatcatattttgcttttgagtatcaattttgttaacttttacaatttaattagattataaattaatttaatttttaaaaattaaaatttaaatattcaatatgttgaacgatacaactttaaatttgaataaaattcttatcgtttgacttccgaaaaatgattgaatggag

SEQ ID NO: 152 - DNA, 669 bp, Solanum melongena
  source 1..669: mol_type = other DNA
atggaggaacgtagcgatggaattggaattaaaatgtacagtgcatcgaaacgcgtcgataattcttcatcgtaccctactgatgtaccaatttcagaattagtggaaccatcaatggttgttggtaaaaaacgaagagctatggcaaatggtgttcaaaaaacactttcaaaaacatcattgcttgttaattttttaccaacaggcacacttttaacatttgaaatgttacttccatcagtatttggtaaaggggattgttcaccaattactacttttatgatgttgacacttcttggactttgcactttgtcatgttttttctttcattttaccgatagttttcgcagtcccgatgggaaggtttactatggtttcgttacaccaacaggtttgaaagttttcaagactggacttgggattgatgtgccaaaagaccaaaggtacattgtggggttgacagattttgtacatgcaatgatgtctgttttggtgtttgtggcaatagcattttcagatcatagagtgacactttgtctatttcctggacatgcaaaagaacttgatgaaattatgaggagttttccattaatggtgggagttatttgtagtggactttttcttgtttttcctaatactagatatggtgtcggatgtatgtctgcttag

SEQ ID NO: 153 - protein, 222 aa, Solanum lycopersicum
MEERSDGIGIKMYSASKRVDNSSSYPTDVPISELVEPSMVVGKKRRAMANGVQKTLSKTSLLVNFLPTGTLLTFEMLLPSVFGKGDCSPITTFMMLTLLGLCTLSCFFFHFTDSFRSPDGKVYYGFVTPTGLKVFKTGLGIDVPKDQRYIVGLTDFVHAMMSVLVFVAIAFSDHRVTLCLFPGHAKELDEIMRSFPLMVGVICSGLFLVFPNTRYGVGCMSA

SEQ ID NO: 154 - DNA, 3289 bp, Capsicum annuum
  source 1..3289: mol_type = genomic DNA
tttgagattgccatttctcgacatggtttcctgttcagatagttcttccttcttttcgttgtgcatttttgttgtatagcatttagcagtctcttacccctcagtccgctaagttttatttctatcatattaacatcccttgtctatcgcaaacaacctctgaggtaagggtaaagtcttcgtatacttctcagactccactttatgggactatactgagtatgttggtgtaattgttatttcgcctatagcctatcaaaaagagaaaaaacctcctgtaattcattcacgaaaaacttcttgtaccaaccatatacttcgtgtcacctgaaacgaaaaaagaaaaaaagaaaagaaaaagctgaagtagacatggaacttttccgttactgtatttttttattttttttttaagttgcaaattccagttattaagatggttaacttttacgtgaggaaatttagctattaagcctctttaagtttctaattagcaaaatgtctaaccctcttcaagttttcaattagcaaaatgacctacttttattttctcatttgtcggacaagtaatagatctgtcggattgataatcgatctgtctatatatttatcggacagataatagatctgttggattgataatcgatttgtctaaatatatttgtcttaaaaatgcatcatttcactaaataaaaaatttatggtccatttaattaaaaaatagacttaaaaggtctatttaacaaagattcctcttttagagttacaattttaaaaatttcttaaagatgtggcaatggttgccaagagtcagttactaaccgttttaaaaaaattcaaaaattgttgtaagtgaccaaaactgtaaataaaccaacaaaacacatatatataatcacatatcttaatactccaaaattttggttttatcttttttccgaaaaaccattaaaacttcattcctattctgcaaatcttcaccattttctcataaaaaaagatggagcaaagtagtgagggaattggaataaaaatctacagtgcatcaaagcgcgtcgataattcttcgtcttcaatgtaccctactagtttaccagaagatgttccaattccagaattgcctcaacaagcatcaattggtggcaaaaaaagtagagcaatggcaagtggtgttcaaaaaacactttcgaaaacttcactgcttgtgaattttctaccaacaggaacattattaacatttgaaatgttacttccatcagtatttggtaaaggggattgttcaccaattactacatttatgattttgacacttcttggattatgcacattgtcatgcttcttcttccattttactgatagttttcgcggtcctgatgggaaagtttactatggttttgttacaccaagaggattgaaagttttcaagactggacttggtgtcgaaatcccaaaagatgaaaggtaattttttagtattgtatagtctgttgtaatatttgtgaaataaagcgcacttagccacgaatacaaattgtgacagaatatttctgaatatagattttcattaaaaaaatggagacatttttatagttgtgacaaaaaattgttcgtgcaaatcgtgacaatttattgttgggacgcaatatttccgttatattcatcaaattgtaaattgggacgaaatatttctgttacattcatcaaattgcgacagtattattcaatataacacaatttgtgaattttttttcatcacaattttttgacaattttatggttttgacgattttttttccgtcacaaatcgagtcagttttacggttgtgacgaaatgttactgaccaaaggtttttcaccataaaattatgacacttttattatacgtagaattttatcaatatagacaaaatttgtgacactgttttattgtccatcacaattttttttcaggttttaacttctaatttgtggtggattgtgacagattctatcataaaaaatattgctattctttttataatgagttttgattccacgccttaaagctattgtttcaccattaaattgtgacagttttatggcaaaatcttcaatattgtggacgaaatttgtgacgtgtttttttccttccatcagttatgcaacgttcgaattactgatggactgacgaattcttctaccgtcacaaatattgtttattttgtaaatatcgtgagttgatttcacgagtcaaattcgatctcgttcttgtgttaattaatctatcttttacatctttttgtgtaataggtacattgtgggattgacagattttgtacatgcaatgatgtctgtgttggtgtttgtagcaattgcattttcagatcatagagtgacactttgtctatttcctggacatgcaaaagaacttgatgaaattatgaggagttttccattaatggttggagttatttgcagtggactttttcttgtttttccgaatactagatatggtgttggatgtatgtctgcttaattaccaattttagggattgctaattttattataagtatatgtgattttttttttctttcaattagttctctatggtaggggtactatttgagtatgtatgttgtaattttagcaatgtctatttatttttggtgtattataatgttgacagtgggtcaatgtttatatatctatggatgattaatttatgcaaaaattacctaaaaccacaacataactatctaaacttttaaaaatttcctacttcttaaaaattacttaaatcccaacatttcatattttttactatttctgagatacaagttaaccctacatgtatctaatatatgtatctactgttgtttgtgatacaagttaatcacattagatacatgtatcaacagtatgcatctaatgtaattaacttgtatcatcagaggtcaaatgttgaaattttaggagattttaaaaaatgttgggatatttagtaattaaggataaacatgtcggtatatatgtaaaatttccttaatttatcttattaaaggggtgttttttctgtctgtcaattgctaattgtatttgtaattgtaattaagagaagggaataagggaattcagagtggattttataccctccccgatgtcgtttaacaaatgaaacacacacaaatataggtatatatataccctcgctgtttaatgaataatgtacgtctacatttttcattacgattgcaaatagaaccaatcattaaacgaagggcgggaagtgccgtgagaaaagaaaatact

SEQ ID NO: 155 - DNA, 669 bp, Capsicum annuum
  source 1..669: mol_type = other DNA
atggagcaaagtagtgagggaattggaataaaaatctacagtgcatcaaagcgcgtcgataattcttcgtcttcaatgtaccctactagtttaccagaagatgttccaattccagaattgcctcaacaagcatcaattggtggcaaaaaaagtagagcaatggcaagtggtgttcaaaaaacactttcgaaaacttcactgcttgtgaattttctaccaacaggaacattattaacatttgaaatgttacttccatcagtatttggtaaaggggattgttcaccaattactacatttatgattttgacacttcttggattatgcacattgtcatgcttcttcttccattttactgatagttttcgcggtcctgatgggaaagtttactatggttttgttacaccaagaggattgaaagttttcaagactggacttggtgtcgaaatcccaaaagatgaaaggtacattgtgggattgacagattttgtacatgcaatgatgtctgtgttggtgtttgtagcaattgcattttcagatcatagagtgacactttgtctatttcctggacatgcaaaagaacttgatgaaattatgaggagttttccattaatggttggagttatttgcagtggactttttcttgtttttccgaatactagatatggtgtt

SEQ ID NO: 156 - protein, 223 aa, Capsicum annuum
MEQSSEGIGIKIYSASKRVDNSSSSMYPTSLPEDVPIPELPQQASIGGKKSRAMASGVQKTLSKTSLLVNFLPTGTLLTFEMLLPSVFGKGDCSPITTFMILTLLGLCTLSCFFFHFTDSFRGPDGKVYYGFVTPRGLKVFKTGLGVEIPKDERYIVGLTDFVHAMMSVLVFVAIAFSDHRVTLCLFPGHAKELDEIMRSFPLMVGVICSGLFLVFPNTRYGV

SEQ ID NO: 157 - DNA, 20 bp, synthetic construct
  source 1..20: mol_type = other DNA
tatcctactaatttaccaca

SEQ ID NO: 158 - DNA, 20 bp, synthetic construct
  source 1..20: mol_type = other DNA
tctcctttaccaaatactga

SEQ ID NO: 159 - DNA, 20 bp, synthetic construct
  source 1..20: mol_type = other DNA
tctcaacctgcattaccaat

SEQ ID NO: 160 - DNA, 20 bp, synthetic construct
  source 1..20: mol_type = other DNA
tctcctttaccaaatactga